European Patent Application EP 4 410 842 A1, published August 7, 2024. Title: A fusion polypeptide and its use. Applicant: 杭州阿诺生物医药科技有限公司. Application WO. The sequence listing filed with the application follows.

SEQUENCE LISTING (190 sequences)

SEQ ID NO: 1 - protein, 288 aa, synthetic construct
  REGION 1..288: note = CD80
MGHTRRQGTSPSKCPYLNFFQLLVLAGLSHFCSGVIHVTKEVKEVATLSCGHNVSVEELAQTRIYWQKEKKMVLTMMSGDMNIWPEYKNRTIFDITNNLSIVILALRPSDEGTYECVVLKYEKDAFKREHLAEVTLSVKADFPTPSISDFEIPTSNIRRIICSTSGGFPEPHLSWLENGEELNAINTTVSQDPETELYAVSSKLDFNMTTNHSFMCLIKYGHLRVNQTFNWNTTKQEHFPDNLLPSWAITLISVNGIFVICCLTYCFAPRCRERRRNERLRRESVRPV

SEQ ID NO: 2 - protein, 208 aa, synthetic construct [sequence omitted]

SEQ ID NO: 3 - protein, 460 aa, synthetic construct
  REGION 1..460: note = JS003
QGQLQESGPSLVKPSQTLSLTCTVSGDSITRGYWNWIRKHPGKGLEYIGYISYTGSTYSNLSLKSRVTISRDTSKNQYYLKLSSVTAADTAVYYCATSTGWLDPVDYWGQGTLVTVSSASTKGPSVFPLAPCSRSTSESTAALGCLVKDYFPEPVTVSWNSGALTSGVHTFPAVLQSSGLYSLSSVVTVPSSSLGTKTYTCNVDHKPSNTKVDKRVESKYGPPCPPCPEPKSCDKTHTCPPCPAPEFEGGPSVFLFPPKPKDTLMISRTPEVTCVVVDVSHEDPEVKFNWYVDGVEVHNAKTKPREEQYNSTYRVVSVLTVLHQDWLNGKEYKCKVSNKALPASIEKTISKAKGQPREPQVYTLPPSREEMTKNQVSLTCLVKGFYPSDIAVEWESNGQPENNYKTTPPVLDSDGSFFLYSKLTVDKSRWQQGNVFSCSVMHEALHNHYTQKSLSLSPGK

SEQ ID NO: 4 - protein, 451 aa, synthetic construct
  REGION 1..451: note = Durvalumab(MEDI4736)
EVQLVESGGGLVQPGGSLRLSCAASGFTFSRYWMSWVRQAPGKGLEWVANIKQDGSEKYYVDSVKGRFTISRDNAKNSLYLQMNSLRAEDTAVYYCAREGGWFGELAFDYWGQGTLVTVSSASTKGPSVFPLAPSSKSTSGGTAALGCLVKDYFPEPVTVSWNSGALTSGVHTFPAVLQSSGLYSLSSVVTVPSSSLGTQTYICNVNHKPSNTKVDKRVEPKSCDKTHTCPPCPAPEFEGGPSVFLFPPKPKDTLMISRTPEVTCVVVDVSHEDPEVKFNWYVDGVEVHNAKTKPREEQYNSTYRVVSVLTVLHQDWLNGKEYKCKVSNKALPASIEKTISKAKGQPREPQVYTLPPSREEMTKNQVSLTCLVKGFYPSDIAVEWESNGQPENNYKTTPPVLDSDGSFFLYSKLTVDKSRWQQGNVFSCSVMHEALHNHYTQKSLSLSPGK

SEQ ID NO: 5 - protein, 448 aa, synthetic construct
  REGION 1..448: note = atezolizumabMPDL3280A
EVQLVESGGGLVQPGGSLRLSCAASGFTFSDSWIHWVRQAPGKGLEWVAWISPYGGSTYYADSVKGRFTISADTSKNTAYLQMNSLRAEDTAVYYCARRHWPGGFDYWGQGTLVTVSSASTKGPSVFPLAPSSKSTSGGTAALGCLVKDYFPEPVTVSWNSGALTSGVHTFPAVLQSSGLYSLSSVVTVPSSSLGTQTYICNVNHKPSNTKVDKKVEPKSCDKTHTCPPCPAPELLGGPSVFLFPPKPKDTLMISRTPEVTCVVVDVSHEDPEVKFNWYVDGVEVHNAKTKPREEQYASTYRVVSVLTVLHQDWLNGKEYKCKVSNKALPAPIEKTISKAKGQPREPQVYTLPPSREEMTKNQVSLTCLVKGFYPSDIAVEWESNGQPENNYKTTPPVLDSDGSFFLYSKLTVDKSRWQQGNVFSCSVMHEALHNHYTQKSLSLSPGK

SEQ ID NO: 6 - protein, 450 aa, synthetic construct
  REGION 1..450: note = Avelumab(MSB0010718C)
EVQLLESGGGLVQPGGSLRLSCAASGFTFSSYIMMWVRQAPGKGLEWVSSIYPSGGITFYADTVKGRFTISRDNSKNTLYLQMNSLRAEDTAVYYCARIKLGTVTTVDYWGQGTLVTVSSASTKGPSVFPLAPSSKSTSGGTAALGCLVKDYFPEPVTVSWNSGALTSGVHTFPAVLQSSGLYSLSSVVTVPSSSLGTQTYICNVNHKPSNTKVDKKVEPKSCDKTHTCPPCPAPELLGGPSVFLFPPKPKDTLMISRTPEVTCVVVDVSHEDPEVKFNWYVDGVEVHNAKTKPREEQYNSTYRVVSVLTVLHQDWLNGKEYKCKVSNKALPAPIEKTISKAKGQPREPQVYTLPPSRDELTKNQVSLTCLVKGFYPSDIAVEWESNGQPENNYKTTPPVLDSDGSFFLYSKLTVDKSRWQQGNVFSCSVMHEALHNHYTQKSLSLSPGK

SEQ ID NO: 7 - protein, 360 aa, synthetic construct
  REGION 1..360: note = Envafolimab(KN035)
QVQLVESGGGLVQPGGSLRLSCAASGKMSSRRCMAWFRQAPGKERERVAKLLTTSGSTYLADSVKGRFTISRDNSKNTVYLQMNSLRAEDTAVYYCAADSFEDPTCTLVTSSGAFQYWGQGTLVTVSSEPKSSDKTHTCPPCPAPELLGGPSVFLFPPKPKDTLMISRTPEVTCVVVAVSHEDPEVKFNWYVDGVEVHNAKTKPREEQYNSTYRVVSVLTVLHQDWLNGKEYKCKVSNKALPAGIEKTISKAKGQPREPQVYTLPPSRDELTKNQVSLTCLVKGFYPSDIAVEWESNGQPENNYKTTPPVLDSDGSFFLYSKLTVDKSRWQQGNVFSCSVMHEALHNHYTQKSLSLSPGK

SEQ ID NO: 8 - protein, 447 aa, synthetic construct
  REGION 1..447: note = Permbrolizumab (MK-3475)
QVQLVQSGVEVKKPGASVKVSCKASGYTFTNYYMYWVRQAPGQGLEWMGGINPSNGGTNFNEKFKNRVTLTTDSSTTTAYMELKSLQFDDTAVYYCARRDYRFDMGFDYWGQGTTVTVSSASTKGPSVFPLAPCSRSTSESTAALGCLVKDYFPEPVTVSWNSGALTSGVHTFPAVLQSSGLYSLSSVVTVPSSSLGTKTYTCNVDHKPSNTKVDKRVESKYGPPCPPCPAPEFLGGPSVFLFPPKPKDTLMISRTPEVTCVVVDVSQEDPEVQFNWYVDGVEVHNAKTKPREEQFNSTYRVVSVLTVLHQDWLNGKEYKCKVSNKGLPSSIEKTISKAKGQPREPQVYTLPPSQEEMTKNQVSLTCLVKGFYPSDIAVEWESNGQPENNYKTTPPVLDSDGSFFLYSRLTVDKSRWQEGNVFSCSVMHEALHNHYTQKSLSLSLGK

SEQ ID NO: 9 - protein, 440 aa, synthetic construct
  REGION 1..440: note = Nivolumab(BMS-936558)
QVQLVESGGGVVQPGRSLRLDCKASGITFSNSGMHWVRQAPGKGLEWVAVIWYDGSKRYYADSVKGRFTISRDNSKNTLFLQMNSLRAEDTAVYYCATNDDYWGQGTLVTVSSASTKGPSVFPLAPCSRSTSESTAALGCLVKDYFPEPVTVSWNSGALTSGVHTFPAVLQSSGLYSLSSVVTVPSSSLGTKTYTCNVDHKPSNTKVDKRVESKYGPPCPPCPAPEFLGGPSVFLFPPKPKDTLMISRTPEVTCVVVDVSQEDPEVQFNWYVDGVEVHNAKTKPREEQFNSTYRVVSVLTVLHQDWLNGKEYKCKVSNKGLPSSIEKTISKAKGQPREPQVYTLPPSQEEMTKNQVSLTCLVKGFYPSDIAVEWESNGQPENNYKTTPPVLDSDGSFFLYSRLTVDKSRWQEGNVFSCSVMHEALHNHYTQKSLSLSLGK

SEQ ID NO: 10 - protein, 525 aa, synthetic construct
  REGION 1..525: note = LAG3
MWEAQFLGLLFLQPLWVAPVKPLQPGAEVPVVWAQEGAPAQLPCSPTIPLQDLSLLRRAGVTWQHQPDSGPPAAAPGHPLAPGPHPAAPSSWGPRPRRYTVLSVGPGGLRSGRLPLQPRVQLDERGRQRGDFSLWLRPARRADAGEYRAAVHLRDRALSCRLRLRLGQASMTASPPGSLRASDWVILNCSFSRPDRPASVHWFRNRGQGRVPVRESPHHHLAESFLFLPQVSPMDSGPWGCILTYRDGFNVSIMYNLTVLGLEPPTPLTVYAGAGSRVGLPCRLPAGVGTRSFLTAKWTPPGGGPDLLVTGDNGDFTLRLEDVSQAQAGTYTCHIHLQEQQLNATVTLAIITVTPKSFGSPGSLGKLLCEVTPVSGQERFVWSSLDTPSQRSFSGPWLEAQEAQLLSQPWQCQLYQGERLLGAAVYFTELSSPGAQRSGRAPGALPAGHLLLFLILGVLSLLLLVTGAFGFHLWRRQWRPRRFSALEQGIHPPQAQSKIEELEQEPEPEPEPEPEPEPEPEPEQL

SEQ ID NO: 11 - protein, 428 aa, synthetic construct
  REGION 1..428: note = LAG3
LQPGAEVPVVWAQEGAPAQLPCSPTIPLQDLSLLRRAGVTWQHQPDSGPPAAAPGHPLAPGPHPAAPSSWGPRPRRYTVLSVGPGGLRSGRLPLQPRVQLDERGRQRGDFSLWLRPARRADAGEYRAAVHLRDRALSCRLRLRLGQASMTASPPGSLRASDWVILNCSFSRPDRPASVHWFRNRGQGRVPVRESPHHHLAESFLFLPQVSPMDSGPWGCILTYRDGFNVSIMYNLTVLGLEPPTPLTVYAGAGSRVGLPCRLPAGVGTRSFLTAKWTPPGGGPDLLVTGDNGDFTLRLEDVSQAQAGTYTCHIHLQEQQLNATVTLAIITVTPKSFGSPGSLGKLLCEVTPVSGQERFVWSSLDTPSQRSFSGPWLEAQEAQLLSQPWQCQLYQGERLLGAAVYFTELSSPGAQRSGRAPGALPAGHL

SEQ ID NO: 12 - protein, 866 aa, synthetic construct
  REGION 1..866: note = LAG3
LQPGAEVPVVWAQEGAPAQLPCSPTIPLQDLSLLRRAGVTWQHQPDSGPPAAAPGHPLAPGPHPAAPSSWGPRPRRYTVLSVGPGGLRSGRLPLQPRVQLDERGRQRGDFSLWLRPARRADAGEYRAAVHLRDRALSCRLRLRLGQASMTASPPGSLRASDWVILNCSFSRPDRPASVHWFRNRGQGRVPVRESPHHHLAESFLFLPQVSPMDSGPWGCILTYRDGFNVSIMYNLTVLGLEPPTPLTVYAGAGSRVGLPCRLPAGVGTRSFLTAKWTPPGGGPDLLVTGDNGDFTLRLEDVSQAQAGTYTCHIHLQEQQLNATVTLAIITVTPKSFGSPGSLGKLLCEVTPVSGQERFVWSSLDTPSQRSFSGPWLEAQEAQLLSQPWQCQLYQGERLLGAAVYFTELSSPGAQRSGRAPGALPAGHLGGGGSGGGGSLQPGAEVPVVWAQEGAPAQLPCSPTIPLQDLSLLRRAGVTWQHQPDSGPPAAAPGHPLAPGPHPAAPSSWGPRPRRYTVLSVGPGGLRSGRLPLQPRVQLDERGRQRGDFSLWLRPARRADAGEYRAAVHLRDRALSCRLRLRLGQASMTASPPGSLRASDWVILNCSFSRPDRPASVHWFRNRGQGRVPVRESPHHHLAESFLFLPQVSPMDSGPWGCILTYRDGFNVSIMYNLTVLGLEPPTPLTVYAGAGSRVGLPCRLPAGVGTRSFLTAKWTPPGGGPDLLVTGDNGDFTLRLEDVSQAQAGTYTCHIHLQEQQLNATVTLAIITVTPKSFGSPGSLGKLLCEVTPVSGQERFVWSSLDTPSQRSFSGPWLEAQEAQLLSQPWQCQLYQGERLLGAAVYFTELSSPGAQRSGRAPGALPAGHL

SEQ ID NO: 13 - protein, 131 aa, synthetic construct
  REGION 1..131: note = LAG3-IgD1
GAPAQLPCSPTIPLQDLSLLRRAGVTWQHQPDSGPPAAAPGHPLAPGPHPAAPSSWGPRPRRYTVLSVGPGGLRSGRLPLQPRVQLDERGRQRGDFSLWLRPARRADAGEYRAAVHLRDRALSCRLRLRLG

SEQ ID NO: 14 - protein, 85 aa, synthetic construct
  REGION 1..85: note = LAG3-IgD2
QASMTASPPGSLRASDWVILNCSFSRPDRPASVHWFRNRGQGRVPVRESPHHHLAESFLFLPQVSPMDSGPWGCILTYRDGFNVS

SEQ ID NO: 15 - protein, 79 aa, synthetic construct
  REGION 1..79: note = LAG3-IgD3
PTPLTVYAGAGSRVGLPCRLPAGVGTRSFLTAKWTPPGGGPDLLVTGDNGDFTLRLEDVSQAQAGTYTCHIHLQEQQLN

SEQ ID NO: 16 - protein, 72 aa, synthetic construct
  REGION 1..72: note = LAG3-IgD4
LAIITVTPKSFGSPGSLGKLLCEVTPVSGQERFVWSSLDTPSQRSFSGPWLEAQEAQLLSQPWQCQLYQGER

SEQ ID NO: 17 - protein, 216 aa, synthetic construct
  REGION 1..216: note = LAG3-IgD1/IgD2
GAPAQLPCSPTIPLQDLSLLRRAGVTWQHQPDSGPPAAAPGHPLAPGPHPAAPSSWGPRPRRYTVLSVGPGGLRSGRLPLQPRVQLDERGRQRGDFSLWLRPARRADAGEYRAAVHLRDRALSCRLRLRLGQASMTASPPGSLRASDWVILNCSFSRPDRPASVHWFRNRGQGRVPVRESPHHHLAESFLFLPQVSPMDSGPWGCILTYRDGFNVS

SEQ ID NO: 18 - protein, 307 aa, synthetic construct
  REGION 1..307: note = LAG3-IgD1/IgD2/IgD3
GAPAQLPCSPTIPLQDLSLLRRAGVTWQHQPDSGPPAAAPGHPLAPGPHPAAPSSWGPRPRRYTVLSVGPGGLRSGRLPLQPRVQLDERGRQRGDFSLWLRPARRADAGEYRAAVHLRDRALSCRLRLRLGQASMTASPPGSLRASDWVILNCSFSRPDRPASVHWFRNRGQGRVPVRESPHHHLAESFLFLPQVSPMDSGPWGCILTYRDGFNVSIMYNLTVLGLEPPTPLTVYAGAGSRVGLPCRLPAGVGTRSFLTAKWTPPGGGPDLLVTGDNGDFTLRLEDVSQAQAGTYTCHIHLQEQQLN

SEQ ID NO: 19 - protein, 383 aa, synthetic construct
  REGION 1..383: note = LAG3-IgD1/IgD2/IgD3/IgD4
GAPAQLPCSPTIPLQDLSLLRRAGVTWQHQPDSGPPAAAPGHPLAPGPHPAAPSSWGPRPRRYTVLSVGPGGLRSGRLPLQPRVQLDERGRQRGDFSLWLRPARRADAGEYRAAVHLRDRALSCRLRLRLGQASMTASPPGSLRASDWVILNCSFSRPDRPASVHWFRNRGQGRVPVRESPHHHLAESFLFLPQVSPMDSGPWGCILTYRDGFNVSIMYNLTVLGLEPPTPLTVYAGAGSRVGLPCRLPAGVGTRSFLTAKWTPPGGGPDLLVTGDNGDFTLRLEDVSQAQAGTYTCHIHLQEQQLNATVTLAIITVTPKSFGSPGSLGKLLCEVTPVSGQERFVWSSLDTPSQRSFSGPWLEAQEAQLLSQPWQCQLYQGER

SEQ ID NO: 20 - protein, 232 aa, synthetic construct
  REGION 1..232: note = IgG1Fc
EPKSCDKTHTCPPCPAPELLGGPSVFLFPPKPKDTLMISRTPEVTCVVVDVSHEDPEVKFNWYVDGVEVHNAKTKPREEQYNSTYRVVSVLTVLHQDWLNGKEYKCKVSNKALPAPIEKTISKAKGQPREPQVYTLPPSRDELTKNQVSLTCLVKGFYPSDIAVEWESNGQPENNYKTTPPVLDSDGSFFLYSKLTVDKSRWQQGNVFSCSVMHEALHNHYTQKSLSLSPGK

SEQ ID NO: 21 - protein, 229 aa, synthetic construct
  REGION 1..229: note = IgG4Fc
ESKYGPPCPSCPAPEFLGGPSVFLFPPKPKDTLMISRTPEVTCVVVDVSQEDPEVQFNWYVDGVEVHNAKTKPREEQFNSTYRVVSVLTVLHQDWLNGKEYKCKVSNKGLPSSIEKTISKAKGQPREPQVYTLPPSQEEMTKNQVSLTCLVKGFYPSDIAVEWESNGQPENNYKTTPPVLDSDGSFFLYSRLTVDKSRWQEGNVFSCSVMHEALHNHYTQKSLSLSLGK

SEQ ID NO: 22 - protein, 5 aa, synthetic construct
  REGION 1..5: note = GGGGS linker
GGGGS

SEQ ID NO: 23 - protein, 10 aa, synthetic construct
  REGION 1..10: note = GGGGSGGGGS linker
GGGGSGGGGS

SEQ ID NO: 24 - protein, 15 aa, synthetic construct
  REGION 1..15: note = GGGGSGGGGSGGGGS linker
GGGGSGGGGSGGGGS

SEQ ID NO: 25 - protein, 20 aa, synthetic construct
  REGION 1..20: note = GGGGSGGGGSGGGGSGGGGSlinker
GGGGSGGGGSGGGGSGGGGS

SEQ ID NO: 26 - protein, 9 aa, synthetic construct
  REGION 1..9: note = GGGGSGGGSlinker
GGGGSGGGS

SEQ ID NO: 27 - protein, 677 aa, synthetic construct
  REGION 1..677: note = AN_Bif_Abs_0017
EVQLLESGGGLVQPGGSLRLSCAASGFTFSSYAMSWVRQAPGKGLEWVSGISGSGGFTYYADSVKGRFTISRDNSKNTLYLQMNSLRAEDTAVYYCAKPPRGYNYGPFDYWGQGTLVTVSSASTKGPSVFPLAPCSRSTSESTAALGCLVKDYFPEPVTVSWNSGALTSGVHTFPAVLQSSGLYSLSSVVTVPSSSLGTKTYTCNVDHKPSNTKVDKRVESKYGPPCPPCPAPEFLGGPSVFLFPPKPKDTLMISRTPEVTCVVVDVSQEDPEVQFNWYVDGVEVHNAKTKPREEQFNSTYRVVSVLTVLHQDWLNGKEYKCKVSNKGLPSSIEKTISKAKGQPREPQVYTLPPSQEEMTKNQVSLTCLVKGFYPSDIAVEWESNGQPENNYKTTPPVLDSDGSFFLYSRLTVDKSRWQEGNVFSCSVMHEALHNHYTQKSLSLSLGAGGGGSGGGGSGGGGSGGGGSGVIHVTKEVKEVATLSCGHNVSVEELAQTRIYWQKEKKMVLTMMSGDMNIWPEYKNRTIFDITNNLSIVILALRPSDEGTYECVVLKYEKDAFKREHLAEVTLSVKADFPTPSISDFEIPTSNIRRIICSTSGGFPEPHLSWLENGEELNAINTTVSQDPETELYAVSSKLDFNMTTNHSFMCLIKYGHLRVNQTFNWNTTKQEHFPDN

SEQ ID NO: 28 - protein, 875 aa, synthetic construct
  REGION 1..875: note = AN_Bif_Abs_0019
EVQLLESGGGLVQPGGSLRLSCAASGFTFSSYAMSWVRQAPGKGLEWVSGISGSGGFTYYADSVKGRFTISRDNSKNTLYLQMNSLRAEDTAVYYCAKPPRGYNYGPFDYWGQGTLVTVSSASTKGPSVFPLAPCSRSTSESTAALGCLVKDYFPEPVTVSWNSGALTSGVHTFPAVLQSSGLYSLSSVVTVPSSSLGTKTYTCNVDHKPSNTKVDKRVESKYGPPCPPCPAPEFLGGPSVFLFPPKPKDTLMISRTPEVTCVVVDVSQEDPEVQFNWYVDGVEVHNAKTKPREEQFNSTYRVVSVLTVLHQDWLNGKEYKCKVSNKGLPSSIEKTISKAKGQPREPQVYTLPPSQEEMTKNQVSLTCLVKGFYPSDIAVEWESNGQPENNYKTTPPVLDSDGSFFLYSRLTVDKSRWQEGNVFSCSVMHEALHNHYTQKSLSLSLGAGGGGSGGGGSGGGGSGGGGSGLQPGAEVPVVWAQEGAPAQLPCSPTIPLQDLSLLRRAGVTWQHQPDSGPPAAAPGHPLAPGPHPAAPSSWGPRPRRYTVLSVGPGGLRSGRLPLQPRVQLDERGRQRGDFSLWLRPARRADAGEYRAAVHLRDRALSCRLRLRLGQASMTASPPGSLRASDWVILNCSFSRPDRPASVHWFRNRGQGRVPVRESPHHHLAESFLFLPQVSPMDSGPWGCILTYRDGFNVSIMYNLTVLGLEPPTPLTVYAGAGSRVGLPCRLPAGVGTRSFLTAKWTPPGGGPDLLVTGDNGDFTLRLEDVSQAQAGTYTCHIHLQEQQLNATVTLAIITVTPKSFGSPGSLGKLLCEVTPVSGQERFVWSSLDTPSQRSFSGPWLEAQEAQLLSQPWQCQLYQGERLLGAAVYFT

SEQ ID NO: 29 - protein, 711 aa, synthetic construct
  REGION 1..711: note = sugemalimab-LAG3 IgD1/D2
EVQLLESGGGLVQPGGSLRLSCAASGFTFSSYAMSWVRQAPGKGLEWVSGISGSGGFTYYADSVKGRFTISRDNSKNTLYLQMNSLRAEDTAVYYCAKPPRGYNYGPFDYWGQGTLVTVSSASTKGPSVFPLAPCSRSTSESTAALGCLVKDYFPEPVTVSWNSGALTSGVHTFPAVLQSSGLYSLSSVVTVPSSSLGTKTYTCNVDHKPSNTKVDKRVESKYGPPCPPCPAPEFLGGPSVFLFPPKPKDTLMISRTPEVTCVVVDVSQEDPEVQFNWYVDGVEVHNAKTKPREEQFNSTYRVVSVLTVLHQDWLNGKEYKCKVSNKGLPSSIEKTISKAKGQPREPQVYTLPPSQEEMTKNQVSLTCLVKGFYPSDIAVEWESNGQPENNYKTTPPVLDSDGSFFLYSRLTVDKSRWQEGNVFSCSVMHEALHNHYTQKSLSLSLGAGGGGSGGGGSGGGGSGGGGSGLQPGAEVPVVWAQEGAPAQLPCSPTIPLQDLSLLRRAGVTWQHQPDSGPPAAAPGHPLAPGPHPAAPSSWGPRPRRYTVLSVGPGGLRSGRLPLQPRVQLDERGRQRGDFSLWLRPARRADAGEYRAAVHLRDRALSCRLRLRLGQASMTASPPGSLRASDWVILNCSFSRPDRPASVHWFRNRGQGRVPVRESPHHHLAESFLFLPQVSPMDSGPWGCILTYRDGFNVSIMYNLTVLGLEP

SEQ ID NO: 30 - protein, 794 aa, synthetic construct
  REGION 1..794: note = sugemalimab-LAG3 IgD1/D2/D3
EVQLLESGGGLVQPGGSLRLSCAASGFTFSSYAMSWVRQAPGKGLEWVSGISGSGGFTYYADSVKGRFTISRDNSKNTLYLQMNSLRAEDTAVYYCAKPPRGYNYGPFDYWGQGTLVTVSSASTKGPSVFPLAPCSRSTSESTAALGCLVKDYFPEPVTVSWNSGALTSGVHTFPAVLQSSGLYSLSSVVTVPSSSLGTKTYTCNVDHKPSNTKVDKRVESKYGPPCPPCPAPEFLGGPSVFLFPPKPKDTLMISRTPEVTCVVVDVSQEDPEVQFNWYVDGVEVHNAKTKPREEQFNSTYRVVSVLTVLHQDWLNGKEYKCKVSNKGLPSSIEKTISKAKGQPREPQVYTLPPSQEEMTKNQVSLTCLVKGFYPSDIAVEWESNGQPENNYKTTPPVLDSDGSFFLYSRLTVDKSRWQEGNVFSCSVMHEALHNHYTQKSLSLSLGAGGGGSGGGGSGGGGSGGGGSGLQPGAEVPVVWAQEGAPAQLPCSPTIPLQDLSLLRRAGVTWQHQPDSGPPAAAPGHPLAPGPHPAAPSSWGPRPRRYTVLSVGPGGLRSGRLPLQPRVQLDERGRQRGDFSLWLRPARRADAGEYRAAVHLRDRALSCRLRLRLGQASMTASPPGSLRASDWVILNCSFSRPDRPASVHWFRNRGQGRVPVRESPHHHLAESFLFLPQVSPMDSGPWGCILTYRDGFNVSIMYNLTVLGLEPPTPLTVYAGAGSRVGLPCRLPAGVGTRSFLTAKWTPPGGGPDLLVTGDNGDFTLRLEDVSQAQAGTYTCHIHLQEQQLNATVT

SEQ ID NO: 31 - protein, 677 aa, synthetic construct
  REGION 1..677: note = CD80-sugemalimab
VIHVTKEVKEVATLSCGHNVSVEELAQTRIYWQKEKKMVLTMMSGDMNIWPEYKNRTIFDITNNLSIVILALRPSDEGTYECVVLKYEKDAFKREHLAEVTLSVKADFPTPSISDFEIPTSNIRRIICSTSGGFPEPHLSWLENGEELNAINTTVSQDPETELYAVSSKLDFNMTTNHSFMCLIKYGHLRVNQTFNWNTTKQEHFPDNGGGGSGGGGSGGGGSGGGGSGEVQLLESGGGLVQPGGSLRLSCAASGFTFSSYAMSWVRQAPGKGLEWVSGISGSGGFTYYADSVKGRFTISRDNSKNTLYLQMNSLRAEDTAVYYCAKPPRGYNYGPFDYWGQGTLVTVSSASTKGPSVFPLAPCSRSTSESTAALGCLVKDYFPEPVTVSWNSGALTSGVHTFPAVLQSSGLYSLSSVVTVPSSSLGTKTYTCNVDHKPSNTKVDKRVESKYGPPCPPCPAPEFLGGPSVFLFPPKPKDTLMISRTPEVTCVVVDVSQEDPEVQFNWYVDGVEVHNAKTKPREEQFNSTYRVVSVLTVLHQDWLNGKEYKCKVSNKGLPSSIEKTISKAKGQPREPQVYTLPPSQEEMTKNQVSLTCLVKGFYPSDIAVEWESNGQPENNYKTTPPVLDSDGSFFLYSRLTVDKSRWQEGNVFSCSVMHEALHNHYTQKSLSLSLGK

SEQ ID NO: 32 - protein, 875 aa, synthetic construct
  REGION 1..875: note = AN_Bif_Abs_0035
LQPGAEVPVVWAQEGAPAQLPCSPTIPLQDLSLLRRAGVTWQHQPDSGPPAAAPGHPLAPGPHPAAPSSWGPRPRRYTVLSVGPGGLRSGRLPLQPRVQLDERGRQRGDFSLWLRPARRADAGEYRAAVHLRDRALSCRLRLRLGQASMTASPPGSLRASDWVILNCSFSRPDRPASVHWFRNRGQGRVPVRESPHHHLAESFLFLPQVSPMDSGPWGCILTYRDGFNVSIMYNLTVLGLEPPTPLTVYAGAGSRVGLPCRLPAGVGTRSFLTAKWTPPGGGPDLLVTGDNGDFTLRLEDVSQAQAGTYTCHIHLQEQQLNATVTLAIITVTPKSFGSPGSLGKLLCEVTPVSGQERFVWSSLDTPSQRSFSGPWLEAQEAQLLSQPWQCQLYQGERLLGAAVYFTGGGGSGGGGSGGGGSGGGGSGEVQLLESGGGLVQPGGSLRLSCAASGFTFSSYAMSWVRQAPGKGLEWVSGISGSGGFTYYADSVKGRFTISRDNSKNTLYLQMNSLRAEDTAVYYCAKPPRGYNYGPFDYWGQGTLVTVSSASTKGPSVFPLAPCSRSTSESTAALGCLVKDYFPEPVTVSWNSGALTSGVHTFPAVLQSSGLYSLSSVVTVPSSSLGTKTYTCNVDHKPSNTKVDKRVESKYGPPCPPCPAPEFLGGPSVFLFPPKPKDTLMISRTPEVTCVVVDVSQEDPEVQFNWYVDGVEVHNAKTKPREEQFNSTYRVVSVLTVLHQDWLNGKEYKCKVSNKGLPSSIEKTISKAKGQPREPQVYTLPPSQEEMTKNQVSLTCLVKGFYPSDIAVEWESNGQPENNYKTTPPVLDSDGSFFLYSRLTVDKSRWQEGNVFSCSVMHEALHNHYTQKSLSLSLGK

SEQ ID NO: 33 - protein, 443 aa, synthetic construct
  REGION 1..443: note = CD80-sugemalimab
VIHVTKEVKEVATLSCGHNVSVEELAQTRIYWQKEKKMVLTMMSGDMNIWPEYKNRTIFDITNNLSIVILALRPSDEGTYECVVLKYEKDAFKREHLAEVTLSVKADFPTPSISDFEIPTSNIRRIICSTSGGFPEPHLSWLENGEELNAINTTVSQDPETELYAVSSKLDFNMTTNHSFMCLIKYGHLRVNQTFNWNTTKQEHFPDNGGGGSGGGGSGGGGSGGGGSGSYVLTQPPSVSVAPGQTARITCGGNNIGSKSVHWYQQKPGQAPVLVVYDDSDRPSGIPERFSGSNSGNTATLTISRVEAGDEADYYCQVWDSSSDHVVFGGGTKLTVLGQPKAAPSVTLFPPSSEELQANKATLVCLISDFYPGAVTVAWKADSSPVKAGVETTTPSKQSNNKYAASSYLSLTPEQWKSHRSYSCQVTHEGSTVEKTVAPTECS

SEQ ID NO: 34 - protein, 641 aa, synthetic construct
  REGION 1..641: note = LAG3-sugemalimab
LQPGAEVPVVWAQEGAPAQLPCSPTIPLQDLSLLRRAGVTWQHQPDSGPPAAAPGHPLAPGPHPAAPSSWGPRPRRYTVLSVGPGGLRSGRLPLQPRVQLDERGRQRGDFSLWLRPARRADAGEYRAAVHLRDRALSCRLRLRLGQASMTASPPGSLRASDWVILNCSFSRPDRPASVHWFRNRGQGRVPVRESPHHHLAESFLFLPQVSPMDSGPWGCILTYRDGFNVSIMYNLTVLGLEPPTPLTVYAGAGSRVGLPCRLPAGVGTRSFLTAKWTPPGGGPDLLVTGDNGDFTLRLEDVSQAQAGTYTCHIHLQEQQLNATVTLAIITVTPKSFGSPGSLGKLLCEVTPVSGQERFVWSSLDTPSQRSFSGPWLEAQEAQLLSQPWQCQLYQGERLLGAAVYFTGGGGSGGGGSGGGGSGGGGSGSYVLTQPPSVSVAPGQTARITCGGNNIGSKSVHWYQQKPGQAPVLVVYDDSDRPSGIPERFSGSNSGNTATLTISRVEAGDEADYYCQVWDSSSDHVVFGGGTKLTVLGQPKAAPSVTLFPPSSEELQANKATLVCLISDFYPGAVTVAWKADSSPVKAGVETTTPSKQSNNKYAASSYLSLTPEQWKSHRSYSCQVTHEGSTVEKTVAPTECS

SEQ ID NO: 35 - protein, 921 aa, synthetic construct
  REGION 1..921: note = AN_Bif_Abs_0052
EVQLLESGGGLVQPGGSLRLSCAASGFTFSSYAMSWVRQAPGKGLEWVSGISGSGGFTYYADSVKGRFTISRDNSKNTLYLQMNSLRAEDTAVYYCAKPPRGYNYGPFDYWGQGTLVTVSSASTKGPSVFPLAPCSRSTSESTAALGCLVKDYFPEPVTVSWNSGALTSGVHTFPAVLQSSGLYSLSSVVTVPSSSLGTKTYTCNVDHKPSNTKVDKRVESKYGPPCPPCPAPEFLGGPSVFLFPPKPKDTLMISRTPEVTCVVVDVSQEDPEVQFNWYVDGVEVHNAKTKPREEQFNSTYRVVSVLTVLHQDWLNGKEYKCKVSNKGLPSSIEKTISKAKGQPREPQVYTLPPSQEEMTKNQVSLTCLVKGFYPSDIAVEWESNGQPENNYKTTPPVLDSDGSFFLYSRLTVDKSRWQEGNVFSCSVMHEALHNHYTQKSLSLSLGAGGGGSGGGGSGVIHVTKEVKEVATLSCGHNVSVEELAQTRIYWQKEKKMVLTMMSGDMNIWPEYKNRTIFDITNNLSIVILALRPSDEGTYECVVLKYEKDAFKREHLAEVTLSVKADFPTPSISDFEIPTSNIRRIICSTSGGFPEPHLSWLENGEELNAINTTVSQDPETELYAVSSKLDFNMTTNHSFMCLIKYGHLRVNQTFNWNTTKQEHFPDNGGGGSGGGGSGSLQPGAEVPVVWAQEGAPAQLPCSPTIPLQDLSLLRRAGVTWQHQPDSGPPAAAPGHPLAPGPHPAAPSSWGPRPRRYTVLSVGPGGLRSGRLPLQPRVQLDERGRQRGDFSLWLRPARRADAGEYRAAVHLRDRALSCRLRLRLGQASMTASPPGSLRASDWVILNCSFSRPDRPASVHWFRNRGQGRVPVRESPHHHLAESFLFLPQVSPMDSGPWGCILTYRDGFNVSIMYNLTVLGLEP

SEQ ID NO: 36 - protein, 1003 aa, synthetic construct
  REGION 1..1003: note = AN_Bif_Abs_0051
EVQLLESGGGLVQPGGSLRLSCAASGFTFSSYAMSWVRQAPGKGLEWVSGISGSGGFTYYADSVKGRFTISRDNSKNTLYLQMNSLRAEDTAVYYCAKPPRGYNYGPFDYWGQGTLVTVSSASTKGPSVFPLAPCSRSTSESTAALGCLVKDYFPEPVTVSWNSGALTSGVHTFPAVLQSSGLYSLSSVVTVPSSSLGTKTYTCNVDHKPSNTKVDKRVESKYGPPCPPCPAPEFLGGPSVFLFPPKPKDTLMISRTPEVTCVVVDVSQEDPEVQFNWYVDGVEVHNAKTKPREEQFNSTYRVVSVLTVLHQDWLNGKEYKCKVSNKGLPSSIEKTISKAKGQPREPQVYTLPPSQEEMTKNQVSLTCLVKGFYPSDIAVEWESNGQPENNYKTTPPVLDSDGSFFLYSRLTVDKSRWQEGNVFSCSVMHEALHNHYTQKSLSLSLGAGGGGSGGGGSGVIHVTKEVKEVATLSCGHNVSVEELAQTRIYWQKEKKMVLTMMSGDMNIWPEYKNRTIFDITNNLSIVILALRPSDEGTYECVVLKYEKDAFKREHLAEVTLSVKADFPTPSISDFEIPTSNIRRIICSTSGGFPEPHLSWLENGEELNAINTTVSQDPETELYAVSSKLDFNMTTNHSFMCLIKYGHLRVNQTFNWNTTKQEHFPDNGGGGSGGGGSGLQPGAEVPVVWAQEGAPAQLPCSPTIPLQDLSLLRRAGVTWQHQPDSGPPAAAPGHPLAPGPHPAAPSSWGPRPRRYTVLSVGPGGLRSGRLPLQPRVQLDERGRQRGDFSLWLRPARRADAGEYRAAVHLRDRALSCRLRLRLGQASMTASPPGSLRASDWVILNCSFSRPDRPASVHWFRNRGQGRVPVRESPHHHLAESFLFLPQVSPMDSGPWGCILTYRDGFNVSIMYNLTVLGLEPPTPLTVYAGAGSRVGLPCRLPAGVGTRSFLTAKWTPPGGGPDLLVTGDNGDFTLRLEDVSQAQAGTYTCHIHLQEQQLNATVT

SEQ ID NO: 37 - protein, 1103 aa, synthetic construct
  REGION 1..1103: note = AN_Bif_Abs_0038
EVQLLESGGGLVQPGGSLRLSCAASGFTFSSYAMSWVRQAPGKGLEWVSGISGSGGFTYYADSVKGRFTISRDNSKNTLYLQMNSLRAEDTAVYYCAKPPRGYNYGPFDYWGQGTLVTVSSASTKGPSVFPLAPCSRSTSESTAALGCLVKDYFPEPVTVSWNSGALTSGVHTFPAVLQSSGLYSLSSVVTVPSSSLGTKTYTCNVDHKPSNTKVDKRVESKYGPPCPPCPAPEFLGGPSVFLFPPKPKDTLMISRTPEVTCVVVDVSQEDPEVQFNWYVDGVEVHNAKTKPREEQFNSTYRVVSVLTVLHQDWLNGKEYKCKVSNKGLPSSIEKTISKAKGQPREPQVYTLPPSQEEMTKNQVSLTCLVKGFYPSDIAVEWESNGQPENNYKTTPPVLDSDGSFFLYSRLTVDKSRWQEGNVFSCSVMHEALHNHYTQKSLSLSLGAGGGGSGGGGSGGGGSGGGSGVIHVTKEVKEVATLSCGHNVSVEELAQTRIYWQKEKKMVLTMMSGDMNIWPEYKNRTIFDITNNLSIVILALRPSDEGTYECVVLKYEKDAFKREHLAEVTLSVKADFPTPSISDFEIPTSNIRRIICSTSGGFPEPHLSWLENGEELNAINTTVSQDPETELYAVSSKLDFNMTTNHSFMCLIKYGHLRVNQTFNWNTTKQEHFPDNGGGGSGGGGSGGGGSGGGGSGLQPGAEVPVVWAQEGAPAQLPCSPTIPLQDLSLLRRAGVTWQHQPDSGPPAAAPGHPLAPGPHPAAPSSWGPRPRRYTVLSVGPGGLRSGRLPLQPRVQLDERGRQRGDFSLWLRPARRADAGEYRAAVHLRDRALSCRLRLRLGQASMTASPPGSLRASDWVILNCSFSRPDRPASVHWFRNRGQGRVPVRESPHHHLAESFLFLPQVSPMDSGPWGCILTYRDGFNVSIMYNLTVLGLEPPTPLTVYAGAGSRVGLPCRLPAGVGTRSFLTAKWTPPGGGPDLLVTGDNGDFTLRLEDVSQAQAGTYTCHIHLQEQQLNATVTLAIITVTPKSFGSPGSLGKLLCEVTPVSGQERFVWSSLDTPSQRSFSGPWLEAQEAQLLSQPWQCQLYQGERLLGAAVYFT

SEQ ID NO: 38 - protein, 921 aa, synthetic construct
  REGION 1..921: note = sugemalimab-LAG3 IgD1/D2-CD80
EVQLLESGGGLVQPGGSLRLSCAASGFTFSSYAMSWVRQAPGKGLEWVSGISGSGGFTYYADSVKGRFTISRDNSKNTLYLQMNSLRAEDTAVYYCAKPPRGYNYGPFDYWGQGTLVTVSSASTKGPSVFPLAPCSRSTSESTAALGCLVKDYFPEPVTVSWNSGALTSGVHTFPAVLQSSGLYSLSSVVTVPSSSLGTKTYTCNVDHKPSNTKVDKRVESKYGPPCPPCPAPEFLGGPSVFLFPPKPKDTLMISRTPEVTCVVVDVSQEDPEVQFNWYVDGVEVHNAKTKPREEQFNSTYRVVSVLTVLHQDWLNGKEYKCKVSNKGLPSSIEKTISKAKGQPREPQVYTLPPSQEEMTKNQVSLTCLVKGFYPSDIAVEWESNGQPENNYKTTPPVLDSDGSFFLYSRLTVDKSRWQEGNVFSCSVMHEALHNHYTQKSLSLSLGAGGGGSGGGGSGSLQPGAEVPVVWAQEGAPAQLPCSPTIPLQDLSLLRRAGVTWQHQPDSGPPAAAPGHPLAPGPHPAAPSSWGPRPRRYTVLSVGPGGLRSGRLPLQPRVQLDERGRQRGDFSLWLRPARRADAGEYRAAVHLRDRALSCRLRLRLGQASMTASPPGSLRASDWVILNCSFSRPDRPASVHWFRNRGQGRVPVRESPHHHLAESFLFLPQVSPMDSGPWGCILTYRDGFNVSIMYNLTVLGLEPGGGGSGGGGSGVIHVTKEVKEVATLSCGHNVSVEELAQTRIYWQKEKKMVLTMMSGDMNIWPEYKNRTIFDITNNLSIVILALRPSDEGTYECVVLKYEKDAFKREHLAEVTLSVKADFPTPSISDFEIPTSNIRRIICSTSGGFPEPHLSWLENGEELNAINTTVSQDPETELYAVSSKLDFNMTTNHSFMCLIKYGHLRVNQTFNWNTTKQEHFPDN

SEQ ID NO: 39 - protein, 1003 aa, synthetic construct
  REGION 1..1003: note = sugemalimab-LAG3 IgD1/D2/D3-CD80
EVQLLESGGGLVQPGGSLRLSCAASGFTFSSYAMSWVRQAPGKGLEWVSGISGSGGFTYYADSVKGRFTISRDNSKNTLYLQMNSLRAEDTAVYYCAKPPRGYNYGPFDYWGQGTLVTVSSASTKGPSVFPLAPCSRSTSESTAALGCLVKDYFPEPVTVSWNSGALTSGVHTFPAVLQSSGLYSLSSVVTVPSSSLGTKTYTCNVDHKPSNTKVDKRVESKYGPPCPPCPAPEFLGGPSVFLFPPKPKDTLMISRTPEVTCVVVDVSQEDPEVQFNWYVDGVEVHNAKTKPREEQFNSTYRVVSVLTVLHQDWLNGKEYKCKVSNKGLPSSIEKTISKAKGQPREPQVYTLPPSQEEMTKNQVSLTCLVKGFYPSDIAVEWESNGQPENNYKTTPPVLDSDGSFFLYSRLTVDKSRWQEGNVFSCSVMHEALHNHYTQKSLSLSLGAGGGGSGGGGSGLQPGAEVPVVWAQEGAPAQLPCSPTIPLQDLSLLRRAGVTWQHQPDSGPPAAAPGHPLAPGPHPAAPSSWGPRPRRYTVLSVGPGGLRSGRLPLQPRVQLDERGRQRGDFSLWLRPARRADAGEYRAAVHLRDRALSCRLRLRLGQASMTASPPGSLRASDWVILNCSFSRPDRPASVHWFRNRGQGRVPVRESPHHHLAESFLFLPQVSPMDSGPWGCILTYRDGFNVSIMYNLTVLGLEPPTPLTVYAGAGSRVGLPCRLPAGVGTRSFLTAKWTPPGGGPDLLVTGDNGDFTLRLEDVSQAQAGTYTCHIHLQEQQLNATVTGGGGSGGGGSGVIHVTKEVKEVATLSCGHNVSVEELAQTRIYWQKEKKMVLTMMSGDMNIWPEYKNRTIFDITNNLSIVILALRPSDEGTYECVVLKYEKDAFKREHLAEVTLSVKADFPTPSISDFEIPTSNIRRIICSTSGGFPEPHLSWLENGEELNAINTTVSQDPETELYAVSSKLDFNMTTNHSFMCLIKYGHLRVNQTFNWNTTKQEHFPDN

SEQ ID NO: 40 - protein, 1103 aa, synthetic construct
  REGION 1..1103: note = AN_Bif_Abs_0037
EVQLLESGGGLVQPGGSLRLSCAASGFTFSSYAMSWVRQAPGKGLEWVSGISGSGGFTYYADSVKGRFTISRDNSKNTLYLQMNSLRAEDTAVYYCAKPPRGYNYGPFDYWGQGTLVTVSSASTKGPSVFPLAPCSRSTSESTAALGCLVKDYFPEPVTVSWNSGALTSGVHTFPAVLQSSGLYSLSSVVTVPSSSLGTKTYTCNVDHKPSNTKVDKRVESKYGPPCPPCPAPEFLGGPSVFLFPPKPKDTLMISRTPEVTCVVVDVSQEDPEVQFNWYVDGVEVHNAKTKPREEQFNSTYRVVSVLTVLHQDWLNGKEYKCKVSNKGLPSSIEKTISKAKGQPREPQVYTLPPSQEEMTKNQVSLTCLVKGFYPSDIAVEWESNGQPENNYKTTPPVLDSDGSFFLYSRLTVDKSRWQEGNVFSCSVMHEALHNHYTQKSLSLSLGAGGGGSGGGGSGGGGSGGGGSGLQPGAEVPVVWAQEGAPAQLPCSPTIPLQDLSLLRRAGVTWQHQPDSGPPAAAPGHPLAPGPHPAAPSSWGPRPRRYTVLSVGPGGLRSGRLPLQPRVQLDERGRQRGDFSLWLRPARRADAGEYRAAVHLRDRALSCRLRLRLGQASMTASPPGSLRASDWVILNCSFSRPDRPASVHWFRNRGQGRVPVRESPHHHLAESFLFLPQVSPMDSGPWGCILTYRDGFNVSIMYNLTVLGLEPPTPLTVYAGAGSRVGLPCRLPAGVGTRSFLTAKWTPPGGGPDLLVTGDNGDFTLRLEDVSQAQAGTYTCHIHLQEQQLNATVTLAIITVTPKSFGSPGSLGKLLCEVTPVSGQERFVWSSLDTPSQRSFSGPWLEAQEAQLLSQPWQCQLYQGERLLGAAVYFTGGGGSGGGGSGGGGSGGGSGVIHVTKEVKEVATLSCGHNVSVEELAQTRIYWQKEKKMVLTMMSGDMNIWPEYKNRTIFDITNNLSIVILALRPSDEGTYECVVLKYEKDAFKREHLAEVTLSVKADFPTPSISDFEIPTSNIRRIICSTSGGFPEPHLSWLENGEELNAINTTVSQDPETELYAVSSKLDFNMTTNHSFMCLIKYGHLRVNQTFNWNTTKQEHFPDN

SEQ ID NO: 41 - protein, 1103 aa, synthetic construct
  REGION 1..1103: note = AN_Bif_Abs_0036
LQPGAEVPVVWAQEGAPAQLPCSPTIPLQDLSLLRRAGVTWQHQPDSGPPAAAPGHPLAPGPHPAAPSSWGPRPRRYTVLSVGPGGLRSGRLPLQPRVQLDERGRQRGDFSLWLRPARRADAGEYRAAVHLRDRALSCRLRLRLGQASMTASPPGSLRASDWVILNCSFSRPDRPASVHWFRNRGQGRVPVRESPHHHLAESFLFLPQVSPMDSGPWGCILTYRDGFNVSIMYNLTVLGLEPPTPLTVYAGAGSRVGLPCRLPAGVGTRSFLTAKWTPPGGGPDLLVTGDNGDFTLRLEDVSQAQAGTYTCHIHLQEQQLNATVTLAIITVTPKSFGSPGSLGKLLCEVTPVSGQERFVWSSLDTPSQRSFSGPWLEAQEAQLLSQPWQCQLYQGERLLGAAVYFTGGGGSGGGGSGGGGSGGGSGEVQLLESGGGLVQPGGSLRLSCAASGFTFSSYAMSWVRQAPGKGLEWVSGISGSGGFTYYADSVKGRFTISRDNSKNTLYLQMNSLRAEDTAVYYCAKPPRGYNYGPFDYWGQGTLVTVSSASTKGPSVFPLAPCSRSTSESTAALGCLVKDYFPEPVTVSWNSGALTSGVHTFPAVLQSSGLYSLSSVVTVPSSSLGTKTYTCNVDHKPSNTKVDKRVESKYGPPCPPCPAPEFLGGPSVFLFPPKPKDTLMISRTPEVTCVVVDVSQEDPEVQFNWYVDGVEVHNAKTKPREEQFNSTYRVVSVLTVLHQDWLNGKEYKCKVSNKGLPSSIEKTISKAKGQPREPQVYTLPPSQEEMTKNQVSLTCLVKGFYPSDIAVEWESNGQPENNYKTTPPVLDSDGSFFLYSRLTVDKSRWQEGNVFSCSVMHEALHNHYTQKSLSLSLGAGGGGSGGGGSGGGGSGGGGSGVIHVTKEVKEVATLSCGHNVSVEELAQTRIYWQKEKKMVLTMMSGDMNIWPEYKNRTIFDITNNLSIVILALRPSDEGTYECVVLKYEKDAFKREHLAEVTLSVKADFPTPSISDFEIPTSNIRRIICSTSGGFPEPHLSWLENGEELNAINTTVSQDPETELYAVSSKLDFNMTTNHSFMCLIKYGHLRVNQTFNWNTTKQEHFPDN

SEQ ID NO: 42 - protein, 1103 aa, synthetic construct
  REGION 1..1103: note = CD80-sugemalimab-LAG3
VIHVTKEVKEVATLSCGHNVSVEELAQTRIYWQKEKKMVLTMMSGDMNIWPEYKNRTIFDITNNLSIVILALRPSDEGTYECVVLKYEKDAFKREHLAEVTLSVKADFPTPSISDFEIPTSNIRRIICSTSGGFPEPHLSWLENGEELNAINTTVSQDPETELYAVSSKLDFNMTTNHSFMCLIKYGHLRVNQTFNWNTTKQEHFPDNGGGGSGGGGSGGGGSGGGSGEVQLLESGGGLVQPGGSLRLSCAASGFTFSSYAMSWVRQAPGKGLEWVSGISGSGGFTYYADSVKGRFTISRDNSKNTLYLQMNSLRAEDTAVYYCAKPPRGYNYGPFDYWGQGTLVTVSSASTKGPSVFPLAPCSRSTSESTAALGCLVKDYFPEPVTVSWNSGALTSGVHTFPAVLQSSGLYSLSSVVTVPSSSLGTKTYTCNVDHKPSNTKVDKRVESKYGPPCPPCPAPEFLGGPSVFLFPPKPKDTLMISRTPEVTCVVVDVSQEDPEVQFNWYVDGVEVHNAKTKPREEQFNSTYRVVSVLTVLHQDWLNGKEYKCKVSNKGLPSSIEKTISKAKGQPREPQVYTLPPSQEEMTKNQVSLTCLVKGFYPSDIAVEWESNGQPENNYKTTPPVLDSDGSFFLYSRLTVDKSRWQEGNVFSCSVMHEALHNHYTQKSLSLSLGAGGGGSGGGGSGGGGSGGGGSGLQPGAEVPVVWAQEGAPAQLPCSPTIPLQDLSLLRRAGVTWQHQPDSGPPAAAPGHPLAPGPHPAAPSSWGPRPRRYTVLSVGPGGLRSGRLPLQPRVQLDERGRQRGDFSLWLRPARRADAGEYRAAVHLRDRALSCRLRLRLGQASMTASPPGSLRASDWVILNCSFSRPDRPASVHWFRNRGQGRVPVRESPHHHLAESFLFLPQVSPMDSGPWGCILTYRDGFNVSIMYNLTVLGLEPPTPLTVYAGAGSRVGLPCRLPAGVGTRSFLTAKWTPPGGGPDLLVTGDNGDFTLRLEDVSQAQAGTYTCHIHLQEQQLNATVTLAIITVTPKSFGSPGSLGKLLCEVTPVSGQERFVWSSLDTPSQRSFSGPWLEAQEAQLLSQPWQCQLYQGERLLGAAVYFT

SEQ ID NO: 43 - protein, 680 aa, synthetic construct
  REGION 1..680: note = Durvalumab-CD80
EVQLVESGGGLVQPGGSLRLSCAASGFTFSRYWMSWVRQAPGKGLEWVANIKQDGSEKYYVDSVKGRFTISRDNAKNSLYLQMNSLRAEDTAVYYCAREGGWFGELAFDYWGQGTLVTVSSASTKGPSVFPLAPSSKSTSGGTAALGCLVKDYFPEPVTVSWNSGALTSGVHTFPAVLQSSGLYSLSSVVTVPSSSLGTQTYICNVNHKPSNTKVDKRVEPKSCDKTHTCPPCPAPEFEGGPSVFLFPPKPKDTLMISRTPEVTCVVVDVSHEDPEVKFNWYVDGVEVHNAKTKPREEQYNSTYRVVSVLTVLHQDWLNGKEYKCKVSNKALPASIEKTISKAKGQPREPQVYTLPPSREEMTKNQVSLTCLVKGFYPSDIAVEWESNGQPENNYKTTPPVLDSDGSFFLYSKLTVDKSRWQQGNVFSCSVMHEALHNHYTQKSLSLSPGAGGGGSGGGGSGGGGSGGGGSGVIHVTKEVKEVATLSCGHNVSVEELAQTRIYWQKEKKMVLTMMSGDMNIWPEYKNRTIFDITNNLSIVILALRPSDEGTYECVVLKYEKDAFKREHLAEVTLSVKADFPTPSISDFEIPTSNIRRIICSTSGGFPEPHLSWLENGEELNAINTTVSQDPETELYAVSSKLDFNMTTNHSFMCLIKYGHLRVNQTFNWNTTKQEHFPDN

SEQ ID NO: 44 - protein, 878 aa, synthetic construct
  REGION 1..878: note = Durvalumab-LAG3
EVQLVESGGGLVQPGGSLRLSCAASGFTFSRYWMSWVRQAPGKGLEWVANIKQDGSEKYYVDSVKGRFTISRDNAKNSLYLQMNSLRAEDTAVYYCAREGGWFGELAFDYWGQGTLVTVSSASTKGPSVFPLAPSSKSTSGGTAALGCLVKDYFPEPVTVSWNSGALTSGVHTFPAVLQSSGLYSLSSVVTVPSSSLGTQTYICNVNHKPSNTKVDKRVEPKSCDKTHTCPPCPAPEFEGGPSVFLFPPKPKDTLMISRTPEVTCVVVDVSHEDPEVKFNWYVDGVEVHNAKTKPREEQYNSTYRVVSVLTVLHQDWLNGKEYKCKVSNKALPASIEKTISKAKGQPREPQVYTLPPSREEMTKNQVSLTCLVKGFYPSDIAVEWESNGQPENNYKTTPPVLDSDGSFFLYSKLTVDKSRWQQGNVFSCSVMHEALHNHYTQKSLSLSPGAGGGGSGGGGSGGGGSGGGGSGLQPGAEVPVVWAQEGAPAQLPCSPTIPLQDLSLLRRAGVTWQHQPDSGPPAAAPGHPLAPGPHPAAPSSWGPRPRRYTVLSVGPGGLRSGRLPLQPRVQLDERGRQRGDFSLWLRPARRADAGEYRAAVHLRDRALSCRLRLRLGQASMTASPPGSLRASDWVILNCSFSRPDRPASVHWFRNRGQGRVPVRESPHHHLAESFLFLPQVSPMDSGPWGCILTYRDGFNVSIMYNLTVLGLEPPTPLTVYAGAGSRVGLPCRLPAGVGTRSFLTAKWTPPGGGPDLLVTGDNGDFTLRLEDVSQAQAGTYTCHIHLQEQQLNATVTLAIITVTPKSFGSPGSLGKLLCEVTPVSGQERFVWSSLDTPSQRSFSGPWLEAQEAQLLSQPWQCQLYQGERLLGAAVYFT

SEQ ID NO: 45 - protein, 714 aa, synthetic construct
  REGION 1..714: note = Durvalumab-LAG3 IgD1/D2
EVQLVESGGGLVQPGGSLRLSCAASGFTFSRYWMSWVRQAPGKGLEWVANIKQDGSEKYYVDSVKGRFTISRDNAKNSLYLQMNSLRAEDTAVYYCAREGGWFGELAFDYWGQGTLVTVSSASTKGPSVFPLAPSSKSTSGGTAALGCLVKDYFPEPVTVSWNSGALTSGVHTFPAVLQSSGLYSLSSVVTVPSSSLGTQTYICNVNHKPSNTKVDKRVEPKSCDKTHTCPPCPAPEFEGGPSVFLFPPKPKDTLMISRTPEVTCVVVDVSHEDPEVKFNWYVDGVEVHNAKTKPREEQYNSTYRVVSVLTVLHQDWLNGKEYKCKVSNKALPASIEKTISKAKGQPREPQVYTLPPSREEMTKNQVSLTCLVKGFYPSDIAVEWESNGQPENNYKTTPPVLDSDGSFFLYSKLTVDKSRWQQGNVFSCSVMHEALHNHYTQKSLSLSPGAGGGGSGGGGSGGGGSGGGGSGLQPGAEVPVVWAQEGAPAQLPCSPTIPLQDLSLLRRAGVTWQHQPDSGPPAAAPGHPLAPGPHPAAPSSWGPRPRRYTVLSVGPGGLRSGRLPLQPRVQLDERGRQRGDFSLWLRPARRADAGEYRAAVHLRDRALSCRLRLRLGQASMTASPPGSLRASDWVILNCSFSRPDRPASVHWFRNRGQGRVPVRESPHHHLAESFLFLPQVSPMDSGPWGCILTYRDGFNVSIMYNLTVLGLEP

SEQ ID NO: 46 - protein, 797 aa, synthetic construct
  REGION 1..797: note = Durvalumab-LAG3 IgD1/D2/D3
EVQLVESGGGLVQPGGSLRLSCAASGFTFSRYWMSWVRQAPGKGLEWVANIKQDGSEKYYVDSVKGRFTISRDNAKNSLYLQMNSLRAEDTAVYYCAREGGWFGELAFDYWGQGTLVTVSSASTKGPSVFPLAPSSKSTSGGTAALGCLVKDYFPEPVTVSWNSGALTSGVHTFPAVLQSSGLYSLSSVVTVPSSSLGTQTYICNVNHKPSNTKVDKRVEPKSCDKTHTCPPCPAPEFEGGPSVFLFPPKPKDTLMISRTPEVTCVVVDVSHEDPEVKFNWYVDGVEVHNAKTKPREEQYNSTYRVVSVLTVLHQDWLNGKEYKCKVSNKALPASIEKTISKAKGQPREPQVYTLPPSREEMTKNQVSLTCLVKGFYPSDIAVEWESNGQPENNYKTTPPVLDSDGSFFLYSKLTVDKSRWQQGNVFSCSVMHEALHNHYTQKSLSLSPGAGGGGSGGGGSGGGGSGGGGSGLQPGAEVPVVWAQEGAPAQLPCSPTIPLQDLSLLRRAGVTWQHQPDSGPPAAAPGHPLAPGPHPAAPSSWGPRPRRYTVLSVGPGGLRSGRLPLQPRVQLDERGRQRGDFSLWLRPARRADAGEYRAAVHLRDRALSCRLRLRLGQASMTASPPGSLRASDWVILNCSFSRPDRPASVHWFRNRGQGRVPVRESPHHHLAESFLFLPQVSPMDSGPWGCILTYRDGFNVSIMYNLTVLGLEPPTPLTVYAGAGSRVGLPCRLPAGVGTRSFLTAKWTPPGGGPDLLVTGDNGDFTLRLEDVSQAQAGTYTCHIHLQEQQLNATVT

SEQ ID NO: 47 - protein, 680 aa, synthetic construct
  REGION 1..680: note = CD80-Durvalumab
VIHVTKEVKEVATLSCGHNVSVEELAQTRIYWQKEKKMVLTMMSGDMNIWPEYKNRTIFDITNNLSIVILALRPSDEGTYECVVLKYEKDAFKREHLAEVTLSVKADFPTPSISDFEIPTSNIRRIICSTSGGFPEPHLSWLENGEELNAINTTVSQDPETELYAVSSKLDFNMTTNHSFMCLIKYGHLRVNQTFNWNTTKQEHFPDNGGGGSGGGGSGGGGSGGGGSGEVQLVESGGGLVQPGGSLRLSCAASGFTFSRYWMSWVRQAPGKGLEWVANIKQDGSEKYYVDSVKGRFTISRDNAKNSLYLQMNSLRAEDTAVYYCAREGGWFGELAFDYWGQGTLVTVSSASTKGPSVFPLAPSSKSTSGGTAALGCLVKDYFPEPVTVSWNSGALTSGVHTFPAVLQSSGLYSLSSVVTVPSSSLGTQTYICNVNHKPSNTKVDKRVEPKSCDKTHTCPPCPAPEFEGGPSVFLFPPKPKDTLMISRTPEVTCVVVDVSHEDPEVKFNWYVDGVEVHNAKTKPREEQYNSTYRVVSVLTVLHQDWLNGKEYKCKVSNKALPASIEKTISKAKGQPREPQVYTLPPSREEMTKNQVSLTCLVKGFYPSDIAVEWESNGQPENNYKTTPPVLDSDGSFFLYSKLTVDKSRWQQGNVFSCSVMHEALHNHYTQKSLSLSPGK

SEQ ID NO: 48 - protein, 878 aa, synthetic construct
  REGION 1..878: note = LAG3-Durvalumab
LQPGAEVPVVWAQEGAPAQLPCSPTIPLQDLSLLRRAGVTWQHQPDSGPPAAAPGHPLAPGPHPAAPSSWGPRPRRYTVLSVGPGGLRSGRLPLQPRVQLDERGRQRGDFSLWLRPARRADAGEYRAAVHLRDRALSCRLRLRLGQASMTASPPGSLRASDWVILNCSFSRPDRPASVHWFRNRGQGRVPVRESPHHHLAESFLFLPQVSPMDSGPWGCILTYRDGFNVSIMYNLTVLGLEPPTPLTVYAGAGSRVGLPCRLPAGVGTRSFLTAKWTPPGGGPDLLVTGDNGDFTLRLEDVSQAQAGTYTCHIHLQEQQLNATVTLAIITVTPKSFGSPGSLGKLLCEVTPVSGQERFVWSSLDTPSQRSFSGPWLEAQEAQLLSQPWQCQLYQGERLLGAAVYFTGGGGSGGGGSGGGGSGGGGSGEVQLVESGGGLVQPGGSLRLSCAASGFTFSRYWMSWVRQAPGKGLEWVANIKQDGSEKYYVDSVKGRFTISRDNAKNSLYLQMNSLRAEDTAVYYCAREGGWFGELAFDYWGQGTLVTVSSASTKGPSVFPLAPSSKSTSGGTAALGCLVKDYFPEPVTVSWNSGALTSGVHTFPAVLQSSGLYSLSSVVTVPSSSLGTQTYICNVNHKPSNTKVDKRVEPKSCDKTHTCPPCPAPEFEGGPSVFLFPPKPKDTLMISRTPEVTCVVVDVSHEDPEVKFNWYVDGVEVHNAKTKPREEQYNSTYRVVSVLTVLHQDWLNGKEYKCKVSNKALPASIEKTISKAKGQPREPQVYTLPPSREEMTKNQVSLTCLVKGFYPSDIAVEWESNGQPENNYKTTPPVLDSDGSFFLYSKLTVDKSRWQQGNVFSCSVMHEALHNHYTQKSLSLSPGK

SEQ ID NO: 49 - protein, 444 aa, synthetic construct
  REGION 1..444: note = CD80-Durvalumab
VIHVTKEVKEVATLSCGHNVSVEELAQTRIYWQKEKKMVLTMMSGDMNIWPEYKNRTIFDITNNLSIVILALRPSDEGTYECVVLKYEKDAFKREHLAEVTLSVKADFPTPSISDFEIPTSNIRRIICSTSGGFPEPHLSWLENGEELNAINTTVSQDPETELYAVSSKLDFNMTTNHSFMCLIKYGHLRVNQTFNWNTTKQEHFPDNGGGGSGGGGSGGGGSGGGGSGEIVLTQSPGTLSLSPGERATLSCRASQRVSSSYLAWYQQKPGQAPRLLIYDASSRATGIPDRFSGSGSGTDFTLTISRLEPEDFAVYYCQQYGSLPWTFGQGTKVEIKRTVAAPSVFIFPPSDEQLKSGTASVVCLLNNFYPREAKVQWKVDNALQSGNSQESVTEQDSKDSTYSLSSTLTLSKADYEKHKVYACEVTHQGLSSPVTKSFNRGEC

SEQ ID NO: 50 - protein, 642 aa, synthetic construct
  REGION 1..642: note = LAG3-Durvalumab
LQPGAEVPVVWAQEGAPAQLPCSPTIPLQDLSLLRRAGVTWQHQPDSGPPAAAPGHPLAPGPHPAAPSSWGPRPRRYTVLSVGPGGLRSGRLPLQPRVQLDERGRQRGDFSLWLRPARRADAGEYRAAVHLRDRALSCRLRLRLGQASMTASPPGSLRASDWVILNCSFSRPDRPASVHWFRNRGQGRVPVRESPHHHLAESFLFLPQVSPMDSGPWGCILTYRDGFNVSIMYNLTVLGLEPPTPLTVYAGAGSRVGLPCRLPAGVGTRSFLTAKWTPPGGGPDLLVTGDNGDFTLRLEDVSQAQAGTYTCHIHLQEQQLNATVTLAIITVTPKSFGSPGSLGKLLCEVTPVSGQERFVWSSLDTPSQRSFSGPWLEAQEAQLLSQPWQCQLYQGERLLGAAVYFTGGGGSGGGGSGGGGSGGGGSGEIVLTQSPGTLSLSPGERATLSCRASQRVSSSYLAWYQQKPGQAPRLLIYDASSRATGIPDRFSGSGSGTDFTLTISRLEPEDFAVYYCQQYGSLPWTFGQGTKVEIKRTVAAPSVFIFPPSDEQLKSGTASVVCLLNNFYPREAKVQWKVDNALQSGNSQESVTEQDSKDSTYSLSSTLTLSKADYEKHKVYACEVTHQGLSSPVTKSFNRGEC

SEQ ID NO: 51 - protein, 924 aa, synthetic construct
  REGION 1..924: note = Durvalumab-LAG3 IgD1/D2-CD80
EVQLVESGGGLVQPGGSLRLSCAASGFTFSRYWMSWVRQAPGKGLEWVANIKQDGSEKYYVDSVKGRFTISRDNAKNSLYLQMNSLRAEDTAVYYCAREGGWFGELAFDYWGQGTLVTVSSASTKGPSVFPLAPSSKSTSGGTAALGCLVKDYFPEPVTVSWNSGALTSGVHTFPAVLQSSGLYSLSSVVTVPSSSLGTQTYICNVNHKPSNTKVDKRVEPKSCDKTHTCPPCPAPEFEGGPSVFLFPPKPKDTLMISRTPEVTCVVVDVSHEDPEVKFNWYVDGVEVHNAKTKPREEQYNSTYRVVSVLTVLHQDWLNGKEYKCKVSNKALPASIEKTISKAKGQPREPQVYTLPPSREEMTKNQVSLTCLVKGFYPSDIAVEWESNGQPENNYKTTPPVLDSDGSFFLYSKLTVDKSRWQQGNVFSCSVMHEALHNHYTQKSLSLSPGAGGGGSGGGGSGVIHVTKEVKEVATLSCGHNVSVEELAQTRIYWQKEKKMVLTMMSGDMNIWPEYKNRTIFDITNNLSIVILALRPSDEGTYECVVLKYEKDAFKREHLAEVTLSVKADFPTPSISDFEIPTSNIRRIICSTSGGFPEPHLSWLENGEELNAINTTVSQDPETELYAVSSKLDFNMTTNHSFMCLIKYGHLRVNQTFNWNTTKQEHFPDNGGGGSGGGGSGSLQPGAEVPVVWAQEGAPAQLPCSPTIPLQDLSLLRRAGVTWQHQPDSGPPAAAPGHPLAPGPHPAAPSSWGPRPRRYTVLSVGPGGLRSGRLPLQPRVQLDERGRQRGDFSLWLRPARRADAGEYRAAVHLRDRALSCRLRLRLGQASMTASPPGSLRASDWVILNCSFSRPDRPASVHWFRNRGQGRVPVRESPHHHLAESFLFLPQVSPMDSGPWGCILTYRDGFNVSIMYNLTVLGLEP

SEQ ID NO: 52 - protein, 1006 aa, synthetic construct
  REGION 1..1006: note = Durvalumab-LAG3 IgD1/D2/D3-CD80
EVQLVESGGGLVQPGGSLRLSCAASGFTFSRYWMSWVRQAPGKGLEWVANIKQDGSEKYYVDSVKGRFTISRDNAKNSLYLQMNSLRAEDTAVYYCAREGGWFGELAFDYWGQGTLVTVSSASTKGPSVFPLAPSSKSTSGGTAALGCLVKDYFPEPVTVSWNSGALTSGVHTFPAVLQSSGLYSLSSVVTVPSSSLGTQTYICNVNHKPSNTKVDKRVEPKSCDKTHTCPPCPAPEFEGGPSVFLFPPKPKDTLMISRTPEVTCVVVDVSHEDPEVKFNWYVDGVEVHNAKTKPREEQYNSTYRVVSVLTVLHQDWLNGKEYKCKVSNKALPASIEKTISKAKGQPREPQVYTLPPSREEMTKNQVSLTCLVKGFYPSDIAVEWESNGQPENNYKTTPPVLDSDGSFFLYSKLTVDKSRWQQGNVFSCSVMHEALHNHYTQKSLSLSPGAGGGGSGGGGSGVIHVTKEVKEVATLSCGHNVSVEELAQTRIYWQKEKKMVLTMMSGDMNIWPEYKNRTIFDITNNLSIVILALRPSDEGTYECVVLKYEKDAFKREHLAEVTLSVKADFPTPSISDFEIPTSNIRRIICSTSGGFPEPHLSWLENGEELNAINTTVSQDPETELYAVSSKLDFNMTTNHSFMCLIKYGHLRVNQTFNWNTTKQEHFPDNGGGGSGGGGSGLQPGAEVPVVWAQEGAPAQLPCSPTIPLQDLSLLRRAGVTWQHQPDSGPPAAAPGHPLAPGPHPAAPSSWGPRPRRYTVLSVGPGGLRSGRLPLQPRVQLDERGRQRGDFSLWLRPARRADAGEYRAAVHLRDRALSCRLRLRLGQASMTASPPGSLRASDWVILNCSFSRPDRPASVHWFRNRGQGRVPVRESPHHHLAESFLFLPQVSPMDSGPWGCILTYRDGFNVSIMYNLTVLGLEPPTPLTVYAGAGSRVGLPCRLPAGVGTRSFLTAKWTPPGGGPDLLVTGDNGDFTLRLEDVSQAQAGTYTCHIHLQEQQLNATVT

SEQ ID NO: 53 - protein, 1106 aa, synthetic construct
  REGION 1..1106: note = Durvalumab-LAG3-CD80
EVQLVESGGGLVQPGGSLRLSCAASGFTFSRYWMSWVRQAPGKGLEWVANIKQDGSEKYYVDSVKGRFTISRDNAKNSLYLQMNSLRAEDTAVYYCAREGGWFGELAFDYWGQGTLVTVSSASTKGPSVFPLAPSSKSTSGGTAALGCLVKDYFPEPVTVSWNSGALTSGVHTFPAVLQSSGLYSLSSVVTVPSSSLGTQTYICNVNHKPSNTKVDKRVEPKSCDKTHTCPPCPAPEFEGGPSVFLFPPKPKDTLMISRTPEVTCVVVDVSHEDPEVKFNWYVDGVEVHNAKTKPREEQYNSTYRVVSVLTVLHQDWLNGKEYKCKVSNKALPASIEKTISKAKGQPREPQVYTLPPSREEMTKNQVSLTCLVKGFYPSDIAVEWESNGQPENNYKTTPPVLDSDGSFFLYSKLTVDKSRWQQGNVFSCSVMHEALHNHYTQKSLSLSPGAGGGGSGGGGSGGGGSGGGSGVIHVTKEVKEVATLSCGHNVSVEELAQTRIYWQKEKKMVLTMMSGDMNIWPEYKNRTIFDITNNLSIVILALRPSDEGTYECVVLKYEKDAFKREHLAEVTLSVKADFPTPSISDFEIPTSNIRRIICSTSGGFPEPHLSWLENGEELNAINTTVSQDPETELYAVSSKLDFNMTTNHSFMCLIKYGHLRVNQTFNWNTTKQEHFPDNGGGGSGGGGSGGGGSGGGGSGLQPGAEVPVVWAQEGAPAQLPCSPTIPLQDLSLLRRAGVTWQHQPDSGPPAAAPGHPLAPGPHPAAPSSWGPRPRRYTVLSVGPGGLRSGRLPLQPRVQLDERGRQRGDFSLWLRPARRADAGEYRAAVHLRDRALSCRLRLRLGQASMTASPPGSLRASDWVILNCSFSRPDRPASVHWFRNRGQGRVPVRESPHHHLAESFLFLPQVSPMDSGPWGCILTYRDGFNVSIMYNLTVLGLEPPTPLTVYAGAGSRVGLPCRLPAGVGTRSFLTAKWTPPGGGPDLLVTGDNGDFTLRLEDVSQAQAGTYTCHIHLQEQQLNATVTLAIITVTPKSFGSPGSLGKLLCEVTPVSGQERFVWSSLDTPSQRSFSGPWLEAQEAQLLSQPWQCQLYQGERLLGAAVYFT

SEQ ID NO: 54 - protein, 924 aa, synthetic construct
  REGION 1..924: note = Durvalumab-CD80-LAG3 IgD1/D2
EVQLVESGGGLVQPGGSLRLSCAASGFTFSRYWMSWVRQAPGKGLEWVANIKQDGSEKYYVDSVKGRFTISRDNAKNSLYLQMNSLRAEDTAVYYCAREGGWFGELAFDYWGQGTLVTVSSASTKGPSVFPLAPSSKSTSGGTAALGCLVKDYFPEPVTVSWNSGALTSGVHTFPAVLQSSGLYSLSSVVTVPSSSLGTQTYICNVNHKPSNTKVDKRVEPKSCDKTHTCPPCPAPEFEGGPSVFLFPPKPKDTLMISRTPEVTCVVVDVSHEDPEVKFNWYVDGVEVHNAKTKPREEQYNSTYRVVSVLTVLHQDWLNGKEYKCKVSNKALPASIEKTISKAKGQPREPQVYTLPPSREEMTKNQVSLTCLVKGFYPSDIAVEWESNGQPENNYKTTPPVLDSDGSFFLYSKLTVDKSRWQQGNVFSCSVMHEALHNHYTQKSLSLSPGAGGGGSGGGGSGSLQPGAEVPVVWAQEGAPAQLPCSPTIPLQDLSLLRRAGVTWQHQPDSGPPAAAPGHPLAPGPHPAAPSSWGPRPRRYTVLSVGPGGLRSGRLPLQPRVQLDERGRQRGDFSLWLRPARRADAGEYRAAVHLRDRALSCRLRLRLGQASMTASPPGSLRASDWVILNCSFSRPDRPASVHWFRNRGQGRVPVRESPHHHLAESFLFLPQVSPMDSGPWGCILTYRDGFNVSIMYNLTVLGLEPGGGGSGGGGSGVIHVTKEVKEVATLSCGHNVSVEELAQTRIYWQKEKKMVLTMMSGDMNIWPEYKNRTIFDITNNLSIVILALRPSDEGTYECVVLKYEKDAFKREHLAEVTLSVKADFPTPSISDFEIPTSNIRRIICSTSGGFPEPHLSWLENGEELNAINTTVSQDPETELYAVSSKLDFNMTTNHSFMCLIKYGHLRVNQTFNWNTTKQEHFPDN

SEQ ID NO: 55 - protein, 1006 aa, synthetic construct
  REGION 1..1006: note = Durvalumab-CD80-LAG3 IgD1/D2/D3
EVQLVESGGGLVQPGGSLRLSCAASGFTFSRYWMSWVRQAPGKGLEWVANIKQDGSEKYYVDSVKGRFTISRDNAKNSLYLQMNSLRAEDTAVYYCAREGGWFGELAFDYWGQGTLVTVSSASTKGPSVFPLAPSSKSTSGGTAALGCLVKDYFPEPVTVSWNSGALTSGVHTFPAVLQSSGLYSLSSVVTVPSSSLGTQTYICNVNHKPSNTKVDKRVEPKSCDKTHTCPPCPAPEFEGGPSVFLFPPKPKDTLMISRTPEVTCVVVDVSHEDPEVKFNWYVDGVEVHNAKTKPREEQYNSTYRVVSVLTVLHQDWLNGKEYKCKVSNKALPASIEKTISKAKGQPREPQVYTLPPSREEMTKNQVSLTCLVKGFYPSDIAVEWESNGQPENNYKTTPPVLDSDGSFFLYSKLTVDKSRWQQGNVFSCSVMHEALHNHYTQKSLSLSPGAGGGGSGGGGSGLQPGAEVPVVWAQEGAPAQLPCSPTIPLQDLSLLRRAGVTWQHQPDSGPPAAAPGHPLAPGPHPAAPSSWGPRPRRYTVLSVGPGGLRSGRLPLQPRVQLDERGRQRGDFSLWLRPARRADAGEYRAAVHLRDRALSCRLRLRLGQASMTASPPGSLRASDWVILNCSFSRPDRPASVHWFRNRGQGRVPVRESPHHHLAESFLFLPQVSPMDSGPWGCILTYRDGFNVSIMYNLTVLGLEPPTPLTVYAGAGSRVGLPCRLPAGVGTRSFLTAKWTPPGGGPDLLVTGDNGDFTLRLEDVSQAQAGTYTCHIHLQEQQLNATVTGGGGSGGGGSGVIHVTKEVKEVATLSCGHNVSVEELAQTRIYWQKEKKMVLTMMSGDMNIWPEYKNRTIFDITNNLSIVILALRPSDEGTYECVVLKYEKDAFKREHLAEVTLSVKADFPTPSISDFEIPTSNIRRIICSTSGGFPEPHLSWLENGEELNAINTTVSQDPETELYAVSSKLDFNMTTNHSFMCLIKYGHLRVNQTFNWNTTKQEHFPDN

SEQ ID NO: 56 - protein, 1106 aa, synthetic construct
  REGION 1..1106: note = Durvalumab-CD80-LAG3
EVQLVESGGGLVQPGGSLRLSCAASGFTFSRYWMSWVRQAPGKGLEWVANIKQDGSEKYYVDSVKGRFTISRDNAKNSLYLQMNSLRAEDTAVYYCAREGGWFGELAFDYWGQGTLVTVSSASTKGPSVFPLAPSSKSTSGGTAALGCLVKDYFPEPVTVSWNSGALTSGVHTFPAVLQSSGLYSLSSVVTVPSSSLGTQTYICNVNHKPSNTKVDKRVEPKSCDKTHTCPPCPAPEFEGGPSVFLFPPKPKDTLMISRTPEVTCVVVDVSHEDPEVKFNWYVDGVEVHNAKTKPREEQYNSTYRVVSVLTVLHQDWLNGKEYKCKVSNKALPASIEKTISKAKGQPREPQVYTLPPSREEMTKNQVSLTCLVKGFYPSDIAVEWESNGQPENNYKTTPPVLDSDGSFFLYSKLTVDKSRWQQGNVFSCSVMHEALHNHYTQKSLSLSPGAGGGGSGGGGSGGGGSGGGGSGLQPGAEVPVVWAQEGAPAQLPCSPTIPLQDLSLLRRAGVTWQHQPDSGPPAAAPGHPLAPGPHPAAPSSWGPRPRRYTVLSVGPGGLRSGRLPLQPRVQLDERGRQRGDFSLWLRPARRADAGEYRAAVHLRDRALSCRLRLRLGQASMTASPPGSLRASDWVILNCSFSRPDRPASVHWFRNRGQGRVPVRESPHHHLAESFLFLPQVSPMDSGPWGCILTYRDGFNVSIMYNLTVLGLEPPTPLTVYAGAGSRVGLPCRLPAGVGTRSFLTAKWTPPGGGPDLLVTGDNGDFTLRLEDVSQAQAGTYTCHIHLQEQQLNATVTLAIITVTPKSFGSPGSLGKLLCEVTPVSGQERFVWSSLDTPSQRSFSGPWLEAQEAQLLSQPWQCQLYQGERLLGAAVYFTGGGGSGGGGSGGGGSGGGSGVIHVTKEVKEVATLSCGHNVSVEELAQTRIYWQKEKKMVLTMMSGDMNIWPEYKNRTIFDITNNLSIVILALRPSDEGTYECVVLKYEKDAFKREHLAEVTLSVKADFPTPSISDFEIPTSNIRRIICSTSGGFPEPHLSWLENGEELNAINTTVSQDPETELYAVSSKLDFNMTTNHSFMCLIKYGHLRVNQTFNWNTTKQEHFPDN

SEQ ID NO: 57 - protein, 1106 aa, synthetic construct
  REGION 1..1106: note = LAG3-Durvalumab-CD80
LQPGAEVPVVWAQEGAPAQLPCSPTIPLQDLSLLRRAGVTWQHQPDSGPPAAAPGHPLAPGPHPAAPSSWGPRPRRYTVLSVGPGGLRSGRLPLQPRVQLDERGRQRGDFSLWLRPARRADAGEYRAAVHLRDRALSCRLRLRLGQASMTASPPGSLRASDWVILNCSFSRPDRPASVHWFRNRGQGRVPVRESPHHHLAESFLFLPQVSPMDSGPWGCILTYRDGFNVSIMYNLTVLGLEPPTPLTVYAGAGSRVGLPCRLPAGVGTRSFLTAKWTPPGGGPDLLVTGDNGDFTLRLEDVSQAQAGTYTCHIHLQEQQLNATVTLAIITVTPKSFGSPGSLGKLLCEVTPVSGQERFVWSSLDTPSQRSFSGPWLEAQEAQLLSQPWQCQLYQGERLLGAAVYFTGGGGSGGGGSGGGGSGGGSGEVQLVESGGGLVQPGGSLRLSCAASGFTFSRYWMSWVRQAPGKGLEWVANIKQDGSEKYYVDSVKGRFTISRDNAKNSLYLQMNSLRAEDTAVYYCAREGGWFGELAFDYWGQGTLVTVSSASTKGPSVFPLAPSSKSTSGGTAALGCLVKDYFPEPVTVSWNSGALTSGVHTFPAVLQSSGLYSLSSVVTVPSSSLGTQTYICNVNHKPSNTKVDKRVEPKSCDKTHTCPPCPAPEFEGGPSVFLFPPKPKDTLMISRTPEVTCVVVDVSHEDPEVKFNWYVDGVEVHNAKTKPREEQYNSTYRVVSVLTVLHQDWLNGKEYKCKVSNKALPASIEKTISKAKGQPREPQVYTLPPSREEMTKNQVSLTCLVKGFYPSDIAVEWESNGQPENNYKTTPPVLDSDGSFFLYSKLTVDKSRWQQGNVFSCSVMHEALHNHYTQKSLSLSPGAGGGGSGGGGSGGGGSGGGGSGVIHVTKEVKEVATLSCGHNVSVEELAQTRIYWQKEKKMVLTMMSGDMNIWPEYKNRTIFDITNNLSIVILALRPSDEGTYECVVLKYEKDAFKREHLAEVTLSVKADFPTPSISDFEIPTSNIRRIICSTSGGFPEPHLSWLENGEELNAINTTVSQDPETELYAVSSKLDFNMTTNHSFMCLIKYGHLRVNQTFNWNTTKQEHFPDN

SEQ ID NO: 58 - protein, 1106 aa, synthetic construct
  REGION 1..1106: note = CD80-Durvalumab-LAG3
VIHVTKEVKEVATLSCGHNVSVEELAQTRIYWQKEKKMVLTMMSGDMNIWPEYKNRTIFDITNNLSIVILALRPSDEGTYECVVLKYEKDAFKREHLAEVTLSVKADFPTPSISDFEIPTSNIRRIICSTSGGFPEPHLSWLENGEELNAINTTVSQDPETELYAVSSKLDFNMTTNHSFMCLIKYGHLRVNQTFNWNTTKQEHFPDNGGGGSGGGGSGGGGSGGGSGEVQLVESGGGLVQPGGSLRLSCAASGFTFSRYWMSWVRQAPGKGLEWVANIKQDGSEKYYVDSVKGRFTISRDNAKNSLYLQMNSLRAEDTAVYYCAREGGWFGELAFDYWGQGTLVTVSSASTKGPSVFPLAPSSKSTSGGTAALGCLVKDYFPEPVTVSWNSGALTSGVHTFPAVLQSSGLYSLSSVVTVPSSSLGTQTYICNVNHKPSNTKVDKRVEPKSCDKTHTCPPCPAPEFEGGPSVFLFPPKPKDTLMISRTPEVTCVVVDVSHEDPEVKFNWYVDGVEVHNAKTKPREEQYNSTYRVVSVLTVLHQDWLNGKEYKCKVSNKALPASIEKTISKAKGQPREPQVYTLPPSREEMTKNQVSLTCLVKGFYPSDIAVEWESNGQPENNYKTTPPVLDSDGSFFLYSKLTVDKSRWQQGNVFSCSVMHEALHNHYTQKSLSLSPGAGGGGSGGGGSGGGGSGGGGSGLQPGAEVPVVWAQEGAPAQLPCSPTIPLQDLSLLRRAGVTWQHQPDSGPPAAAPGHPLAPGPHPAAPSSWGPRPRRYTVLSVGPGGLRSGRLPLQPRVQLDERGRQRGDFSLWLRPARRADAGEYRAAVHLRDRALSCRLRLRLGQASMTASPPGSLRASDWVILNCSFSRPDRPASVHWFRNRGQGRVPVRESPHHHLAESFLFLPQVSPMDSGPWGCILTYRDGFNVSIMYNLTVLGLEPPTPLTVYAGAGSRVGLPCRLPAGVGTRSFLTAKWTPPGGGPDLLVTGDNGDFTLRLEDVSQAQAGTYTCHIHLQEQQLNATVTLAIITVTPKSFGSPGSLGKLLCEVTPVSGQERFVWSSLDTPSQRSFSGPWLEAQEAQLLSQPWQCQLYQGERLLGAAVYFT

SEQ ID NO: 59 - protein, 677 aa, synthetic construct
  REGION 1..677: note = Atezolizumab-CD80
EVQLVESGGGLVQPGGSLRLSCAASGFTFSDSWIHWVRQAPGKGLEWVAWISPYGGSTYYADSVKGRFTISADTSKNTAYLQMNSLRAEDTAVYYCARRHWPGGFDYWGQGTLVTVSSASTKGPSVFPLAPSSKSTSGGTAALGCLVKDYFPEPVTVSWNSGALTSGVHTFPAVLQSSGLYSLSSVVTVPSSSLGTQTYICNVNHKPSNTKVDKKVEPKSCDKTHTCPPCPAPELLGGPSVFLFPPKPKDTLMISRTPEVTCVVVDVSHEDPEVKFNWYVDGVEVHNAKTKPREEQYASTYRVVSVLTVLHQDWLNGKEYKCKVSNKALPAPIEKTISKAKGQPREPQVYTLPPSREEMTKNQVSLTCLVKGFYPSDIAVEWESNGQPENNYKTTPPVLDSDGSFFLYSKLTVDKSRWQQGNVFSCSVMHEALHNHYTQKSLSLSPGAGGGGSGGGGSGGGGSGGGGSGVIHVTKEVKEVATLSCGHNVSVEELAQTRIYWQKEKKMVLTMMSGDMNIWPEYKNRTIFDITNNLSIVILALRPSDEGTYECVVLKYEKDAFKREHLAEVTLSVKADFPTPSISDFEIPTSNIRRIICSTSGGFPEPHLSWLENGEELNAINTTVSQDPETELYAVSSKLDFNMTTNHSFMCLIKYGHLRVNQTFNWNTTKQEHFPDN

SEQ ID NO: 60 - protein, 875 aa, synthetic construct
  REGION 1..875: note = Atezolizumab-LAG3
EVQLVESGGGLVQPGGSLRLSCAASGFTFSDSWIHWVRQAPGKGLEWVAWISPYGGSTYYADSVKGRFTISADTSKNTAYLQMNSLRAEDTAVYYCARRHWPGGFDYWGQGTLVTVSSASTKGPSVFPLAPSSKSTSGGTAALGCLVKDYFPEPVTVSWNSGALTSGVHTFPAVLQSSGLYSLSSVVTVPSSSLGTQTYICNVNHKPSNTKVDKKVEPKSCDKTHTCPPCPAPELLGGPSVFLFPPKPKDTLMISRTPEVTCVVVDVSHEDPEVKFNWYVDGVEVHNAKTKPREEQYASTYRVVSVLTVLHQDWLNGKEYKCKVSNKALPAPIEKTISKAKGQPREPQVYTLPPSREEMTKNQVSLTCLVKGFYPSDIAVEWESNGQPENNYKTTPPVLDSDGSFFLYSKLTVDKSRWQQGNVFSCSVMHEALHNHYTQKSLSLSPGAGGGGSGGGGSGGGGSGGGGSGLQPGAEVPVVWAQEGAPAQLPCSPTIPLQDLSLLRRAGVTWQHQPDSGPPAAAPGHPLAPGPHPAAPSSWGPRPRRYTVLSVGPGGLRSGRLPLQPRVQLDERGRQRGDFSLWLRPARRADAGEYRAAVHLRDRALSCRLRLRLGQASMTASPPGSLRASDWVILNCSFSRPDRPASVHWFRNRGQGRVPVRESPHHHLAESFLFLPQVSPMDSGPWGCILTYRDGFNVSIMYNLTVLGLEPPTPLTVYAGAGSRVGLPCRLPAGVGTRSFLTAKWTPPGGGPDLLVTGDNGDFTLRLEDVSQAQAGTYTCHIHLQEQQLNATVTLAIITVTPKSFGSPGSLGKLLCEVTPVSGQERFVWSSLDTPSQRSFSGPWLEAQEAQLLSQPWQCQLYQGERLLGAAVYFT

SEQ ID NO: 61 - protein, 711 aa, synthetic construct
  REGION 1..711: note = Atezolizumab-LAG3 IgD1/D2
EVQLVESGGGLVQPGGSLRLSCAASGFTFSDSWIHWVRQAPGKGLEWVAWISPYGGSTYYADSVKGRFTISADTSKNTAYLQMNSLRAEDTAVYYCARRHWPGGFDYWGQGTLVTVSSASTKGPSVFPLAPSSKSTSGGTAALGCLVKDYFPEPVTVSWNSGALTSGVHTFPAVLQSSGLYSLSSVVTVPSSSLGTQTYICNVNHKPSNTKVDKKVEPKSCDKTHTCPPCPAPELLGGPSVFLFPPKPKDTLMISRTPEVTCVVVDVSHEDPEVKFNWYVDGVEVHNAKTKPREEQYASTYRVVSVLTVLHQDWLNGKEYKCKVSNKALPAPIEKTISKAKGQPREPQVYTLPPSREEMTKNQVSLTCLVKGFYPSDIAVEWESNGQPENNYKTTPPVLDSDGSFFLYSKLTVDKSRWQQGNVFSCSVMHEALHNHYTQKSLSLSPGAGGGGSGGGGSGGGGSGGGGSGLQPGAEVPVVWAQEGAPAQLPCSPTIPLQDLSLLRRAGVTWQHQPDSGPPAAAPGHPLAPGPHPAAPSSWGPRPRRYTVLSVGPGGLRSGRLPLQPRVQLDERGRQRGDFSLWLRPARRADAGEYRAAVHLRDRALSCRLRLRLGQASMTASPPGSLRASDWVILNCSFSRPDRPASVHWFRNRGQGRVPVRESPHHHLAESFLFLPQVSPMDSGPWGCILTYRDGFNVSIMYNLTVLGLEP

SEQ ID NO: 62 - protein, 794 aa, synthetic construct
  REGION 1..794: note = Atezolizumab-LAG3 IgD1/D2/D3
EVQLVESGGGLVQPGGSLRLSCAASGFTFSDSWIHWVRQAPGKGLEWVAWISPYGGSTYYADSVKGRFTISADTSKNTAYLQMNSLRAEDTAVYYCARRHWPGGFDYWGQGTLVTVSSASTKGPSVFPLAPSSKSTSGGTAALGCLVKDYFPEPVTVSWNSGALTSGVHTFPAVLQSSGLYSLSSVVTVPSSSLGTQTYICNVNHKPSNTKVDKKVEPKSCDKTHTCPPCPAPELLGGPSVFLFPPKPKDTLMISRTPEVTCVVVDVSHEDPEVKFNWYVDGVEVHNAKTKPREEQYASTYRVVSVLTVLHQDWLNGKEYKCKVSNKALPAPIEKTISKAKGQPREPQVYTLPPSREEMTKNQVSLTCLVKGFYPSDIAVEWESNGQPENNYKTTPPVLDSDGSFFLYSKLTVDKSRWQQGNVFSCSVMHEALHNHYTQKSLSLSPGAGGGGSGGGGSGGGGSGGGGSGLQPGAEVPVVWAQEGAPAQLPCSPTIPLQDLSLLRRAGVTWQHQPDSGPPAAAPGHPLAPGPHPAAPSSWGPRPRRYTVLSVGPGGLRSGRLPLQPRVQLDERGRQRGDFSLWLRPARRADAGEYRAAVHLRDRALSCRLRLRLGQASMTASPPGSLRASDWVILNCSFSRPDRPASVHWFRNRGQGRVPVRESPHHHLAESFLFLPQVSPMDSGPWGCILTYRDGFNVSIMYNLTVLGLEPPTPLTVYAGAGSRVGLPCRLPAGVGTRSFLTAKWTPPGGGPDLLVTGDNGDFTLRLEDVSQAQAGTYTCHIHLQEQQLNATVT

SEQ ID NO: 63 - protein, 677 aa, synthetic construct
  REGION 1..677: note = CD80-Atezolizumab
VIHVTKEVKEVATLSCGHNVSVEELAQTRIYWQKEKKMVLTMMSGDMNIWPEYKNRTIFDITNNLSIVILALRPSDEGTYECVVLKYEKDAFKREHLAEVTLSVKADFPTPSISDFEIPTSNIRRIICSTSGGFPEPHLSWLENGEELNAINTTVSQDPETELYAVSSKLDFNMTTNHSFMCLIKYGHLRVNQTFNWNTTKQEHFPDNGGGGSGGGGSGGGGSGGGGSGEVQLVESGGGLVQPGGSLRLSCAASGFTFSDSWIHWVRQAPGKGLEWVAWISPYGGSTYYADSVKGRFTISADTSKNTAYLQMNSLRAEDTAVYYCARRHWPGGFDYWGQGTLVTVSSASTKGPSVFPLAPSSKSTSGGTAALGCLVKDYFPEPVTVSWNSGALTSGVHTFPAVLQSSGLYSLSSVVTVPSSSLGTQTYICNVNHKPSNTKVDKKVEPKSCDKTHTCPPCPAPELLGGPSVFLFPPKPKDTLMISRTPEVTCVVVDVSHEDPEVKFNWYVDGVEVHNAKTKPREEQYASTYRVVSVLTVLHQDWLNGKEYKCKVSNKALPAPIEKTISKAKGQPREPQVYTLPPSREEMTKNQVSLTCLVKGFYPSDIAVEWESNGQPENNYKTTPPVLDSDGSFFLYSKLTVDKSRWQQGNVFSCSVMHEALHNHYTQKSLSLSPGK

SEQ ID NO: 64 - protein, 875 aa, synthetic construct
  REGION 1..875: note = LAG3-Atezolizumab
LQPGAEVPVVWAQEGAPAQLPCSPTIPLQDLSLLRRAGVTWQHQPDSGPPAAAPGHPLAPGPHPAAPSSWGPRPRRYTVLSVGPGGLRSGRLPLQPRVQLDERGRQRGDFSLWLRPARRADAGEYRAAVHLRDRALSCRLRLRLGQASMTASPPGSLRASDWVILNCSFSRPDRPASVHWFRNRGQGRVPVRESPHHHLAESFLFLPQVSPMDSGPWGCILTYRDGFNVSIMYNLTVLGLEPPTPLTVYAGAGSRVGLPCRLPAGVGTRSFLTAKWTPPGGGPDLLVTGDNGDFTLRLEDVSQAQAGTYTCHIHLQEQQLNATVTLAIITVTPKSFGSPGSLGKLLCEVTPVSGQERFVWSSLDTPSQRSFSGPWLEAQEAQLLSQPWQCQLYQGERLLGAAVYFTGGGGSGGGGSGGGGSGGGGSGEVQLVESGGGLVQPGGSLRLSCAASGFTFSDSWIHWVRQAPGKGLEWVAWISPYGGSTYYADSVKGRFTISADTSKNTAYLQMNSLRAEDTAVYYCARRHWPGGFDYWGQGTLVTVSSASTKGPSVFPLAPSSKSTSGGTAALGCLVKDYFPEPVTVSWNSGALTSGVHTFPAVLQSSGLYSLSSVVTVPSSSLGTQTYICNVNHKPSNTKVDKKVEPKSCDKTHTCPPCPAPELLGGPSVFLFPPKPKDTLMISRTPEVTCVVVDVSHEDPEVKFNWYVDGVEVHNAKTKPREEQYASTYRVVSVLTVLHQDWLNGKEYKCKVSNKALPAPIEKTISKAKGQPREPQVYTLPPSREEMTKNQVSLTCLVKGFYPSDIAVEWESNGQPENNYKTTPPVLDSDGSFFLYSKLTVDKSRWQQGNVFSCSVMHEALHNHYTQKSLSLSPGK

SEQ ID NO: 65 - protein, 443 aa, synthetic construct
  REGION 1..443: note = CD80-Atezolizumab
VIHVTKEVKEVATLSCGHNVSVEELAQTRIYWQKEKKMVLTMMSGDMNIWPEYKNRTIFDITNNLSIVILALRPSDEGTYECVVLKYEKDAFKREHLAEVTLSVKADFPTPSISDFEIPTSNIRRIICSTSGGFPEPHLSWLENGEELNAINTTVSQDPETELYAVSSKLDFNMTTNHSFMCLIKYGHLRVNQTFNWNTTKQEHFPDNGGGGSGGGGSGGGGSGGGGSGDIQMTQSPSSLSASVGDRVTITCRASQDVSTAVAWYQQKPGKAPKLLIYSASFLYSGVPSRFSGSGSGTDFTLTISSLQPEDFATYYCQQYLYHPATFGQGTKVEIKRTVAAPSVFIFPPSDEQLKSGTASVVCLLNNFYPREAKVQWKVDNALQSGNSQESVTEQDSKDSTYSLSSTLTLSKADYEKHKVYACEVTHQGLSSPVTKSFNRGEC

SEQ ID NO: 66 - protein, 641 aa, synthetic construct
  REGION 1..641: note = LAG3-Atezolizumab
LQPGAEVPVVWAQEGAPAQLPCSPTIPLQDLSLLRRAGVTWQHQPDSGPPAAAPGHPLAPGPHPAAPSSWGPRPRRYTVLSVGPGGLRSGRLPLQPRVQLDERGRQRGDFSLWLRPARRADAGEYRAAVHLRDRALSCRLRLRLGQASMTASPPGSLRASDWVILNCSFSRPDRPASVHWFRNRGQGRVPVRESPHHHLAESFLFLPQVSPMDSGPWGCILTYRDGFNVSIMYNLTVLGLEPPTPLTVYAGAGSRVGLPCRLPAGVGTRSFLTAKWTPPGGGPDLLVTGDNGDFTLRLEDVSQAQAGTYTCHIHLQEQQLNATVTLAIITVTPKSFGSPGSLGKLLCEVTPVSGQERFVWSSLDTPSQRSFSGPWLEAQEAQLLSQPWQCQLYQGERLLGAAVYFTGGGGSGGGGSGGGGSGGGGSGDIQMTQSPSSLSASVGDRVTITCRASQDVSTAVAWYQQKPGKAPKLLIYSASFLYSGVPSRFSGSGSGTDFTLTISSLQPEDFATYYCQQYLYHPATFGQGTKVEIKRTVAAPSVFIFPPSDEQLKSGTASVVCLLNNFYPREAKVQWKVDNALQSGNSQESVTEQDSKDSTYSLSSTLTLSKADYEKHKVYACEVTHQGLSSPVTKSFNRGEC

SEQ ID NO: 67 - protein, 921 aa, synthetic construct
  REGION 1..921: note = Atezolizumab-LAG3 IgD1/D2-CD80
EVQLVESGGGLVQPGGSLRLSCAASGFTFSDSWIHWVRQAPGKGLEWVAWISPYGGSTYYADSVKGRFTISADTSKNTAYLQMNSLRAEDTAVYYCARRHWPGGFDYWGQGTLVTVSSASTKGPSVFPLAPSSKSTSGGTAALGCLVKDYFPEPVTVSWNSGALTSGVHTFPAVLQSSGLYSLSSVVTVPSSSLGTQTYICNVNHKPSNTKVDKKVEPKSCDKTHTCPPCPAPELLGGPSVFLFPPKPKDTLMISRTPEVTCVVVDVSHEDPEVKFNWYVDGVEVHNAKTKPREEQYASTYRVVSVLTVLHQDWLNGKEYKCKVSNKALPAPIEKTISKAKGQPREPQVYTLPPSREEMTKNQVSLTCLVKGFYPSDIAVEWESNGQPENNYKTTPPVLDSDGSFFLYSKLTVDKSRWQQGNVFSCSVMHEALHNHYTQKSLSLSPGAGGGGSGGGGSGVIHVTKEVKEVATLSCGHNVSVEELAQTRIYWQKEKKMVLTMMSGDMNIWPEYKNRTIFDITNNLSIVILALRPSDEGTYECVVLKYEKDAFKREHLAEVTLSVKADFPTPSISDFEIPTSNIRRIICSTSGGFPEPHLSWLENGEELNAINTTVSQDPETELYAVSSKLDFNMTTNHSFMCLIKYGHLRVNQTFNWNTTKQEHFPDNGGGGSGGGGSGSLQPGAEVPVVWAQEGAPAQLPCSPTIPLQDLSLLRRAGVTWQHQPDSGPPAAAPGHPLAPGPHPAAPSSWGPRPRRYTVLSVGPGGLRSGRLPLQPRVQLDERGRQRGDFSLWLRPARRADAGEYRAAVHLRDRALSCRLRLRLGQASMTASPPGSLRASDWVILNCSFSRPDRPASVHWFRNRGQGRVPVRESPHHHLAESFLFLPQVSPMDSGPWGCILTYRDGFNVSIMYNLTVLGLEP

SEQ ID NO: 68 - protein, 1003 aa, synthetic construct
  REGION 1..1003: note = Atezolizumab-LAG3 IgD1/D2/D3-CD80
EVQLVESGGGLVQPGGSLRLSCAASGFTFSDSWIHWVRQAPGKGLEWVAWISPYGGSTYYADSVKGRFTISADTSKNTAYLQMNSLRAEDTAVYYCARRHWPGGFDYWGQGTLVTVSSASTKGPSVFPLAPSSKSTSGGTAALGCLVKDYFPEPVTVSWNSGALTSGVHTFPAVLQSSGLYSLSSVVTVPSSSLGTQTYICNVNHKPSNTKVDKKVEPKSCDKTHTCPPCPAPELLGGPSVFLFPPKPKDTLMISRTPEVTCVVVDVSHEDPEVKFNWYVDGVEVHNAKTKPREEQYASTYRVVSVLTVLHQDWLNGKEYKCKVSNKALPAPIEKTISKAKGQPREPQVYTLPPSREEMTKNQVSLTCLVKGFYPSDIAVEWESNGQPENNYKTTPPVLDSDGSFFLYSKLTVDKSRWQQGNVFSCSVMHEALHNHYTQKSLSLSPGAGGGGSGGGGSGVIHVTKEVKEVATLSCGHNVSVEELAQTRIYWQKEKKMVLTMMSGDMNIWPEYKNRTIFDITNNLSIVILALRPSDEGTYECVVLKYEKDAFKREHLAEVTLSVKADFPTPSISDFEIPTSNIRRIICSTSGGFPEPHLSWLENGEELNAINTTVSQDPETELYAVSSKLDFNMTTNHSFMCLIKYGHLRVNQTFNWNTTKQEHFPDNGGGGSGGGGSGLQPGAEVPVVWAQEGAPAQLPCSPTIPLQDLSLLRRAGVTWQHQPDSGPPAAAPGHPLAPGPHPAAPSSWGPRPRRYTVLSVGPGGLRSGRLPLQPRVQLDERGRQRGDFSLWLRPARRADAGEYRAAVHLRDRALSCRLRLRLGQASMTASPPGSLRASDWVILNCSFSRPDRPASVHWFRNRGQGRVPVRESPHHHLAESFLFLPQVSPMDSGPWGCILTYRDGFNVSIMYNLTVLGLEPPTPLTVYAGAGSRVGLPCRLPAGVGTRSFLTAKWTPPGGGPDLLVTGDNGDFTLRLEDVSQAQAGTYTCHIHLQEQQLNATVT

SEQ ID NO: 69 - protein, 1103 aa, synthetic construct
  REGION 1..1103: note = Atezolizumab-LAG3-CD80
EVQLVESGGGLVQPGGSLRLSCAASGFTFSDSWIHWVRQAPGKGLEWVAWISPYGGSTYYADSVKGRFTISADTSKNTAYLQMNSLRAEDTAVYYCARRHWPGGFDYWGQGTLVTVSSASTKGPSVFPLAPSSKSTSGGTAALGCLVKDYFPEPVTVSWNSGALTSGVHTFPAVLQSSGLYSLSSVVTVPSSSLGTQTYICNVNHKPSNTKVDKKVEPKSCDKTHTCPPCPAPELLGGPSVFLFPPKPKDTLMISRTPEVTCVVVDVSHEDPEVKFNWYVDGVEVHNAKTKPREEQYASTYRVVSVLTVLHQDWLNGKEYKCKVSNKALPAPIEKTISKAKGQPREPQVYTLPPSREEMTKNQVSLTCLVKGFYPSDIAVEWESNGQPENNYKTTPPVLDSDGSFFLYSKLTVDKSRWQQGNVFSCSVMHEALHNHYTQKSLSLSPGAGGGGSGGGGSGGGGSGGGSGVIHVTKEVKEVATLSCGHNVSVEELAQTRIYWQKEKKMVLTMMSGDMNIWPEYKNRTIFDITNNLSIVILALRPSDEGTYECVVLKYEKDAFKREHLAEVTLSVKADFPTPSISDFEIPTSNIRRIICSTSGGFPEPHLSWLENGEELNAINTTVSQDPETELYAVSSKLDFNMTTNHSFMCLIKYGHLRVNQTFNWNTTKQEHFPDNGGGGSGGGGSGGGGSGGGGSGLQPGAEVPVVWAQEGAPAQLPCSPTIPLQDLSLLRRAGVTWQHQPDSGPPAAAPGHPLAPGPHPAAPSSWGPRPRRYTVLSVGPGGLRSGRLPLQPRVQLDERGRQRGDFSLWLRPARRADAGEYRAAVHLRDRALSCRLRLRLGQASMTASPPGSLRASDWVILNCSFSRPDRPASVHWFRNRGQGRVPVRESPHHHLAESFLFLPQVSPMDSGPWGCILTYRDGFNVSIMYNLTVLGLEPPTPLTVYAGAGSRVGLPCRLPAGVGTRSFLTAKWTPPGGGPDLLVTGDNGDFTLRLEDVSQAQAGTYTCHIHLQEQQLNATVTLAIITVTPKSFGSPGSLGKLLCEVTPVSGQERFVWSSLDTPSQRSFSGPWLEAQEAQLLSQPWQCQLYQGERLLGAAVYFT

SEQ ID NO: 70 - protein, 921 aa, synthetic construct
  REGION 1..921: note = Atezolizumab-CD80-LAG3 IgD1/D2
EVQLVESGGGLVQPGGSLRLSCAASGFTFSDSWIHWVRQAPGKGLEWVAWISPYGGSTYYADSVKGRFTISADTSKNTAYLQMNSLRAEDTAVYYCARRHWPGGFDYWGQGTLVTVSSASTKGPSVFPLAPSSKSTSGGTAALGCLVKDYFPEPVTVSWNSGALTSGVHTFPAVLQSSGLYSLSSVVTVPSSSLGTQTYICNVNHKPSNTKVDKKVEPKSCDKTHTCPPCPAPELLGGPSVFLFPPKPKDTLMISRTPEVTCVVVDVSHEDPEVKFNWYVDGVEVHNAKTKPREEQYASTYRVVSVLTVLHQDWLNGKEYKCKVSNKALPAPIEKTISKAKGQPREPQVYTLPPSREEMTKNQVSLTCLVKGFYPSDIAVEWESNGQPENNYKTTPPVLDSDGSFFLYSKLTVDKSRWQQGNVFSCSVMHEALHNHYTQKSLSLSPGAGGGGSGGGGSGSLQPGAEVPVVWAQEGAPAQLPCSPTIPLQDLSLLRRAGVTWQHQPDSGPPAAAPGHPLAPGPHPAAPSSWGPRPRRYTVLSVGPGGLRSGRLPLQPRVQLDERGRQRGDFSLWLRPARRADAGEYRAAVHLRDRALSCRLRLRLGQASMTASPPGSLRASDWVILNCSFSRPDRPASVHWFRNRGQGRVPVRESPHHHLAESFLFLPQVSPMDSGPWGCILTYRDGFNVSIMYNLTVLGLEPGGGGSGGGGSGVIHVTKEVKEVATLSCGHNVSVEELAQTRIYWQKEKKMVLTMMSGDMNIWPEYKNRTIFDITNNLSIVILALRPSDEGTYECVVLKYEKDAFKREHLAEVTLSVKADFPTPSISDFEIPTSNIRRIICSTSGGFPEPHLSWLENGEELNAINTTVSQDPETELYAVSSKLDFNMTTNHSFMCLIKYGHLRVNQTFNWNTTKQEHFPDN

SEQ ID NO: 71 - protein, 1003 aa, synthetic construct
  REGION 1..1003: note = Atezolizumab-CD80-LAG3 IgD1/D2/D3
EVQLVESGGGLVQPGGSLRLSCAASGFTFSDSWIHWVRQAPGKGLEWVAWISPYGGSTYYADSVKGRFTISADTSKNTAYLQMNSLRAEDTAVYYCARRHWPGGFDYWGQGTLVTVSSASTKGPSVFPLAPSSKSTSGGTAALGCLVKDYFPEPVTVSWNSGALTSGVHTFPAVLQSSGLYSLSSVVTVPSSSLGTQTYICNVNHKPSNTKVDKKVEPKSCDKTHTCPPCPAPELLGGPSVFLFPPKPKDTLMISRTPEVTCVVVDVSHEDPEVKFNWYVDGVEVHNAKTKPREEQYASTYRVVSVLTVLHQDWLNGKEYKCKVSNKALPAPIEKTISKAKGQPREPQVYTLPPSREEMTKNQVSLTCLVKGFYPSDIAVEWESNGQPENNYKTTPPVLDSDGSFFLYSKLTVDKSRWQQGNVFSCSVMHEALHNHYTQKSLSLSPGAGGGGSGGGGSGLQPGAEVPVVWAQEGAPAQLPCSPTIPLQDLSLLRRAGVTWQHQPDSGPPAAAPGHPLAPGPHPAAPSSWGPRPRRYTVLSVGPGGLRSGRLPLQPRVQLDERGRQRGDFSLWLRPARRADAGEYRAAVHLRDRALSCRLRLRLGQASMTASPPGSLRASDWVILNCSFSRPDRPASVHWFRNRGQGRVPVRESPHHHLAESFLFLPQVSPMDSGPWGCILTYRDGFNVSIMYNLTVLGLEPPTPLTVYAGAGSRVGLPCRLPAGVGTRSFLTAKWTPPGGGPDLLVTGDNGDFTLRLEDVSQAQAGTYTCHIHLQEQQLNATVTGGGGSGGGGSGVIHVTKEVKEVATLSCGHNVSVEELAQTRIYWQKEKKMVLTMMSGDMNIWPEYKNRTIFDITNNLSIVILALRPSDEGTYECVVLKYEKDAFKREHLAEVTLSVKADFPTPSISDFEIPTSNIRRIICSTSGGFPEPHLSWLENGEELNAINTTVSQDPETELYAVSSKLDFNMTTNHSFMCLIKYGHLRVNQTFNWNTTKQEHFPDN

SEQ ID NO: 72 - protein, 1103 aa, synthetic construct
  REGION 1..1103: note = Atezolizumab-CD80-LAG3
EVQLVESGGGLVQPGGSLRLSCAASGFTFSDSWIHWVRQAPGKGLEWVAWISPYGGSTYYADSVKGRFTISADTSKNTAYLQMNSLRAEDTAVYYCARRHWPGGFDYWGQGTLVTVSSASTKGPSVFPLAPSSKSTSGGTAALGCLVKDYFPEPVTVSWNSGALTSGVHTFPAVLQSSGLYSLSSVVTVPSSSLGTQTYICNVNHKPSNTKVDKKVEPKSCDKTHTCPPCPAPELLGGPSVFLFPPKPKDTLMISRTPEVTCVVVDVSHEDPEVKFNWYVDGVEVHNAKTKPREEQYASTYRVVSVLTVLHQDWLNGKEYKCKVSNKALPAPIEKTISKAKGQPREPQVYTLPPSREEMTKNQVSLTCLVKGFYPSDIAVEWESNGQPENNYKTTPPVLDSDGSFFLYSKLTVDKSRWQQGNVFSCSVMHEALHNHYTQKSLSLSPGAGGGGSGGGGSGGGGSGGGGSGLQPGAEVPVVWAQEGAPAQLPCSPTIPLQDLSLLRRAGVTWQHQPDSGPPAAAPGHPLAPGPHPAAPSSWGPRPRRYTVLSVGPGGLRSGRLPLQPRVQLDERGRQRGDFSLWLRPARRADAGEYRAAVHLRDRALSCRLRLRLGQASMTASPPGSLRASDWVILNCSFSRPDRPASVHWFRNRGQGRVPVRESPHHHLAESFLFLPQVSPMDSGPWGCILTYRDGFNVSIMYNLTVLGLEPPTPLTVYAGAGSRVGLPCRLPAGVGTRSFLTAKWTPPGGGPDLLVTGDNGDFTLRLEDVSQAQAGTYTCHIHLQEQQLNATVTLAIITVTPKSFGSPGSLGKLLCEVTPVSGQERFVWSSLDTPSQRSFSGPWLEAQEAQLLSQPWQCQLYQGERLLGAAVYFTGGGGSGGGGSGGGGSGGGSGVIHVTKEVKEVATLSCGHNVSVEELAQTRIYWQKEKKMVLTMMSGDMNIWPEYKNRTIFDITNNLSIVILALRPSDEGTYECVVLKYEKDAFKREHLAEVTLSVKADFPTPSISDFEIPTSNIRRIICSTSGGFPEPHLSWLENGEELNAINTTVSQDPETELYAVSSKLDFNMTTNHSFMCLIKYGHLRVNQTFNWNTTKQEHFPDN

SEQ ID NO: 73 - protein, 1103 aa, synthetic construct
  REGION 1..1103: note = LAG3-Atezolizumab-CD80
LQPGAEVPVVWAQEGAPAQLPCSPTIPLQDLSLLRRAGVTWQHQPDSGPPAAAPGHPLAPGPHPAAPSSWGPRPRRYTVLSVGPGGLRSGRLPLQPRVQLDERGRQRGDFSLWLRPARRADAGEYRAAVHLRDRALSCRLRLRLGQASMTASPPGSLRASDWVILNCSFSRPDRPASVHWFRNRGQGRVPVRESPHHHLAESFLFLPQVSPMDSGPWGCILTYRDGFNVSIMYNLTVLGLEPPTPLTVYAGAGSRVGLPCRLPAGVGTRSFLTAKWTPPGGGPDLLVTGDNGDFTLRLEDVSQAQAGTYTCHIHLQEQQLNATVTLAIITVTPKSFGSPGSLGKLLCEVTPVSGQERFVWSSLDTPSQRSFSGPWLEAQEAQLLSQPWQCQLYQGERLLGAAVYFTGGGGSGGGGSGGGGSGGGSGEVQLVESGGGLVQPGGSLRLSCAASGFTFSDSWIHWVRQAPGKGLEWVAWISPYGGSTYYADSVKGRFTISADTSKNTAYLQMNSLRAEDTAVYYCARRHWPGGFDYWGQGTLVTVSSASTKGPSVFPLAPSSKSTSGGTAALGCLVKDYFPEPVTVSWNSGALTSGVHTFPAVLQSSGLYSLSSVVTVPSSSLGTQTYICNVNHKPSNTKVDKKVEPKSCDKTHTCPPCPAPELLGGPSVFLFPPKPKDTLMISRTPEVTCVVVDVSHEDPEVKFNWYVDGVEVHNAKTKPREEQYASTYRVVSVLTVLHQDWLNGKEYKCKVSNKALPAPIEKTISKAKGQPREPQVYTLPPSREEMTKNQVSLTCLVKGFYPSDIAVEWESNGQPENNYKTTPPVLDSDGSFFLYSKLTVDKSRWQQGNVFSCSVMHEALHNHYTQKSLSLSPGAGGGGSGGGGSGGGGSGGGGSGVIHVTKEVKEVATLSCGHNVSVEELAQTRIYWQKEKKMVLTMMSGDMNIWPEYKNRTIFDITNNLSIVILALRPSDEGTYECVVLKYEKDAFKREHLAEVTLSVKADFPTPSISDFEIPTSNIRRIICSTSGGFPEPHLSWLENGEELNAINTTVSQDPETELYAVSSKLDFNMTTNHSFMCLIKYGHLRVNQTFNWNTTKQEHFPDN

SEQ ID NO: 74 - protein, 1103 aa, synthetic construct
  REGION 1..1103: note = CD80-Atezolizumab-LAG3
VIHVTKEVKEVATLSCGHNVSVEELAQTRIYWQKEKKMVLTMMSGDMNIWPEYKNRTIFDITNNLSIVILALRPSDEGTYECVVLKYEKDAFKREHLAEVTLSVKADFPTPSISDFEIPTSNIRRIICSTSGGFPEPHLSWLENGEELNAINTTVSQDPETELYAVSSKLDFNMTTNHSFMCLIKYGHLRVNQTFNWNTTKQEHFPDNGGGGSGGGGSGGGGSGGGSGEVQLVESGGGLVQPGGSLRLSCAASGFTFSDSWIHWVRQAPGKGLEWVAWISPYGGSTYYADSVKGRFTISADTSKNTAYLQMNSLRAEDTAVYYCARRHWPGGFDYWGQGTLVTVSSASTKGPSVFPLAPSSKSTSGGTAALGCLVKDYFPEPVTVSWNSGALTSGVHTFPAVLQSSGLYSLSSVVTVPSSSLGTQTYICNVNHKPSNTKVDKKVEPKSCDKTHTCPPCPAPELLGGPSVFLFPPKPKDTLMISRTPEVTCVVVDVSHEDPEVKFNWYVDGVEVHNAKTKPREEQYASTYRVVSVLTVLHQDWLNGKEYKCKVSNKALPAPIEKTISKAKGQPREPQVYTLPPSREEMTKNQVSLTCLVKGFYPSDIAVEWESNGQPENNYKTTPPVLDSDGSFFLYSKLTVDKSRWQQGNVFSCSVMHEALHNHYTQKSLSLSPGAGGGGSGGGGSGGGGSGGGGSGLQPGAEVPVVWAQEGAPAQLPCSPTIPLQDLSLLRRAGVTWQHQPDSGPPAAAPGHPLAPGPHPAAPSSWGPRPRRYTVLSVGPGGLRSGRLPLQPRVQLDERGRQRGDFSLWLRPARRADAGEYRAAVHLRDRALSCRLRLRLGQASMTASPPGSLRASDWVILNCSFSRPDRPASVHWFRNRGQGRVPVRESPHHHLAESFLFLPQVSPMDSGPWGCILTYRDGFNVSIMYNLTVLGLEPPTPLTVYAGAGSRVGLPCRLPAGVGTRSFLTAKWTPPGGGPDLLVTGDNGDFTLRLEDVSQAQAGTYTCHIHLQEQQLNATVTLAIITVTPKSFGSPGSLGKLLCEVTPVSGQERFVWSSLDTPSQRSFSGPWLEAQEAQLLSQPWQCQLYQGERLLGAAVYFT

SEQ ID NO: 75 - protein, 679 aa, synthetic construct
  REGION 1..679: note = Avelumab-CD80
EVQLLESGGGLVQPGGSLRLSCAASGFTFSSYIMMWVRQAPGKGLEWVSSIYPSGGITFYADTVKGRFTISRDNSKNTLYLQMNSLRAEDTAVYYCARIKLGTVTTVDYWGQGTLVTVSSASTKGPSVFPLAPSSKSTSGGTAALGCLVKDYFPEPVTVSWNSGALTSGVHTFPAVLQSSGLYSLSSVVTVPSSSLGTQTYICNVNHKPSNTKVDKKVEPKSCDKTHTCPPCPAPELLGGPSVFLFPPKPKDTLMISRTPEVTCVVVDVSHEDPEVKFNWYVDGVEVHNAKTKPREEQYNSTYRVVSVLTVLHQDWLNGKEYKCKVSNKALPAPIEKTISKAKGQPREPQVYTLPPSRDELTKNQVSLTCLVKGFYPSDIAVEWESNGQPENNYKTTPPVLDSDGSFFLYSKLTVDKSRWQQGNVFSCSVMHEALHNHYTQKSLSLSPGAGGGGSGGGGSGGGGSGGGGSGVIHVTKEVKEVATLSCGHNVSVEELAQTRIYWQKEKKMVLTMMSGDMNIWPEYKNRTIFDITNNLSIVILALRPSDEGTYECVVLKYEKDAFKREHLAEVTLSVKADFPTPSISDFEIPTSNIRRIICSTSGGFPEPHLSWLENGEELNAINTTVSQDPETELYAVSSKLDFNMTTNHSFMCLIKYGHLRVNQTFNWNTTKQEHFPDN

SEQ ID NO: 76 - protein, 877 aa, synthetic construct
  REGION 1..877: note = Avelumab-LAG3
EVQLLESGGGLVQPGGSLRLSCAASGFTFSSYIMMWVRQAPGKGLEWVSSIYPSGGITFYADTVKGRFTISRDNSKNTLYLQMNSLRAEDTAVYYCARIKLGTVTTVDYWGQGTLVTVSSASTKGPSVFPLAPSSKSTSGGTAALGCLVKDYFPEPVTVSWNSGALTSGVHTFPAVLQSSGLYSLSSVVTVPSSSLGTQTYICNVNHKPSNTKVDKKVEPKSCDKTHTCPPCPAPELLGGPSVFLFPPKPKDTLMISRTPEVTCVVVDVSHEDPEVKFNWYVDGVEVHNAKTKPREEQYNSTYRVVSVLTVLHQDWLNGKEYKCKVSNKALPAPIEKTISKAKGQPREPQVYTLPPSRDELTKNQVSLTCLVKGFYPSDIAVEWESNGQPENNYKTTPPVLDSDGSFFLYSKLTVDKSRWQQGNVFSCSVMHEALHNHYTQKSLSLSPGAGGGGSGGGGSGGGGSGGGGSGLQPGAEVPVVWAQEGAPAQLPCSPTIPLQDLSLLRRAGVTWQHQPDSGPPAAAPGHPLAPGPHPAAPSSWGPRPRRYTVLSVGPGGLRSGRLPLQPRVQLDERGRQRGDFSLWLRPARRADAGEYRAAVHLRDRALSCRLRLRLGQASMTASPPGSLRASDWVILNCSFSRPDRPASVHWFRNRGQGRVPVRESPHHHLAESFLFLPQVSPMDSGPWGCILTYRDGFNVSIMYNLTVLGLEPPTPLTVYAGAGSRVGLPCRLPAGVGTRSFLTAKWTPPGGGPDLLVTGDNGDFTLRLEDVSQAQAGTYTCHIHLQEQQLNATVTLAIITVTPKSFGSPGSLGKLLCEVTPVSGQERFVWSSLDTPSQRSFSGPWLEAQEAQLLSQPWQCQLYQGERLLGAAVYFT

SEQ ID NO: 77 - protein, 713 aa, synthetic construct
  REGION 1..713: note = Avelumab-LAG3 IgD1/D2
EVQLLESGGGLVQPGGSLRLSCAASGFTFSSYIMMWVRQAPGKGLEWVSSIYPSGGITFYADTVKGRFTISRDNSKNTLYLQMNSLRAEDTAVYYCARIKLGTVTTVDYWGQGTLVTVSSASTKGPSVFPLAPSSKSTSGGTAALGCLVKDYFPEPVTVSWNSGALTSGVHTFPAVLQSSGLYSLSSVVTVPSSSLGTQTYICNVNHKPSNTKVDKKVEPKSCDKTHTCPPCPAPELLGGPSVFLFPPKPKDTLMISRTPEVTCVVVDVSHEDPEVKFNWYVDGVEVHNAKTKPREEQYNSTYRVVSVLTVLHQDWLNGKEYKCKVSNKALPAPIEKTISKAKGQPREPQVYTLPPSRDELTKNQVSLTCLVKGFYPSDIAVEWESNGQPENNYKTTPPVLDSDGSFFLYSKLTVDKSRWQQGNVFSCSVMHEALHNHYTQKSLSLSPGAGGGGSGGGGSGGGGSGGGGSGLQPGAEVPVVWAQEGAPAQLPCSPTIPLQDLSLLRRAGVTWQHQPDSGPPAAAPGHPLAPGPHPAAPSSWGPRPRRYTVLSVGPGGLRSGRLPLQPRVQLDERGRQRGDFSLWLRPARRADAGEYRAAVHLRDRALSCRLRLRLGQASMTASPPGSLRASDWVILNCSFSRPDRPASVHWFRNRGQGRVPVRESPHHHLAESFLFLPQVSPMDSGPWGCILTYRDGFNVSIMYNLTVLGLEP

SEQ ID NO: 78 - protein, 796 aa, synthetic construct
  REGION 1..796: note = Avelumab-LAG3 IgD1/D2/D3
EVQLLESGGGLVQPGGSLRLSCAASGFTFSSYIMMWVRQAPGKGLEWVSSIYPSGGITFYADTVKGRFTISRDNSKNTLYLQMNSLRAEDTAVYYCARIKLGTVTTVDYWGQGTLVTVSSASTKGPSVFPLAPSSKSTSGGTAALGCLVKDYFPEPVTVSWNSGALTSGVHTFPAVLQSSGLYSLSSVVTVPSSSLGTQTYICNVNHKPSNTKVDKKVEPKSCDKTHTCPPCPAPELLGGPSVFLFPPKPKDTLMISRTPEVTCVVVDVSHEDPEVKFNWYVDGVEVHNAKTKPREEQYNSTYRVVSVLTVLHQDWLNGKEYKCKVSNKALPAPIEKTISKAKGQPREPQVYTLPPSRDELTKNQVSLTCLVKGFYPSDIAVEWESNGQPENNYKTTPPVLDSDGSFFLYSKLTVDKSRWQQGNVFSCSVMHEALHNHYTQKSLSLSPGAGGGGSGGGGSGGGGSGGGGSGLQPGAEVPVVWAQEGAPAQLPCSPTIPLQDLSLLRRAGVTWQHQPDSGPPAAAPGHPLAPGPHPAAPSSWGPRPRRYTVLSVGPGGLRSGRLPLQPRVQLDERGRQRGDFSLWLRPARRADAGEYRAAVHLRDRALSCRLRLRLGQASMTASPPGSLRASDWVILNCSFSRPDRPASVHWFRNRGQGRVPVRESPHHHLAESFLFLPQVSPMDSGPWGCILTYRDGFNVSIMYNLTVLGLEPPTPLTVYAGAGSRVGLPCRLPAGVGTRSFLTAKWTPPGGGPDLLVTGDNGDFTLRLEDVSQAQAGTYTCHIHLQEQQLNATVT

SEQ ID NO: 79 - protein, 679 aa, synthetic construct
  REGION 1..679: note = CD80-Avelumab
VIHVTKEVKEVATLSCGHNVSVEELAQTRIYWQKEKKMVLTMMSGDMNIWPEYKNRTIFDITNNLSIVILALRPSDEGTYECVVLKYEKDAFKREHLAEVTLSVKADFPTPSISDFEIPTSNIRRIICSTSGGFPEPHLSWLENGEELNAINTTVSQDPETELYAVSSKLDFNMTTNHSFMCLIKYGHLRVNQTFNWNTTKQEHFPDNGGGGSGGGGSGGGGSGGGGSGEVQLLESGGGLVQPGGSLRLSCAASGFTFSSYIMMWVRQAPGKGLEWVSSIYPSGGITFYADTVKGRFTISRDNSKNTLYLQMNSLRAEDTAVYYCARIKLGTVTTVDYWGQGTLVTVSSASTKGPSVFPLAPSSKSTSGGTAALGCLVKDYFPEPVTVSWNSGALTSGVHTFPAVLQSSGLYSLSSVVTVPSSSLGTQTYICNVNHKPSNTKVDKKVEPKSCDKTHTCPPCPAPELLGGPSVFLFPPKPKDTLMISRTPEVTCVVVDVSHEDPEVKFNWYVDGVEVHNAKTKPREEQYNSTYRVVSVLTVLHQDWLNGKEYKCKVSNKALPAPIEKTISKAKGQPREPQVYTLPPSRDELTKNQVSLTCLVKGFYPSDIAVEWESNGQPENNYKTTPPVLDSDGSFFLYSKLTVDKSRWQQGNVFSCSVMHEALHNHYTQKSLSLSPGK

SEQ ID NO: 80 - protein, 877 aa, synthetic construct
  REGION 1..877: note = LAG3-Avelumab
LQPGAEVPVVWAQEGAPAQLPCSPTIPLQDLSLLRRAGVTWQHQPDSGPPAAAPGHPLAPGPHPAAPSSWGPRPRRYTVLSVGPGGLRSGRLPLQPRVQLDERGRQRGDFSLWLRPARRADAGEYRAAVHLRDRALSCRLRLRLGQASMTASPPGSLRASDWVILNCSFSRPDRPASVHWFRNRGQGRVPVRESPHHHLAESFLFLPQVSPMDSGPWGCILTYRDGFNVSIMYNLTVLGLEPPTPLTVYAGAGSRVGLPCRLPAGVGTRSFLTAKWTPPGGGPDLLVTGDNGDFTLRLEDVSQAQAGTYTCHIHLQEQQLNATVTLAIITVTPKSFGSPGSLGKLLCEVTPVSGQERFVWSSLDTPSQRSFSGPWLEAQEAQLLSQPWQCQLYQGERLLGAAVYFTGGGGSGGGGSGGGGSGGGGSGEVQLLESGGGLVQPGGSLRLSCAASGFTFSSYIMMWVRQAPGKGLEWVSSIYPSGGITFYADTVKGRFTISRDNSKNTLYLQMNSLRAEDTAVYYCARIKLGTVTTVDYWGQGTLVTVSSASTKGPSVFPLAPSSKSTSGGTAALGCLVKDYFPEPVTVSWNSGALTSGVHTFPAVLQSSGLYSLSSVVTVPSSSLGTQTYICNVNHKPSNTKVDKKVEPKSCDKTHTCPPCPAPELLGGPSVFLFPPKPKDTLMISRTPEVTCVVVDVSHEDPEVKFNWYVDGVEVHNAKTKPREEQYNSTYRVVSVLTVLHQDWLNGKEYKCKVSNKALPAPIEKTISKAKGQPREPQVYTLPPSRDELTKNQVSLTCLVKGFYPSDIAVEWESNGQPENNYKTTPPVLDSDGSFFLYSKLTVDKSRWQQGNVFSCSVMHEALHNHYTQKSLSLSPGK

SEQ ID NO: 81 - protein, 445 aa, synthetic construct
  REGION 1..445: note = CD80-Avelumab
VIHVTKEVKEVATLSCGHNVSVEELAQTRIYWQKEKKMVLTMMSGDMNIWPEYKNRTIFDITNNLSIVILALRPSDEGTYECVVLKYEKDAFKREHLAEVTLSVKADFPTPSISDFEIPTSNIRRIICSTSGGFPEPHLSWLENGEELNAINTTVSQDPETELYAVSSKLDFNMTTNHSFMCLIKYGHLRVNQTFNWNTTKQEHFPDNGGGGSGGGGSGGGGSGGGGSGQSALTQPASVSGSPGQSITISCTGTSSDVGGYNYVSWYQQHPGKAPKLMIYDVSNRPSGVSNRFSGSKSGNTASLTISGLQAEDEADYYCSSYTSSSTRVFGTGTKVTVLGQPKANPTVTLFPPSSEELQANKATLVCLISDFYPGAVTVAWKADGSPVKAGVETTKPSKQSNNKYAASSYLSLTPEQWKSHRSYSCQVTHEGSTVEKTVAPTECS

SEQ ID NO: 82 - protein, 643 aa, synthetic construct
  REGION 1..643: note = LAG3-Avelumab
LQPGAEVPVVWAQEGAPAQLPCSPTIPLQDLSLLRRAGVTWQHQPDSGPPAAAPGHPLAPGPHPAAPSSWGPRPRRYTVLSVGPGGLRSGRLPLQPRVQLDERGRQRGDFSLWLRPARRADAGEYRAAVHLRDRALSCRLRLRLGQASMTASPPGSLRASDWVILNCSFSRPDRPASVHWFRNRGQGRVPVRESPHHHLAESFLFLPQVSPMDSGPWGCILTYRDGFNVSIMYNLTVLGLEPPTPLTVYAGAGSRVGLPCRLPAGVGTRSFLTAKWTPPGGGPDLLVTGDNGDFTLRLEDVSQAQAGTYTCHIHLQEQQLNATVTLAIITVTPKSFGSPGSLGKLLCEVTPVSGQERFVWSSLDTPSQRSFSGPWLEAQEAQLLSQPWQCQLYQGERLLGAAVYFTGGGGSGGGGSGGGGSGGGGSGQSALTQPASVSGSPGQSITISCTGTSSDVGGYNYVSWYQQHPGKAPKLMIYDVSNRPSGVSNRFSGSKSGNTASLTISGLQAEDEADYYCSSYTSSSTRVFGTGTKVTVLGQPKANPTVTLFPPSSEELQANKATLVCLISDFYPGAVTVAWKADGSPVKAGVETTKPSKQSNNKYAASSYLSLTPEQWKSHRSYSCQVTHEGSTVEKTVAPTECS

SEQ ID NO: 83 - protein, 923 aa, synthetic construct
  REGION 1..923: note = Avelumab-LAG3 IgD1/D2-CD80
EVQLLESGGGLVQPGGSLRLSCAASGFTFSSYIMMWVRQAPGKGLEWVSSIYPSGGITFYADTVKGRFTISRDNSKNTLYLQMNSLRAEDTAVYYCARIKLGTVTTVDYWGQGTLVTVSSASTKGPSVFPLAPSSKSTSGGTAALGCLVKDYFPEPVTVSWNSGALTSGVHTFPAVLQSSGLYSLSSVVTVPSSSLGTQTYICNVNHKPSNTKVDKKVEPKSCDKTHTCPPCPAPELLGGPSVFLFPPKPKDTLMISRTPEVTCVVVDVSHEDPEVKFNWYVDGVEVHNAKTKPREEQYNSTYRVVSVLTVLHQDWLNGKEYKCKVSNKALPAPIEKTISKAKGQPREPQVYTLPPSRDELTKNQVSLTCLVKGFYPSDIAVEWESNGQPENNYKTTPPVLDSDGSFFLYSKLTVDKSRWQQGNVFSCSVMHEALHNHYTQKSLSLSPGAGGGGSGGGGSGVIHVTKEVKEVATLSCGHNVSVEELAQTRIYWQKEKKMVLTMMSGDMNIWPEYKNRTIFDITNNLSIVILALRPSDEGTYECVVLKYEKDAFKREHLAEVTLSVKADFPTPSISDFEIPTSNIRRIICSTSGGFPEPHLSWLENGEELNAINTTVSQDPETELYAVSSKLDFNMTTNHSFMCLIKYGHLRVNQTFNWNTTKQEHFPDNGGGGSGGGGSGSLQPGAEVPVVWAQEGAPAQLPCSPTIPLQDLSLLRRAGVTWQHQPDSGPPAAAPGHPLAPGPHPAAPSSWGPRPRRYTVLSVGPGGLRSGRLPLQPRVQLDERGRQRGDFSLWLRPARRADAGEYRAAVHLRDRALSCRLRLRLGQASMTASPPGSLRASDWVILNCSFSRPDRPASVHWFRNRGQGRVPVRESPHHHLAESFLFLPQVSPMDSGPWGCILTYRDGFNVSIMYNLTVLGLEP

SEQ ID NO: 84 - protein, 1005 aa, synthetic construct
  REGION 1..1005: note = Avelumab-LAG3 IgD1/D2/D3-CD80
EVQLLESGGGLVQPGGSLRLSCAASGFTFSSYIMMWVRQAPGKGLEWVSSIYPSGGITFYADTVKGRFTISRDNSKNTLYLQMNSLRAEDTAVYYCARIKLGTVTTVDYWGQGTLVTVSSASTKGPSVFPLAPSSKSTSGGTAALGCLVKDYFPEPVTVSWNSGALTSGVHTFPAVLQSSGLYSLSSVVTVPSSSLGTQTYICNVNHKPSNTKVDKKVEPKSCDKTHTCPPCPAPELLGGPSVFLFPPKPKDTLMISRTPEVTCVVVDVSHEDPEVKFNWYVDGVEVHNAKTKPREEQYNSTYRVVSVLTVLHQDWLNGKEYKCKVSNKALPAPIEKTISKAKGQPREPQVYTLPPSRDELTKNQVSLTCLVKGFYPSDIAVEWESNGQPENNYKTTPPVLDSDGSFFLYSKLTVDKSRWQQGNVFSCSVMHEALHNHYTQKSLSLSPGAGGGGSGGGGSGVIHVTKEVKEVATLSCGHNVSVEELAQTRIYWQKEKKMVLTMMSGDMNIWPEYKNRTIFDITNNLSIVILALRPSDEGTYECVVLKYEKDAFKREHLAEVTLSVKADFPTPSISDFEIPTSNIRRIICSTSGGFPEPHLSWLENGEELNAINTTVSQDPETELYAVSSKLDFNMTTNHSFMCLIKYGHLRVNQTFNWNTTKQEHFPDNGGGGSGGGGSGLQPGAEVPVVWAQEGAPAQLPCSPTIPLQDLSLLRRAGVTWQHQPDSGPPAAAPGHPLAPGPHPAAPSSWGPRPRRYTVLSVGPGGLRSGRLPLQPRVQLDERGRQRGDFSLWLRPARRADAGEYRAAVHLRDRALSCRLRLRLGQASMTASPPGSLRASDWVILNCSFSRPDRPASVHWFRNRGQGRVPVRESPHHHLAESFLFLPQVSPMDSGPWGCILTYRDGFNVSIMYNLTVLGLEPPTPLTVYAGAGSRVGLPCRLPAGVGTRSFLTAKWTPPGGGPDLLVTGDNGDFTLRLEDVSQAQAGTYTCHIHLQEQQLNATVT

SEQ ID NO: 85 - protein, 1105 aa, synthetic construct
  REGION 1..1105: note = Avelumab-LAG3-CD80
EVQLLESGGGLVQPGGSLRLSCAASGFTFSSYIMMWVRQAPGKGLEWVSSIYPSGGITFYADTVKGRFTISRDNSKNTLYLQMNSLRAEDTAVYYCARIKLGTVTTVDYWGQGTLVTVSSASTKGPSVFPLAPSSKSTSGGTAALGCLVKDYFPEPVTVSWNSGALTSGVHTFPAVLQSSGLYSLSSVVTVPSSSLGTQTYICNVNHKPSNTKVDKKVEPKSCDKTHTCPPCPAPELLGGPSVFLFPPKPKDTLMISRTPEVTCVVVDVSHEDPEVKFNWYVDGVEVHNAKTKPREEQYNSTYRVVSVLTVLHQDWLNGKEYKCKVSNKALPAPIEKTISKAKGQPREPQVYTLPPSRDELTKNQVSLTCLVKGFYPSDIAVEWESNGQPENNYKTTPPVLDSDGSFFLYSKLTVDKSRWQQGNVFSCSVMHEALHNHYTQKSLSLSPGAGGGGSGGGGSGGGGSGGGSGVIHVTKEVKEVATLSCGHNVSVEELAQTRIYWQKEKKMVLTMMSGDMNIWPEYKNRTIFDITNNLSIVILALRPSDEGTYECVVLKYEKDAFKREHLAEVTLSVKADFPTPSISDFEIPTSNIRRIICSTSGGFPEPHLSWLENGEELNAINTTVSQDPETELYAVSSKLDFNMTTNHSFMCLIKYGHLRVNQTFNWNTTKQEHFPDNGGGGSGGGGSGGGGSGGGGSGLQPGAEVPVVWAQEGAPAQLPCSPTIPLQDLSLLRRAGVTWQHQPDSGPPAAAPGHPLAPGPHPAAPSSWGPRPRRYTVLSVGPGGLRSGRLPLQPRVQLDERGRQRGDFSLWLRPARRADAGEYRAAVHLRDRALSCRLRLRLGQASMTASPPGSLRASDWVILNCSFSRPDRPASVHWFRNRGQGRVPVRESPHHHLAESFLFLPQVSPMDSGPWGCILTYRDGFNVSIMYNLTVLGLEPPTPLTVYAGAGSRVGLPCRLPAGVGTRSFLTAKWTPPGGGPDLLVTGDNGDFTLRLEDVSQAQAGTYTCHIHLQEQQLNATVTLAIITVTPKSFGSPGSLGKLLCEVTPVSGQERFVWSSLDTPSQRSFSGPWLEAQEAQLLSQPWQCQLYQGERLLGAAVYFT

SEQ ID NO: 86 - protein, 923 aa, synthetic construct
  REGION 1..923: note = Avelumab-CD80-LAG3 IgD1/D2
EVQLLESGGGLVQPGGSLRLSCAASGFTFSSYIMMWVRQAPGKGLEWVSSIYPSGGITFYADTVKGRFTISRDNSKNTLYLQMNSLRAEDTAVYYCARIKLGTVTTVDYWGQGTLVTVSSASTKGPSVFPLAPSSKSTSGGTAALGCLVKDYFPEPVTVSWNSGALTSGVHTFPAVLQSSGLYSLSSVVTVPSSSLGTQTYICNVNHKPSNTKVDKKVEPKSCDKTHTCPPCPAPELLGGPSVFLFPPKPKDTLMISRTPEVTCVVVDVSHEDPEVKFNWYVDGVEVHNAKTKPREEQYNSTYRVVSVLTVLHQDWLNGKEYKCKVSNKALPAPIEKTISKAKGQPREPQVYTLPPSRDELTKNQVSLTCLVKGFYPSDIAVEWESNGQPENNYKTTPPVLDSDGSFFLYSKLTVDKSRWQQGNVFSCSVMHEALHNHYTQKSLSLSPGAGGGGSGGGGSGSLQPGAEVPVVWAQEGAPAQLPCSPTIPLQDLSLLRRAGVTWQHQPDSGPPAAAPGHPLAPGPHPAAPSSWGPRPRRYTVLSVGPGGLRSGRLPLQPRVQLDERGRQRGDFSLWLRPARRADAGEYRAAVHLRDRALSCRLRLRLGQASMTASPPGSLRASDWVILNCSFSRPDRPASVHWFRNRGQGRVPVRESPHHHLAESFLFLPQVSPMDSGPWGCILTYRDGFNVSIMYNLTVLGLEPGGGGSGGGGSGVIHVTKEVKEVATLSCGHNVSVEELAQTRIYWQKEKKMVLTMMSGDMNIWPEYKNRTIFDITNNLSIVILALRPSDEGTYECVVLKYEKDAFKREHLAEVTLSVKADFPTPSISDFEIPTSNIRRIICSTSGGFPEPHLSWLENGEELNAINTTVSQDPETELYAVSSKLDFNMTTNHSFMCLIKYGHLRVNQTFNWNTTKQEHFPDN

SEQ ID NO: 87 - protein, 1005 aa, synthetic construct
  REGION 1..1005: note = Avelumab-CD80-LAG3 IgD1/D2/D3
EVQLLESGGGLVQPGGSLRLSCAASGFTFSSYIMMWVRQAPGKGLEWVSSIYPSGGITFYADTVKGRFTISRDNSKNTLYLQMNSLRAEDTAVYYCARIKLGTVTTVDYWGQGTLVTVSSASTKGPSVFPLAPSSKSTSGGTAALGCLVKDYFPEPVTVSWNSGALTSGVHTFPAVLQSSGLYSLSSVVTVPSSSLGTQTYICNVNHKPSNTKVDKKVEPKSCDKTHTCPPCPAPELLGGPSVFLFPPKPKDTLMISRTPEVTCVVVDVSHEDPEVKFNWYVDGVEVHNAKTKPREEQYNSTYRVVSVLTVLHQDWLNGKEYKCKVSNKALPAPIEKTISKAKGQPREPQVYTLPPSRDELTKNQVSLTCLVKGFYPSDIAVEWESNGQPENNYKTTPPVLDSDGSFFLYSKLTVDKSRWQQGNVFSCSVMHEALHNHYTQKSLSLSPGAGGGGSGGGGSGLQPGAEVPVVWAQEGAPAQLPCSPTIPLQDLSLLRRAGVTWQHQPDSGPPAAAPGHPLAPGPHPAAPSSWGPRPRRYTVLSVGPGGLRSGRLPLQPRVQLDERGRQRGDFSLWLRPARRADAGEYRAAVHLRDRALSCRLRLRLGQASMTASPPGSLRASDWVILNCSFSRPDRPASVHWFRNRGQGRVPVRESPHHHLAESFLFLPQVSPMDSGPWGCILTYRDGFNVSIMYNLTVLGLEPPTPLTVYAGAGSRVGLPCRLPAGVGTRSFLTAKWTPPGGGPDLLVTGDNGDFTLRLEDVSQAQAGTYTCHIHLQEQQLNATVTGGGGSGGGGSGVIHVTKEVKEVATLSCGHNVSVEELAQTRIYWQKEKKMVLTMMSGDMNIWPEYKNRTIFDITNNLSIVILALRPSDEGTYECVVLKYEKDAFKREHLAEVTLSVKADFPTPSISDFEIPTSNIRRIICSTSGGFPEPHLSWLENGEELNAINTTVSQDPETELYAVSSKLDFNMTTNHSFMCLIKYGHLRVNQTFNWNTTKQEHFPDN

SEQ ID NO: 88 - protein, 1105 aa, synthetic construct
  REGION 1..1105: note = Avelumab-CD80-LAG3
EVQLLESGGGLVQPGGSLRLSCAASGFTFSSYIMMWVRQAPGKGLEWVSSIYPSGGITFYADTVKGRFTISRDNSKNTLYLQMNSLRAEDTAVYYCARIKLGTVTTVDYWGQGTLVTVSSASTKGPSVFPLAPSSKSTSGGTAALGCLVKDYFPEPVTVSWNSGALTSGVHTFPAVLQSSGLYSLSSVVTVPSSSLGTQTYICNVNHKPSNTKVDKKVEPKSCDKTHTCPPCPAPELLGGPSVFLFPPKPKDTLMISRTPEVTCVVVDVSHEDPEVKFNWYVDGVEVHNAKTKPREEQYNSTYRVVSVLTVLHQDWLNGKEYKCKVSNKALPAPIEKTISKAKGQPREPQVYTLPPSRDELTKNQVSLTCLVKGFYPSDIAVEWESNGQPENNYKTTPPVLDSDGSFFLYSKLTVDKSRWQQGNVFSCSVMHEALHNHYTQKSLSLSPGAGGGGSGGGGSGGGGSGGGGSGLQPGAEVPVVWAQEGAPAQLPCSPTIPLQDLSLLRRAGVTWQHQPDSGPPAAAPGHPLAPGPHPAAPSSWGPRPRRYTVLSVGPGGLRSGRLPLQPRVQLDERGRQRGDFSLWLRPARRADAGEYRAAVHLRDRALSCRLRLRLGQASMTASPPGSLRASDWVILNCSFSRPDRPASVHWFRNRGQGRVPVRESPHHHLAESFLFLPQVSPMDSGPWGCILTYRDGFNVSIMYNLTVLGLEPPTPLTVYAGAGSRVGLPCRLPAGVGTRSFLTAKWTPPGGGPDLLVTGDNGDFTLRLEDVSQAQAGTYTCHIHLQEQQLNATVTLAIITVTPKSFGSPGSLGKLLCEVTPVSGQERFVWSSLDTPSQRSFSGPWLEAQEAQLLSQPWQCQLYQGERLLGAAVYFTGGGGSGGGGSGGGGSGGGSGVIHVTKEVKEVATLSCGHNVSVEELAQTRIYWQKEKKMVLTMMSGDMNIWPEYKNRTIFDITNNLSIVILALRPSDEGTYECVVLKYEKDAFKREHLAEVTLSVKADFPTPSISDFEIPTSNIRRIICSTSGGFPEPHLSWLENGEELNAINTTVSQDPETELYAVSSKLDFNMTTNHSFMCLIKYGHLRVNQTFNWNTTKQEHFPDN

SEQ ID NO: 89 - protein, 1105 aa, synthetic construct
  REGION 1..1105: note = LAG3-Avelumab-CD80
LQPGAEVPVVWAQEGAPAQLPCSPTIPLQDLSLLRRAGVTWQHQPDSGPPAAAPGHPLAPGPHPAAPSSWGPRPRRYTVLSVGPGGLRSGRLPLQPRVQLDERGRQRGDFSLWLRPARRADAGEYRAAVHLRDRALSCRLRLRLGQASMTASPPGSLRASDWVILNCSFSRPDRPASVHWFRNRGQGRVPVRESPHHHLAESFLFLPQVSPMDSGPWGCILTYRDGFNVSIMYNLTVLGLEPPTPLTVYAGAGSRVGLPCRLPAGVGTRSFLTAKWTPPGGGPDLLVTGDNGDFTLRLEDVSQAQAGTYTCHIHLQEQQLNATVTLAIITVTPKSFGSPGSLGKLLCEVTPVSGQERFVWSSLDTPSQRSFSGPWLEAQEAQLLSQPWQCQLYQGERLLGAAVYFTGGGGSGGGGSGGGGSGGGSGEVQLLESGGGLVQPGGSLRLSCAASGFTFSSYIMMWVRQAPGKGLEWVSSIYPSGGITFYADTVKGRFTISRDNSKNTLYLQMNSLRAEDTAVYYCARIKLGTVTTVDYWGQGTLVTVSSASTKGPSVFPLAPSSKSTSGGTAALGCLVKDYFPEPVTVSWNSGALTSGVHTFPAVLQSSGLYSLSSVVTVPSSSLGTQTYICNVNHKPSNTKVDKKVEPKSCDKTHTCPPCPAPELLGGPSVFLFPPKPKDTLMISRTPEVTCVVVDVSHEDPEVKFNWYVDGVEVHNAKTKPREEQYNSTYRVVSVLTVLHQDWLNGKEYKCKVSNKALPAPIEKTISKAKGQPREPQVYTLPPSRDELTKNQVSLTCLVKGFYPSDIAVEWESNGQPENNYKTTPPVLDSDGSFFLYSKLTVDKSRWQQGNVFSCSVMHEALHNHYTQKSLSLSPGAGGGGSGGGGSGGGGSGGGGSGVIHVTKEVKEVATLSCGHNVSVEELAQTRIYWQKEKKMVLTMMSGDMNIWPEYKNRTIFDITNNLSIVILALRPSDEGTYECVVLKYEKDAFKREHLAEVTLSVKADFPTPSISDFEIPTSNIRRIICSTSGGFPEPHLSWLENGEELNAINTTVSQDPETELYAVSSKLDFNMTTNHSFMCLIKYGHLRVNQTFNWNTTKQEHFPDN

SEQ ID NO: 90 - protein, 1105 aa, synthetic construct
  REGION 1..1105: note = CD80-Avelumab-LAG3
VIHVTKEVKEVATLSCGHNVSVEELAQTRIYWQKEKKMVLTMMSGDMNIWPEYKNRTIFDITNNLSIVILALRPSDEGTYECVVLKYEKDAFKREHLAEVTLSVKADFPTPSISDFEIPTSNIRRIICSTSGGFPEPHLSWLENGEELNAINTTVSQDPETELYAVSSKLDFNMTTNHSFMCLIKYGHLRVNQTFNWNTTKQEHFPDNGGGGSGGGGSGGGGSGGGSGEVQLLESGGGLVQPGGSLRLSCAASGFTFSSYIMMWVRQAPGKGLEWVSSIYPSGGITFYADTVKGRFTISRDNSKNTLYLQMNSLRAEDTAVYYCARIKLGTVTTVDYWGQGTLVTVSSASTKGPSVFPLAPSSKSTSGGTAALGCLVKDYFPEPVTVSWNSGALTSGVHTFPAVLQSSGLYSLSSVVTVPSSSLGTQTYICNVNHKPSNTKVDKKVEPKSCDKTHTCPPCPAPELLGGPSVFLFPPKPKDTLMISRTPEVTCVVVDVSHEDPEVKFNWYVDGVEVHNAKTKPREEQYNSTYRVVSVLTVLHQDWLNGKEYKCKVSNKALPAPIEKTISKAKGQPREPQVYTLPPSRDELTKNQVSLTCLVKGFYPSDIAVEWESNGQPENNYKTTPPVLDSDGSFFLYSKLTVDKSRWQQGNVFSCSVMHEALHNHYTQKSLSLSPGAGGGGSGGGGSGGGGSGGGGSGLQPGAEVPVVWAQEGAPAQLPCSPTIPLQDLSLLRRAGVTWQHQPDSGPPAAAPGHPLAPGPHPAAPSSWGPRPRRYTVLSVGPGGLRSGRLPLQPRVQLDERGRQRGDFSLWLRPARRADAGEYRAAVHLRDRALSCRLRLRLGQASMTASPPGSLRASDWVILNCSFSRPDRPASVHWFRNRGQGRVPVRESPHHHLAESFLFLPQVSPMDSGPWGCILTYRDGFNVSIMYNLTVLGLEPPTPLTVYAGAGSRVGLPCRLPAGVGTRSFLTAKWTPPGGGPDLLVTGDNGDFTLRLEDVSQAQAGTYTCHIHLQEQQLNATVTLAIITVTPKSFGSPGSLGKLLCEVTPVSGQERFVWSSLDTPSQRSFSGPWLEAQEAQLLSQPWQCQLYQGERLLGAAVYFT

SEQ ID NO: 91 - protein, 589 aa, synthetic construct
  REGION 1..589: note = Envafolimab-CD80
QVQLVESGGGLVQPGGSLRLSCAASGKMSSRRCMAWFRQAPGKERERVAKLLTTSGSTYLADSVKGRFTISRDNSKNTVYLQMNSLRAEDTAVYYCAADSFEDPTCTLVTSSGAFQYWGQGTLVTVSSEPKSSDKTHTCPPCPAPELLGGPSVFLFPPKPKDTLMISRTPEVTCVVVAVSHEDPEVKFNWYVDGVEVHNAKTKPREEQYNSTYRVVSVLTVLHQDWLNGKEYKCKVSNKALPAGIEKTISKAKGQPREPQVYTLPPSRDELTKNQVSLTCLVKGFYPSDIAVEWESNGQPENNYKTTPPVLDSDGSFFLYSKLTVDKSRWQQGNVFSCSVMHEALHNHYTQKSLSLSPGAGGGGSGGGGSGGGGSGGGGSGVIHVTKEVKEVATLSCGHNVSVEELAQTRIYWQKEKKMVLTMMSGDMNIWPEYKNRTIFDITNNLSIVILALRPSDEGTYECVVLKYEKDAFKREHLAEVTLSVKADFPTPSISDFEIPTSNIRRIICSTSGGFPEPHLSWLENGEELNAINTTVSQDPETELYAVSSKLDFNMTTNHSFMCLIKYGHLRVNQTFNWNTTKQEHFPDN

SEQ ID NO: 92 - protein, 787 aa, synthetic construct
  REGION 1..787: note = Envafolimab-LAG3
QVQLVESGGGLVQPGGSLRLSCAASGKMSSRRCMAWFRQAPGKERERVAKLLTTSGSTYLADSVKGRFTISRDNSKNTVYLQMNSLRAEDTAVYYCAADSFEDPTCTLVTSSGAFQYWGQGTLVTVSSEPKSSDKTHTCPPCPAPELLGGPSVFLFPPKPKDTLMISRTPEVTCVVVAVSHEDPEVKFNWYVDGVEVHNAKTKPREEQYNSTYRVVSVLTVLHQDWLNGKEYKCKVSNKALPAGIEKTISKAKGQPREPQVYTLPPSRDELTKNQVSLTCLVKGFYPSDIAVEWESNGQPENNYKTTPPVLDSDGSFFLYSKLTVDKSRWQQGNVFSCSVMHEALHNHYTQKSLSLSPGAGGGGSGGGGSGGGGSGGGGSGLQPGAEVPVVWAQEGAPAQLPCSPTIPLQDLSLLRRAGVTWQHQPDSGPPAAAPGHPLAPGPHPAAPSSWGPRPRRYTVLSVGPGGLRSGRLPLQPRVQLDERGRQRGDFSLWLRPARRADAGEYRAAVHLRDRALSCRLRLRLGQASMTASPPGSLRASDWVILNCSFSRPDRPASVHWFRNRGQGRVPVRESPHHHLAESFLFLPQVSPMDSGPWGCILTYRDGFNVSIMYNLTVLGLEPPTPLTVYAGAGSRVGLPCRLPAGVGTRSFLTAKWTPPGGGPDLLVTGDNGDFTLRLEDVSQAQAGTYTCHIHLQEQQLNATVTLAIITVTPKSFGSPGSLGKLLCEVTPVSGQERFVWSSLDTPSQRSFSGPWLEAQEAQLLSQPWQCQLYQGERLLGAAVYFT

SEQ ID NO: 93 - protein, 623 aa, synthetic construct
  REGION 1..623: note = Envafolimab-LAG3 IgD1/D2
QVQLVESGGGLVQPGGSLRLSCAASGKMSSRRCMAWFRQAPGKERERVAKLLTTSGSTYLADSVKGRFTISRDNSKNTVYLQMNSLRAEDTAVYYCAADSFEDPTCTLVTSSGAFQYWGQGTLVTVSSEPKSSDKTHTCPPCPAPELLGGPSVFLFPPKPKDTLMISRTPEVTCVVVAVSHEDPEVKFNWYVDGVEVHNAKTKPREEQYNSTYRVVSVLTVLHQDWLNGKEYKCKVSNKALPAGIEKTISKAKGQPREPQVYTLPPSRDELTKNQVSLTCLVKGFYPSDIAVEWESNGQPENNYKTTPPVLDSDGSFFLYSKLTVDKSRWQQGNVFSCSVMHEALHNHYTQKSLSLSPGAGGGGSGGGGSGGGGSGGGGSGLQPGAEVPVVWAQEGAPAQLPCSPTIPLQDLSLLRRAGVTWQHQPDSGPPAAAPGHPLAPGPHPAAPSSWGPRPRRYTVLSVGPGGLRSGRLPLQPRVQLDERGRQRGDFSLWLRPARRADAGEYRAAVHLRDRALSCRLRLRLGQASMTASPPGSLRASDWVILNCSFSRPDRPASVHWFRNRGQGRVPVRESPHHHLAESFLFLPQVSPMDSGPWGCILTYRDGFNVSIMYNLTVLGLEP

SEQ ID NO: 94 - protein, 706 aa, synthetic construct
  REGION 1..706: note = Envafolimab-LAG3 IgD1/D2/D3
QVQLVESGGGLVQPGGSLRLSCAASGKMSSRRCMAWFRQAPGKERERVAKLLTTSGSTYLADSVKGRFTISRDNSKNTVYLQMNSLRAEDTAVYYCAADSFEDPTCTLVTSSGAFQYWGQGTLVTVSSEPKSSDKTHTCPPCPAPELLGGPSVFLFPPKPKDTLMISRTPEVTCVVVAVSHEDPEVKFNWYVDGVEVHNAKTKPREEQYNSTYRVVSVLTVLHQDWLNGKEYKCKVSNKALPAGIEKTISKAKGQPREPQVYTLPPSRDELTKNQVSLTCLVKGFYPSDIAVEWESNGQPENNYKTTPPVLDSDGSFFLYSKLTVDKSRWQQGNVFSCSVMHEALHNHYTQKSLSLSPGAGGGGSGGGGSGGGGSGGGGSGLQPGAEVPVVWAQEGAPAQLPCSPTIPLQDLSLLRRAGVTWQHQPDSGPPAAAPGHPLAPGPHPAAPSSWGPRPRRYTVLSVGPGGLRSGRLPLQPRVQLDERGRQRGDFSLWLRPARRADAGEYRAAVHLRDRALSCRLRLRLGQASMTASPPGSLRASDWVILNCSFSRPDRPASVHWFRNRGQGRVPVRESPHHHLAESFLFLPQVSPMDSGPWGCILTYRDGFNVSIMYNLTVLGLEPPTPLTVYAGAGSRVGLPCRLPAGVGTRSFLTAKWTPPGGGPDLLVTGDNGDFTLRLEDVSQAQAGTYTCHIHLQEQQLNATVT

SEQ ID NO: 95 - protein, 589 aa, synthetic construct
  REGION 1..589: note = CD80-Envafolimab
VIHVTKEVKEVATLSCGHNVSVEELAQTRIYWQKEKKMVLTMMSGDMNIWPEYKNRTIFDITNNLSIVILALRPSDEGTYECVVLKYEKDAFKREHLAEVTLSVKADFPTPSISDFEIPTSNIRRIICSTSGGFPEPHLSWLENGEELNAINTTVSQDPETELYAVSSKLDFNMTTNHSFMCLIKYGHLRVNQTFNWNTTKQEHFPDNGGGGSGGGGSGGGGSGGGGSGQVQLVESGGGLVQPGGSLRLSCAASGKMSSRRCMAWFRQAPGKERERVAKLLTTSGSTYLADSVKGRFTISRDNSKNTVYLQMNSLRAEDTAVYYCAADSFEDPTCTLVTSSGAFQYWGQGTLVTVSSEPKSSDKTHTCPPCPAPELLGGPSVFLFPPKPKDTLMISRTPEVTCVVVAVSHEDPEVKFNWYVDGVEVHNAKTKPREEQYNSTYRVVSVLTVLHQDWLNGKEYKCKVSNKALPAGIEKTISKAKGQPREPQVYTLPPSRDELTKNQVSLTCLVKGFYPSDIAVEWESNGQPENNYKTTPPVLDSDGSFFLYSKLTVDKSRWQQGNVFSCSVMHEALHNHYTQKSLSLSPGK

SEQ ID NO: 96 - protein, 787 aa, synthetic construct
  REGION 1..787: note = LAG3-Envafolimab
LQPGAEVPVVWAQEGAPAQLPCSPTIPLQDLSLLRRAGVTWQHQPDSGPPAAAPGHPLAPGPHPAAPSSWGPRPRRYTVLSVGPGGLRSGRLPLQPRVQLDERGRQRGDFSLWLRPARRADAGEYRAAVHLRDRALSCRLRLRLGQASMTASPPGSLRASDWVILNCSFSRPDRPASVHWFRNRGQGRVPVRESPHHHLAESFLFLPQVSPMDSGPWGCILTYRDGFNVSIMYNLTVLGLEPPTPLTVYAGAGSRVGLPCRLPAGVGTRSFLTAKWTPPGGGPDLLVTGDNGDFTLRLEDVSQAQAGTYTCHIHLQEQQLNATVTLAIITVTPKSFGSPGSLGKLLCEVTPVSGQERFVWSSLDTPSQRSFSGPWLEAQEAQLLSQPWQCQLYQGERLLGAAVYFTGGGGSGGGGSGGGGSGGGGSGQVQLVESGGGLVQPGGSLRLSCAASGKMSSRRCMAWFRQAPGKERERVAKLLTTSGSTYLADSVKGRFTISRDNSKNTVYLQMNSLRAEDTAVYYCAADSFEDPTCTLVTSSGAFQYWGQGTLVTVSSEPKSSDKTHTCPPCPAPELLGGPSVFLFPPKPKDTLMISRTPEVTCVVVAVSHEDPEVKFNWYVDGVEVHNAKTKPREEQYNSTYRVVSVLTVLHQDWLNGKEYKCKVSNKALPAGIEKTISKAKGQPREPQVYTLPPSRDELTKNQVSLTCLVKGFYPSDIAVEWESNGQPENNYKTTPPVLDSDGSFFLYSKLTVDKSRWQQGNVFSCSVMHEALHNHYTQKSLSLSPGK

SEQ ID NO: 97 - protein, 833 aa, synthetic construct
  REGION 1..833: note = Envafolimab-LAG3 IgD1/D2-CD80
QVQLVESGGGLVQPGGSLRLSCAASGKMSSRRCMAWFRQAPGKERERVAKLLTTSGSTYLADSVKGRFTISRDNSKNTVYLQMNSLRAEDTAVYYCAADSFEDPTCTLVTSSGAFQYWGQGTLVTVSSEPKSSDKTHTCPPCPAPELLGGPSVFLFPPKPKDTLMISRTPEVTCVVVAVSHEDPEVKFNWYVDGVEVHNAKTKPREEQYNSTYRVVSVLTVLHQDWLNGKEYKCKVSNKALPAGIEKTISKAKGQPREPQVYTLPPSRDELTKNQVSLTCLVKGFYPSDIAVEWESNGQPENNYKTTPPVLDSDGSFFLYSKLTVDKSRWQQGNVFSCSVMHEALHNHYTQKSLSLSPGAGGGGSGGGGSGVIHVTKEVKEVATLSCGHNVSVEELAQTRIYWQKEKKMVLTMMSGDMNIWPEYKNRTIFDITNNLSIVILALRPSDEGTYECVVLKYEKDAFKREHLAEVTLSVKADFPTPSISDFEIPTSNIRRIICSTSGGFPEPHLSWLENGEELNAINTTVSQDPETELYAVSSKLDFNMTTNHSFMCLIKYGHLRVNQTFNWNTTKQEHFPDNGGGGSGGGGSGSLQPGAEVPVVWAQEGAPAQLPCSPTIPLQDLSLLRRAGVTWQHQPDSGPPAAAPGHPLAPGPHPAAPSSWGPRPRRYTVLSVGPGGLRSGRLPLQPRVQLDERGRQRGDFSLWLRPARRADAGEYRAAVHLRDRALSCRLRLRLGQASMTASPPGSLRASDWVILNCSFSRPDRPASVHWFRNRGQGRVPVRESPHHHLAESFLFLPQVSPMDSGPWGCILTYRDGFNVSIMYNLTVLGLEP

SEQ ID NO: 98 - protein, 915 aa, synthetic construct
  REGION 1..915: note = Envafolimab-LAG3 IgD1/D2/D3-CD80
QVQLVESGGGLVQPGGSLRLSCAASGKMSSRRCMAWFRQAPGKERERVAKLLTTSGSTYLADSVKGRFTISRDNSKNTVYLQMNSLRAEDTAVYYCAADSFEDPTCTLVTSSGAFQYWGQGTLVTVSSEPKSSDKTHTCPPCPAPELLGGPSVFLFPPKPKDTLMISRTPEVTCVVVAVSHEDPEVKFNWYVDGVEVHNAKTKPREEQYNSTYRVVSVLTVLHQDWLNGKEYKCKVSNKALPAGIEKTISKAKGQPREPQVYTLPPSRDELTKNQVSLTCLVKGFYPSDIAVEWESNGQPENNYKTTPPVLDSDGSFFLYSKLTVDKSRWQQGNVFSCSVMHEALHNHYTQKSLSLSPGAGGGGSGGGGSGVIHVTKEVKEVATLSCGHNVSVEELAQTRIYWQKEKKMVLTMMSGDMNIWPEYKNRTIFDITNNLSIVILALRPSDEGTYECVVLKYEKDAFKREHLAEVTLSVKADFPTPSISDFEIPTSNIRRIICSTSGGFPEPHLSWLENGEELNAINTTVSQDPETELYAVSSKLDFNMTTNHSFMCLIKYGHLRVNQTFNWNTTKQEHFPDNGGGGSGGGGSGLQPGAEVPVVWAQEGAPAQLPCSPTIPLQDLSLLRRAGVTWQHQPDSGPPAAAPGHPLAPGPHPAAPSSWGPRPRRYTVLSVGPGGLRSGRLPLQPRVQLDERGRQRGDFSLWLRPARRADAGEYRAAVHLRDRALSCRLRLRLGQASMTASPPGSLRASDWVILNCSFSRPDRPASVHWFRNRGQGRVPVRESPHHHLAESFLFLPQVSPMDSGPWGCILTYRDGFNVSIMYNLTVLGLEPPTPLTVYAGAGSRVGLPCRLPAGVGTRSFLTAKWTPPGGGPDLLVTGDNGDFTLRLEDVSQAQAGTYTCHIHLQEQQLNATVT

SEQ ID NO: 99 - protein, 1015 aa, synthetic construct
  REGION 1..1015: note = Envafolimab-LAG3-CD80
QVQLVESGGGLVQPGGSLRLSCAASGKMSSRRCMAWFRQAPGKERERVAKLLTTSGSTYLADSVKGRFTISRDNSKNTVYLQMNSLRAEDTAVYYCAADSFEDPTCTLVTSSGAFQYWGQGTLVTVSSEPKSSDKTHTCPPCPAPELLGGPSVFLFPPKPKDTLMISRTPEVTCVVVAVSHEDPEVKFNWYVDGVEVHNAKTKPREEQYNSTYRVVSVLTVLHQDWLNGKEYKCKVSNKALPAGIEKTISKAKGQPREPQVYTLPPSRDELTKNQVSLTCLVKGFYPSDIAVEWESNGQPENNYKTTPPVLDSDGSFFLYSKLTVDKSRWQQGNVFSCSVMHEALHNHYTQKSLSLSPGAGGGGSGGGGSGGGGSGGGSGVIHVTKEVKEVATLSCGHNVSVEELAQTRIYWQKEKKMVLTMMSGDMNIWPEYKNRTIFDITNNLSIVILALRPSDEGTYECVVLKYEKDAFKREHLAEVTLSVKADFPTPSISDFEIPTSNIRRIICSTSGGFPEPHLSWLENGEELNAINTTVSQDPETELYAVSSKLDFNMTTNHSFMCLIKYGHLRVNQTFNWNTTKQEHFPDNGGGGSGGGGSGGGGSGGGGSGLQPGAEVPVVWAQEGAPAQLPCSPTIPLQDLSLLRRAGVTWQHQPDSGPPAAAPGHPLAPGPHPAAPSSWGPRPRRYTVLSVGPGGLRSGRLPLQPRVQLDERGRQRGDFSLWLRPARRADAGEYRAAVHLRDRALSCRLRLRLGQASMTASPPGSLRASDWVILNCSFSRPDRPASVHWFRNRGQGRVPVRESPHHHLAESFLFLPQVSPMDSGPWGCILTYRDGFNVSIMYNLTVLGLEPPTPLTVYAGAGSRVGLPCRLPAGVGTRSFLTAKWTPPGGGPDLLVTGDNGDFTLRLEDVSQAQAGTYTCHIHLQEQQLNATVTLAIITVTPKSFGSPGSLGKLLCEVTPVSGQERFVWSSLDTPSQRSFSGPWLEAQEAQLLSQPWQCQLYQGERLLGAAVYFT

SEQ ID NO: 100 - protein, 833 aa, synthetic construct
  REGION 1..833: note = Envafolimab-CD80-LAG3 IgD1/D2
QVQLVESGGGLVQPGGSLRLSCAASGKMSSRRCMAWFRQAPGKERERVAKLLTTSGSTYLADSVKGRFTISRDNSKNTVYLQMNSLRAEDTAVYYCAADSFEDPTCTLVTSSGAFQYWGQGTLVTVSSEPKSSDKTHTCPPCPAPELLGGPSVFLFPPKPKDTLMISRTPEVTCVVVAVSHEDPEVKFNWYVDGVEVHNAKTKPREEQYNSTYRVVSVLTVLHQDWLNGKEYKCKVSNKALPAGIEKTISKAKGQPREPQVYTLPPSRDELTKNQVSLTCLVKGFYPSDIAVEWESNGQPENNYKTTPPVLDSDGSFFLYSKLTVDKSRWQQGNVFSCSVMHEALHNHYTQKSLSLSPGAGGGGSGGGGSGSLQPGAEVPVVWAQEGAPAQLPCSPTIPLQDLSLLRRAGVTWQHQPDSGPPAAAPGHPLAPGPHPAAPSSWGPRPRRYTVLSVGPGGLRSGRLPLQPRVQLDERGRQRGDFSLWLRPARRADAGEYRAAVHLRDRALSCRLRLRLGQASMTASPPGSLRASDWVILNCSFSRPDRPASVHWFRNRGQGRVPVRESPHHHLAESFLFLPQVSPMDSGPWGCILTYRDGFNVSIMYNLTVLGLEPGGGGSGGGGSGVIHVTKEVKEVATLSCGHNVSVEELAQTRIYWQKEKKMVLTMMSGDMNIWPEYKNRTIFDITNNLSIVILALRPSDEGTYECVVLKYEKDAFKREHLAEVTLSVKADFPTPSISDFEIPTSNIRRIICSTSGGFPEPHLSWLENGEELNAINTTVSQDPETELYAVSSKLDFNMTTNHSFMCLIKYGHLRVNQTFNWNTTKQEHFPDN

SEQ ID NO: 101 - protein, 915 aa, synthetic construct
  REGION 1..915: note = Envafolimab-CD80-LAG3 IgD1/D2/D3
QVQLVESGGGLVQPGGSLRLSCAASGKMSSRRCMAWFRQAPGKERERVAKLLTTSGSTYLADSVKGRFTISRDNSKNTVYLQMNSLRAEDTAVYYCAADSFEDPTCTLVTSSGAFQYWGQGTLVTVSSEPKSSDKTHTCPPCPAPELLGGPSVFLFPPKPKDTLMISRTPEVTCVVVAVSHEDPEVKFNWYVDGVEVHNAKTKPREEQYNSTYRVVSVLTVLHQDWLNGKEYKCKVSNKALPAGIEKTISKAKGQPREPQVYTLPPSRDELTKNQVSLTCLVKGFYPSDIAVEWESNGQPENNYKTTPPVLDSDGSFFLYSKLTVDKSRWQQGNVFSCSVMHEALHNHYTQKSLSLSPGAGGGGSGGGGSGLQPGAEVPVVWAQEGAPAQLPCSPTIPLQDLSLLRRAGVTWQHQPDSGPPAAAPGHPLAPGPHPAAPSSWGPRPRRYTVLSVGPGGLRSGRLPLQPRVQLDERGRQRGDFSLWLRPARRADAGEYRAAVHLRDRALSCRLRLRLGQASMTASPPGSLRASDWVILNCSFSRPDRPASVHWFRNRGQGRVPVRESPHHHLAESFLFLPQVSPMDSGPWGCILTYRDGFNVSIMYNLTVLGLEPPTPLTVYAGAGSRVGLPCRLPAGVGTRSFLTAKWTPPGGGPDLLVTGDNGDFTLRLEDVSQAQAGTYTCHIHLQEQQLNATVTGGGGSGGGGSGVIHVTKEVKEVATLSCGHNVSVEELAQTRIYWQKEKKMVLTMMSGDMNIWPEYKNRTIFDITNNLSIVILALRPSDEGTYECVVLKYEKDAFKREHLAEVTLSVKADFPTPSISDFEIPTSNIRRIICSTSGGFPEPHLSWLENGEELNAINTTVSQDPETELYAVSSKLDFNMTTNHSFMCLIKYGHLRVNQTFNWNTTKQEHFPDN

SEQ ID NO: 102 - protein, 1015 aa, synthetic construct
  REGION 1..1015: note = Envafolimab-CD80-LAG3
QVQLVESGGGLVQPGGSLRLSCAASGKMSSRRCMAWFRQAPGKERERVAKLLTTSGSTYLADSVKGRFTISRDNSKNTVYLQMNSLRAEDTAVYYCAADSFEDPTCTLVTSSGAFQYWGQGTLVTVSSEPKSSDKTHTCPPCPAPELLGGPSVFLFPPKPKDTLMISRTPEVTCVVVAVSHEDPEVKFNWYVDGVEVHNAKTKPREEQYNSTYRVVSVLTVLHQDWLNGKEYKCKVSNKALPAGIEKTISKAKGQPREPQVYTLPPSRDELTKNQVSLTCLVKGFYPSDIAVEWESNGQPENNYKTTPPVLDSDGSFFLYSKLTVDKSRWQQGNVFSCSVMHEALHNHYTQKSLSLSPGAGGGGSGGGGSGGGGSGGGGSGLQPGAEVPVVWAQEGAPAQLPCSPTIPLQDLSLLRRAGVTWQHQPDSGPPAAAPGHPLAPGPHPAAPSSWGPRPRRYTVLSVGPGGLRSGRLPLQPRVQLDERGRQRGDFSLWLRPARRADAGEYRAAVHLRDRALSCRLRLRLGQASMTASPPGSLRASDWVILNCSFSRPDRPASVHWFRNRGQGRVPVRESPHHHLAESFLFLPQVSPMDSGPWGCILTYRDGFNVSIMYNLTVLGLEPPTPLTVYAGAGSRVGLPCRLPAGVGTRSFLTAKWTPPGGGPDLLVTGDNGDFTLRLEDVSQAQAGTYTCHIHLQEQQLNATVTLAIITVTPKSFGSPGSLGKLLCEVTPVSGQERFVWSSLDTPSQRSFSGPWLEAQEAQLLSQPWQCQLYQGERLLGAAVYFTGGGGSGGGGSGGGGSGGGSGVIHVTKEVKEVATLSCGHNVSVEELAQTRIYWQKEKKMVLTMMSGDMNIWPEYKNRTIFDITNNLSIVILALRPSDEGTYECVVLKYEKDAFKREHLAEVTLSVKADFPTPSISDFEIPTSNIRRIICSTSGGFPEPHLSWLENGEELNAINTTVSQDPETELYAVSSKLDFNMTTNHSFMCLIKYGHLRVNQTFNWNTTKQEHFPDN

SEQ ID NO: 103 - protein, 1015 aa, synthetic construct
  REGION 1..1015: note = LAG3-Envafolimab-CD80
LQPGAEVPVVWAQEGAPAQLPCSPTIPLQDLSLLRRAGVTWQHQPDSGPPAAAPGHPLAPGPHPAAPSSWGPRPRRYTVLSVGPGGLRSGRLPLQPRVQLDERGRQRGDFSLWLRPARRADAGEYRAAVHLRDRALSCRLRLRLGQASMTASPPGSLRASDWVILNCSFSRPDRPASVHWFRNRGQGRVPVRESPHHHLAESFLFLPQVSPMDSGPWGCILTYRDGFNVSIMYNLTVLGLEPPTPLTVYAGAGSRVGLPCRLPAGVGTRSFLTAKWTPPGGGPDLLVTGDNGDFTLRLEDVSQAQAGTYTCHIHLQEQQLNATVTLAIITVTPKSFGSPGSLGKLLCEVTPVSGQERFVWSSLDTPSQRSFSGPWLEAQEAQLLSQPWQCQLYQGERLLGAAVYFTGGGGSGGGGSGGGGSGGGSGQVQLVESGGGLVQPGGSLRLSCAASGKMSSRRCMAWFRQAPGKERERVAKLLTTSGSTYLADSVKGRFTISRDNSKNTVYLQMNSLRAEDTAVYYCAADSFEDPTCTLVTSSGAFQYWGQGTLVTVSSEPKSSDKTHTCPPCPAPELLGGPSVFLFPPKPKDTLMISRTPEVTCVVVAVSHEDPEVKFNWYVDGVEVHNAKTKPREEQYNSTYRVVSVLTVLHQDWLNGKEYKCKVSNKALPAGIEKTISKAKGQPREPQVYTLPPSRDELTKNQVSLTCLVKGFYPSDIAVEWESNGQPENNYKTTPPVLDSDGSFFLYSKLTVDKSRWQQGNVFSCSVMHEALHNHYTQKSLSLSPGAGGGGSGGGGSGGGGSGGGGSGVIHVTKEVKEVATLSCGHNVSVEELAQTRIYWQKEKKMVLTMMSGDMNIWPEYKNRTIFDITNNLSIVILALRPSDEGTYECVVLKYEKDAFKREHLAEVTLSVKADFPTPSISDFEIPTSNIRRIICSTSGGFPEPHLSWLENGEELNAINTTVSQDPETELYAVSSKLDFNMTTNHSFMCLIKYGHLRVNQTFNWNTTKQEHFPDN

SEQ ID NO: 104 - protein, 1015 aa, synthetic construct
  REGION 1..1015: note = CD80-Envafolimab-LAG3
VIHVTKEVKEVATLSCGHNVSVEELAQTRIYWQKEKKMVLTMMSGDMNIWPEYKNRTIFDITNNLSIVILALRPSDEGTYECVVLKYEKDAFKREHLAEVTLSVKADFPTPSISDFEIPTSNIRRIICSTSGGFPEPHLSWLENGEELNAINTTVSQDPETELYAVSSKLDFNMTTNHSFMCLIKYGHLRVNQTFNWNTTKQEHFPDNGGGGSGGGGSGGGGSGGGSGQVQLVESGGGLVQPGGSLRLSCAASGKMSSRRCMAWFRQAPGKERERVAKLLTTSGSTYLADSVKGRFTISRDNSKNTVYLQMNSLRAEDTAVYYCAADSFEDPTCTLVTSSGAFQYWGQGTLVTVSSEPKSSDKTHTCPPCPAPELLGGPSVFLFPPKPKDTLMISRTPEVTCVVVAVSHEDPEVKFNWYVDGVEVHNAKTKPREEQYNSTYRVVSVLTVLHQDWLNGKEYKCKVSNKALPAGIEKTISKAKGQPREPQVYTLPPSRDELTKNQVSLTCLVKGFYPSDIAVEWESNGQPENNYKTTPPVLDSDGSFFLYSKLTVDKSRWQQGNVFSCSVMHEALHNHYTQKSLSLSPGAGGGGSGGGGSGGGGSGGGGSGLQPGAEVPVVWAQEGAPAQLPCSPTIPLQDLSLLRRAGVTWQHQPDSGPPAAAPGHPLAPGPHPAAPSSWGPRPRRYTVLSVGPGGLRSGRLPLQPRVQLDERGRQRGDFSLWLRPARRADAGEYRAAVHLRDRALSCRLRLRLGQASMTASPPGSLRASDWVILNCSFSRPDRPASVHWFRNRGQGRVPVRESPHHHLAESFLFLPQVSPMDSGPWGCILTYRDGFNVSIMYNLTVLGLEPPTPLTVYAGAGSRVGLPCRLPAGVGTRSFLTAKWTPPGGGPDLLVTGDNGDFTLRLEDVSQAQAGTYTCHIHLQEQQLNATVTLAIITVTPKSFGSPGSLGKLLCEVTPVSGQERFVWSSLDTPSQRSFSGPWLEAQEAQLLSQPWQCQLYQGERLLGAAVYFT

SEQ ID NO: 105 - protein, 669 aa, synthetic construct
  REGION 1..669: note = Nivolumab-CD80
QVQLVESGGGVVQPGRSLRLDCKASGITFSNSGMHWVRQAPGKGLEWVAVIWYDGSKRYYADSVKGRFTISRDNSKNTLFLQMNSLRAEDTAVYYCATNDDYWGQGTLVTVSSASTKGPSVFPLAPCSRSTSESTAALGCLVKDYFPEPVTVSWNSGALTSGVHTFPAVLQSSGLYSLSSVVTVPSSSLGTKTYTCNVDHKPSNTKVDKRVESKYGPPCPPCPAPEFLGGPSVFLFPPKPKDTLMISRTPEVTCVVVDVSQEDPEVQFNWYVDGVEVHNAKTKPREEQFNSTYRVVSVLTVLHQDWLNGKEYKCKVSNKGLPSSIEKTISKAKGQPREPQVYTLPPSQEEMTKNQVSLTCLVKGFYPSDIAVEWESNGQPENNYKTTPPVLDSDGSFFLYSRLTVDKSRWQEGNVFSCSVMHEALHNHYTQKSLSLSLGAGGGGSGGGGSGGGGSGGGGSGVIHVTKEVKEVATLSCGHNVSVEELAQTRIYWQKEKKMVLTMMSGDMNIWPEYKNRTIFDITNNLSIVILALRPSDEGTYECVVLKYEKDAFKREHLAEVTLSVKADFPTPSISDFEIPTSNIRRIICSTSGGFPEPHLSWLENGEELNAINTTVSQDPETELYAVSSKLDFNMTTNHSFMCLIKYGHLRVNQTFNWNTTKQEHFPDN

SEQ ID NO: 106 - protein, 867 aa, synthetic construct
  REGION 1..867: note = Nivolumab-LAG3
QVQLVESGGGVVQPGRSLRLDCKASGITFSNSGMHWVRQAPGKGLEWVAVIWYDGSKRYYADSVKGRFTISRDNSKNTLFLQMNSLRAEDTAVYYCATNDDYWGQGTLVTVSSASTKGPSVFPLAPCSRSTSESTAALGCLVKDYFPEPVTVSWNSGALTSGVHTFPAVLQSSGLYSLSSVVTVPSSSLGTKTYTCNVDHKPSNTKVDKRVESKYGPPCPPCPAPEFLGGPSVFLFPPKPKDTLMISRTPEVTCVVVDVSQEDPEVQFNWYVDGVEVHNAKTKPREEQFNSTYRVVSVLTVLHQDWLNGKEYKCKVSNKGLPSSIEKTISKAKGQPREPQVYTLPPSQEEMTKNQVSLTCLVKGFYPSDIAVEWESNGQPENNYKTTPPVLDSDGSFFLYSRLTVDKSRWQEGNVFSCSVMHEALHNHYTQKSLSLSLGAGGGGSGGGGSGGGGSGGGGSGLQPGAEVPVVWAQEGAPAQLPCSPTIPLQDLSLLRRAGVTWQHQPDSGPPAAAPGHPLAPGPHPAAPSSWGPRPRRYTVLSVGPGGLRSGRLPLQPRVQLDERGRQRGDFSLWLRPARRADAGEYRAAVHLRDRALSCRLRLRLGQASMTASPPGSLRASDWVILNCSFSRPDRPASVHWFRNRGQGRVPVRESPHHHLAESFLFLPQVSPMDSGPWGCILTYRDGFNVSIMYNLTVLGLEPPTPLTVYAGAGSRVGLPCRLPAGVGTRSFLTAKWTPPGGGPDLLVTGDNGDFTLRLEDVSQAQAGTYTCHIHLQEQQLNATVTLAIITVTPKSFGSPGSLGKLLCEVTPVSGQERFVWSSLDTPSQRSFSGPWLEAQEAQLLSQPWQCQLYQGERLLGAAVYFT

SEQ ID NO: 107 - protein, 703 aa, synthetic construct
  REGION 1..703: note = Nivolumab-LAG3 IgD1/D2
QVQLVESGGGVVQPGRSLRLDCKASGITFSNSGMHWVRQAPGKGLEWVAVIWYDGSKRYYADSVKGRFTISRDNSKNTLFLQMNSLRAEDTAVYYCATNDDYWGQGTLVTVSSASTKGPSVFPLAPCSRSTSESTAALGCLVKDYFPEPVTVSWNSGALTSGVHTFPAVLQSSGLYSLSSVVTVPSSSLGTKTYTCNVDHKPSNTKVDKRVESKYGPPCPPCPAPEFLGGPSVFLFPPKPKDTLMISRTPEVTCVVVDVSQEDPEVQFNWYVDGVEVHNAKTKPREEQFNSTYRVVSVLTVLHQDWLNGKEYKCKVSNKGLPSSIEKTISKAKGQPREPQVYTLPPSQEEMTKNQVSLTCLVKGFYPSDIAVEWESNGQPENNYKTTPPVLDSDGSFFLYSRLTVDKSRWQEGNVFSCSVMHEALHNHYTQKSLSLSLGAGGGGSGGGGSGGGGSGGGGSGLQPGAEVPVVWAQEGAPAQLPCSPTIPLQDLSLLRRAGVTWQHQPDSGPPAAAPGHPLAPGPHPAAPSSWGPRPRRYTVLSVGPGGLRSGRLPLQPRVQLDERGRQRGDFSLWLRPARRADAGEYRAAVHLRDRALSCRLRLRLGQASMTASPPGSLRASDWVILNCSFSRPDRPASVHWFRNRGQGRVPVRESPHHHLAESFLFLPQVSPMDSGPWGCILTYRDGFNVSIMYNLTVLGLEP

SEQ ID NO: 108 - protein, 786 aa, synthetic construct
  REGION 1..786: note = Nivolumab-LAG3 IgD1/D2/D3
QVQLVESGGGVVQPGRSLRLDCKASGITFSNSGMHWVRQAPGKGLEWVAVIWYDGSKRYYADSVKGRFTISRDNSKNTLFLQMNSLRAEDTAVYYCATNDDYWGQGTLVTVSSASTKGPSVFPLAPCSRSTSESTAALGCLVKDYFPEPVTVSWNSGALTSGVHTFPAVLQSSGLYSLSSVVTVPSSSLGTKTYTCNVDHKPSNTKVDKRVESKYGPPCPPCPAPEFLGGPSVFLFPPKPKDTLMISRTPEVTCVVVDVSQEDPEVQFNWYVDGVEVHNAKTKPREEQFNSTYRVVSVLTVLHQDWLNGKEYKCKVSNKGLPSSIEKTISKAKGQPREPQVYTLPPSQEEMTKNQVSLTCLVKGFYPSDIAVEWESNGQPENNYKTTPPVLDSDGSFFLYSRLTVDKSRWQEGNVFSCSVMHEALHNHYTQKSLSLSLGAGGGGSGGGGSGGGGSGGGGSGLQPGAEVPVVWAQEGAPAQLPCSPTIPLQDLSLLRRAGVTWQHQPDSGPPAAAPGHPLAPGPHPAAPSSWGPRPRRYTVLSVGPGGLRSGRLPLQPRVQLDERGRQRGDFSLWLRPARRADAGEYRAAVHLRDRALSCRLRLRLGQASMTASPPGSLRASDWVILNCSFSRPDRPASVHWFRNRGQGRVPVRESPHHHLAESFLFLPQVSPMDSGPWGCILTYRDGFNVSIMYNLTVLGLEPPTPLTVYAGAGSRVGLPCRLPAGVGTRSFLTAKWTPPGGGPDLLVTGDNGDFTLRLEDVSQAQAGTYTCHIHLQEQQLNATVT

SEQ ID NO: 109 - protein, 669 aa, synthetic construct
  REGION 1..669: note = CD80-Nivolumab
VIHVTKEVKEVATLSCGHNVSVEELAQTRIYWQKEKKMVLTMMSGDMNIWPEYKNRTIFDITNNLSIVILALRPSDEGTYECVVLKYEKDAFKREHLAEVTLSVKADFPTPSISDFEIPTSNIRRIICSTSGGFPEPHLSWLENGEELNAINTTVSQDPETELYAVSSKLDFNMTTNHSFMCLIKYGHLRVNQTFNWNTTKQEHFPDNGGGGSGGGGSGGGGSGGGGSGQVQLVESGGGVVQPGRSLRLDCKASGITFSNSGMHWVRQAPGKGLEWVAVIWYDGSKRYYADSVKGRFTISRDNSKNTLFLQMNSLRAEDTAVYYCATNDDYWGQGTLVTVSSASTKGPSVFPLAPCSRSTSESTAALGCLVKDYFPEPVTVSWNSGALTSGVHTFPAVLQSSGLYSLSSVVTVPSSSLGTKTYTCNVDHKPSNTKVDKRVESKYGPPCPPCPAPEFLGGPSVFLFPPKPKDTLMISRTPEVTCVVVDVSQEDPEVQFNWYVDGVEVHNAKTKPREEQFNSTYRVVSVLTVLHQDWLNGKEYKCKVSNKGLPSSIEKTISKAKGQPREPQVYTLPPSQEEMTKNQVSLTCLVKGFYPSDIAVEWESNGQPENNYKTTPPVLDSDGSFFLYSRLTVDKSRWQEGNVFSCSVMHEALHNHYTQKSLSLSLGK

SEQ ID NO: 110 - protein, 867 aa, synthetic construct
  REGION 1..867: note = LAG3-Nivolumab
LQPGAEVPVVWAQEGAPAQLPCSPTIPLQDLSLLRRAGVTWQHQPDSGPPAAAPGHPLAPGPHPAAPSSWGPRPRRYTVLSVGPGGLRSGRLPLQPRVQLDERGRQRGDFSLWLRPARRADAGEYRAAVHLRDRALSCRLRLRLGQASMTASPPGSLRASDWVILNCSFSRPDRPASVHWFRNRGQGRVPVRESPHHHLAESFLFLPQVSPMDSGPWGCILTYRDGFNVSIMYNLTVLGLEPPTPLTVYAGAGSRVGLPCRLPAGVGTRSFLTAKWTPPGGGPDLLVTGDNGDFTLRLEDVSQAQAGTYTCHIHLQEQQLNATVTLAIITVTPKSFGSPGSLGKLLCEVTPVSGQERFVWSSLDTPSQRSFSGPWLEAQEAQLLSQPWQCQLYQGERLLGAAVYFTGGGGSGGGGSGGGGSGGGGSGQVQLVESGGGVVQPGRSLRLDCKASGITFSNSGMHWVRQAPGKGLEWVAVIWYDGSKRYYADSVKGRFTISRDNSKNTLFLQMNSLRAEDTAVYYCATNDDYWGQGTLVTVSSASTKGPSVFPLAPCSRSTSESTAALGCLVKDYFPEPVTVSWNSGALTSGVHTFPAVLQSSGLYSLSSVVTVPSSSLGTKTYTCNVDHKPSNTKVDKRVESKYGPPCPPCPAPEFLGGPSVFLFPPKPKDTLMISRTPEVTCVVVDVSQEDPEVQFNWYVDGVEVHNAKTKPREEQFNSTYRVVSVLTVLHQDWLNGKEYKCKVSNKGLPSSIEKTISKAKGQPREPQVYTLPPSQEEMTKNQVSLTCLVKGFYPSDIAVEWESNGQPENNYKTTPPVLDSDGSFFLYSRLTVDKSRWQEGNVFSCSVMHEALHNHYTQKSLSLSLGK

SEQ ID NO: 111 - protein, 443 aa, synthetic construct
  REGION 1..443: note = CD80-Nivolumab
VIHVTKEVKEVATLSCGHNVSVEELAQTRIYWQKEKKMVLTMMSGDMNIWPEYKNRTIFDITNNLSIVILALRPSDEGTYECVVLKYEKDAFKREHLAEVTLSVKADFPTPSISDFEIPTSNIRRIICSTSGGFPEPHLSWLENGEELNAINTTVSQDPETELYAVSSKLDFNMTTNHSFMCLIKYGHLRVNQTFNWNTTKQEHFPDNGGGGSGGGGSGGGGSGGGGSGEIVLTQSPATLSLSPGERATLSCRASQSVSSYLAWYQQKPGQAPRLLIYDASNRATGIPARFSGSGSGTDFTLTISSLEPEDFAVYYCQQSSNWPRTFGQGTKVEIKRTVAAPSVFIFPPSDEQLKSGTASVVCLLNNFYPREAKVQWKVDNALQSGNSQESVTEQDSKDSTYSLSSTLTLSKADYEKHKVYACEVTHQGLSSPVTKSFNRGEC

SEQ ID NO: 112 - protein, 641 aa, synthetic construct
  REGION 1..641: note = LAG3-Nivolumab
LQPGAEVPVVWAQEGAPAQLPCSPTIPLQDLSLLRRAGVTWQHQPDSGPPAAAPGHPLAPGPHPAAPSSWGPRPRRYTVLSVGPGGLRSGRLPLQPRVQLDERGRQRGDFSLWLRPARRADAGEYRAAVHLRDRALSCRLRLRLGQASMTASPPGSLRASDWVILNCSFSRPDRPASVHWFRNRGQGRVPVRESPHHHLAESFLFLPQVSPMDSGPWGCILTYRDGFNVSIMYNLTVLGLEPPTPLTVYAGAGSRVGLPCRLPAGVGTRSFLTAKWTPPGGGPDLLVTGDNGDFTLRLEDVSQAQAGTYTCHIHLQEQQLNATVTLAIITVTPKSFGSPGSLGKLLCEVTPVSGQERFVWSSLDTPSQRSFSGPWLEAQEAQLLSQPWQCQLYQGERLLGAAVYFTGGGGSGGGGSGGGGSGGGGSGEIVLTQSPATLSLSPGERATLSCRASQSVSSYLAWYQQKPGQAPRLLIYDASNRATGIPARFSGSGSGTDFTLTISSLEPEDFAVYYCQQSSNWPRTFGQGTKVEIKRTVAAPSVFIFPPSDEQLKSGTASVVCLLNNFYPREAKVQWKVDNALQSGNSQESVTEQDSKDSTYSLSSTLTLSKADYEKHKVYACEVTHQGLSSPVTKSFNRGEC

SEQ ID NO: 113 - protein, 913 aa, synthetic construct
  REGION 1..913: note = Nivolumab-LAG3 IgD1/D2-CD80
QVQLVESGGGVVQPGRSLRLDCKASGITFSNSGMHWVRQAPGKGLEWVAVIWYDGSKRYYADSVKGRFTISRDNSKNTLFLQMNSLRAEDTAVYYCATNDDYWGQGTLVTVSSASTKGPSVFPLAPCSRSTSESTAALGCLVKDYFPEPVTVSWNSGALTSGVHTFPAVLQSSGLYSLSSVVTVPSSSLGTKTYTCNVDHKPSNTKVDKRVESKYGPPCPPCPAPEFLGGPSVFLFPPKPKDTLMISRTPEVTCVVVDVSQEDPEVQFNWYVDGVEVHNAKTKPREEQFNSTYRVVSVLTVLHQDWLNGKEYKCKVSNKGLPSSIEKTISKAKGQPREPQVYTLPPSQEEMTKNQVSLTCLVKGFYPSDIAVEWESNGQPENNYKTTPPVLDSDGSFFLYSRLTVDKSRWQEGNVFSCSVMHEALHNHYTQKSLSLSLGAGGGGSGGGGSGVIHVTKEVKEVATLSCGHNVSVEELAQTRIYWQKEKKMVLTMMSGDMNIWPEYKNRTIFDITNNLSIVILALRPSDEGTYECVVLKYEKDAFKREHLAEVTLSVKADFPTPSISDFEIPTSNIRRIICSTSGGFPEPHLSWLENGEELNAINTTVSQDPETELYAVSSKLDFNMTTNHSFMCLIKYGHLRVNQTFNWNTTKQEHFPDNGGGGSGGGGSGSLQPGAEVPVVWAQEGAPAQLPCSPTIPLQDLSLLRRAGVTWQHQPDSGPPAAAPGHPLAPGPHPAAPSSWGPRPRRYTVLSVGPGGLRSGRLPLQPRVQLDERGRQRGDFSLWLRPARRADAGEYRAAVHLRDRALSCRLRLRLGQASMTASPPGSLRASDWVILNCSFSRPDRPASVHWFRNRGQGRVPVRESPHHHLAESFLFLPQVSPMDSGPWGCILTYRDGFNVSIMYNLTVLGLEP

SEQ ID NO: 114 - protein, 995 aa, synthetic construct
  REGION 1..995: note = Nivolumab-LAG3 IgD1/D2/D3-CD80
QVQLVESGGGVVQPGRSLRLDCKASGITFSNSGMHWVRQAPGKGLEWVAVIWYDGSKRYYADSVKGRFTISRDNSKNTLFLQMNSLRAEDTAVYYCATNDDYWGQGTLVTVSSASTKGPSVFPLAPCSRSTSESTAALGCLVKDYFPEPVTVSWNSGALTSGVHTFPAVLQSSGLYSLSSVVTVPSSSLGTKTYTCNVDHKPSNTKVDKRVESKYGPPCPPCPAPEFLGGPSVFLFPPKPKDTLMISRTPEVTCVVVDVSQEDPEVQFNWYVDGVEVHNAKTKPREEQFNSTYRVVSVLTVLHQDWLNGKEYKCKVSNKGLPSSIEKTISKAKGQPREPQVYTLPPSQEEMTKNQVSLTCLVKGFYPSDIAVEWESNGQPENNYKTTPPVLDSDGSFFLYSRLTVDKSRWQEGNVFSCSVMHEALHNHYTQKSLSLSLGAGGGGSGGGGSGVIHVTKEVKEVATLSCGHNVSVEELAQTRIYWQKEKKMVLTMMSGDMNIWPEYKNRTIFDITNNLSIVILALRPSDEGTYECVVLKYEKDAFKREHLAEVTLSVKADFPTPSISDFEIPTSNIRRIICSTSGGFPEPHLSWLENGEELNAINTTVSQDPETELYAVSSKLDFNMTTNHSFMCLIKYGHLRVNQTFNWNTTKQEHFPDNGGGGSGGGGSGLQPGAEVPVVWAQEGAPAQLPCSPTIPLQDLSLLRRAGVTWQHQPDSGPPAAAPGHPLAPGPHPAAPSSWGPRPRRYTVLSVGPGGLRSGRLPLQPRVQLDERGRQRGDFSLWLRPARRADAGEYRAAVHLRDRALSCRLRLRLGQASMTASPPGSLRASDWVILNCSFSRPDRPASVHWFRNRGQGRVPVRESPHHHLAESFLFLPQVSPMDSGPWGCILTYRDGFNVSIMYNLTVLGLEPPTPLTVYAGAGSRVGLPCRLPAGVGTRSFLTAKWTPPGGGPDLLVTGDNGDFTLRLEDVSQAQAGTYTCHIHLQEQQLNATVT

SEQ ID NO: 115 - protein, 1095 aa, synthetic construct
  REGION 1..1095: note = Nivolumab-LAG3-CD80
QVQLVESGGGVVQPGRSLRLDCKASGITFSNSGMHWVRQAPGKGLEWVAVIWYDGSKRYYADSVKGRFTISRDNSKNTLFLQMNSLRAEDTAVYYCATNDDYWGQGTLVTVSSASTKGPSVFPLAPCSRSTSESTAALGCLVKDYFPEPVTVSWNSGALTSGVHTFPAVLQSSGLYSLSSVVTVPSSSLGTKTYTCNVDHKPSNTKVDKRVESKYGPPCPPCPAPEFLGGPSVFLFPPKPKDTLMISRTPEVTCVVVDVSQEDPEVQFNWYVDGVEVHNAKTKPREEQFNSTYRVVSVLTVLHQDWLNGKEYKCKVSNKGLPSSIEKTISKAKGQPREPQVYTLPPSQEEMTKNQVSLTCLVKGFYPSDIAVEWESNGQPENNYKTTPPVLDSDGSFFLYSRLTVDKSRWQEGNVFSCSVMHEALHNHYTQKSLSLSLGAGGGGSGGGGSGGGGSGGGSGVIHVTKEVKEVATLSCGHNVSVEELAQTRIYWQKEKKMVLTMMSGDMNIWPEYKNRTIFDITNNLSIVILALRPSDEGTYECVVLKYEKDAFKREHLAEVTLSVKADFPTPSISDFEIPTSNIRRIICSTSGGFPEPHLSWLENGEELNAINTTVSQDPETELYAVSSKLDFNMTTNHSFMCLIKYGHLRVNQTFNWNTTKQEHFPDNGGGGSGGGGSGGGGSGGGGSGLQPGAEVPVVWAQEGAPAQLPCSPTIPLQDLSLLRRAGVTWQHQPDSGPPAAAPGHPLAPGPHPAAPSSWGPRPRRYTVLSVGPGGLRSGRLPLQPRVQLDERGRQRGDFSLWLRPARRADAGEYRAAVHLRDRALSCRLRLRLGQASMTASPPGSLRASDWVILNCSFSRPDRPASVHWFRNRGQGRVPVRESPHHHLAESFLFLPQVSPMDSGPWGCILTYRDGFNVSIMYNLTVLGLEPPTPLTVYAGAGSRVGLPCRLPAGVGTRSFLTAKWTPPGGGPDLLVTGDNGDFTLRLEDVSQAQAGTYTCHIHLQEQQLNATVTLAIITVTPKSFGSPGSLGKLLCEVTPVSGQERFVWSSLDTPSQRSFSGPWLEAQEAQLLSQPWQCQLYQGERLLGAAVYFT

SEQ ID NO: 116 - protein, 913 aa, synthetic construct
  REGION 1..913: note = Nivolumab-CD80-LAG3 IgD1/D2
QVQLVESGGGVVQPGRSLRLDCKASGITFSNSGMHWVRQAPGKGLEWVAVIWYDGSKRYYADSVKGRFTISRDNSKNTLFLQMNSLRAEDTAVYYCATNDDYWGQGTLVTVSSASTKGPSVFPLAPCSRSTSESTAALGCLVKDYFPEPVTVSWNSGALTSGVHTFPAVLQSSGLYSLSSVVTVPSSSLGTKTYTCNVDHKPSNTKVDKRVESKYGPPCPPCPAPEFLGGPSVFLFPPKPKDTLMISRTPEVTCVVVDVSQEDPEVQFNWYVDGVEVHNAKTKPREEQFNSTYRVVSVLTVLHQDWLNGKEYKCKVSNKGLPSSIEKTISKAKGQPREPQVYTLPPSQEEMTKNQVSLTCLVKGFYPSDIAVEWESNGQPENNYKTTPPVLDSDGSFFLYSRLTVDKSRWQEGNVFSCSVMHEALHNHYTQKSLSLSLGAGGGGSGGGGSGSLQPGAEVPVVWAQEGAPAQLPCSPTIPLQDLSLLRRAGVTWQHQPDSGPPAAAPGHPLAPGPHPAAPSSWGPRPRRYTVLSVGPGGLRSGRLPLQPRVQLDERGRQRGDFSLWLRPARRADAGEYRAAVHLRDRALSCRLRLRLGQASMTASPPGSLRASDWVILNCSFSRPDRPASVHWFRNRGQGRVPVRESPHHHLAESFLFLPQVSPMDSGPWGCILTYRDGFNVSIMYNLTVLGLEPGGGGSGGGGSGVIHVTKEVKEVATLSCGHNVSVEELAQTRIYWQKEKKMVLTMMSGDMNIWPEYKNRTIFDITNNLSIVILALRPSDEGTYECVVLKYEKDAFKREHLAEVTLSVKADFPTPSISDFEIPTSNIRRIICSTSGGFPEPHLSWLENGEELNAINTTVSQDPETELYAVSSKLDFNMTTNHSFMCLIKYGHLRVNQTFNWNTTKQEHFPDN

SEQ ID NO: 117 - protein, 995 aa, synthetic construct
  REGION 1..995: note = Nivolumab-CD80-LAG3 IgD1/D2/D3
QVQLVESGGGVVQPGRSLRLDCKASGITFSNSGMHWVRQAPGKGLEWVAVIWYDGSKRYYADSVKGRFTISRDNSKNTLFLQMNSLRAEDTAVYYCATNDDYWGQGTLVTVSSASTKGPSVFPLAPCSRSTSESTAALGCLVKDYFPEPVTVSWNSGALTSGVHTFPAVLQSSGLYSLSSVVTVPSSSLGTKTYTCNVDHKPSNTKVDKRVESKYGPPCPPCPAPEFLGGPSVFLFPPKPKDTLMISRTPEVTCVVVDVSQEDPEVQFNWYVDGVEVHNAKTKPREEQFNSTYRVVSVLTVLHQDWLNGKEYKCKVSNKGLPSSIEKTISKAKGQPREPQVYTLPPSQEEMTKNQVSLTCLVKGFYPSDIAVEWESNGQPENNYKTTPPVLDSDGSFFLYSRLTVDKSRWQEGNVFSCSVMHEALHNHYTQKSLSLSLGAGGGGSGGGGSGLQPGAEVPVVWAQEGAPAQLPCSPTIPLQDLSLLRRAGVTWQHQPDSGPPAAAPGHPLAPGPHPAAPSSWGPRPRRYTVLSVGPGGLRSGRLPLQPRVQLDERGRQRGDFSLWLRPARRADAGEYRAAVHLRDRALSCRLRLRLGQASMTASPPGSLRASDWVILNCSFSRPDRPASVHWFRNRGQGRVPVRESPHHHLAESFLFLPQVSPMDSGPWGCILTYRDGFNVSIMYNLTVLGLEPPTPLTVYAGAGSRVGLPCRLPAGVGTRSFLTAKWTPPGGGPDLLVTGDNGDFTLRLEDVSQAQAGTYTCHIHLQEQQLNATVTGGGGSGGGGSGVIHVTKEVKEVATLSCGHNVSVEELAQTRIYWQKEKKMVLTMMSGDMNIWPEYKNRTIFDITNNLSIVILALRPSDEGTYECVVLKYEKDAFKREHLAEVTLSVKADFPTPSISDFEIPTSNIRRIICSTSGGFPEPHLSWLENGEELNAINTTVSQDPETELYAVSSKLDFNMTTNHSFMCLIKYGHLRVNQTFNWNTTKQEHFPDN

SEQ ID NO: 118 - protein, 1095 aa, synthetic construct
  REGION 1..1095: note = Nivolumab-CD80-LAG3
QVQLVESGGGVVQPGRSLRLDCKASGITFSNSGMHWVRQAPGKGLEWVAVIWYDGSKRYYADSVKGRFTISRDNSKNTLFLQMNSLRAEDTAVYYCATNDDYWGQGTLVTVSSASTKGPSVFPLAPCSRSTSESTAALGCLVKDYFPEPVTVSWNSGALTSGVHTFPAVLQSSGLYSLSSVVTVPSSSLGTKTYTCNVDHKPSNTKVDKRVESKYGPPCPPCPAPEFLGGPSVFLFPPKPKDTLMISRTPEVTCVVVDVSQEDPEVQFNWYVDGVEVHNAKTKPREEQFNSTYRVVSVLTVLHQDWLNGKEYKCKVSNKGLPSSIEKTISKAKGQPREPQVYTLPPSQEEMTKNQVSLTCLVKGFYPSDIAVEWESNGQPENNYKTTPPVLDSDGSFFLYSRLTVDKSRWQEGNVFSCSVMHEALHNHYTQKSLSLSLGAGGGGSGGGGSGGGGSGGGGSGLQPGAEVPVVWAQEGAPAQLPCSPTIPLQDLSLLRRAGVTWQHQPDSGPPAAAPGHPLAPGPHPAAPSSWGPRPRRYTVLSVGPGGLRSGRLPLQPRVQLDERGRQRGDFSLWLRPARRADAGEYRAAVHLRDRALSCRLRLRLGQASMTASPPGSLRASDWVILNCSFSRPDRPASVHWFRNRGQGRVPVRESPHHHLAESFLFLPQVSPMDSGPWGCILTYRDGFNVSIMYNLTVLGLEPPTPLTVYAGAGSRVGLPCRLPAGVGTRSFLTAKWTPPGGGPDLLVTGDNGDFTLRLEDVSQAQAGTYTCHIHLQEQQLNATVTLAIITVTPKSFGSPGSLGKLLCEVTPVSGQERFVWSSLDTPSQRSFSGPWLEAQEAQLLSQPWQCQLYQGERLLGAAVYFTGGGGSGGGGSGGGGSGGGSGVIHVTKEVKEVATLSCGHNVSVEELAQTRIYWQKEKKMVLTMMSGDMNIWPEYKNRTIFDITNNLSIVILALRPSDEGTYECVVLKYEKDAFKREHLAEVTLSVKADFPTPSISDFEIPTSNIRRIICSTSGGFPEPHLSWLENGEELNAINTTVSQDPETELYAVSSKLDFNMTTNHSFMCLIKYGHLRVNQTFNWNTTKQEHFPDN

SEQ ID NO: 119 - protein, 1095 aa, synthetic construct
  REGION 1..1095: note = LAG3-Nivolumab-CD80
LQPGAEVPVVWAQEGAPAQLPCSPTIPLQDLSLLRRAGVTWQHQPDSGPPAAAPGHPLAPGPHPAAPSSWGPRPRRYTVLSVGPGGLRSGRLPLQPRVQLDERGRQRGDFSLWLRPARRADAGEYRAAVHLRDRALSCRLRLRLGQASMTASPPGSLRASDWVILNCSFSRPDRPASVHWFRNRGQGRVPVRESPHHHLAESFLFLPQVSPMDSGPWGCILTYRDGFNVSIMYNLTVLGLEPPTPLTVYAGAGSRVGLPCRLPAGVGTRSFLTAKWTPPGGGPDLLVTGDNGDFTLRLEDVSQAQAGTYTCHIHLQEQQLNATVTLAIITVTPKSFGSPGSLGKLLCEVTPVSGQERFVWSSLDTPSQRSFSGPWLEAQEAQLLSQPWQCQLYQGERLLGAAVYFTGGGGSGGGGSGGGGSGGGSGQVQLVESGGGVVQPGRSLRLDCKASGITFSNSGMHWVRQAPGKGLEWVAVIWYDGSKRYYADSVKGRFTISRDNSKNTLFLQMNSLRAEDTAVYYCATNDDYWGQGTLVTVSSASTKGPSVFPLAPCSRSTSESTAALGCLVKDYFPEPVTVSWNSGALTSGVHTFPAVLQSSGLYSLSSVVTVPSSSLGTKTYTCNVDHKPSNTKVDKRVESKYGPPCPPCPAPEFLGGPSVFLFPPKPKDTLMISRTPEVTCVVVDVSQEDPEVQFNWYVDGVEVHNAKTKPREEQFNSTYRVVSVLTVLHQDWLNGKEYKCKVSNKGLPSSIEKTISKAKGQPREPQVYTLPPSQEEMTKNQVSLTCLVKGFYPSDIAVEWESNGQPENNYKTTPPVLDSDGSFFLYSRLTVDKSRWQEGNVFSCSVMHEALHNHYTQKSLSLSLGAGGGGSGGGGSGGGGSGGGGSGVIHVTKEVKEVATLSCGHNVSVEELAQTRIYWQKEKKMVLTMMSGDMNIWPEYKNRTIFDITNNLSIVILALRPSDEGTYECVVLKYEKDAFKREHLAEVTLSVKADFPTPSISDFEIPTSNIRRIICSTSGGFPEPHLSWLENGEELNAINTTVSQDPETELYAVSSKLDFNMTTNHSFMCLIKYGHLRVNQTFNWNTTKQEHFPDN

SEQ ID NO: 120 - protein, 1095 aa, synthetic construct
  REGION 1..1095: note = CD80-Nivolumab-LAG3
VIHVTKEVKEVATLSCGHNVSVEELAQTRIYWQKEKKMVLTMMSGDMNIWPEYKNRTIFDITNNLSIVILALRPSDEGTYECVVLKYEKDAFKREHLAEVTLSVKADFPTPSISDFEIPTSNIRRIICSTSGGFPEPHLSWLENGEELNAINTTVSQDPETELYAVSSKLDFNMTTNHSFMCLIKYGHLRVNQTFNWNTTKQEHFPDNGGGGSGGGGSGGGGSGGGSGQVQLVESGGGVVQPGRSLRLDCKASGITFSNSGMHWVRQAPGKGLEWVAVIWYDGSKRYYADSVKGRFTISRDNSKNTLFLQMNSLRAEDTAVYYCATNDDYWGQGTLVTVSSASTKGPSVFPLAPCSRSTSESTAALGCLVKDYFPEPVTVSWNSGALTSGVHTFPAVLQSSGLYSLSSVVTVPSSSLGTKTYTCNVDHKPSNTKVDKRVESKYGPPCPPCPAPEFLGGPSVFLFPPKPKDTLMISRTPEVTCVVVDVSQEDPEVQFNWYVDGVEVHNAKTKPREEQFNSTYRVVSVLTVLHQDWLNGKEYKCKVSNKGLPSSIEKTISKAKGQPREPQVYTLPPSQEEMTKNQVSLTCLVKGFYPSDIAVEWESNGQPENNYKTTPPVLDSDGSFFLYSRLTVDKSRWQEGNVFSCSVMHEALHNHYTQKSLSLSLGAGGGGSGGGGSGGGGSGGGGSGLQPGAEVPVVWAQEGAPAQLPCSPTIPLQDLSLLRRAGVTWQHQPDSGPPAAAPGHPLAPGPHPAAPSSWGPRPRRYTVLSVGPGGLRSGRLPLQPRVQLDERGRQRGDFSLWLRPARRADAGEYRAAVHLRDRALSCRLRLRLGQASMTASPPGSLRASDWVILNCSFSRPDRPASVHWFRNRGQGRVPVRESPHHHLAESFLFLPQVSPMDSGPWGCILTYRDGFNVSIMYNLTVLGLEPPTPLTVYAGAGSRVGLPCRLPAGVGTRSFLTAKWTPPGGGPDLLVTGDNGDFTLRLEDVSQAQAGTYTCHIHLQEQQLNATVTLAIITVTPKSFGSPGSLGKLLCEVTPVSGQERFVWSSLDTPSQRSFSGPWLEAQEAQLLSQPWQCQLYQGERLLGAAVYFT

SEQ ID NO: 121 - protein, 448 aa, synthetic construct
  REGION 1..448: note = sugemalimab
EVQLLESGGGLVQPGGSLRLSCAASGFTFSSYAMSWVRQAPGKGLEWVSGISGSGGFTYYADSVKGRFTISRDNSKNTLYLQMNSLRAEDTAVYYCAKPPRGYNYGPFDYWGQGTLVTVSSASTKGPSVFPLAPCSRSTSESTAALGCLVKDYFPEPVTVSWNSGALTSGVHTFPAVLQSSGLYSLSSVVTVPSSSLGTKTYTCNVDHKPSNTKVDKRVESKYGPPCPPCPAPEFLGGPSVFLFPPKPKDTLMISRTPEVTCVVVDVSQEDPEVQFNWYVDGVEVHNAKTKPREEQFNSTYRVVSVLTVLHQDWLNGKEYKCKVSNKGLPSSIEKTISKAKGQPREPQVYTLPPSQEEMTKNQVSLTCLVKGFYPSDIAVEWESNGQPENNYKTTPPVLDSDGSFFLYSRLTVDKSRWQEGNVFSCSVMHEALHNHYTQKSLSLSLGK

SEQ ID NO: 122 - protein, 214 aa, synthetic construct
  REGION 1..214: note = sugemalimab
SYVLTQPPSVSVAPGQTARITCGGNNIGSKSVHWYQQKPGQAPVLVVYDDSDRPSGIPERFSGSNSGNTATLTISRVEAGDEADYYCQVWDSSSDHVVFGGGTKLTVLGQPKAAPSVTLFPPSSEELQANKATLVCLISDFYPGAVTVAWKADSSPVKAGVETTTPSKQSNNKYAASSYLSLTPEQWKSHRSYSCQVTHEGSTVEKTVAPTECS

SEQ ID NO: 123 - DNA, 1401 bp, synthetic construct
  misc_feature 1..1401: note = sugemalimabDNA
  source 1..1401: mol_type = other DNA
atgcacagctcagcactgctctgttgcctggtcctcctgactggggtgagggccgaggtgcagctgctggagagcggggggggactggtgcagccaggaggaagcctgagactgagctgtgccgccagcgggtttacatttagcagctatgccatgagctgggtgagacaggcccctggcaaaggcctggagtgggtgagcggaatctccggcagcgggggatttacatactacgccgatagtgtgaagggcagatttacaatcagcagagacaacagcaagaacacactgtacctgcagatgaacagcctgagagccgaggacaccgccgtgtactattgcgccaagccccccagaggatataactacggacccttcgactactggggacagggcaccctggtgacagtgtccagcgctagcaccaagggcccatcggtcttccccctggcgccctgctccaggagcacctccgagagcacagccgccctgggctgcctggtcaaggactacttccccgaaccggtgacggtgtcgtggaactcaggcgccctgaccagcggcgtgcacaccttcccggctgtcctacagtcctcaggactctactccctcagcagcgtggtgaccgtgccctccagcagcttgggcacgaagacctacacctgcaacgtagatcacaagcccagcaacaccaaggtggacaagagagttgagtccaaatatggtcccccatgcccaccatgcccagcacctgagttcctggggggaccatcagtcttcctgttccccccaaaacccaaggacactctcatgatctcccggacccctgaggtcacgtgcgtggtggtggacgtgagccaggaagaccccgaggtccagttcaactggtacgtggatggcgtggaggtgcataatgccaagacaaagccgcgggaggagcagttcaacagcacgtaccgtgtggtcagcgtcctcaccgtcctgcaccaggactggctgaacggcaaggagtacaagtgcaaggtctccaacaaaggcctcccgtcctccatcgagaaaaccatctccaaagccaaagggcagccccgagagccacaggtgtacaccctgcccccatcccaggaggagatgaccaagaaccaggtcagcctgacctgcctggtcaaaggcttctaccccagcgacatcgccgtggagtgggagagcaatgggcagccggagaacaactacaagaccacgcctcccgtgctggactccgacggctccttcttcctctacagcaggctaaccgtggacaagagcaggtggcaggaggggaatgtcttctcatgctccgtgatgcatgaggctctgcacaaccactacacacagaagagcctctccctgtctctgggtaaatga

SEQ ID NO: 124 - DNA, 702 bp, synthetic construct
  misc_feature 1..702: note = sugemalimabDNA
  source 1..702: mol_type = other DNA
atgggttggagttgcatcatcctatttctagtcgctaccgctacaggagtgcacagcagctacgtgctgacccaacctccatctgtttccgtcgcccctggacagaccgccagaatcacctgtggcggcaataacatcggctctaagtccgtgcactggtaccagcagaagcctggccaggctcctgtgctggtcgtgtacgacgactctgaccggccttctggcatccctgagcggttttctggcagcaactccggcaacaccgccaccctcaccatctctagagtggaagctggcgacgaggccgactactactgccaggtgtgggattccagctccgatcacgtggtgttcggcggaggcaccaagctgaccgtgctgggccagcctaaggctgctccctctgtgaccctgttcccccccagctccgaggaactgcaggccaacaaagccaccctggtgtgcctgatctccgacttctaccctggcgccgtgacagtggcttggaaagctgattcttctccagtgaaggccggcgtggaaaccaccacaccttcgaagcagtccaacaacaagtacgccgcctcctcttacctgtccctgacacccgagcagtggaagtctcatagatcctattcctgccaagtgacccacgagggctccaccgtggagaagaccgtggcccctaccgagtgctcctga

SEQ ID NO: 125 - DNA, 2088 bp, synthetic construct
  misc_feature 1..2088: note = AN_Bif_Abs_0017DNA
  source 1..2088: mol_type = other DNA
atgcacagctcagcactgctctgttgcctggtcctcctgactggggtgagggccgaggtgcagctgctggagagcggggggggactggtgcagccaggaggaagcctgagactgagctgtgccgccagcgggtttacatttagcagctatgccatgagctgggtgagacaggcccctggcaaaggcctggagtgggtgagcggaatctccggcagcgggggatttacatactacgccgatagtgtgaagggcagatttacaatcagcagagacaacagcaagaacacactgtacctgcagatgaacagcctgagagccgaggacaccgccgtgtactattgcgccaagccccccagaggatataactacggacccttcgactactggggacagggcaccctggtgacagtgtccagcgctagcaccaagggcccatcggtcttccccctggcgccctgctccaggagcacctccgagagcacagccgccctgggctgcctggtcaaggactacttccccgaaccggtgacggtgtcgtggaactcaggcgccctgaccagcggcgtgcacaccttcccggctgtcctacagtcctcaggactctactccctcagcagcgtggtgaccgtgccctccagcagcttgggcacgaagacctacacctgcaacgtagatcacaagcccagcaacaccaaggtggacaagagagttgagtccaaatatggtcccccatgcccaccatgcccagcacctgagttcctggggggaccatcagtcttcctgttccccccaaaacccaaggacactctcatgatctcccggacccctgaggtcacgtgcgtggtggtggacgtgagccaggaagaccccgaggtccagttcaactggtacgtggatggcgtggaggtgcataatgccaagacaaagccgcgggaggagcagttcaacagcacgtaccgtgtggtcagcgtcctcaccgtcctgcaccaggactggctgaacggcaaggagtacaagtgcaaggtctccaacaaaggcctcccgtcctccatcgagaaaaccatctccaaagccaaagggcagccccgagagccacaggtgtacaccctgcccccatcccaggaggagatgaccaagaaccaggtcagcctgacctgcctggtcaaaggcttctaccccagcgacatcgccgtggagtgggagagcaatgggcagccggagaacaactacaagaccacgcctcccgtgctggactccgacggctccttcttcctctacagcaggctaaccgtggacaagagcaggtggcaggaggggaatgtcttctcatgctccgtgatgcatgaggctctgcacaaccactacacacagaagagcctctccctgtctctgggtgccggcggaggtggctccggtggaggcggaagcggtggaggcggtagtggtggaggcggaagcggcgttatccacgtgaccaaggaagtgaaagaagtggcaacgctgtcctgtggtcacaatgtttctgttgaagagctggcacaaactcgcatctactggcaaaaggagaagaaaatggtgctgactatgatgtctggggacatgaatatatggcccgagtacaagaaccggaccatctttgatatcactaataacctctccattgtgatcctggctctgcgcccatctgacgagggcacatacgagtgtgttgttctgaagtatgaaaaagacgctttcaagcgggaacacctggctgaagtgacgttatcagtcaaagctgacttccctacacctagtatatctgactttgaaattccaacttctaatattagaaggataatttgctcaacctctggaggttttccagagcctcacctctcctggttggaaaatggagaagaattaaatgccatcaacacaacagtttcccaagatcctgaaactgagctctatgctgttagcagcaaactggatttcaatatgacaaccaaccacagcttcatgtgtctcatcaagtatggacatttaagagtgaatcagaccttcaactggaatacaaccaagcaagagcattttcctgataactga

SEQ ID NO: 126 - protein, 684 aa, synthetic construct
  REGION 1..684: note = AN_Bif_Abs_0025
EVQLLESGGGLVQPGGSLRLSCAASGFTFSNYAMSWVRQAPGKGLEWVSAISASGHSTYLADSVKGRFTISRDNSKNTLYLQMNSLRAEDTAVYYCAKDREVTMIVVLNGGFDYWGQGTRVTVSSASTKGPSVFPLAPSSKSTSGGTAALGCLVKDYFPEPVTVSWNSGALTSGVHTFPAVLQSSGLYSLSSVVTVPSSSLGTQTYICNVNHKPSNTKVDKRVEPKSCDKTHTCPPCPAPEFEGGPSVFLFPPKPKDTLMISRTPEVTCVVVDVSHEDPEVKFNWYVDGVEVHNAKTKPREEQYNSTYRVVSVLTVLHQDWLNGKEYKCKVSNKALPASIEKTISKAKGQPREPQVYTLPPSREEMTKNQVSLTCLVKGFYPSDIAVEWESNGQPENNYKTTPPVLDSDGSFFLYSKLTVDKSRWQQGNVFSCSVMHEALHNHYTQKSLSLSPGAGGGGSGGGGSGGGGSGGGGSGVIHVTKEVKEVATLSCGHNVSVEELAQTRIYWQKEKKMVLTMMSGDMNIWPEYKNRTIFDITNNLSIVILALRPSDEGTYECVVLKYEKDAFKREHLAEVTLSVKADFPTPSISDFEIPTSNIRRIICSTSGGFPEPHLSWLENGEELNAINTTVSQDPETELYAVSSKLDFNMTTNHSFMCLIKYGHLRVNQTFNWNTTKQEHFPDN

SEQ ID NO: 127 - protein, 214 aa, synthetic construct
  REGION 1..214: note = AN_Bif_Abs_0025
EIVLTQSPATLSLSPGERATLACRASQTASRYLAWYQQKPGQAPRLLIYDTSNRATGIPARFSGSGSGTDFTLSISSLEPEDFAVYYCQQRFNWPWTFGQGTKVEFKRTVAAPSVFIFPPSDEQLKSGTASVVCLLNNFYPREAKVQWKVDNALQSGNSQESVTEQDSKDSTYSLSSTLTLSKADYEKHKVYACEVTHQGLSSPVTKSFNRGEC

SEQ ID NO: 128 - DNA, 2109 bp, synthetic construct
  misc_feature 1..2109: note = AN_Bif_Abs_0025DNA
  source 1..2109: mol_type = other DNA
atgcacagctcagcactgctctgttgcctggtcctcctgactggggtgagggccgaggtgcagctgctggagagcggggggggactggtgcagccaggaggaagcctgagactgagctgtgccgccagcgggtttacatttagcaactatgccatgagctgggtgagacaggcccccggaaaaggactggagtgggtgagcgccattagcgccagtggacacagcacctacctggctgattccgtgaaggggcggttcacaatctccagagacaacagcaagaacacactgtacctgcagatgaacagcctgagagccgaggacaccgccgtgtactactgcgccaaggacagagaggtgaccatgattgtggtgctgaacggcggattcgactactggggccagggcacccgggtgaccgtgtcaagcgctagcaccaagggcccatcggtcttccccctggcaccctcctccaagagcacctctgggggcacagcggccctgggctgcctggtcaaggactacttccccgaaccggtgacggtgtcgtggaactcaggcgccctgaccagcggcgtgcacaccttcccggctgtcctacagtcctcaggactctactccctcagcagcgtggtgaccgtgccctccagcagcttgggcacccagacctacatctgcaacgtgaatcacaagcccagcaacaccaaggtggacaagagagttgagcccaaatcttgtgacaaaactcacacatgcccaccgtgcccagcacctgaattcgaggggggaccgtcagtcttcctcttccccccaaaacccaaggacaccctcatgatctcccggacccccgaggtcacatgcgtggtggtggacgtgagccacgaagaccctgaggtcaagttcaactggtacgtggacggcgtggaggtgcataatgccaagacaaagccgcgggaggagcagtacaacagcacgtaccgtgtggtcagcgtcctcaccgtcctgcaccaggactggctgaatggcaaggagtacaagtgcaaggtctccaacaaagccctcccagccagcatcgagaaaaccatctccaaagccaaagggcagccccgagaaccacaggtgtacaccctgcccccatcccgggaggagatgaccaagaaccaggtcagcctgacctgcctggtcaaaggcttctatcccagcgacatcgccgtggagtgggagagcaatgggcagccggagaacaactacaagaccacgcctcccgtgctggactccgacggctccttcttcctctacagcaagctcaccgtggacaagagcaggtggcagcaggggaacgtcttctcatgctccgtgatgcatgaggctctgcacaaccactacacgcagaagagcctctccctgtctccgggtgccggaggaggaggaagcggaggaggagggagcggaggagggggaagcggaggcggaggatccggcgttatccacgtgaccaaggaagtgaaagaagtggcaacgctgtcctgtggtcacaatgtttctgttgaagagctggcacaaactcgcatctactggcaaaaggagaagaaaatggtgctgactatgatgtctggggacatgaatatatggcccgagtacaagaaccggaccatctttgatatcactaataacctctccattgtgatcctggctctgcgcccatctgacgagggcacatacgagtgtgttgttctgaagtatgaaaaagacgctttcaagcgggaacacctggctgaagtgacgttatcagtcaaagctgacttccctacacctagtatatctgactttgaaattccaacttctaatattagaaggataatttgctcaacctctggaggttttccagagcctcacctctcctggttggaaaatggagaagaattaaatgccatcaacacaacagtttcccaagatcctgaaactgagctctatgctgttagcagcaaactggatttcaatatgacaaccaaccacagcttcatgtgtctcatcaagtatggacatttaagagtgaatcagaccttcaactggaatacaaccaagcaagagcattttcctgataactga

SEQ ID NO: 129 - DNA, 699 bp, synthetic construct
  misc_feature 1..699: note = AN_Bif_Abs_0025DNA
  source 1..699: mol_type = other DNA
atgcacagctcagcactgctctgttgcctggtcctcctgactggggtgagggccgagattgtgctgacccagagccccgccacactgagtctgagtcccggcgagagagccacactggcctgtagagctagtcagaccgccagcagatacctggcctggtatcagcagaagcccggccaggcccccagactgctgatttacgacacctccaacagagccaccggaatccctgccagattcagcggaagcggaagcggcacagacttcaccctgagcattagcagcctggaacccgaggatttcgccgtgtactactgccagcagcgcttcaactggccctggaccttcggccagggcaccaaggtggagttcaagcgtacggtggctgcaccatctgtcttcatcttcccgccatctgatgagcagttgaaatctggaactgcctctgttgtgtgcctgctgaataacttctatcccagagaggccaaagtacagtggaaggtggataacgccctccaatcgggtaactcccaggagagtgtcacagagcaggacagcaaggacagcacctacagcctcagcagcaccctgacgctgagcaaagcagactacgagaaacacaaagtctacgcctgcgaagtcacccatcagggcctgagttcgcccgtcacaaagagcttcaacaggggagagtgttga

SEQ ID NO: 130 - protein, 672 aa, synthetic construct
  REGION 1..672: note = AN_Bif_Abs_0042
EVQLLESGGGLVQPGGSLRLSCAASGFTFSSYAMSWVRQAPGKGLEWVSGISGSGGFTYYADSVKGRFTISRDNSKNTLYLQMNSLRAEDTAVYYCAKPPRGYNYGPFDYWGQGTLVTVSSASTKGPSVFPLAPCSRSTSESTAALGCLVKDYFPEPVTVSWNSGALTSGVHTFPAVLQSSGLYSLSSVVTVPSSSLGTKTYTCNVDHKPSNTKVDKRVESKYGPPCPPCPAPEFLGGPSVFLFPPKPKDTLMISRTPEVTCVVVDVSQEDPEVQFNWYVDGVEVHNAKTKPREEQFNSTYRVVSVLTVLHQDWLNGKEYKCKVSNKGLPSSIEKTISKAKGQPREPQVYTLPPSQEEMTKNQVSLTCLVKGFYPSDIAVEWESNGQPENNYKTTPPVLDSDGSFFLYSRLTVDKSRWQEGNVFSCSVMHEALHNHYTQKSLSLSLGAGGGGSGGGGSGGGGSGVIHVTKEVKEVATLSCGHNVSVEELAQTRIYWQKEKKMVLTMMSGDMNIWPEYKNRTIFDITNNLSIVILALRPSDEGTYECVVLKYEKDAFKREHLAEVTLSVKADFPTPSISDFEIPTSNIRRIICSTSGGFPEPHLSWLENGEELNAINTTVSQDPETELYAVSSKLDFNMTTNHSFMCLIKYGHLRVNQTFNWNTTKQEHFPDN

SEQ ID NO: 131 - DNA, 2073 bp, synthetic construct
  misc_feature 1..2073: note = AN_Bif_Abs_0042DNA
  source 1..2073: mol_type = other DNA
atgggttggagttgcatcatcctatttctagttgctaccgctaccggcgtgcatagcgaggtccagctgctggaatctggcggcggactggtgcagcctggcggcagcctacggctgtcctgtgccgcctctggctttaccttcagttcctacgccatgagctgggtcagacaggcccctggcaagggcctggagtgggtgtccggcatttctggctccggcggcttcacctactacgccgactccgtgaagggacggttcaccatctccagagataactccaagaacaccctgtacctgcagatgaactccctcagggccgaagataccgctgtgtactactgcgccaagcctccaagaggctacaactatggccctttcgactactggggccagggcaccctggtgaccgtctcaagcgcctctaccaaaggcccgtctgtgttccctctggctccttgctctcggtctacctccgagagcaccgccgctctgggctgcctggtcaaggactacttccccgaacctgtgacagtgtcctggaactctggcgctctgacctctggcgtgcacacctttcctgccgtgctgcagtcctccggcctgtactctctgtcttccgtggtgaccgtgcctagctcctccctgggcaccaagacctatacctgcaatgtggaccacaagccctccaacaccaaagtggataagcgggtggagtccaagtatggccccccttgtcctccatgccctgctcccgagttcctgggcggacccagcgtctttctgttccctcccaagcctaaggataccctgatgatctcccgcacacctgaagtgacctgcgtggtggtggacgtgtcccaagaggaccctgaggtgcagttcaactggtacgtcgacggcgtggaagtgcataacgccaagaccaagcctcgggaagagcagtttaactctacatacagagtggtgagcgtactgaccgtgctgcaccaggactggctgaacggcaaagagtacaagtgcaaggtgtctaacaagggcctcccatcttccatcgagaagacaatcagcaaggctaagggacagcctagagagcctcaggtgtacaccctgcctccatctcaggaagagatgaccaagaatcaagtgtctctgacctgtctggtcaaaggcttctacccttccgacatcgccgtggaatgggagtccaatggccagcccgagaacaactacaaaaccaccccacctgtgctggactctgatggctcattcttcctgtactccagactgacagtggacaagtctagatggcaagaaggcaacgtgttctcctgctccgtgatgcacgaggccctgcacaaccactacacccagaagtccctgagcctgtctctgggagctggcggtggcggctctggaggcggcggctccggaggtggaggctccggcgtgatccacgtgaccaaagaggtgaaagaagtggctacactgtcttgtggccacaacgtgtctgtggaagagctggcccagaccagaatttactggcagaaagaaaagaagatggtgctgaccatgatgtccggcgacatgaacatctggcctgagtacaagaaccggaccatcttcgacatcaccaacaacctgtccatcgtgatcctggctctgagaccttctgacgagggaacatacgagtgcgtggtgctgaagtacgagaaggacgccttcaagagagaacacctggccgaggtaaccctgtccgtgaaggccgacttccctaccccttccatcagtgacttcgagatccccacctccaacatccggcggatcatctgctccactagcgggggctttcctgagcctcacctctcctggctggaaaacggcgaggaactgaatgccatcaacaccaccgtatcccaggatcctgagacagagctgtatgctgtgtcttctaagctggatttcaacatgaccacaaaccactccttcatgtgcctgatcaagtacggccatctgagagtgaaccagacattcaattggaacactaccaagcaggaacacttccccgacaac

SEQ ID NO: 132 - protein, 667 aa, synthetic construct
  REGION 1..667: note = AN_Bif_Abs_0043
EVQLLESGGGLVQPGGSLRLSCAASGFTFSSYAMSWVRQAPGKGLEWVSGISGSGGFTYYADSVKGRFTISRDNSKNTLYLQMNSLRAEDTAVYYCAKPPRGYNYGPFDYWGQGTLVTVSSASTKGPSVFPLAPCSRSTSESTAALGCLVKDYFPEPVTVSWNSGALTSGVHTFPAVLQSSGLYSLSSVVTVPSSSLGTKTYTCNVDHKPSNTKVDKRVESKYGPPCPPCPAPEFLGGPSVFLFPPKPKDTLMISRTPEVTCVVVDVSQEDPEVQFNWYVDGVEVHNAKTKPREEQFNSTYRVVSVLTVLHQDWLNGKEYKCKVSNKGLPSSIEKTISKAKGQPREPQVYTLPPSQEEMTKNQVSLTCLVKGFYPSDIAVEWESNGQPENNYKTTPPVLDSDGSFFLYSRLTVDKSRWQEGNVFSCSVMHEALHNHYTQKSLSLSLGAGGGGSGGGGSGVIHVTKEVKEVATLSCGHNVSVEELAQTRIYWQKEKKMVLTMMSGDMNIWPEYKNRTIFDITNNLSIVILALRPSDEGTYECVVLKYEKDAFKREHLAEVTLSVKADFPTPSISDFEIPTSNIRRIICSTSGGFPEPHLSWLENGEELNAINTTVSQDPETELYAVSSKLDFNMTTNHSFMCLIKYGHLRVNQTFNWNTTKQEHFPDN

SEQ ID NO: 133 - DNA, 2058 bp, synthetic construct
  misc_feature 1..2058: note = AN_Bif_Abs_0043DNA
  source 1..2058: mol_type = other DNA
atgggttggagttgcatcatcctatttctagtggctaccgccaccggcgtgcattccgaagtgcagctgctggaaagcggaggcggcctggtgcagcccggcggctctctgagactgtcctgcgccgcttctggctttaccttctcttcctacgccatgtcttgggtgagacaggcccccggcaagggtctggaatgggtctccggcatctcgggctctggcggattcacctactacgctgactctgtcaaaggcagattcaccatctctcgggacaactccaagaacaccctctacctgcagatgaattctctgagagccgaggacaccgctgtgtactactgcgccaagcctcctagaggctacaactacggacctttcgactactggggccagggcacactggtaacagtgtcatctgcctctaccaagggcccctccgtgttccctctggctccctgttctaggtccacctccgagtccacagctgccctcggctgcctggtcaaggattacttccccgagcctgtgaccgtgtcttggaactctggcgccctgaccagcggcgtgcacacctttcctgccgtgctgcaatcctccggactgtactctctgtcttccgtcgtgaccgtgccttcttcttccctgggaaccaagacctacacctgcaacgtggaccacaagccatccaatacaaaggtggataagagagtcgaatctaagtacgggcctccttgcccaccttgccctgctcctgagttcctgggcggccctagcgtgtttctgttcccccctaagcccaaggacaccctgatgatctcccgcacacctgaagtgacctgtgtggtcgtcgacgtgtcccaagaggatcctgaagtgcagttcaattggtacgtggatggcgtggaagtccataacgctaaaacgaagcccagagaggaacagtttaacagtacctacagagtggtgtctgtgctgacagttctgcaccaggattggctgaatggcaaagagtacaagtgcaaggtgtccaacaagggcctgccttcttcaatcgagaagacaatttctaaggccaagggacagcctagagaacctcaggtgtacaccctgcctccaagccaagaggaaatgaccaagaaccaggtgtctctgacctgtttggtgaagggcttctaccctagcgacatcgccgtagagtgggagtccaacggccagcctgaaaacaactacaagaccacccctcctgtgctggactccgatggctccttcttcctctactcccggctcaccgtggacaaatctcggtggcaggagggcaacgtgttctcttgcagtgtgatgcacgaggccctgcacaaccactacacccagaagtccctgtccctgagcctgggcgctggcggcggaggcagcggtgggggcggctccggcgtgatccacgtgaccaaagaggtgaaagaggtggccaccctgagctgtggccacaacgtgtccgtggaagagctggctcagaccagaatctactggcagaaagaaaagaagatggtgctgactatgatgtccggcgacatgaacatctggcctgagtacaagaaccggaccatcttcgatatcaccaataacctgtccatcgtgatcctggctctgagaccttccgacgagggaacatatgagtgcgtggtgctgaagtacgagaaagacgccttcaagcgggaacacctggcagaagtgaccctctctgtgaaggccgactttcctaccccttccatcagcgacttcgagatccccacctctaacatccggcggatcatctgctccacctccggcggcttcccagagcctcacctgtcctggctggagaacggcgaggagctgaacgccatcaacaccacagtgtcccaggaccccgagacagaactgtatgccgtgtccagcaagctggacttcaacatgaccaccaaccactccttcatgtgcctgatcaagtatggccatctgcgggtgaaccagaccttcaactggaacaccaccaagcaggagcacttccctgacaac

SEQ ID NO: 134 - DNA, 2745 bp, synthetic construct
  misc_feature 1..2745: note = AN_Bif_Abs_0019DNA
  source 1..2745: mol_type = other DNA
atgcacagctcagcactgctctgttgcctggtcctcctgactggggtgagggccgaggtgcagctgctggagagcggggggggactggtgcagccaggaggaagcctgagactgagctgtgccgccagcgggtttacatttagcagctatgccatgagctgggtgagacaggcccctggcaaaggcctggagtgggtgagcggaatctccggcagcgggggatttacatactacgccgatagtgtgaagggcagatttacaatcagcagagacaacagcaagaacacactgtacctgcagatgaacagcctgagagccgaggacaccgccgtgtactattgcgccaagccccccagaggatataactacggacccttcgactactggggacagggcaccctggtgacagtgtccagcgctagcaccaagggcccatcggtcttccccctggcgccctgctccaggagcacctccgagagcacagccgccctgggctgcctggtcaaggactacttccccgaaccggtgacggtgtcgtggaactcaggcgccctgaccagcggcgtgcacaccttcccggctgtcctacagtcctcaggactctactccctcagcagcgtggtgaccgtgccctccagcagcttgggcacgaagacctacacctgcaacgtagatcacaagcccagcaacaccaaggtggacaagagagttgagtccaaatatggtcccccatgcccaccatgcccagcacctgagttcctggggggaccatcagtcttcctgttccccccaaaacccaaggacactctcatgatctcccggacccctgaggtcacgtgcgtggtggtggacgtgagccaggaagaccccgaggtccagttcaactggtacgtggatggcgtggaggtgcataatgccaagacaaagccgcgggaggagcagttcaacagcacgtaccgtgtggtcagcgtcctcaccgtcctgcaccaggactggctgaacggcaaggagtacaagtgcaaggtctccaacaaaggcctcccgtcctccatcgagaaaaccatctccaaagccaaagggcagccccgagagccacaggtgtacaccctgcccccatcccaggaggagatgaccaagaaccaggtcagcctgacctgcctggtcaaaggcttctaccccagcgacatcgccgtggagtgggagagcaatgggcagccggagaacaactacaagaccacgcctcccgtgctggactccgacggctccttcttcctctacagcaggctaaccgtggacaagagcaggtggcaggaggggaatgtcttctcatgctccgtgatgcatgaggctctgcacaaccactacacacagaagagcctctccctgtctctgggtgccggcggaggtggctccggtggaggcggaagcggtggaggcggtagtggtggaggcggaagcctgcagcctggcgctgaagtgcccgtggtgtgggcccaggagggcgctcctgctcagctgccttgctcccccaccatccccctgcaggacctgagcctgctgagaagagccggagtgacctggcagcaccagccagattccggacctcccgccgccgctccaggacatcctctggctcccggcccccacccagctgctccttctagctggggaccccggccaagaagatacaccgtgctgagcgtgggacccggcggcctgagatccggaagattgcctttacagccccgcgtgcagctggacgaaagaggaaggcaacgtggtgacttcagcctgtggctgaggcctgccaggagagccgatgccggagagtatagagccgccgtgcacctgagagacagagccctgagttgcagactgagactgagactgggccaggcttccatgaccgcctctccccccggctccctgagagctagcgactgggtgatcctgaactgtagcttctccagacccgacagacccgcctccgtgcactggtttagaaatagaggccagggccgcgtgcccgtgagagagtctccccaccaccacctggccgaaagtttcctgttcctgccccaggtgagccccatggacagcggcccttggggatgcatcctgacctacagagacggattcaatgtgtctatcatgtacaacctgaccgtgctgggcctggagccccctacccctctgaccgtgtacgccggagccggatctcgcgtgggcctgccttgcagactgcccgctggcgtgggcaccagatcctttctgaccgccaaatggaccccccctggcggcggaccagacctgctggtgaccggagacaatggagactttaccctgagactggaggacgtgagccaggctcaggctggcacctacacctgccacatccacctgcaggaacagcagctgaacgccaccgtgaccctggccatcatcaccgtgacccccaaatcctttggcagccccggcagcctgggcaagctgctgtgcgaggtgacccccgtgagcggccaggagagattcgtgtggagtagcctggacaccccctcccagagatccttttccggcccctggctggaggcccaggaggctcagctgctgtctcagccctggcagtgccagctgtatcagggggagaggctgctgggcgccgccgtgtatttcaccgagctgagctcccccggcgcccagagaagcggaagagccccaggcgccctgcccgctggacatctgtga

SEQ ID NO: 135 - protein, 870 aa, synthetic construct
  REGION 1..870: note = AN_Bif_Abs_0044
EVQLLESGGGLVQPGGSLRLSCAASGFTFSSYAMSWVRQAPGKGLEWVSGISGSGGFTYYADSVKGRFTISRDNSKNTLYLQMNSLRAEDTAVYYCAKPPRGYNYGPFDYWGQGTLVTVSSASTKGPSVFPLAPCSRSTSESTAALGCLVKDYFPEPVTVSWNSGALTSGVHTFPAVLQSSGLYSLSSVVTVPSSSLGTKTYTCNVDHKPSNTKVDKRVESKYGPPCPPCPAPEFLGGPSVFLFPPKPKDTLMISRTPEVTCVVVDVSQEDPEVQFNWYVDGVEVHNAKTKPREEQFNSTYRVVSVLTVLHQDWLNGKEYKCKVSNKGLPSSIEKTISKAKGQPREPQVYTLPPSQEEMTKNQVSLTCLVKGFYPSDIAVEWESNGQPENNYKTTPPVLDSDGSFFLYSRLTVDKSRWQEGNVFSCSVMHEALHNHYTQKSLSLSLGAGGGGSGGGGSGGGGSGLQPGAEVPVVWAQEGAPAQLPCSPTIPLQDLSLLRRAGVTWQHQPDSGPPAAAPGHPLAPGPHPAAPSSWGPRPRRYTVLSVGPGGLRSGRLPLQPRVQLDERGRQRGDFSLWLRPARRADAGEYRAAVHLRDRALSCRLRLRLGQASMTASPPGSLRASDWVILNCSFSRPDRPASVHWFRNRGQGRVPVRESPHHHLAESFLFLPQVSPMDSGPWGCILTYRDGFNVSIMYNLTVLGLEPPTPLTVYAGAGSRVGLPCRLPAGVGTRSFLTAKWTPPGGGPDLLVTGDNGDFTLRLEDVSQAQAGTYTCHIHLQEQQLNATVTLAIITVTPKSFGSPGSLGKLLCEVTPVSGQERFVWSSLDTPSQRSFSGPWLEAQEAQLLSQPWQCQLYQGERLLGAAVYFT

SEQ ID NO: 136 - DNA, 2667 bp, synthetic construct
  misc_feature 1..2667: note = AN_Bif_Abs_0044DNA
  source 1..2667: mol_type = other DNA
atgggttggagttgcatcatcctatttctagtggccaccgccaccggcgtgcactccgaggtgcagctgctggagtctggcggcggcctggtgcagcctggaggcagcctgagactgtcctgcgccgcctccggcttcaccttctcctcctacgccatgtcctgggtcagacaggcacccggcaagggactggagtgggtgtccggcatctccggatccggcggcttcacctactacgccgactccgtgaagggccggttcaccatttcccgggacaactccaagaacaccctgtacctgcagatgaactcccttagagccgaggataccgctgtgtactattgcgccaaacctcctcggggctacaactatggccctttcgactactgggggcagggcacgctggtcaccgtctcctctgcttctaccaagggcccatccgtgttccctctggctccctgctccaggtccacatccgaaagcaccgccgccctgggctgtctggtgaaggactacttccccgagcctgtgaccgtgtcttggaactccggcgctctgacatccggagtgcacacctttcctgccgtgctgcagtcttccggcttgtactccctgtcctctgtggtgaccgtgccttcttcttctctgggcaccaaaacatacacctgcaacgtggaccacaagccttctaacaccaaggttgacaagcgggtcgaatccaagtacggccccccttgccctccttgtcctgctcccgagttcctgggcggaccctccgtctttctgtttcctcccaagcctaaggacaccctgatgatctctagaacccccgaagtgacctgtgtggtggtggacgtctcccaagaggaccctgaggtgcagttcaactggtacgtggatggcgtggaagtgcacaacgccaagaccaagcctagagaggaacagttcaattccacctacagagtggtgtctgtcctgacagtgctgcatcaggattggctgaacggcaaagagtacaagtgcaaggtatccaacaagggcctgccctcctccatcgagaagaccatctctaaggccaagggccagcctagagaacctcaagtgtatacgctccctccttctcaagaagagatgaccaagaaccaggtgtctctgacatgcctggtgaagggcttctacccttccgacatcgccgtggaatgggagtccaacggccagcctgagaacaactacaagaccacccctcccgtgctggatagcgacggctccttcttcctgtactctaggctgaccgtggacaagtctagatggcaggagggcaacgtgttctcatgtagcgtgatgcacgaggccctgcacaaccactacacccagaaatctctgtccctgtctctgggcgctggcggcggaggctcaggcggcggtggctccggcggcggcggctctggcctccagcccggcgccgaggtgcccgtcgtgtgggcccaggaaggcgcccctgcccagttgccttgttctcctaccatccctctgcaggacctgtctctgctgagaagagctggcgtgacctggcagcaccagcctgattctggccccccggccgcagctcctggccaccccctggcccctggccctcatcctgccgctccatctagctggggtcctagacccagaagatacaccgtgctgtctgtcggacctggcggcctgcggtctggcagactaccactgcagcctagagtccagctggacgagcggggacggcagcggggcgatttctccctgtggctgcggcctgccagacgggccgatgccggcgagtaccgggccgctgtgcacctgcgggaccgggctctgtcctgccggctgagactgagactgggacaggcctccatgaccgcctctcctcccggcagtctgagggcttctgactgggtgatcctgaactgcagcttctccagacctgaccgcccagccagtgtgcactggttcagaaacagaggccagggcagagtgcctgtgcgcgagtcccctcaccaccatctggctgaatccttcctgttcctgcctcaggtgagccctatggactccggaccttggggctgcatcctgacctatcgggatgggttcaacgtgagtatcatgtacaatctgactgtgctgggcctggaaccacctacacccctgaccgtttacgctggcgctggctccagagtgggcctgccttgcagattacccgccggcgtgggcacccggtcttttctgaccgctaagtggaccccgcctggcggcggaccggacctgctggtgacaggcgacaatggggacttcacactgcggctggaggacgtgtcccaggcccaggccggcacctacacatgtcacatccacctgcaagagcagcagctgaatgctaccgtgaccctggccatcatcaccgtgacccctaagagcttcggctctcccggatctttaggcaagctgctgtgcgaggtgacacctgtgtccggccaagaaagattcgtgtggagctccctggacaccccttcccagagatccttcagcggaccttggctggaagctcaagaggctcagctgctctctcagccttggcagtgccagctgtaccagggcgagcgactgctgggcgctgccgtgtactttaca

SEQ ID NO: 137 - protein, 865 aa, synthetic construct
  REGION 1..865: note = AN_Bif_Abs_0045
EVQLLESGGGLVQPGGSLRLSCAASGFTFSSYAMSWVRQAPGKGLEWVSGISGSGGFTYYADSVKGRFTISRDNSKNTLYLQMNSLRAEDTAVYYCAKPPRGYNYGPFDYWGQGTLVTVSSASTKGPSVFPLAPCSRSTSESTAALGCLVKDYFPEPVTVSWNSGALTSGVHTFPAVLQSSGLYSLSSVVTVPSSSLGTKTYTCNVDHKPSNTKVDKRVESKYGPPCPPCPAPEFLGGPSVFLFPPKPKDTLMISRTPEVTCVVVDVSQEDPEVQFNWYVDGVEVHNAKTKPREEQFNSTYRVVSVLTVLHQDWLNGKEYKCKVSNKGLPSSIEKTISKAKGQPREPQVYTLPPSQEEMTKNQVSLTCLVKGFYPSDIAVEWESNGQPENNYKTTPPVLDSDGSFFLYSRLTVDKSRWQEGNVFSCSVMHEALHNHYTQKSLSLSLGAGGGGSGGGGSGLQPGAEVPVVWAQEGAPAQLPCSPTIPLQDLSLLRRAGVTWQHQPDSGPPAAAPGHPLAPGPHPAAPSSWGPRPRRYTVLSVGPGGLRSGRLPLQPRVQLDERGRQRGDFSLWLRPARRADAGEYRAAVHLRDRALSCRLRLRLGQASMTASPPGSLRASDWVILNCSFSRPDRPASVHWFRNRGQGRVPVRESPHHHLAESFLFLPQVSPMDSGPWGCILTYRDGFNVSIMYNLTVLGLEPPTPLTVYAGAGSRVGLPCRLPAGVGTRSFLTAKWTPPGGGPDLLVTGDNGDFTLRLEDVSQAQAGTYTCHIHLQEQQLNATVTLAIITVTPKSFGSPGSLGKLLCEVTPVSGQERFVWSSLDTPSQRSFSGPWLEAQEAQLLSQPWQCQLYQGERLLGAAVYFT

SEQ ID NO: 138 - DNA, 2652 bp, synthetic construct
  misc_feature 1..2652: note = AN_Bif_Abs_0045DNA
  source 1..2652: mol_type = other DNA
atgggttggagttgcatcatcctatttctagtggccacagccaccggcgtccactccgaggtgcagctgctggaatctggcggcggcctggtgcagcctggcggatcccttcgcctgtcttgcgctgcttctggcttcaccttcagctcctatgctatgtcctgggtcagacaggctcctgggaaaggcctggagtgggtgagcggcatcagcggctctggcggctttacctactatgctgactctgtgaagggcagattcaccatctctcgggataattctaagaacacactgtacctccagatgaacagtctgcgggctgaggatacagctgtgtactactgcgccaagcctcctagaggctacaactacggccccttcgactactggggccagggcaccctggtgaccgtgagttctgcctccaccaagggacctagcgtgtttccactggccccttgctctcggtccacctctgagtctaccgccgccctgggctgtctggtgaaagactacttccccgagcctgtgacagtgtcctggaactccggcgctttgacctccggcgtgcacacctttcctgccgtgctgcagtccagcggactgtacagcctgtcttctgtggtgaccgttccttcctcttccctgggcaccaagacctatacatgcaacgtggaccacaagccctccaacactaaagtggataagcgggtggaatccaagtacggcccgccttgtcctccctgtcctgcgcccgaattcctgggaggccctagcgtgttcctattccctcctaagcccaaggacaccctgatgatctcccggacccctgaggttacatgcgtggtggtcgacgtgagccaggaggaccccgaagtgcagttcaactggtacgtggacggcgtggaagtgcacaacgccaagaccaaacctagagaggaacagttcaattctacctacagagtggtgtccgttctgaccgtactgcaccaggactggctgaacggcaaagagtacaagtgcaaggtgtccaacaagggcctgccatccagcatcgagaagaccatctccaaggccaagggacagcctcgcgagcctcaagtgtacaccctgcctccttctcaagaagagatgaccaagaaccaggtgtctcttacctgcctggtgaagggcttctacccttctgacatcgccgtggaatgggagtccaatggccaaccagagaacaactacaaaaccacccctcccgttctggattccgacggctccttcttcctgtactcgcggctgacggtggacaagtccagatggcaagagggcaacgtgttcagctgctccgtgatgcacgaggctctgcataaccactacacccagaagtccctgtctctgtccctgggtgcaggcggaggcggatctggtggcggaggctctggcctgcagccaggcgccgaagtgcctgttgtgtgggcccaggaaggcgcccctgctcagctgccctgctctcccaccattccactccaggatctgagtctgctgcggagagccggcgtgacctggcagcaccagcctgactccggcccaccggccgctgcacctggccaccctctggcccctggccctcatcctgctgctccttcctcttggggcccccggcctcggagatacaccgtgctgtccgtgggacccggcggtctgagatctggtagactccctctgcaacccagagtgcagctggacgagcggggaagacagagaggcgacttctccctgtggctgaggcctgccagaagagccgacgccggcgagtaccgcgccgctgtgcacctgcgggacagagctctgtcctgcagactgagactgaggctgggccaggcctccatgaccgcctccccacctggctccctgcgagcttccgattgggtgatcctgaactgttctttctccagacctgacagacccgcctcagtgcactggttcagaaacagaggccaaggccgggtgcccgtgcgggagtctcctcaccaccatctggccgagtccttcctgtttctgcctcaggtgtcgcccatggactccggcccttggggctgcatcctcacctatagggatggcttcaacgtgtccatcatgtacaacctgacagtgctgggcctggaacctcctacccctctgacagtgtacgccggcgccggctctcgggtgggcctgccttgtcggctgcctgccggcgtgggcaccagatccttcctcaccgctaagtggacccctcctggcggaggccccgatctgctggtcacaggcgataacggcgacttcaccctgagactggaggacgtatcacaggcccaggctgggacctacacctgtcacatccacctgcaggagcagcagctgaatgctaccgtcaccctggccatcatcaccgtgactcctaagagcttcggctcgccgggctccctgggcaagctgctgtgcgaggtgacacccgtgtctggccaggaaagattcgtctggtcctctctggacaccccatcccagcggagcttttctgggccttggctcgaagcccaggaggcccagctgctgtctcagccctggcagtgccagctgtaccagggcgagcgcctgctgggagctgctgtgtactttacc

SEQ ID NO: 139 - protein, 860 aa, synthetic construct
  REGION 1..860: note = AN_Bif_Abs_0046
EVQLLESGGGLVQPGGSLRLSCAASGFTFSSYAMSWVRQAPGKGLEWVSGISGSGGFTYYADSVKGRFTISRDNSKNTLYLQMNSLRAEDTAVYYCAKPPRGYNYGPFDYWGQGTLVTVSSASTKGPSVFPLAPCSRSTSESTAALGCLVKDYFPEPVTVSWNSGALTSGVHTFPAVLQSSGLYSLSSVVTVPSSSLGTKTYTCNVDHKPSNTKVDKRVESKYGPPCPPCPAPEFLGGPSVFLFPPKPKDTLMISRTPEVTCVVVDVSQEDPEVQFNWYVDGVEVHNAKTKPREEQFNSTYRVVSVLTVLHQDWLNGKEYKCKVSNKGLPSSIEKTISKAKGQPREPQVYTLPPSQEEMTKNQVSLTCLVKGFYPSDIAVEWESNGQPENNYKTTPPVLDSDGSFFLYSRLTVDKSRWQEGNVFSCSVMHEALHNHYTQKSLSLSLGAGGGGSGLQPGAEVPVVWAQEGAPAQLPCSPTIPLQDLSLLRRAGVTWQHQPDSGPPAAAPGHPLAPGPHPAAPSSWGPRPRRYTVLSVGPGGLRSGRLPLQPRVQLDERGRQRGDFSLWLRPARRADAGEYRAAVHLRDRALSCRLRLRLGQASMTASPPGSLRASDWVILNCSFSRPDRPASVHWFRNRGQGRVPVRESPHHHLAESFLFLPQVSPMDSGPWGCILTYRDGFNVSIMYNLTVLGLEPPTPLTVYAGAGSRVGLPCRLPAGVGTRSFLTAKWTPPGGGPDLLVTGDNGDFTLRLEDVSQAQAGTYTCHIHLQEQQLNATVTLAIITVTPKSFGSPGSLGKLLCEVTPVSGQERFVWSSLDTPSQRSFSGPWLEAQEAQLLSQPWQCQLYQGERLLGAAVYFT

SEQ ID NO: 140 - DNA, 2637 bp, synthetic construct
  misc_feature 1..2637: note = AN_Bif_Abs_0046DNA
  source 1..2637: mol_type = other DNA
atgggttggagttgcatcatcctatttctagtggccaccgccacaggcgtgcactccgaggttcagctgctggaaagcggcggcggacttgtgcagcctggtggctccttgcggctgtcctgtgccgcctctggatttaccttctcttcctacgccatgtcctgggtgcggcaagctccgggcaagggcctggagtgggtcagcggcatctctggatctggcggatttacctactacgccgactccgtgaaaggccggttcaccatctcccgggacaactccaagaataccctgtacctgcagatgaacagcctgcgggccgaggacaccgctgtgtactactgcgccaagcctcctagaggctacaactatggccctttcgactactggggccagggcacactggtcaccgtgtcttccgcttctaccaagggcccttctgtgttccctctggctccttgctctagatccacctctgagagcaccgctgctcttggctgcctggtgaaggactactttcctgagcctgtgaccgtctcctggaactccggcgctctgacctccggagtgcacaccttcccagccgtgctgcagtctagcggcctgtattccctgtcctccgtggtaaccgtgccctcgtcctccctgggcacgaaaacctacacctgcaacgtggaccacaagccttctaacaccaaagtggacaagcgggtggaatccaagtacggccccccttgcccaccttgtcctgctcctgagttcctgggcggccccagtgtgttcctgttcccccctaaacccaaggacacactgatgatcagcagaacccctgaggtgacttgcgtggtggtggatgtcagtcaagaggaccctgaagtgcagttcaactggtacgtggacggcgtggaagtgcacaacgccaaaaccaagcctagagaggaacagttcaactctacctaccgggtggtctccgtgctgaccgtgctgcaccaggattggctgaatggcaaagagtacaagtgcaaggtgtccaacaagggcctgccttcctctatcgagaagaccattagcaaggccaagggccagcctcgggaacctcaggtgtacacgctgcctccttcccaagaagagatgaccaagaaccaggtgtctctgacctgtctggtgaagggattctacccttccgacatcgccgtggaatgggagtccaatggccagcctgagaacaactacaagaccacgcctcctgtgctggattctgatggctccttcttcctctactcccgtttaacagtggacaagtccagatggcaggaaggcaacgtgttctcttgctccgtgatgcacgaggccctgcacaatcactacacccagaagagcctctctctgtccctgggagctggcggcggcggctctggcctgcagccaggcgccgaagtgcctgtggtgtgggctcaggagggcgcccctgcccagctgccctgttctcccactatccctctgcaggacctgtccctgctgagacgggctggagtcacctggcagcaccagcctgacagcggcccacctgccgctgctcctggccaccctttggctcccggccctcatcctgccgccccttcttcttggggcccaagacctcggagatacaccgtgctgtccgtcggaccaggcggactgagatctggcagactgcccctccagcctcgggtgcaactggacgagagaggcagacagagaggcgatttctccctgtggctgcggcccgccagaagagcagacgccggcgagtacagagccgctgtgcatctgagggatagagcactgtcgtgcagactacgcctgagactgggccaggcctccatgaccgccagcccgcctggatctctgagggcctcagactgggtgatcctgaactgcagcttctcccggccagaccgtcctgcttctgtgcactggttccggaaccggggacagggcagagtgcctgtgagagagtcccctcaccaccatctggctgagtctttcctgtttctgcctcaggtctcacctatggactctggcccctggggatgcatcctgacctatagagacggcttcaatgtgtccatcatgtacaacctgacagtgctgggcctggaaccccctacacctctgaccgtgtacgccggagctggctccagagtgggcctgccatgtagactgcctgccggcgtgggcacccggtcctttctgaccgcgaagtggacccctcccggcggcggccccgatctgctggtgaccggcgataacggtgacttcaccctgcggctggaggatgtgtcccaggcccaggctggcacctacacctgtcacatccacctgcaagagcagcagctgaacgctaccgtgacactggccatcatcaccgtgacacctaagagcttcggctctcccggctctctgggcaagctgctgtgcgaggtgacgcccgtgtctggccaagagcggttcgtgtggtcctctctggacaccccttcccagagatcttttagcgggccatggctggaagctcaggaggcccagctgctgtctcagccctggcagtgccagctgtaccagggcgaacgcctgctgggtgctgccgtgtacttcacc

SEQ ID NO: 141 - DNA, 2682 bp, synthetic construct
  misc_feature 1..2682: note = AN_Bif_Abs_0035DNA
  source 1..2682: mol_type = other DNA
atgcacagctcagcactgctctgttgcctggtcctcctgactggggtgagggccctgcagcctggagctgaagtgcccgtggtgtgggcccaggagggtgctcctgctcagctgccttgctcccccaccatccccctgcaggacctgtccctgctgaggagggccggagtgacctggcagcaccagccagattctggacctcccgccgccgctccaggtcatcctctggctcctggcccccaccctgctgctccttcttcctggggccctcggccaaggaggtacaccgtgctgtccgtgggacccggcggtctgagatccggtagactgcccctgcagccccgggtgcagctggacgagagaggaaggcagcggggcgacttctccctgtggctgaggcctgcaaggagggctgacgccggagaatatagggccgctgtgcacctgagggacagggctctgtcttgccggctgaggctgaggctgggccaggcttctatgaccgcctcccccccaggctccctgagagcttctgactgggtgatcctgaattgttccttctccaggcccgaccggcccgcttctgtgcattggttccggaacagaggccagggcagggtgcccgtgagagagtctccccaccaccatctggccgagtctttcctgttcctgccccaggtgtcccccatggactccggaccttggggctgcatcctgacctacagggacgggttcaatgtgtctatcatgtacaacctgaccgtgctgggactggagccccctacccctctgaccgtgtacgccggagccggtagtcgcgtgggactgccttgcagactgccagccggggtgggaaccaggtccttcctgaccgccaagtggacccctcccggcggaggacctgatctgctggtgaccggagacaacggggactttacactgaggctggaggacgtgagccaggctcaggctggcacctacacctgccacatccacctgcaggagcagcagctgaacgctactgtgaccctggccatcatcaccgtgacccccaagtccttcggctcccccggaagcctgggcaagctgctgtgcgaggtgacccccgtgtccggacaggaaaggtttgtgtggtcctccctggacaccccaagccagaggtctttctccggcccctggctggaggcccaggaagctcagctgctgtcccagccctggcagtgccagctgtaccagggcgagcggctgctgggtgctgctgtgtacttcaccggtggcggagggtctggtggtggaggatcagggggtggaggttcaggaggcgggggaagtggtgaggtgcagctgctggagtccggaggagggctggtgcagccaggaggaagcctgaggctgtcctgtgccgcaagcgggttcacatttagttcctacgcaatgtcctgggtgaggcaggcccccggaaaaggcctggagtgggtgtccggaatttccggcagcgggggatttacctactacgcagatagtgtgaagggcagatttaccatttccagggacaacagcaagaacaccctgtacctgcagatgaacagcctgagggccgaggacaccgctgtgtattactgtgcaaagccacccaggggatataactacggccccttcgactactggggacagggaaccctggtgactgtgtcctccgctagcaccaagggcccatcggtcttccccctggcgccctgctccaggagcacctccgagagcacagccgccctgggctgcctggtcaaggactacttccccgaaccggtgacggtgtcgtggaactcaggcgccctgaccagcggcgtgcacaccttcccggctgtcctacagtcctcaggactctactccctcagcagcgtggtgaccgtgccctccagcagcttgggcacgaagacctacacctgcaacgtagatcacaagcccagcaacaccaaggtggacaagagagttgagtccaaatatggtcccccatgcccaccatgcccagcacctgagttcctggggggaccatcagtcttcctgttccccccaaaacccaaggacactctcatgatctcccggacccctgaggtcacgtgcgtggtggtggacgtgagccaggaagaccccgaggtccagttcaactggtacgtggatggcgtggaggtgcataatgccaagacaaagccgcgggaggagcagttcaacagcacgtaccgtgtggtcagcgtcctcaccgtcctgcaccaggactggctgaacggcaaggagtacaagtgcaaggtctccaacaaaggcctcccgtcctccatcgagaaaaccatctccaaagccaaagggcagccccgagagccacaggtgtacaccctgcccccatcccaggaggagatgaccaagaaccaggtcagcctgacctgcctggtcaaaggcttctaccccagcgacatcgccgtggagtgggagagcaatgggcagccggagaacaactacaagaccacgcctcccgtgctggactccgacggctccttcttcctctacagcaggctaaccgtggacaagagcaggtggcaggaggggaatgtcttctcatgctccgtgatgcatgaggctctgcacaaccactacacacagaagagcctctccctgtctctgggtaaatga

SEQ ID NO: 142 - DNA, 2439 bp, synthetic construct
  misc_feature 1..2439: note = AN_Bif_Abs_0047DNA
  source 1..2439: mol_type = other DNA
atgggttggagttgcatcatcctatttctagtggccaccgctaccggcgtgcactctgaggtccagctgctggaatccggcggcggcctggtgcagcctggcggcagcctgagactgtcttgcgctgcctccggctttaccttttcctcctacgccatgtcctgggtcagacaggcccctggcaagggcctggaatgggtgtccggcatctcgggatctggcggatttacctactacgctgactccgtgaaaggccggttcaccatctcccgggacaactccaagaacactctgtacctgcagatgaactctctgagagccgaagacaccgccgtgtactactgcgccaagccacctagaggctacaattacggccctttcgactactggggccagggcaccctggtgaccgtgtcctccgcctctacgaagggcccttccgtgttccctctcgccccctgctctcggtccacctccgagagcaccgctgctctgggatgcctggtgaaggactatttccccgaacctgtgaccgtgtcctggaacagtggcgctctgacatccggcgtgcacaccttcccagccgtgctgcagtccagcggcctgtactccttgagctcagtggtgacagtgccttcttcctctctgggcacaaagacctacacctgcaacgtggaccacaagccttctaacaccaaggtggacaagagagtggaatctaagtacggacctccatgtcctccttgccctgctcctgagttcctgggaggcccttctgtgttcctgttcccccccaaacctaaggacacactgatgatctccagaacccctgaggtgacctgcgtggtcgtcgatgtttcccaggaggatcctgaagtgcagtttaattggtacgtggatggggtggaagtgcataatgccaagacaaagcccagagaggaacagttcaactccacctaccgggtggttagcgtacttaccgtgctgcaccaggactggctgaacggcaaagagtacaagtgcaaggtgtccaacaagggcctgccctcctccatcgagaagaccatttccaaggccaaaggccagccccgcgagcctcaagtgtacacattgcctccctctcaggaagagatgaccaagaaccaggtgagcctgacctgtctggtgaagggcttctaccccagcgacatcgccgtcgagtgggagtccaacggacagcccgagaacaactacaaaaccaccccacctgtgctggactccgatggatctttcttcctgtactctagactcaccgtggacaagtctagatggcaggaaggcaacgtgttctcttgtagcgtgatgcacgaggccctccacaaccactacacccagaagagcctgtctctgtccctgggtgccgggggcggcggctctggcggaggaggctccggcggcggcggatctggcggcggcggctccggcctccagcctggcgctgaggtgcctgtggtgtgggctcaagagggcgctcctgcccagctgccctgtagccctacaatccctctgcaggatctgtctctgttgagacgggctggcgtgacctggcagcaccagcctgattctggcccccctgctgcagctcctggccaccccctggcccccggccctcaccctgccgcccctagctcctggggccctcggccccgcagatacaccgtgctgtccgtgggccccggcggcctgcggtccgggagactgcctctgcagcctagggtgcagctggacgagcgcggccggcagcggggcgatttctccctgtggctgcggcctgctagacgggccgacgccggcgagtaccgggccgctgtgcatctgagagacagagccctgtcctgcagacttagactgaggctcggccaggcttccatgaccgcctctcctccaggatctctccgggcttctgattgggtgatcctgaactgcagcttcagcagacctgaccggcctgcctctgtgcactggttccggaaccgaggccaaggtagagtgcccgtgcgggagtctccccaccaccatctggccgagtcctttctgttcctgccacaagtgagtcctatggactctggaccttggggctgcatcctgacctatagagacggcttcaatgtgtccatcatgtacaacctgacagtgctgggcctcgaaccccctacccctctgacagtgtacgccggcgctggctctagagtgggcctgccttgccggctgcctgccggcgttggcaccagatccttcctgaccgccaagtggaccccacctggcggtggcccagacctgctggtcaccggcgacaacggcgatttcaccctgcgcctggaagacgtgtcccaggcccaggctggtacctatacctgtcacatccacctgcaagagcagcagctgaacgccaccgtgaca

SEQ ID NO: 143 - DNA, 2190 bp, synthetic construct
  misc_feature 1..2190: note = AN_Bif_Abs_0048DNA
  source 1..2190: mol_type = other DNA
atgggttggagttgcatcatcctatttctagtggccaccgccacaggcgtgcattctgaagtccagctgctggaatctggcggcggcctggtgcagcctggcggctctctgagactgtcctgtgccgcctctggctttaccttttcctcttacgccatgtcctgggtccgacaggctcctggcaagggcctggagtgggtcagcggcatctctggctctgggggcttcacgtactacgctgactctgtgaaaggcagattcacaatctcccgggacaactccaagaacaccctgtacctgcagatgaacagcctgagagccgaggacaccgctgtgtactactgcgccaagcctccacggggctacaactacggccctttcgactactggggacaaggcaccctggtgacagtttcttctgcttctacaaagggcccttcagtatttcctctggctccttgcagtagatccacctccgagtccaccgctgcactgggctgtctggtgaaggactacttccccgagcctgttacagtgtcttggaactccggcgccctaaccagcggcgtgcacacctttcctgctgtactccagtcctccggactgtatagcctgtcctccgtggtgaccgtgcctagctccagcctgggaaccaagacctacacctgcaacgtggaccacaagccctccaacaccaaagtggacaagcgggtggaatccaagtacggccctccttgtcctccatgccctgccccagagttcctcggtggaccttctgtgtttctgttccctcctaagcctaaagacacactgatgatctccagaaccccagaggtgacctgcgtggtcgtcgacgtgtcccaggaggatcctgaagtgcagttcaactggtacgtggatggcgtcgaggtgcacaacgccaagaccaagcccagagaggaacagttcaattccacctacagagtggtgtccgtcctgaccgtgctgcaccaggactggctgaacggcaaagagtacaagtgcaaggtgtccaacaagggcctgccatcttctatcgagaagaccatcagcaaggccaaaggtcagcctagagaacctcaagtgtacaccctgcctccatcccaagaagagatgaccaagaaccaggtgtctctgacatgcctggtgaagggcttctatccttccgacatcgccgtggaatgggagagcaatggccagcctgagaacaactacaagaccacccctcctgtgctggattctgacggatccttcttcctgtactccagactgaccgtggacaagtctagatggcaggagggcaacgtgttctcttgctccgtgatgcacgaggccctgcacaaccactacacccagaagtccctgtctctgtctctgggagccggaggcggtggctccggaggcggcggctctggcggcggcggctccggcggcggcggctctggcctgcagcctggagctgaggtgcctgtggtgtgggctcaggaaggcgctccagcccagctgccctgtagtcctaccatccccctgcaggatctgagcctgctgcggcgggctggcgtgacctggcagcaccagcctgattcgggcccccctgccgctgcccccggccatcctctggcccctggcccccaccccgccgctccctcgtcctggggccctcggccccgccggtacaccgtgctgtctgtgggccctggcggattacggtctggccgcctgcctctgcagcccagagtgcagctggacgagagaggccggcagcggggcgacttctcactgtggctgcggcctgccaggagagccgacgccggcgagtatagagccgccgtgcatctgagagaccgggctctgtcttgcagactgagactgagactgggccaagcctccatgaccgcctcccccccgggctccctgcgcgcttctgattgggtgatcctgaactgctccttcagccggcctgacagacctgcttctgtgcactggttccggaaccggggacagggcagagtgcccgtgcgcgagtcccctcaccaccacctggccgagtccttcctgttcctgccacaggtgtctcctatggactccggcccttggggctgcatcctgacctacagagatggcttcaatgtgtccatcatgtacaacctgactgtgctgggcctggaacct

SEQ ID NO: 144 - DNA, 3369 bp, synthetic construct
  misc_feature 1..3369: note = AN_Bif_Abs_0036DNA
  source 1..3369: mol_type = other DNA
atgcacagctcagcactgctctgttgcctggtcctcctgactggggtgagggccctgcagcctggcgctgaagtgcccgtggtgtgggcccaggagggcgctcctgctcagctgccttgctcccccaccatccccctgcaggacctgagcctgctgagaagagccggagtgacctggcagcaccagccagattccggacctcccgccgccgctccaggacatcctctggctcccggcccccacccagctgctccttctagctggggaccccggccaagaagatacaccgtgctgagcgtgggacccggcggcctgagatccggaagattgcctttacagccccgcgtgcagctggacgaaagaggaaggcaacgtggtgacttcagcctgtggctgaggcctgccaggagagccgatgccggagagtatagagccgccgtgcacctgagagacagagccctgagttgcagactgagactgagactgggccaggcttccatgaccgcctctccccccggctccctgagagctagcgactgggtgatcctgaactgtagcttctccagacccgacagacccgcctccgtgcactggtttagaaatagaggccagggccgcgtgcccgtgagagagtctccccaccaccacctggccgaaagtttcctgttcctgccccaggtgagccccatggacagcggcccttggggatgcatcctgacctacagagacggattcaatgtgtctatcatgtacaacctgaccgtgctgggcctggagccccctacccctctgaccgtgtacgccggagccggatctcgcgtgggcctgccttgcagactgcccgctggcgtgggcaccagatcctttctgaccgccaaatggaccccccctggcggcggaccagacctgctggtgaccggagacaatggagactttaccctgagactggaggacgtgagccaggctcaggctggcacctacacctgccacatccacctgcaggaacagcagctgaacgccaccgtgaccctggccatcatcaccgtgacccccaaatcctttggcagccccggcagcctgggcaagctgctgtgcgaggtgacccccgtgagcggccaggagagattcgtgtggagtagcctggacaccccctcccagagatccttttccggcccctggctggaggcccaggaggctcagctgctgtctcagccctggcagtgccagctgtatcagggggagaggctgctgggcgccgccgtgtatttcaccggagggggtggaagtggcggaggtggttctggaggtggtgggtctggtggaggcggttcaggagaggtgcagctgctggagagcggggggggactggtgcagccaggaggaagcctgagactgagctgtgccgccagcgggtttacatttagcagctatgccatgagctgggtgagacaggcccctggcaaaggcctggagtgggtgagcggaatctccggcagcgggggatttacatactacgccgatagtgtgaagggcagatttacaatcagcagagacaacagcaagaacacactgtacctgcagatgaacagcctgagagccgaggacaccgccgtgtactattgcgccaagccccccagaggatataactacggacccttcgactactggggacagggcaccctggtgacagtgtccagcgctagcaccaagggcccatcggtcttccccctggcgccctgctccaggagcacctccgagagcacagccgccctgggctgcctggtcaaggactacttccccgaaccggtgacggtgtcgtggaactcaggcgccctgaccagcggcgtgcacaccttcccggctgtcctacagtcctcaggactctactccctcagcagcgtggtgaccgtgccctccagcagcttgggcacgaagacctacacctgcaacgtagatcacaagcccagcaacaccaaggtggacaagagagttgagtccaaatatggtcccccatgcccaccatgcccagcacctgagttcctggggggaccatcagtcttcctgttccccccaaaacccaaggacactctcatgatctcccggacccctgaggtcacgtgcgtggtggtggacgtgagccaggaagaccccgaggtccagttcaactggtacgtggatggcgtggaggtgcataatgccaagacaaagccgcgggaggagcagttcaacagcacgtaccgtgtggtcagcgtcctcaccgtcctgcaccaggactggctgaacggcaaggagtacaagtgcaaggtctccaacaaaggcctcccgtcctccatcgagaaaaccatctccaaagccaaagggcagccccgagagccacaggtgtacaccctgcccccatcccaggaggagatgaccaagaaccaggtcagcctgacctgcctggtcaaaggcttctaccccagcgacatcgccgtggagtgggagagcaatgggcagccggagaacaactacaagaccacgcctcccgtgctggactccgacggctccttcttcctctacagcaggctaaccgtggacaagagcaggtggcaggaggggaatgtcttctcatgctccgtgatgcatgaggctctgcacaaccactacacacagaagagcctctccctgtctctgggtgccggcggaggtggctccggtggaggcggaagcggtggaggcggtagtggtggaggcggaagcggcgttatccacgtgaccaaggaagtgaaagaagtggcaacgctgtcctgtggtcacaatgtttctgttgaagagctggcacaaactcgcatctactggcaaaaggagaagaaaatggtgctgactatgatgtctggggacatgaatatatggcccgagtacaagaaccggaccatctttgatatcactaataacctctccattgtgatcctggctctgcgcccatctgacgagggcacatacgagtgtgttgttctgaagtatgaaaaagacgctttcaagcgggaacacctggctgaagtgacgttatcagtcaaagctgacttccctacacctagtatatctgactttgaaattccaacttctaatattagaaggataatttgctcaacctctggaggttttccagagcctcacctctcctggttggaaaatggagaagaattaaatgccatcaacacaacagtttcccaagatcctgaaactgagctctatgctgttagcagcaaactggatttcaatatgacaaccaaccacagcttcatgtgtctcatcaagtatggacatttaagagtgaatcagaccttcaactggaatacaaccaagcaagagcattttcctgataactga

SEQ ID NO: 145 - DNA, 3369 bp, synthetic construct
  misc_feature 1..3369: note = AN_Bif_Abs_0037DNA
  source 1..3369: mol_type = other DNA
atgcacagctcagcactgctctgttgcctggtcctcctgactggggtgagggccgaggtgcagctgctggagagcggggggggactggtgcagccaggaggaagcctgagactgagctgtgccgccagcgggtttacatttagcagctatgccatgagctgggtgagacaggcccctggcaaaggcctggagtgggtgagcggaatctccggcagcgggggatttacatactacgccgatagtgtgaagggcagatttacaatcagcagagacaacagcaagaacacactgtacctgcagatgaacagcctgagagccgaggacaccgccgtgtactattgcgccaagccccccagaggatataactacggacccttcgactactggggacagggcaccctggtgacagtgtccagcgctagcaccaagggcccatcggtcttccccctggcgccctgctccaggagcacctccgagagcacagccgccctgggctgcctggtcaaggactacttccccgaaccggtgacggtgtcgtggaactcaggcgccctgaccagcggcgtgcacaccttcccggctgtcctacagtcctcaggactctactccctcagcagcgtggtgaccgtgccctccagcagcttgggcacgaagacctacacctgcaacgtagatcacaagcccagcaacaccaaggtggacaagagagttgagtccaaatatggtcccccatgcccaccatgcccagcacctgagttcctggggggaccatcagtcttcctgttccccccaaaacccaaggacactctcatgatctcccggacccctgaggtcacgtgcgtggtggtggacgtgagccaggaagaccccgaggtccagttcaactggtacgtggatggcgtggaggtgcataatgccaagacaaagccgcgggaggagcagttcaacagcacgtaccgtgtggtcagcgtcctcaccgtcctgcaccaggactggctgaacggcaaggagtacaagtgcaaggtctccaacaaaggcctcccgtcctccatcgagaaaaccatctccaaagccaaagggcagccccgagagccacaggtgtacaccctgcccccatcccaggaggagatgaccaagaaccaggtcagcctgacctgcctggtcaaaggcttctaccccagcgacatcgccgtggagtgggagagcaatgggcagccggagaacaactacaagaccacgcctcccgtgctggactccgacggctccttcttcctctacagcaggctaaccgtggacaagagcaggtggcaggaggggaatgtcttctcatgctccgtgatgcatgaggctctgcacaaccactacacacagaagagcctctccctgtctctgggtgccggagggggtggaagtggcggaggtggttctggaggtggtgggtctggtggaggcggttcaggactgcagcctggcgctgaagtgcccgtggtgtgggcccaggagggcgctcctgctcagctgccttgctcccccaccatccccctgcaggacctgagcctgctgagaagagccggagtgacctggcagcaccagccagattccggacctcccgccgccgctccaggacatcctctggctcccggcccccacccagctgctccttctagctggggaccccggccaagaagatacaccgtgctgagcgtgggacccggcggcctgagatccggaagattgcctttacagccccgcgtgcagctggacgaaagaggaaggcaacgtggtgacttcagcctgtggctgaggcctgccaggagagccgatgccggagagtatagagccgccgtgcacctgagagacagagccctgagttgcagactgagactgagactgggccaggcttccatgaccgcctctccccccggctccctgagagctagcgactgggtgatcctgaactgtagcttctccagacccgacagacccgcctccgtgcactggtttagaaatagaggccagggccgcgtgcccgtgagagagtctccccaccaccacctggccgaaagtttcctgttcctgccccaggtgagccccatggacagcggcccttggggatgcatcctgacctacagagacggattcaatgtgtctatcatgtacaacctgaccgtgctgggcctggagccccctacccctctgaccgtgtacgccggagccggatctcgcgtgggcctgccttgcagactgcccgctggcgtgggcaccagatcctttctgaccgccaaatggaccccccctggcggcggaccagacctgctggtgaccggagacaatggagactttaccctgagactggaggacgtgagccaggctcaggctggcacctacacctgccacatccacctgcaggaacagcagctgaacgccaccgtgaccctggccatcatcaccgtgacccccaaatcctttggcagccccggcagcctgggcaagctgctgtgcgaggtgacccccgtgagcggccaggagagattcgtgtggagtagcctggacaccccctcccagagatccttttccggcccctggctggaggcccaggaggctcagctgctgtctcagccctggcagtgccagctgtatcagggggagaggctgctgggcgccgccgtgtatttcaccggcggaggtggctccggtggaggcggaagcggtggaggcggtagtggtggaggcggaagcggcgttatccacgtgaccaaggaagtgaaagaagtggcaacgctgtcctgtggtcacaatgtttctgttgaagagctggcacaaactcgcatctactggcaaaaggagaagaaaatggtgctgactatgatgtctggggacatgaatatatggcccgagtacaagaaccggaccatctttgatatcactaataacctctccattgtgatcctggctctgcgcccatctgacgagggcacatacgagtgtgttgttctgaagtatgaaaaagacgctttcaagcgggaacacctggctgaagtgacgttatcagtcaaagctgacttccctacacctagtatatctgactttgaaattccaacttctaatattagaaggataatttgctcaacctctggaggttttccagagcctcacctctcctggttggaaaatggagaagaattaaatgccatcaacacaacagtttcccaagatcctgaaactgagctctatgctgttagcagcaaactggatttcaatatgacaaccaaccacagcttcatgtgtctcatcaagtatggacatttaagagtgaatcagaccttcaactggaatacaaccaagcaagagcattttcctgataactga

SEQ ID NO: 146 - DNA, 3369 bp, synthetic construct
  misc_feature 1..3369: note = AN_Bif_Abs_0038DNA
  source 1..3369: mol_type = other DNA
atgcacagctcagcactgctctgttgcctggtcctcctgactggggtgagggccgaggtgcagctgctggagagcggggggggactggtgcagccaggaggaagcctgagactgagctgtgccgccagcgggtttacatttagcagctatgccatgagctgggtgagacaggcccctggcaaaggcctggagtgggtgagcggaatctccggcagcgggggatttacatactacgccgatagtgtgaagggcagatttacaatcagcagagacaacagcaagaacacactgtacctgcagatgaacagcctgagagccgaggacaccgccgtgtactattgcgccaagccccccagaggatataactacggacccttcgactactggggacagggcaccctggtgacagtgtccagcgctagcaccaagggcccatcggtcttccccctggcgccctgctccaggagcacctccgagagcacagccgccctgggctgcctggtcaaggactacttccccgaaccggtgacggtgtcgtggaactcaggcgccctgaccagcggcgtgcacaccttcccggctgtcctacagtcctcaggactctactccctcagcagcgtggtgaccgtgccctccagcagcttgggcacgaagacctacacctgcaacgtagatcacaagcccagcaacaccaaggtggacaagagagttgagtccaaatatggtcccccatgcccaccatgcccagcacctgagttcctggggggaccatcagtcttcctgttccccccaaaacccaaggacactctcatgatctcccggacccctgaggtcacgtgcgtggtggtggacgtgagccaggaagaccccgaggtccagttcaactggtacgtggatggcgtggaggtgcataatgccaagacaaagccgcgggaggagcagttcaacagcacgtaccgtgtggtcagcgtcctcaccgtcctgcaccaggactggctgaacggcaaggagtacaagtgcaaggtctccaacaaaggcctcccgtcctccatcgagaaaaccatctccaaagccaaagggcagccccgagagccacaggtgtacaccctgcccccatcccaggaggagatgaccaagaaccaggtcagcctgacctgcctggtcaaaggcttctaccccagcgacatcgccgtggagtgggagagcaatgggcagccggagaacaactacaagaccacgcctcccgtgctggactccgacggctccttcttcctctacagcaggctaaccgtggacaagagcaggtggcaggaggggaatgtcttctcatgctccgtgatgcatgaggctctgcacaaccactacacacagaagagcctctccctgtctctgggtgccggagggggtggaagtggcggaggtggttctggaggtggtgggtctggtggaggcggttcaggcgttatccacgtgaccaaggaagtgaaagaagtggcaacgctgtcctgtggtcacaatgtttctgttgaagagctggcacaaactcgcatctactggcaaaaggagaagaaaatggtgctgactatgatgtctggggacatgaatatatggcccgagtacaagaaccggaccatctttgatatcactaataacctctccattgtgatcctggctctgcgcccatctgacgagggcacatacgagtgtgttgttctgaagtatgaaaaagacgctttcaagcgggaacacctggctgaagtgacgttatcagtcaaagctgacttccctacacctagtatatctgactttgaaattccaacttctaatattagaaggataatttgctcaacctctggaggttttccagagcctcacctctcctggttggaaaatggagaagaattaaatgccatcaacacaacagtttcccaagatcctgaaactgagctctatgctgttagcagcaaactggatttcaatatgacaaccaaccacagcttcatgtgtctcatcaagtatggacatttaagagtgaatcagaccttcaactggaatacaaccaagcaagagcattttcctgataacggcggaggtggctccggtggaggcggaagcggtggaggcggtagtggtggaggcggaagcggactgcagcctggcgctgaagtgcccgtggtgtgggcccaggagggcgctcctgctcagctgccttgctcccccaccatccccctgcaggacctgagcctgctgagaagagccggagtgacctggcagcaccagccagattccggacctcccgccgccgctccaggacatcctctggctcccggcccccacccagctgctccttctagctggggaccccggccaagaagatacaccgtgctgagcgtgggacccggcggcctgagatccggaagattgcctttacagccccgcgtgcagctggacgaaagaggaaggcaacgtggtgacttcagcctgtggctgaggcctgccaggagagccgatgccggagagtatagagccgccgtgcacctgagagacagagccctgagttgcagactgagactgagactgggccaggcttccatgaccgcctctccccccggctccctgagagctagcgactgggtgatcctgaactgtagcttctccagacccgacagacccgcctccgtgcactggtttagaaatagaggccagggccgcgtgcccgtgagagagtctccccaccaccacctggccgaaagtttcctgttcctgccccaggtgagccccatggacagcggcccttggggatgcatcctgacctacagagacggattcaatgtgtctatcatgtacaacctgaccgtgctgggcctggagccccctacccctctgaccgtgtacgccggagccggatctcgcgtgggcctgccttgcagactgcccgctggcgtgggcaccagatcctttctgaccgccaaatggaccccccctggcggcggaccagacctgctggtgaccggagacaatggagactttaccctgagactggaggacgtgagccaggctcaggctggcacctacacctgccacatccacctgcaggaacagcagctgaacgccaccgtgaccctggccatcatcaccgtgacccccaaatcctttggcagccccggcagcctgggcaagctgctgtgcgaggtgacccccgtgagcggccaggagagattcgtgtggagtagcctggacaccccctcccagagatccttttccggcccctggctggaggcccaggaggctcagctgctgtctcagccctggcagtgccagctgtatcagggggagaggctgctgggcgccgccgtgtatttcacctga

SEQ ID NO: 147 - protein, 1075 aa, synthetic construct
  REGION 1..1075: note = AN_Bif_Abs_0049
EVQLLESGGGLVQPGGSLRLSCAASGFTFSSYAMSWVRQAPGKGLEWVSGISGSGGFTYYADSVKGRFTISRDNSKNTLYLQMNSLRAEDTAVYYCAKPPRGYNYGPFDYWGQGTLVTVSSASTKGPSVFPLAPCSRSTSESTAALGCLVKDYFPEPVTVSWNSGALTSGVHTFPAVLQSSGLYSLSSVVTVPSSSLGTKTYTCNVDHKPSNTKVDKRVESKYGPPCPPCPAPEFLGGPSVFLFPPKPKDTLMISRTPEVTCVVVDVSQEDPEVQFNWYVDGVEVHNAKTKPREEQFNSTYRVVSVLTVLHQDWLNGKEYKCKVSNKGLPSSIEKTISKAKGQPREPQVYTLPPSQEEMTKNQVSLTCLVKGFYPSDIAVEWESNGQPENNYKTTPPVLDSDGSFFLYSRLTVDKSRWQEGNVFSCSVMHEALHNHYTQKSLSLSLGAGGGGSGGGGSGVIHVTKEVKEVATLSCGHNVSVEELAQTRIYWQKEKKMVLTMMSGDMNIWPEYKNRTIFDITNNLSIVILALRPSDEGTYECVVLKYEKDAFKREHLAEVTLSVKADFPTPSISDFEIPTSNIRRIICSTSGGFPEPHLSWLENGEELNAINTTVSQDPETELYAVSSKLDFNMTTNHSFMCLIKYGHLRVNQTFNWNTTKQEHFPDNGGGGSGGGGSGLQPGAEVPVVWAQEGAPAQLPCSPTIPLQDLSLLRRAGVTWQHQPDSGPPAAAPGHPLAPGPHPAAPSSWGPRPRRYTVLSVGPGGLRSGRLPLQPRVQLDERGRQRGDFSLWLRPARRADAGEYRAAVHLRDRALSCRLRLRLGQASMTASPPGSLRASDWVILNCSFSRPDRPASVHWFRNRGQGRVPVRESPHHHLAESFLFLPQVSPMDSGPWGCILTYRDGFNVSIMYNLTVLGLEPPTPLTVYAGAGSRVGLPCRLPAGVGTRSFLTAKWTPPGGGPDLLVTGDNGDFTLRLEDVSQAQAGTYTCHIHLQEQQLNATVTLAIITVTPKSFGSPGSLGKLLCEVTPVSGQERFVWSSLDTPSQRSFSGPWLEAQEAQLLSQPWQCQLYQGER

SEQ ID NO: 148 - DNA, 3282 bp, synthetic construct
  misc_feature 1..3282: note = AN_Bif_Abs_0049DNA
  source 1..3282: mol_type = other DNA
atgggttggagttgcatcatcctatttctagtggccaccgctaccggggtgcattctgaagtgcagctgctggaatctggaggtggcctggtccagcctggcggctccctcagactgtcctgtgccgcctctggctttaccttttcctcctacgccatgtcttgggtgcggcaggctcctggaaagggcctggagtgggtgtccggcatcagcggatccggcggcttcacctactacgccgacagcgtgaagggcagattcaccatctctcgggacaactccaagaataccctgtacctgcagatgaactccctgagagccgaagataccgccgtttactactgcgccaagcctcctagaggctacaactacggccctttcgactactggggccagggcactctggtcaccgtgtcctccgcctccacgaagggcccttccgtgttccctctggctccatgttcaagatccacctccgaatctaccgctgctctgggctgtctggtgaaggactacttccccgaacccgtgaccgtgtcctggaactccggcgccctgacctctggcgttcacaccttccctgccgtcctgcagtcctccggcctgtactctctgtctagcgtggtgacagtgccctcctcgtctctgggcaccaagacctacacctgcaacgtggaccacaagccttccaacaccaaagtggacaagcgggtggagtccaagtacggccctccttgccctccatgtcctgctcctgagttcctgggcggccctagtgtgttcctgttcccacccaagcccaaggacaccctgatgatctctcggacccctgaagtgacctgtgtggtggtggatgtgtcccaagaggatcctgaagtgcagttcaattggtacgtggacggagtggaagtgcacaacgccaagacaaaacccagagaggaacagttcaactctacctacagagtcgtgtctgtgctgaccgtgctgcatcaggattggctgaacggcaaagagtacaagtgcaaggtgtccaacaagggcctgccatcctccatcgagaaaaccatctccaaagccaagggccaacccagagagcctcaggtgtacacactgcctcccagccaggaagagatgaccaagaaccaggtgagcctgacctgcctggtgaaaggcttctacccctccgacatcgccgtggaatgggagtctaatggacagcctgagaacaactacaagaccacccctcctgtcctggattctgatggctctttcttcctgtactcccggctgaccgtcgacaaatctagatggcaggagggcaacgtgttttcctgctcagtgatgcacgaggctctgcacaatcactacacccagaagtctctgagcctatctttaggcgcagggggcggcggctctggaggcggcggttccggcgtgatccacgtgaccaaggaagtgaaagaggtggctacactgtcttgcggccacaacgtgtccgtggaagagctggcccagacaagaatctactggcagaaagaaaagaagatggtgctgaccatgatgtccggcgacatgaacatctggcctgagtataagaacagaaccatcttcgatatcacaaacaacttgtctatcgtgatcctcgccctgcgccccagcgacgagggcacctatgagtgcgtggtcctgaagtacgagaaggacgccttcaagcgggaacacctggccgaggtgaccctgtccgtgaaggccgactttcccaccccttctatctccgacttcgagatccccaccagcaacatcagacggatcatttgctccactagcggcggcttccctgaacctcacctgtcctggctggagaatggcgaagagctgaatgccatcaacaccaccgtgtctcaggatcctgagacagagctgtacgctgtgagctctaagctggacttcaacatgaccacaaaccacagcttcatgtgcctgatcaagtatggccatctgagggtgaaccagaccttcaactggaacaccaccaagcaggagcacttccctgacaacggcggaggcggaagcggcggaggcggctccggactgcagcctggtgccgaggttcctgtggtgtgggcccaggaaggcgctcctgcccagctgccttgctcccctacaatccctctgcaggacctgtctctgttgcggagagccggagtcacctggcagcaccagcctgactccggccctcccgccgccgctcccggccaccccctggcccctggccctcatcctgctgctccttcatcttggggacctagacctagacggtacaccgtgctgtctgtcggcccggggggcctgagaagcggcagactgcctttgcagcctagagtgcagctcgacgagcggggcagacagcgtggcgatttctctctctggctgcggcctgccagacgggccgacgctggcgagtacagagctgctgtgcacctgagagacagagccctatcctgcagactgagactgagactgggccaagcctccatgaccgcctctcctcctggctccctccgggcttccgactgggtcatcctgaactgctccttttctcggccggacagacccgcgagtgtccactggttccggaacaggggccaaggcagggtgcccgtgagagagtccccccaccaccatctggccgaatctttcctctttcttccacaagtgtctcctatggactccggcccttggggttgtatcctgacctaccgggacggcttcaacgtgtccatcatgtacaacctgacagtgctgggcctggagccccctacccctctaaccgtgtacgctggggctggcagtagagtgggactgccttgcagactgcctgctggtgtgggcacacggtcctttctgacagctaagtggaccccccctggcggaggccccgacctgctggttaccggcgataacggcgacttcaccctgagactggaggacgtgtctcaagcacaggccggcacctacacctgtcacatccacctgcaggagcagcagctgaacgctaccgtgacactggccatcatcaccgtgacccctaagagcttcggctctccaggctccctgggcaagctgctgtgcgaggtgacccctgtttccggacaggaacggttcgtgtggtcctctctggacaccccatcccagcggagcttctccggaccttggctggaggcccaagaggcccagctgctgagccagccttggcagtgccagctgtaccagggcgagaga

SEQ ID NO: 149 - protein, 1049 aa, synthetic construct
  REGION 1..1049: note = AN_Bif_Abs_0050
EVQLLESGGGLVQPGGSLRLSCAASGFTFSSYAMSWVRQAPGKGLEWVSGISGSGGFTYYADSVKGRFTISRDNSKNTLYLQMNSLRAEDTAVYYCAKPPRGYNYGPFDYWGQGTLVTVSSASTKGPSVFPLAPCSRSTSESTAALGCLVKDYFPEPVTVSWNSGALTSGVHTFPAVLQSSGLYSLSSVVTVPSSSLGTKTYTCNVDHKPSNTKVDKRVESKYGPPCPPCPAPEFLGGPSVFLFPPKPKDTLMISRTPEVTCVVVDVSQEDPEVQFNWYVDGVEVHNAKTKPREEQFNSTYRVVSVLTVLHQDWLNGKEYKCKVSNKGLPSSIEKTISKAKGQPREPQVYTLPPSQEEMTKNQVSLTCLVKGFYPSDIAVEWESNGQPENNYKTTPPVLDSDGSFFLYSRLTVDKSRWQEGNVFSCSVMHEALHNHYTQKSLSLSLGAGGGGSGGGGSGVIHVTKEVKEVATLSCGHNVSVEELAQTRIYWQKEKKMVLTMMSGDMNIWPEYKNRTIFDITNNLSIVILALRPSDEGTYECVVLKYEKDAFKREHLAEVTLSVKADFPTPSISDFEIPTSNIRRIICSTSGGFPEPHLSWLENGEELNAINTTVSQDPETELYAVSSKLDFNMTTNHSFMCLIKYGHLRVNQTFNGGGGSGGGGSGGAPAQLPCSPTIPLQDLSLLRRAGVTWQHQPDSGPPAAAPGHPLAPGPHPAAPSSWGPRPRRYTVLSVGPGGLRSGRLPLQPRVQLDERGRQRGDFSLWLRPARRADAGEYRAAVHLRDRALSCRLRLRLGQASMTASPPGSLRASDWVILNCSFSRPDRPASVHWFRNRGQGRVPVRESPHHHLAESFLFLPQVSPMDSGPWGCILTYRDGFNVSIMYNLTVLGLEPPTPLTVYAGAGSRVGLPCRLPAGVGTRSFLTAKWTPPGGGPDLLVTGDNGDFTLRLEDVSQAQAGTYTCHIHLQEQQLNATVTLAIITVTPKSFGSPGSLGKLLCEVTPVSGQERFVWSSLDTPSQRSFSGPWLEAQEAQLLSQPWQCQLYQGER

SEQ ID NO: 150 - DNA, 3204 bp, synthetic construct
  misc_feature 1..3204: note = AN_Bif_Abs_0050DNA
  source 1..3204: mol_type = other DNA
atgggttggagttgcatcatcctatttctagtggccaccgctaccggcgtccactccgaggtgcagctcctggagagtgggggcggcctcgtgcaacctggagggagcctgcgactaagctgtgctgcttctggctttaccttctcttcctacgccatgagctgggtccggcaggcccctggcaaaggcctggagtgggtctctggcatctctggctctggcggcttcacctactacgccgactccgtgaagggcagattcaccatctcccgggacaacagcaaaaataccctgtacctgcagatgaactccctgcgggccgaggacacagccgtgtactactgcgccaaacctcctagaggctataactacggcccttttgactactggggccaaggcaccctggtgacggtgtcgtctgccagcacaaagggaccttccgtgttcccactggccccttgctccagatccacctccgaatccaccgccgccctgggctgcctggtcaaagactacttcccagaacccgttaccgtgtcgtggaactccggcgctctgacctctggcgtgcacaccttcccagctgtgctccagtcctctggcctatactccctgagctccgtggtcacagtgccttcttcctccctgggcacaaaaacctacacttgcaacgtggaccataagccaagcaacaccaaggtggacaagcgggtggaatctaagtatggcccgccttgtcccccctgtcctgcacctgagttcctgggaggccctagcgtgtttctgtttcctcctaaacctaaagacaccctgatgatcagcagaacccctgaagtgacctgcgtggtggtggatgtgtcccaagaggatcctgaggtccagtttaactggtacgtggatggcgtggaagtgcacaatgccaagacaaagcccagggaggaacagttcaattcaacctacagagtcgtgagcgtgctgacagtactgcaccaggactggctgaacggcaaggagtacaagtgtaaggtatccaacaagggcctgccatcttccatcgagaagaccatctctaaggccaagggccagccacgcgagcctcaggtgtacaccctgccccctagccaggaagagatgaccaagaatcaggtgtccctgacctgtctggtgaagggcttctaccccagcgatatcgccgtggaatgggagtctaacggccaacctgagaacaactacaagaccaccccacctgtgctggattctgacggctctttcttcctgtactcccgcctgaccgtcgataagtccagatggcaggaaggcaacgtgttctcctgctccgtgatgcacgaggctctgcacaaccactacacccagaagtccctttccctgtctctgggggctggcggcggcggctccggcggaggcgggtctggagtgatccacgtgaccaaggaagtgaaagaggtggccaccctgtcttgcggccacaacgtgtccgtggaagagctggctcagaccagaatctactggcagaaagaaaagaagatggtgctgaccatgatgtccggcgacatgaacatctggcctgagtataagaaccggaccatcttcgacatcaccaacaacctgtccatcgtgatcctggctctgcgcccttccgacgagggcacttacgaatgtgttgtgctgaagtacgagaaggacgccttcaagagagagcacctggctgaagtgaccctgagcgtcaaggccgatttccctacccctagcatctccgacttcgagatccccacctccaatatcagacggatcatctgctccacctctggaggctttccagagcctcatctgtcttggttggagaacggcgaggaactaaacgctatcaacaccaccgtgtcccaggaccctgagaccgagctgtacgctgtctcctctaagctggacttcaacatgacaaccaatcactctttcatgtgcctgatcaagtacggccatctgcgggtgaaccagacattcaacggaggcggaggctccggcggcggcggttctgggggagctcccgctcagctgccctgctctcctacaatccctctgcaggacctgtccctgctgagaagagctggcgtgacctggcagcaccagcctgactccggccctcctgctgctgccccaggccaccctctggcccctggccctcatcctgccgctccttcttcttggggccccagacctcggagatataccgtcctgtctgtgggacctggcggactgcggtccggccggctgcccctgcagcctagagtgcagctggacgaacggggcagacagagaggcgacttctccctgtggctgcggcctgcccggagagccgacgccggcgagtacagagccgccgtgcacctgagagatagagccctgtcctgcagactgcggctgaggctgggacaggcttccatgaccgcctctcccccaggctccctgagagcctccgattgggtgattctgaactgctctttctctagaccagacagacccgcgtctgtccactggttcagaaacagaggccagggcagagtgcctgtgcgggagtccccacaccaccacctggccgagagctttctgttcctgcctcaggtgtcccctatggacagcggcccttggggatgcatcctgacctaccgggacggattcaatgtgtctatcatgtacaacctgaccgtgctcggcctggaaccccctacccctctgacagtgtacgccggcgccggctcccgggtgggcctgccctgccggctgccggctggcgttggcaccagatccttcctgaccgctaagtggacccctcctggcggaggccctgacctgctagtgaccggcgacaacggcgatttcaccctgagactggaggacgtgtcccaggcccaggctggcacctacacatgccacattcatctgcaagagcagcagctgaacgccaccgtaacactggccatcatcactgtgacacccaagagcttcggctctcccggaagcctgggcaagctgctgtgcgaggtgacccctgtgtccggccaggaacggttcgtgtggtcctctctggacaccccctcccagcggtccttctccggtccttggctggaagctcaagaggcccagctcctgtctcagccttggcagtgccagctgtaccagggcgaaaga

SEQ ID NO: 151 - DNA, 3066 bp, synthetic construct
  misc_feature 1..3066: note = AN_Bif_Abs_0051DNA
  source 1..3066: mol_type = other DNA
atgggttggagttgcatcatcctatttctagtggctaccgccaccggcgtccactccgaggtgcagctcctggagtccggcgggggcctggtccagcctggtggatctctgcgattatcctgtgctgcttctggattcaccttctcttcctacgccatgtcttgggtccggcaggcccccggcaagggcctggagtgggtctctggcatcagcggttcaggcggcttcacctattacgccgactccgtgaagggcagattcacaatctccagagacaattctaaaaacaccctgtacctgcagatgaactccctgagagccgaggacacagccgtgtactactgcgccaaaccacctcgtggctacaactacggccccttcgattactggggccagggcacactggtgacagtgagctccgcctctacaaagggcccctccgtgttccctctggctccttgtagtcggtccacctctgagagcaccgctgctttgggctgtctggtgaaggactacttccctgaaccggtgaccgtgtcctggaactccggcgctctgacctccggcgtccacacctttcctgctgtcctgcagtcctccggcctgtactctctgtcctctgtggttactgtgccatcctcttctctgggcaccaaaacctacacctgcaacgtggaccacaagccttctaacaccaaggtggacaagcgggtcgagtccaaatatggacctccttgtcctccctgccctgctcctgagttcctgggcggcccaagtgtcttcctgtttcctcctaagcccaaggacaccctgatgatcagcagaacccctgaagtgacctgtgtggtggtcgacgtgtctcaagaggaccctgaagtgcagttcaactggtacgtggacggcgtggaagtgcacaacgccaagaccaagcccagagaggaacagttcaactctacctaccgggtggtgtccgtgctgaccgttctgcatcaggactggctgaacggcaaagagtacaagtgcaaggtgtctaacaagggcttgccgtcctccatcgagaagaccatctccaaggctaaaggccagcctagagagccacaagtgtacaccctccctccatctcaggaggagatgaccaagaaccaagtgtctctgacctgcctggtgaagggcttctaccctagcgacatcgccgtcgaatgggagtctaatggccagcctgagaacaactacaagaccacaccccctgtgctggactctgacggcagcttcttcctgtactccaggctgacagtggacaagtccagatggcaggagggcaacgtgttttcctgctccgtgatgcacgaggccctgcacaaccactacacccagaaaagcctgagcctgtcactgggcgctgggggcggcggctccggcggcggcggctcgggggtgatccacgtgaccaaggaagtgaaagaagtggccaccctctcttgcggccacaacgtgagtgtggaagagctggctcagacaagaatctactggcagaaggagaagaagatggtgctgaccatgatgtccggcgacatgaacatctggcctgagtataagaaccggaccatcttcgacatcaccaacaacctgtccatcgtgattctggccctgagaccttccgacgagggcacatacgagtgcgtggtgctgaagtacgagaaggacgccttcaagagagaacatctggccgaggtcaccttgagcgtcaaggccgattttcctaccccttccatctccgacttcgagatccccacctccaacatcagacggatcatctgctccactagcggaggctttcctgaacctcatctgtcctggctggaaaacggcgaggaactgaacgccatcaacaccaccgtgtcccaggaccccgaaaccgagctgtacgctgtgtcttccaagctggacttcaacatgacaacaaaccactctttcatgtgcctgatcaagtacggccacctgagagtgaaccagaccttcaactggaataccaccaagcaggaacacttccccgataatggcggcggcggatctggaggaggcggctctggcctgcagcctggcgccgaggtgcccgtggtgtgggcccaagaaggagctcccgcccagctgccttgctctccaaccatccctctgcaggatctgtctctgctgcgccgggctggcgtgacctggcagcaccagcccgactctggccctccagccgctgctcctggccatcctctggcccctggacctcaccccgccgccccttctagttggggacctagacctcgaagatacaccgtgctgtccgtgggccccggaggcctgcggagcgggagactgcctctccaacctagagtgcagctggatgagagaggcagacaacggggcgacttctccctgtggctgcggcctgccagaagagccgatgccggcgagtacagagccgccgtgcatctgcgcgatcgggccctgtcttgccggctgcggctgcgcttaggccaggcttccatgaccgcttctccccctggctccctgcgggcctccgattgggtgatcctgaactgcagcttttctagaccagaccggcctgcttctgtgcactggttccggaaccggggacagggccgggtgcctgtgcgggaatcccctcaccaccacctggccgaatcttttctgttcctgcctcaggtgtctcctatggactccggcccttgggggtgcatcctgacctacagagatggctttaatgtgtctatcatgtacaacctgaccgtgctgggcctggagcctcctacacccctgacagtgtacgccggcgccggctctagagtcggcctgccttgcagactgcctgctggcgtgggcaccagatctttcctgaccgctaagtggacccctcctggcggcggtcctgacctgctggtgaccggcgacaacggcgatttcaccctgagactggaagatgtgtctcaggcccaggccggaacgtatacctgtcacatccacctgcaggagcagcagctgaacgctaccgtgacc

SEQ ID NO: 152 - DNA, 2817 bp, synthetic construct
  misc_feature 1..2817: note = AN_Bif_Abs_0052DNA
  source 1..2817: mol_type = other DNA
atgggttggagttgcatcatcctatttctagtggctaccgccaccggcgtgcattccgaggtgcagctgctggaatctggcggaggcctggtgcagcccggcggctccctgcggctgtcctgtgccgcctctggcttcaccttttcttcctacgccatgtcttgggtacggcaggctcctggaaagggcctggaatgggtctccggcatctctggctcaggtggctttacctactacgccgactccgtgaaagggagattcaccatctctagagacaactccaagaacaccctgtacctgcagatgaacagcctgagagccgaggataccgctgtgtactactgcgccaagccccctagaggctacaactacggccctttcgattactggggtcagggcacactggtgaccgtttcctctgcctccaccaagggaccatcggtgttccctctggctccctgctcccggtctacctctgagtccaccgccgccctgggctgtctcgtgaaggactacttccctgaacctgtgaccgtgtcttggaattctggcgcgctgacctctggcgtgcacaccttccctgccgtgctgcagtcctccggactgtactccctcagcagcgtggtcactgtgccatcctcctctttaggcaccaaaacctacacctgcaacgtggaccacaagcctagcaataccaaagtggacaagagagtggaatccaagtatggccctccttgtcctccatgccccgcccctgagttcctgggaggacccagtgtgttcctgttcccacctaagcccaaggacaccctgatgatcagccggacccctgaagtcacatgcgtggtggtagacgtgtcccaggaggaccctgaggtgcagttcaattggtacgtggatggcgtggaagtgcacaacgctaagaccaagccgcgcgaagagcagttcaactccacatatcgggtggtgtccgtgctgacagtgctacaccaggattggctgaacggcaaggagtacaagtgcaaggtgtctaacaagggcctgccttcctctatcgagaaaaccatcagcaaggcgaagggccaacccagagagcctcaagtgtacacactgcctccttcccaagaggaaatgaccaagaaccaggtgagcctgacctgtctggtcaagggcttctacccttccgatatcgccgtggagtgggagtccaacggccagcctgagaacaactacaaaaccaccccacctgtgctggatagcgacggctctttcttcctgtattctcgcctgaccgtggacaagtccagatggcaagaaggcaacgtgttctcctgctccgtgatgcacgaggctctgcacaatcactacacccagaaaagcctgtccctgagtctgggcgctggcggcggaggctcaggcggcggcggctccggcgtgatccacgtgaccaaagaggtgaaagaggtggccaccctgtcttgtggccacaatgtgtccgtcgaggaactggcacagacccggatctactggcagaaggaaaagaagatggtcctgaccatgatgtccggcgacatgaacatctggcctgagtacaagaacagaaccatcttcgacatcaccaacaacctgtccatcgtgatcctggctctgaggccttctgacgagggcacctacgagtgtgtggtgctgaagtacgagaaggatgccttcaagcgggagcatctggccgaggtgacgctatccgtgaaggccgactttcctaccccttccatcagcgatttcgagatccccacctccaacatcagaagaatcatctgctctacatccggcggcttccctgagcctcacctgtcctggctggaaaatggcgaggaactgaacgccatcaacacaacggtttcccaggacccggagacagagctgtacgctgtgagttccaagctggacttcaacatgaccacaaaccactcctttatgtgcctgatcaagtacggccacctgagagtgaaccagaccttcaactggaacaccaccaagcaggagcacttccccgacaacggcggcggcggatctggcggaggcggctctggactgcagcctggcgccgaagtgcctgtggtgtgggctcaggaaggcgctcctgctcaactgccttgcagccctacaatccctctgcaggacctgtctctcctgagaagagctggcgtcacctggcagcaccagcctgactctggcccccccgctgccgcccctggccatcctctggcccctggaccccaccctgctgctccatccagctggggccccagacctagaagatacaccgtcctatctgtgggcccaggcgggctgcggagcggccggctgcccctgcaacccagagtgcagctggacgagcggggcagacagagaggagacttcagcctgtggctgagacctgctagacgggccgatgccggcgaatacagagctgccgtgcacctgcgggacagagccctgtcttgcagactgcggctccggctgggccaggcctccatgaccgcctcccctcccggttctctgagggcctccgactgggtaattctgaactgctccttctcccgccctgatagacctgcttctgtgcactggttccggaaccggggccagggcagagtgcccgtgcgcgagtctcctcaccaccatctggccgaaagctttctgttcctgcctcaggtctctcctatggactccggcccttggggctgcatcctgacctacagagacggctttaacgtgtccatcatgtacaacctgaccgtcctgggcctggaaccc

SEQ ID NO: 153 - protein, 1065 aa, synthetic construct
  REGION 1..1065: note = AN_Bif_Abs_0053
EVQLLESGGGLVQPGGSLRLSCAASGFTFSSYAMSWVRQAPGKGLEWVSGISGSGGFTYYADSVKGRFTISRDNSKNTLYLQMNSLRAEDTAVYYCAKPPRGYNYGPFDYWGQGTLVTVSSASTKGPSVFPLAPCSRSTSESTAALGCLVKDYFPEPVTVSWNSGALTSGVHTFPAVLQSSGLYSLSSVVTVPSSSLGTKTYTCNVDHKPSNTKVDKRVESKYGPPCPPCPAPEFLGGPSVFLFPPKPKDTLMISRTPEVTCVVVDVSQEDPEVQFNWYVDGVEVHNAKTKPREEQFNSTYRVVSVLTVLHQDWLNGKEYKCKVSNKGLPSSIEKTISKAKGQPREPQVYTLPPSQEEMTKNQVSLTCLVKGFYPSDIAVEWESNGQPENNYKTTPPVLDSDGSFFLYSRLTVDKSRWQEGNVFSCSVMHEALHNHYTQKSLSLSLGAGGGGSGVIHVTKEVKEVATLSCGHNVSVEELAQTRIYWQKEKKMVLTMMSGDMNIWPEYKNRTIFDITNNLSIVILALRPSDEGTYECVVLKYEKDAFKREHLAEVTLSVKADFPTPSISDFEIPTSNIRRIICSTSGGFPEPHLSWLENGEELNAINTTVSQDPETELYAVSSKLDFNMTTNHSFMCLIKYGHLRVNQTFNWNTTKQEHFPDNGGGGSGLQPGAEVPVVWAQEGAPAQLPCSPTIPLQDLSLLRRAGVTWQHQPDSGPPAAAPGHPLAPGPHPAAPSSWGPRPRRYTVLSVGPGGLRSGRLPLQPRVQLDERGRQRGDFSLWLRPARRADAGEYRAAVHLRDRALSCRLRLRLGQASMTASPPGSLRASDWVILNCSFSRPDRPASVHWFRNRGQGRVPVRESPHHHLAESFLFLPQVSPMDSGPWGCILTYRDGFNVSIMYNLTVLGLEPPTPLTVYAGAGSRVGLPCRLPAGVGTRSFLTAKWTPPGGGPDLLVTGDNGDFTLRLEDVSQAQAGTYTCHIHLQEQQLNATVTLAIITVTPKSFGSPGSLGKLLCEVTPVSGQERFVWSSLDTPSQRSFSGPWLEAQEAQLLSQPWQCQLYQGER

SEQ ID NO: 154 - DNA, 3252 bp, synthetic construct
  misc_feature 1..3252: note = AN_Bif_Abs_0053DNA
  source 1..3252: mol_type = other DNA
atgggttggagttgcatcatcctatttctagtggccacagcaaccggcgtgcattctgaggtgcagctgctggagagtggcggcgggcttgtgcagccaggcggatccctgcgcctgtcctgtgctgcttccggctttaccttctcgtcctacgccatgtcctgggtgcggcaggcccctggaaagggcctggagtgggtgtccggcatctccggctcgggcggcttcacttactacgccgattccgtgaagggcagattcaccatcagcagagacaactccaagaacaccctgtacctgcaaatgaactccctgagggccgaggacaccgccgtgtactactgcgccaaacctcctagaggctacaattatggccctttcgactactggggacagggcacattggtgaccgtcagttccgcctccaccaaaggcccttcggtgttccctctggccccttgctctagatcaacctctgagtctaccgctgccctgggctgtctggtgaaggactacttccccgagcctgtgaccgtttcctggaactccggcgctctgacctctggagtgcacaccttccccgctgtgctgcagtccagtggcctgtacagcctgtcttctgtggtgaccgtgccatcgtcctccttgggaacaaagacctacacctgcaacgtggaccacaagccatccaacaccaaggtggacaagagagtcgaatccaagtacggcccaccttgtcctccttgccctgcccctgagttcctgggcggaccttctgtgttcctgttcccaccgaagcctaaagataccctgatgatcagccggacccctgaagtgacctgtgtggttgtggacgtgtcccaggaggaccctgaagtgcagttcaattggtacgtggacggcgtcgaagtgcacaacgctaagacaaaaccccgggaagagcagttcaactccacctatagagtggtgtctgttctgaccgtgctgcaccaggactggctgaacggcaaagaatacaagtgcaaggtgtccaacaagggcctgccttccagcatcgagaagaccatctctaaggccaagggacagcctagagaacctcaggtgtacacactgcctccatcacaggaagagatgaccaagaatcaagtgtccctgacctgcctggtgaagggcttctacccctccgacatcgccgtggaatgggaaagcaacggccagcccgagaacaactacaaaaccacccctcctgtcctggacagcgacggcagcttcttcctgtactctcggctgaccgtggacaagtctagatggcaagagggaaacgtgttctcctgttctgtgatgcacgaggccctgcacaatcactacacccagaaatctctctccctgagcctcggcgccggcggtggcggctctggcgtgatccacgtgaccaaagaagtgaaagaagtggctacactgagctgtggccacaacgtgagcgtggaggagctggcccagacccggatctactggcagaaggagaagaagatggtgctgaccatgatgtctggcgacatgaacatctggcctgagtacaagaacagaaccatcttcgacatcaccaacaacctgtctatcgtgatcctggctctgagacctagcgacgagggcacctacgagtgcgtggtgctcaagtacgaaaaggacgccttcaagagagaacacctggccgaagtgaccctctccgtcaaggccgacttccctacaccttctatctccgacttcgagattcccacctccaacatcagacggatcatctgcagcacctctggcggatttccagagccccacctgtcttggctggagaatggcgaagaactgaacgccatcaacaccacagtgtctcaggatcccgagacagagctgtatgctgtctcctccaagctggactttaacatgaccaccaaccactctttcatgtgcctgatcaagtacggacatctgagggtgaaccagaccttcaactggaacaccaccaagcaggagcacttccctgacaacggcggcggcggcagtggactgcagcctggagccgaggtgcctgtggtgtgggcccaagaaggcgctcccgctcagctgccttgctccccaacaatccctctgcaggatctctccctcctgcggagagccggcgtcacctggcagcaccagcccgattctggccctcctgctgctgctccaggccatcccctggcccctggccctcaccctgctgctccttctagttggggccccagacctagaagatacaccgtgctgtctgttggaccgggaggcctgcggtccggccgactgcctctgcagccacgggtgcaactggacgaacggggcagacagagaggcgacttttctctgtggctgcggcctgccagacgggctgacgctggcgagtacagagctgctgtgcacctgcgtgacagagccctgagctgcagactgcggctgcgcctgggccaggcctccatgaccgcttctcctccaggctccctgcgggcctctgattgggtgatcctgaactgctctttttctagacctgaccggcctgccagtgtgcactggttccggaacagaggccagggcagggtgcccgtgcgggaaagcccccaccaccatctggccgagtcttttctgtttctgcctcaggtgtcccctatggactctggcccttggggctgcatcctgacatacagagacggcttcaacgtttccatcatgtacaatctgaccgtgctgggcctggagccccctacccccttgacagtctatgctggcgccggcagcagagtgggcctgccctgtagactgcctgccggcgtgggcacccggtccttcctgaccgctaagtggacccctcccggaggaggccctgatctgctggtcaccggcgataacggagatttcaccctgagactggaggatgtatcccaggcccaggccggcacctacacttgccacatccacctgcaagaacagcagttgaatgcaaccgtgaccctggccatcatcacagtgacccctaagtccttcggttctcctggctctctgggaaagctgctgtgcgaggtaactcctgtgtccggccaggagcggttcgtgtggtccagtctggatacaccttcccagcggtccttctccggcccttggttggaggcccaggaggcccagctgctgtctcagccttggcagtgccaactgtatcagggcgagaga

SEQ ID NO: 155 - protein, 1085 aa, synthetic construct
  REGION 1..1085: note = AN_Bif_Abs_0054
EVQLLESGGGLVQPGGSLRLSCAASGFTFSSYAMSWVRQAPGKGLEWVSGISGSGGFTYYADSVKGRFTISRDNSKNTLYLQMNSLRAEDTAVYYCAKPPRGYNYGPFDYWGQGTLVTVSSASTKGPSVFPLAPCSRSTSESTAALGCLVKDYFPEPVTVSWNSGALTSGVHTFPAVLQSSGLYSLSSVVTVPSSSLGTKTYTCNVDHKPSNTKVDKRVESKYGPPCPPCPAPEFLGGPSVFLFPPKPKDTLMISRTPEVTCVVVDVSQEDPEVQFNWYVDGVEVHNAKTKPREEQFNSTYRVVSVLTVLHQDWLNGKEYKCKVSNKGLPSSIEKTISKAKGQPREPQVYTLPPSQEEMTKNQVSLTCLVKGFYPSDIAVEWESNGQPENNYKTTPPVLDSDGSFFLYSRLTVDKSRWQEGNVFSCSVMHEALHNHYTQKSLSLSLGAGGGGSGGGGSGGGGSGVIHVTKEVKEVATLSCGHNVSVEELAQTRIYWQKEKKMVLTMMSGDMNIWPEYKNRTIFDITNNLSIVILALRPSDEGTYECVVLKYEKDAFKREHLAEVTLSVKADFPTPSISDFEIPTSNIRRIICSTSGGFPEPHLSWLENGEELNAINTTVSQDPETELYAVSSKLDFNMTTNHSFMCLIKYGHLRVNQTFNWNTTKQEHFPDNGGGGSGGGGSGGGGSGLQPGAEVPVVWAQEGAPAQLPCSPTIPLQDLSLLRRAGVTWQHQPDSGPPAAAPGHPLAPGPHPAAPSSWGPRPRRYTVLSVGPGGLRSGRLPLQPRVQLDERGRQRGDFSLWLRPARRADAGEYRAAVHLRDRALSCRLRLRLGQASMTASPPGSLRASDWVILNCSFSRPDRPASVHWFRNRGQGRVPVRESPHHHLAESFLFLPQVSPMDSGPWGCILTYRDGFNVSIMYNLTVLGLEPPTPLTVYAGAGSRVGLPCRLPAGVGTRSFLTAKWTPPGGGPDLLVTGDNGDFTLRLEDVSQAQAGTYTCHIHLQEQQLNATVTLAIITVTPKSFGSPGSLGKLLCEVTPVSGQERFVWSSLDTPSQRSFSGPWLEAQEAQLLSQPWQCQLYQGER

SEQ ID NO: 156 - DNA, 3315 bp, synthetic construct
  misc_feature 1..3315: note = AN_Bif_Abs_0054DNA
  source 1..3315: mol_type = other DNA
atgggttggagttgcatcatcctatttctagtggccaccgcaacaggagtgcactctgaggtgcagctgctggaatccggaggcggcctggtgcagcctggcggatctttaagactgtcctgtgccgcttccggatttaccttttcttcctacgccatgtcctgggtgcggcaggcccctggcaagggcctggaatgggtgtctggcatctctggctctggcggattcacctattacgccgatagcgtgaagggcagattcaccatctctcgggacaactccaagaacaccctgtatctgcagatgaactcactgcgggccgaggacaccgctgtgtactactgcgctaagcctccccggggctacaactacggccctttcgactactggggccagggcacgctggtgaccgtttcttctgcctccaccaagggaccaagcgtgttcccactggccccttgcagtaggtctacctccgagtctacagccgctctgggctgcctggtgaaagactacttccccgaacctgttaccgtgtcctggaactctggcgctctgacatcaggcgtgcacaccttcccagccgtgctgcagtcctctggcttgtactctttgtcaagcgtggtgaccgtgccttcctcctcgttgggcacaaaaacatacacctgtaacgtggaccacaagccttccaacaccaaggtggacaagagagtggagtcgaaatatggccctccttgtcctccatgccctgcccccgagttcctgggtggcccatcagtgttcctgttcccacctaagcctaaggacactctgatgatctctagaaccccagaggtgacctgcgtggtggtcgacgtcagccaggaagatcctgaagtgcagttcaattggtacgtggacggcgtcgaggtgcataatgccaaaaccaagcccagagaggaacaattcaactctacctaccgggtggtctccgtgctgaccgtgctgcaccaggattggctgaacggcaaggaatacaagtgcaaggtgagcaacaaggggctgccctccagcatcgagaaaaccatctccaaggctaagggacaacccagagaacctcaggtgtacacactgccccccagccaggaggagatgaccaagaatcaggtctccctgacctgcctggtgaagggcttctacccctctgacatcgccgtggagtgggagtccaatggccagcctgaaaacaactacaagaccacacctcctgtgctggactccgacggctccttcttcctgtactcccggctgaccgtggataagtccagatggcaggagggcaacgtgttctcgtgttccgtgatgcacgaggcgctgcacaaccattacacccagaaatctctctctctgtccctgggcgctggcggtggcggcagcggcggcggaggctctggcggtgggggctctggcgtgatccacgtgaccaaagaggtgaaagaggtggctaccctgagttgtggccacaacgtgtccgtcgaggagctggcccagactcggatctactggcagaaggaaaagaagatggtgctgacaatgatgtccggagacatgaacatctggcctgagtacaagaaccggaccatcttcgacattaccaacaacctgtccatcgtgatcctggccctgagaccctccgacgagggaacatacgagtgcgtcgttctgaagtacgaaaaggatgccttcaagcgcgagcatctggccgaggtcaccttgtccgtgaaggctgactttcctacccctagcatttctgacttcgaaatccctacgtctaacatcagaagaatcatctgcagcaccagcggaggcttccctgaacctcacctgtcctggctggagaacggggaagaactgaacgccatcaacaccacggtgtcccaagaccccgaaacagaactgtacgccgtgtccagcaagctggatttcaacatgaccaccaaccactccttcatgtgcctgatcaagtacggccacctgagagtgaaccagaccttcaactggaataccacaaagcaggagcacttccctgataacggcggcggcggctccggaggcggcggctctggaggcggcggcagcggcctgcagcccggcgctgaggtgcccgtggtctgggcccaggaaggcgctccagctcagctcccttgttctccaacaatccctctgcaagatctgtccctgctgagaagagccggcgtgacctggcagcaccagcccgactccggccctccagctgctgcgcctggacatcctctggctcctgggcctcaccctgctgctccttcctcttggggccctagacctagacggtacactgtgctgtccgtcggccctggtggcctcagaagcggacggctgcctctgcagcctcgggtgcagctggacgagagaggcagacagagaggcgactttagcctgtggctgcggcctgcccggagagctgacgccggcgagtaccgggccgctgtgcacttgcgagacagagccttatcttgcagacttcgcctgcggctgggccaagcctccatgaccgcctctccccctggctcactgcgtgccagcgactgggtcatcctgaactgctctttctccagacccgatagacctgcttccgtgcactggttcaggaacagagggcagggaagagtccctgtgagagagtcaccacatcaccacctggctgagtcctttctgtttctgcctcaagtgtcccctatggactctggcccttggggatgcatcctgacctacagagatggcttcaacgtgtctatcatgtacaacctcaccgtgctgggcctggagcctcctacacctctgaccgtgtacgctggcgccggctctcgggtgggcctgccttgcagactgcccgccggcgtcggcacccggtccttcctgaccgccaaatggacccctccaggcggcggccctgacctgctggtgaccggcgacaacggcgatttcaccctgagactggaggacgtgtcccaggctcaggccggcacttatacatgtcacatccacctgcaggagcagcagctgaacgccaccgtgaccctggccatcatcaccgtgacccctaagtcctttggctctcctgggagtctgggcaagctgctgtgcgaggtcacccctgtgtccggccaggaacggttcgtgtggtccagcctggacaccccctcacaaagatctttctccggcccttggctggaggcccaggaagcccagctgctgtctcagccttggcagtgccaactgtaccagggcgagcggtga

SEQ ID NO: 157 - protein, 893 aa, synthetic construct
  REGION 1..893: note = AN_Bif_Abs_0030
EVQLLESGGGLVQPGGSLRLSCAASGFTFSNYAMSWVRQAPGKGLEWVSAISASGHSTYLADSVKGRFTISRDNSKNTLYLQMNSLRAEDTAVYYCAKDREVTMIVVLNGGFDYWGQGTRVTVSSASTKGPSVFPLAPSSKSTSGGTAALGCLVKDYFPEPVTVSWNSGALTSGVHTFPAVLQSSGLYSLSSVVTVPSSSLGTQTYICNVNHKPSNTKVDKRVEPKSCDKTHTCPPCPAPEFEGGPSVFLFPPKPKDTLMISRTPEVTCVVVDVSHEDPEVKFNWYVDGVEVHNAKTKPREEQYNSTYRVVSVLTVLHQDWLNGKEYKCKVSNKALPASIEKTISKAKGQPREPQVYTLPPSREEMTKNQVSLTCLVKGFYPSDIAVEWESNGQPENNYKTTPPVLDSDGSFFLYSKLTVDKSRWQQGNVFSCSVMHEALHNHYTQKSLSLSPGAGGGGSGGGGSGGGGSGGGGSGLQPGAEVPVVWAQEGAPAQLPCSPTIPLQDLSLLRRAGVTWQHQPDSGPPAAAPGHPLAPGPHPAAPSSWGPRPRRYTVLSVGPGGLRSGRLPLQPRVQLDERGRQRGDFSLWLRPARRADAGEYRAAVHLRDRALSCRLRLRLGQASMTASPPGSLRASDWVILNCSFSRPDRPASVHWFRNRGQGRVPVRESPHHHLAESFLFLPQVSPMDSGPWGCILTYRDGFNVSIMYNLTVLGLEPPTPLTVYAGAGSRVGLPCRLPAGVGTRSFLTAKWTPPGGGPDLLVTGDNGDFTLRLEDVSQAQAGTYTCHIHLQEQQLNATVTLAIITVTPKSFGSPGSLGKLLCEVTPVSGQERFVWSSLDTPSQRSFSGPWLEAQEAQLLSQPWQCQLYQGERLLGAAVYFTELSSPGAQRSG

SEQ ID NO: 158 - DNA, 2736 bp, synthetic construct
  misc_feature 1..2736: note = AN_Bif_Abs_0030DNA
  source 1..2736: mol_type = other DNA
atgcacagctcagcactgctctgttgcctggtcctcctgactggggtgagggccgaggtgcagctgctggagagcggggggggactggtgcagccaggaggaagcctgagactgagctgtgccgccagcgggtttacatttagcaactatgccatgagctgggtgagacaggcccccggaaaaggactggagtgggtgagcgccattagcgccagtggacacagcacctacctggctgattccgtgaaggggcggttcacaatctccagagacaacagcaagaacacactgtacctgcagatgaacagcctgagagccgaggacaccgccgtgtactactgcgccaaggacagagaggtgaccatgattgtggtgctgaacggcggattcgactactggggccagggcacccgggtgaccgtgtcaagcgctagcaccaagggcccatcggtcttccccctggcaccctcctccaagagcacctctgggggcacagcggccctgggctgcctggtcaaggactacttccccgaaccggtgacggtgtcgtggaactcaggcgccctgaccagcggcgtgcacaccttcccggctgtcctacagtcctcaggactctactccctcagcagcgtggtgaccgtgccctccagcagcttgggcacccagacctacatctgcaacgtgaatcacaagcccagcaacaccaaggtggacaagagagttgagcccaaatcttgtgacaaaactcacacatgcccaccgtgcccagcacctgaattcgaggggggaccgtcagtcttcctcttccccccaaaacccaaggacaccctcatgatctcccggacccccgaggtcacatgcgtggtggtggacgtgagccacgaagaccctgaggtcaagttcaactggtacgtggacggcgtggaggtgcataatgccaagacaaagccgcgggaggagcagtacaacagcacgtaccgtgtggtcagcgtcctcaccgtcctgcaccaggactggctgaatggcaaggagtacaagtgcaaggtctccaacaaagccctcccagccagcatcgagaaaaccatctccaaagccaaagggcagccccgagaaccacaggtgtacaccctgcccccatcccgggaggagatgaccaagaaccaggtcagcctgacctgcctggtcaaaggcttctatcccagcgacatcgccgtggagtgggagagcaatgggcagccggagaacaactacaagaccacgcctcccgtgctggactccgacggctccttcttcctctacagcaagctcaccgtggacaagagcaggtggcagcaggggaacgtcttctcatgctccgtgatgcatgaggctctgcacaaccactacacgcagaagagcctctccctgtctccgggtgccggaggaggaggaagcggaggaggagggagcggaggagggggaagcggaggcggaggatccggcctgcagcctggcgctgaagtgcccgtggtgtgggcccaggagggcgctcctgctcagctgccttgctcccccaccatccccctgcaggacctgagcctgctgagaagagccggagtgacctggcagcaccagccagattccggacctcccgccgccgctccaggacatcctctggctcccggcccccacccagctgctccttctagctggggaccccggccaagaagatacaccgtgctgagcgtgggacccggcggcctgagatccggaagattgcctttacagccccgcgtgcagctggacgaaagaggaaggcaacgtggtgacttcagcctgtggctgaggcctgccaggagagccgatgccggagagtatagagccgccgtgcacctgagagacagagccctgagttgcagactgagactgagactgggccaggcttccatgaccgcctctccccccggctccctgagagctagcgactgggtgatcctgaactgtagcttctccagacccgacagacccgcctccgtgcactggtttagaaatagaggccagggccgcgtgcccgtgagagagtctccccaccaccacctggccgaaagtttcctgttcctgccccaggtgagccccatggacagcggcccttggggatgcatcctgacctacagagacggattcaatgtgtctatcatgtacaacctgaccgtgctgggcctggagccccctacccctctgaccgtgtacgccggagccggatctcgcgtgggcctgccttgcagactgcccgctggcgtgggcaccagatcctttctgaccgccaaatggaccccccctggcggcggaccagacctgctggtgaccggagacaatggagactttaccctgagactggaggacgtgagccaggctcaggctggcacctacacctgccacatccacctgcaggaacagcagctgaacgccaccgtgaccctggccatcatcaccgtgacccccaaatcctttggcagccccggcagcctgggcaagctgctgtgcgaggtgacccccgtgagcggccaggagagattcgtgtggagtagcctggacaccccctcccagagatccttttccggcccctggctggaggcccaggaggctcagctgctgtctcagccctggcagtgccagctgtatcagggggagaggctgctgggcgccgccgtgtatttcaccgagctgagctcccccggcgcccagagaagcggatga

SEQ ID NO: 159 - protein, 681 aa, synthetic construct
  REGION 1..681: note = AN_Bif_Abs_0002
EVQLVESGGGLVQPGGSLRLSCAASGFTFSRYWMSWVRQAPGKGLEWVANIKQDGSEKYYVDSVKGRFTISRDNAKNSLYLQMNSLRAEDTAVYYCAREGGWFGELAFDYWGQGTLVTVSSASTKGPSVFPLAPSSKSTSGGTAALGCLVKDYFPEPVTVSWNSGALTSGVHTFPAVLQSSGLYSLSSVVTVPSSSLGTQTYICNVNHKPSNTKVDKRVEPKSCDKTHTCPPCPAPEFEGGPSVFLFPPKPKDTLMISRTPEVTCVVVDVSHEDPEVKFNWYVDGVEVHNAKTKPREEQYNSTYRVVSVLTVLHQDWLNGKEYKCKVSNKALPASIEKTISKAKGQPREPQVYTLPPSREEMTKNQVSLTCLVKGFYPSDIAVEWESNGQPENNYKTTPPVLDSDGSFFLYSKLTVDKSRWQQGNVFSCSVMHEALHNHYTQKSLSLSPGAGGGGSGGGGSGGGGSGGGGSGDVDEQLSKSVKDKVLLPCRYNSPHEDESEDRIYWQKHDKVVLSVIAGKLKVWPEYKNRTLYDNTTYSLIILGLVLSDRGTYSCVVQKKERGTYEVKHLALVKLSIKADFSTPNITESGNPSADTKRITCFASGGFPKPRFSWLENGRELPGINTTISQDPESELYTISSQLDFNTTRNHTIKCLIKYGDAHVSEDFTWEKPPEDPPDSK

SEQ ID NO: 160 - protein, 704 aa, synthetic construct
  REGION 1..704: note = AN_Bif_Abs_0003
MEFGLSWLFLVAILKGVQCEVQLLESGGGLVQPGGSLRLSCAASGFTFSNYAMSWVRQAPGKGLEWVSAISASGHSTYLADSVKGRFTISRDNSKNTLYLQMNSLRAEDTAVYYCAKDREVTMIVVLNGGFDYWGQGTRVTVSSASTKGPSVFPLAPSSKSTSGGTAALGCLVKDYFPEPVTVSWNSGALTSGVHTFPAVLQSSGLYSLSSVVTVPSSSLGTQTYICNVNHKPSNTKVDKRVEPKSCDKTHTCPPCPAPEFEGGPSVFLFPPKPKDTLMISRTPEVTCVVVDVSHEDPEVKFNWYVDGVEVHNAKTKPREEQYNSTYRVVSVLTVLHQDWLNGKEYKCKVSNKALPASIEKTISKAKGQPREPQVYTLPPSREEMTKNQVSLTCLVKGFYPSDIAVEWESNGQPENNYKTTPPVLDSDGSFFLYSKLTVDKSRWQQGNVFSCSVMHEALHNHYTQKSLSLSPGAGGGGSGGGGSGGGGSGGGGSGDVDEQLSKSVKDKVLLPCRYNSPHEDESEDRIYWQKHDKVVLSVIAGKLKVWPEYKNRTLYDNTTYSLIILGLVLSDRGTYSCVVQKKERGTYEVKHLALVKLSIKADFSTPNITESGNPSADTKRITCFASGGFPKPRFSWLENGRELPGINTTISQDPESELYTISSQLDFNTTRNHTIKCLIKYGDAHVSEDFTWEKPPEDPPDSK

SEQ ID NO: 161 - protein, 890 aa, synthetic construct
  REGION 1..890: note = AN_Bif_Abs_0004
EVQLVESGGGLVQPGGSLRLSCAASGFTFSRYWMSWVRQAPGKGLEWVANIKQDGSEKYYVDSVKGRFTISRDNAKNSLYLQMNSLRAEDTAVYYCAREGGWFGELAFDYWGQGTLVTVSSASTKGPSVFPLAPSSKSTSGGTAALGCLVKDYFPEPVTVSWNSGALTSGVHTFPAVLQSSGLYSLSSVVTVPSSSLGTQTYICNVNHKPSNTKVDKRVEPKSCDKTHTCPPCPAPEFEGGPSVFLFPPKPKDTLMISRTPEVTCVVVDVSHEDPEVKFNWYVDGVEVHNAKTKPREEQYNSTYRVVSVLTVLHQDWLNGKEYKCKVSNKALPASIEKTISKAKGQPREPQVYTLPPSREEMTKNQVSLTCLVKGFYPSDIAVEWESNGQPENNYKTTPPVLDSDGSFFLYSKLTVDKSRWQQGNVFSCSVMHEALHNHYTQKSLSLSPGAGGGGSGGGGSGGGGSGGGGSGPGKELPVVWAQEGAPVHLPCSLKSPNLDPNFLRRGGVIWQHQPDSGQPTPIPALDLHQGMPSPRQPAPGRYTVLSVAPGGLRSGRQPLHPHVQLEERGLQRGDFSLWLRPALRTDAGEYHATVRLPNRALSCSLRLRVGQASMIASPSGVLKLSDWVLLNCSFSRPDRPVSVHWFQGQNRVPVYNSPRHFLAETFLLLPQVSPLDSGTWGCVLTYRDGFNVSITYNLKVLGLEPVAPLTVYAAEGSRVELPCHLPPGVGTPSLLIAKWTPPGGGPELPVAGKSGNFTLHLEAVGLAQAGTYTCSIHLQGQQLNATVTLAVITVTPKSFGLPGSRGKLLCEVTPASGKERFVWRPLNNLSRSCPGPVLEIQEARLLAERWQCQLYEGQRLLGATVYAAESSSGAHSARRISGDLKGGHL

SEQ ID NO: 162 - protein, 214 aa, synthetic construct
  REGION 1..214: note = JS003
DIVMTQSPDSLAVSLGERATINCKASQNVDTSVAWFQQKPGQPPKALIYSASFRYSGVPDRFSGSGSGTDFTLTISSLQAEDVAVYFCQQYYGYPFTFGQGTKLEIKRTVAAPSVFIFPPSDEQLKSGTASVVCLLNNFYPREAKVQWKVDNALQSGNSQESVTEQDSKDSTYSLSSTLTLSKADYEKHKVYACEVTHQGLSSPVTKSFNRGEC

SEQ ID NO: 163 - protein, 215 aa, synthetic construct
  REGION 1..215: note = Durvalumab(MEDI4736)
EIVLTQSPGTLSLSPGERATLSCRASQRVSSSYLAWYQQKPGQAPRLLIYDASSRATGIPDRFSGSGSGTDFTLTISRLEPEDFAVYYCQQYGSLPWTFGQGTKVEIKRTVAAPSVFIFPPSDEQLKSGTASVVCLLNNFYPREAKVQWKVDNALQSGNSQESVTEQDSKDSTYSLSSTLTLSKADYEKHKVYACEVTHQGLSSPVTKSFNRGEC

SEQ ID NO: 164 - protein, 214 aa, synthetic construct
  REGION 1..214: note = atezolizumabMPDL3280A
DIQMTQSPSSLSASVGDRVTITCRASQDVSTAVAWYQQKPGKAPKLLIYSASFLYSGVPSRFSGSGSGTDFTLTISSLQPEDFATYYCQQYLYHPATFGQGTKVEIKRTVAAPSVFIFPPSDEQLKSGTASVVCLLNNFYPREAKVQWKVDNALQSGNSQESVTEQDSKDSTYSLSSTLTLSKADYEKHKVYACEVTHQGLSSPVTKSFNRGEC

SEQ ID NO: 165 - protein, 216 aa, synthetic construct
  REGION 1..216: note = Avelumab(MSB0010718C)
QSALTQPASVSGSPGQSITISCTGTSSDVGGYNYVSWYQQHPGKAPKLMIYDVSNRPSGVSNRFSGSKSGNTASLTISGLQAEDEADYYCSSYTSSSTRVFGTGTKVTVLGQPKANPTVTLFPPSSEELQANKATLVCLISDFYPGAVTVAWKADGSPVKAGVETTKPSKQSNNKYAASSYLSLTPEQWKSHRSYSCQVTHEGSTVEKTVAPTECS

SEQ ID NO: 166 - protein, 218 aa, synthetic construct
  REGION 1..218: note = Permbrolizumab (MK-3475)
EIVLTQSPATLSLSPGERATLSCRASKGVSTSGYSYLHWYQQKPGQAPRLLIYLASYLESGVPARFSGSGSGTDFTLTISSLEPEDFAVYYCQHSRDLPLTFGGGTKVEIKRTVAAPSVFIFPPSDEQLKSGTASVVCLLNNFYPREAKVQWKVDNALQSGNSQESVTEQDSKDSTYSLSSTLTLSKADYEKHKVYACEVTHQGLSSPVTKSFNRGEC

SEQ ID NO: 167 - protein, 214 aa, synthetic construct
  REGION 1..214: note = Nivolumab(BMS-936558)
EIVLTQSPATLSLSPGERATLSCRASQSVSSYLAWYQQKPGQAPRLLIYDASNRATGIPARFSGSGSGTDFTLTISSLEPEDFAVYYCQQSSNWPRTFGQGTKVEIKRTVAAPSVFIFPPSDEQLKSGTASVVCLLNNFYPREAKVQWKVDNALQSGNSQESVTEQDSKDSTYSLSSTLTLSKADYEKHKVYACEVTHQGLSSPVTKSFNRGEC

SEQ ID NO: 168 - protein, 959 aa, synthetic construct
  REGION 1..959: note = AN_Bif_Abs_0055
MGWSCIILFLVATATGVHSLQPGAEVPVVWAQEGAPAQLPCSPTIPLQDLSLLRRAGVTWQHQPDSGPPAAAPGHPLAPGPHPAAPSSWGPRPRRYTVLSVGPGGLRSGRLPLQPRVQLDERGRQRGDFSLWLRPARRADAGEYRAAVHLRDRALSCRLRLRLGQASMTASPPGSLRASDWVILNCSFSRPDRPASVHWFRNRGQGRVPVRESPHHHLAESFLFLPQVSPMDSGPWGCILTYRDGFNVSIMYNLTVLGLEPGGGGSGGGGSGGGGSGGGGSGEVQLLESGGGLVQPGGSLRLSCAASGFTFSSYAMSWVRQAPGKGLEWVSGISGSGGFTYYADSVKGRFTISRDNSKNTLYLQMNSLRAEDTAVYYCAKPPRGYNYGPFDYWGQGTLVTVSSASTKGPSVFPLAPCSRSTSESTAALGCLVKDYFPEPVTVSWNSGALTSGVHTFPAVLQSSGLYSLSSVVTVPSSSLGTKTYTCNVDHKPSNTKVDKRVESKYGPPCPPCPAPEFLGGPSVFLFPPKPKDTLMISRTPEVTCVVVDVSQEDPEVQFNWYVDGVEVHNAKTKPREEQFNSTYRVVSVLTVLHQDWLNGKEYKCKVSNKGLPSSIEKTISKAKGQPREPQVYTLPPSQEEMTKNQVSLTCLVKGFYPSDIAVEWESNGQPENNYKTTPPVLDSDGSFFLYSRLTVDKSRWQEGNVFSCSVMHEALHNHYTQKSLSLSLGAGGGGSGGGGSGGGGSGGGGSGVIHVTKEVKEVATLSCGHNVSVEELAQTRIYWQKEKKMVLTMMSGDMNIWPEYKNRTIFDITNNLSIVILALRPSDEGTYECVVLKYEKDAFKREHLAEVTLSVKADFPTPSISDFEIPTSNIRRIICSTSGGFPEPHLSWLENGEELNAINTTVSQDPETELYAVSSKLDFNMTTNHSFMCLIKYGHLRVNQTFNWNTTKQEHFPDN

SEQ ID NO: 169 - DNA, 2877 bp, synthetic construct
  misc_feature 1..2877: note = AN_Bif_Abs_0055DNA
  source 1..2877: mol_type = other DNA
atgggttggagttgcatcatcctatttctagtggctacagctaccggcgtacactctctgcagcctggagccgaggttcccgtggtctgggcccaggagggcgctcctgcccaactgccttgctcgcccaccatccctctgcaagacctgtctctgctgcggcgggctggcgtgacctggcagcaccagcctgattctggcccccctgctgctgctcccggccatcctctggctcctggccctcaccctgcagctccttcctcctggggccctcggcctagaagatacaccgtgctgtccgtgggcccaggcggcctgcggagcggccggctgcctctgcagcctagagtgcagctggatgagcggggaagacagagaggcgacttctctctgtggctgagacctgccagaagagccgacgctggcgagtaccgggctgccgtgcacctgcgggacagagccctctcctgcagactgagactgagactgggccaagcctccatgaccgcttcccctcctggctccctcagagcctccgattgggtcatcctgaactgctccttctcccgccccgatcggcccgcttctgtgcactggttccggaaccgaggccagggaagagtgcctgtgcgggagtcccctcaccaccatctggccgagtccttcctgtttctgccccaggtgtctcctatggactctggcccttggggctgcatcctgacctacagagatggattcaatgtgtctatcatgtacaacctgacagtgctgggcctggaacctggtggcggcggctctggcggaggcggaagtggcggcggtggatcgggcggtggcggctctggcgaggtgcagctgctggaatctggcggcggcctggtgcagcctggcggctccctgaggctgtcctgtgctgcctctggctttaccttctcttcctacgccatgagctgggtgcggcaggctcccggcaagggcctggagtgggtgtccggaatctccggctccggcggcttcacctactacgccgatagcgtgaagggcagattcaccatctctagagacaattccaagaacacactgtacctgcagatgaacagcctgcgagccgaggatactgccgtatactactgcgccaagcctcccagaggctacaactacggccccttcgactactggggacagggcaccctggtgactgtgtcttctgccagcaccaaaggcccttctgtgttccctttagctccttgttctagatccacatctgagtctaccgccgctctgggctgtcttgtgaaggattacttcccagagcctgtgaccgtgtcttggaactctggcgctttgacctctggcgtgcacaccttccctgccgtactgcagtcctctggcctgtacagcctgtccagcgtggtgacagttccctcttcctctctgggcaccaaaacctacacctgcaacgtggaccacaagcccagcaacaccaaggtggacaagagagtggaatccaaatacggcccaccttgtcctccttgccctgctcccgagttcctcggcgggccttccgtgttcctgttcccgcctaagcctaaggacactctgatgatctccagaacccctgaagtgacctgtgttgtggtcgacgtgtcccaagaggaccccgaagtgcagttcaactggtacgtggacggcgtggaggtgcacaatgctaagaccaagcctagagaagagcagttcaactccacctaccgggtggtgtccgtgctgaccgtgctgcaccaggactggctgaacggcaaggagtacaagtgcaaggtctccaacaagggactgccttctagcatcgagaagacaatttccaaggccaagggccagcctcgggaaccacaagtgtatacgctgcctcctagccaggaagagatgacaaagaatcaggtctccctgacctgtctggtcaagggcttctaccccagcgatatcgccgtggaatgggagtccaacggacagccagagaataactacaagaccacaccacccgttctggactccgacggcagcttctttctgtactccagactgaccgtggacaagagccggtggcaggaagggaatgtgttctcctgctctgtgatgcacgaggccctgcacaaccactacacccagaagagcctgagcctgtctctgggcgccggcggcggcggctctggcggcggcggctcgggcggcggaggatctgggggtggcggctctggcgtgatccacgtgacaaaagaggtgaaagaagtggccaccctgtcctgcggccacaacgtgtccgtggaggagctggcccagaccagaatctactggcagaaagaaaagaagatggtgctgaccatgatgtctggcgacatgaacatctggcccgagtacaagaaccggaccatcttcgacatcaccaacaacctctctatcgtgatcctggccctgagaccttctgacgaaggcacctatgagtgcgtggtgctgaagtacgagaaggacgccttcaagcgggagcatctggccgaggtgaccctgtccgtgaaggccgactttccaaccccttccatctctgatttcgagatccctacctccaacatccggcggatcatctgctccacctccggcggttttcctgagcctcatctatcttggctggagaacggcgaagaactgaacgccatcaacaccacagtgtcccaggacccagaaaccgagctgtacgcagtgtcctccaagctggacttcaacatgaccaccaatcattccttcatgtgcctgatcaagtatggacacctgagagtgaaccagacctttaactggaacaccactaagcaggaacacttccctgacaac

SEQ ID NO: 170 - protein, 1037 aa, synthetic construct
  REGION 1..1037: note = AN_Bif_Abs_0056
MGWSCIILFLVATATGVHSLQPGAEVPVVWAQEGAPAQLPCSPTIPLQDLSLLRRAGVTWQHQPDSGPPAAAPGHPLAPGPHPAAPSSWGPRPRRYTVLSVGPGGLRSGRLPLQPRVQLDERGRQRGDFSLWLRPARRADAGEYRAAVHLRDRALSCRLRLRLGQASMTASPPGSLRASDWVILNCSFSRPDRPASVHWFRNRGQGRVPVRESPHHHLAESFLFLPQVSPMDSGPWGCILTYRDGFNVSIMYNLTVLGLEPPTPLTVYAGAGSRVGLPCRLPAGVGTRSFLTAKWTPPGGGPDLLVTGDNGDFTLRLEDVSQAQAGTYTCHIHLQEQQLNGGGGSGGGGSGGGGSGGGSGEVQLLESGGGLVQPGGSLRLSCAASGFTFSSYAMSWVRQAPGKGLEWVSGISGSGGFTYYADSVKGRFTISRDNSKNTLYLQMNSLRAEDTAVYYCAKPPRGYNYGPFDYWGQGTLVTVSSASTKGPSVFPLAPCSRSTSESTAALGCLVKDYFPEPVTVSWNSGALTSGVHTFPAVLQSSGLYSLSSVVTVPSSSLGTKTYTCNVDHKPSNTKVDKRVESKYGPPCPPCPAPEFLGGPSVFLFPPKPKDTLMISRTPEVTCVVVDVSQEDPEVQFNWYVDGVEVHNAKTKPREEQFNSTYRVVSVLTVLHQDWLNGKEYKCKVSNKGLPSSIEKTISKAKGQPREPQVYTLPPSQEEMTKNQVSLTCLVKGFYPSDIAVEWESNGQPENNYKTTPPVLDSDGSFFLYSRLTVDKSRWQEGNVFSCSVMHEALHNHYTQKSLSLSLGAGGGGSGGGGSGGGGSGGGGSGVIHVTKEVKEVATLSCGHNVSVEELAQTRIYWQKEKKMVLTMMSGDMNIWPEYKNRTIFDITNNLSIVILALRPSDEGTYECVVLKYEKDAFKREHLAEVTLSVKADFPTPSISDFEIPTSNIRRIICSTSGGFPEPHLSWLENGEELNAINTTVSQDPETELYAVSSKLDFNMTTNHSFMCLIKYGHLRVNQTFNWNTTKQEHFPDN

SEQ ID NO: 171 - DNA, 3111 bp, synthetic construct
  misc_feature 1..3111: note = AN_Bif_Abs_0056DNA
  source 1..3111: mol_type = other DNA
atgggttggagttgcatcatcctatttctagtggccaccgccaccggcgttcactctctccagcctggcgccgaggtgcctgtggtgtgggctcaggaaggagcaccggcccagctgccttgctcccctaccatccccctgcaggacctgagcctgctgagaagagccggcgtgacctggcagcaccagcctgactccggccctcctgctgctgcccctggccatcctctggcccctggccctcaccctgccgccccctccagctggggccctcgtcctagaagatacaccgtgctgtcagtaggccccggaggcctgagatccggaagactgcctctgcagcccagggtgcagctggacgagagaggccggcagagaggcgacttctccctgtggctgcgccccgccagaagggccgatgcaggagaatacagagctgctgtgcatctgagagaccgggccctgtcctgccggctgcggctaagattaggtcaagcctcgatgacagcctcccctcctggctccttgagagcatccgattgggtgatcctgaactgctcgttcagccggcccgacagacctgcctctgtgcactggttccggaaccggggacagggcagagtcccagtgagagagtccccacatcaccacctggctgaatcctttctctttctgcctcaggtgtctcctatggactccggcccttggggatgcatcctgacctatagagatggcttcaacgtttccatcatgtacaacctgaccgtcctgggccttgaaccgcccaccccgctgaccgtgtatgcgggcgctggctctagagtgggcctgccctgcagactgcctgctggcgtgggcacaagatcttttctgacagctaagtggaccccccctggcggaggacctgatctgctcgtcaccggagataacggcgacttcaccctgcggctggaagatgtttctcaggcccaggccggcacttatacctgtcacatccatctgcaagaacagcagctgaatggcggcggcgggagcggcggaggcggctctggcggcggcggctcaggcggcggcagtggcgaggtgcagctgctggagtccggcggcggcctggtgcagcctggaggaagcctgagactgtcctgcgccgcctccggatttaccttctcctcctacgccatgtcttgggtcagacaagctccaggcaagggcctggaatgggtttctggcatctccggctccggcggtttcacctactacgctgactccgtgaaaggcaggttcaccatcagccgggacaactccaagaataccctgtacctgcagatgaactccctccgggccgaggacaccgccgtgtactactgcgccaagcctcctcggggctacaactacggccctttcgactactggggccagggtaccctcgtgacggtaagttctgcctctaccaagggcccctccgtgtttcctctggccccatgttctcggtccacaagcgagtccaccgccgccctgggctgcctggtgaaggactacttccccgagcctgtgaccgtgtcctggaactctggtgctctaacctctggcgtgcacacctttccagctgtgctgcagtcctcgggtctgtacagcctgtcttctgtcgtgactgtgccctcctcctctctgggcaccaagacctacacctgcaacgtggaccacaagccttccaacaccaaagtcgataagcgggtggaatccaagtacggcccaccttgtcctccctgccccgctcctgagttcctgggcggcccttccgtgttcctgtttcctcctaagcccaaggatacactgatgatctcacggacccctgaggtgacctgtgtggtcgtggacgtgtcccaggaggaccccgaagtgcagttcaactggtacgtggatggcgtggaagtgcacaatgctaagaccaagccacgagaagagcagttcaattctacctacagagtggtgtctgtgctgaccgtgctgcaccaggactggctgaatggcaaggagtacaagtgcaaggtgagcaacaagggcctgccttcctctatcgagaaaacaatctccaaggccaagggccagcccagagaacctcaagtgtacaccctgcccccttcacaagaggagatgaccaagaaccaggtgagcctgacctgtctcgtgaaaggcttctaccctagcgacatcgccgtagagtgggagtccaatggccaacctgagaacaactacaagaccacaccacctgtgctggactctgacggcagcttcttcctgtactctcggctgacagtggacaagtccagatggcaggaaggcaacgtgttctcctgctctgtgatgcacgaggccctgcacaaccactacacacagaagtccctgtccctctccctgggcgccggcggcggaggctctggcggcgggggctccggcggcggcggctccggcgggggcggaagcggcgtgatccacgtgaccaaagaggtgaaagaagtggccacactgtcttgtggccacaacgtgtccgtggaggagctggctcagaccagaatctactggcagaaagagaagaagatggtgctgaccatgatgtccggcgacatgaacatctggcctgagtacaagaacagaacgatcttcgacatcaccaacaacctgtctatcgtgattctggctctgcgtccttccgacgagggcacctacgagtgcgtggtgctgaagtacgagaaggacgccttcaagcgggagcacctggctgaggtgaccctgtctgtgaaggccgacttccctaccccttccatctctgacttcgagatccctactagcaacatcagacggatcatctgctccacctccggcggcttccccgagccacatctgagctggctggaaaacggcgaggaactgaacgccatcaacaccaccgtgagccaggatcctgaaaccgagctgtacgctgtctcttccaagctggacttcaacatgaccaccaaccactccttcatgtgcctgatcaagtacggccacctgcgggtgaaccagaccttcaactggaacaccaccaagcaggaacacttccccgacaac

SEQ ID NO: 172 - protein, 1121 aa, synthetic construct
  REGION 1..1121: note = AN_Bif_Abs_0060
MGWSCIILFLVATATGVHSLQPGAEVPVVWAQEGAPAQLPCSPTIPLQDLSLLRRAGVTWQHQPDSGPPAAAPGHPLAPGPHPAAPSSWGPRPRRYTVLSVGPGGLRSGRLPLQPRVQLDERGRQRGDFSLWLRPARRADAGEYRAAVHLRDRALSCRLRLRLGQASMTASPPGSLRASDWVILNCSFSRPDRPASVHWFRNRGQGRVPVRESPHHHLAESFLFLPQVSPMDSGPWGCILTYRDGFNVSIMYNLTVLGLEPPTPLTVYAGAGSRVGLPCRLPAGVGTRSFLTAKWTPPGGGPDLLVTGDNGDFTLRLEDVSQAQAGTYTCHIHLQEQQLNATVTLAIITVTPKSFGSPGSLGKLLCEVTPVSGQERFVWSSLDTPSQRSFSGPWLEAQEAQLLSQPWQCQLYQGERLLGAAVYFTELSSPGGGGSGGGSGGGSGEVQLLESGGGLVQPGGSLRLSCAASGFTFSSYAMSWVRQAPGKGLEWVSGISGSGGFTYYADSVKGRFTISRDNSKNTLYLQMNSLRAEDTAVYYCAKPPRGYNYGPFDYWGQGTLVTVSSASTKGPSVFPLAPCSRSTSESTAALGCLVKDYFPEPVTVSWNSGALTSGVHTFPAVLQSSGLYSLSSVVTVPSSSLGTKTYTCNVDHKPSNTKVDKRVESKYGPPCPPCPAPEFLGGPSVFLFPPKPKDTLMISRTPEVTCVVVDVSQEDPEVQFNWYVDGVEVHNAKTKPREEQFNSTYRVVSVLTVLHQDWLNGKEYKCKVSNKGLPSSIEKTISKAKGQPREPQVYTLPPSQEEMTKNQVSLTCLVKGFYPSDIAVEWESNGQPENNYKTTPPVLDSDGSFFLYSRLTVDKSRWQEGNVFSCSVMHEALHNHYTQKSLSLSLGAGGGGSGGGGSGGGGSGGGGSGVIHVTKEVKEVATLSCGHNVSVEELAQTRIYWQKEKKMVLTMMSGDMNIWPEYKNRTIFDITNNLSIVILALRPSDEGTYECVVLKYEKDAFKREHLAEVTLSVKADFPTPSISDFEIPTSNIRRIICSTSGGFPEPHLSWLENGEELNAINTTVSQDPETELYAVSSKLDFNMTTNHSFMCLIKYGHLRVNQTFNWNTTKQEHFPDN

SEQ ID NO: 173 - DNA, 3363 bp, synthetic construct
  misc_feature 1..3363: note = AN_Bif_Abs_0060DNA
  source 1..3363: mol_type = other DNA
atgggttggagttgcatcatcctatttctagtggctaccgccaccggcgtgcactccctgcagccaggtgcagaagtgcccgtggtgtgggcccaggagggcgcccctgcccagctgccatgcagccctaccatccctctgcaggacctgtcccttctgagaagagctggcgtgacctggcagcaccagcctgattccgggccacccgctgccgctcctggccatcccctggctcctgggcctcatcctgccgcgccctctagttggggacccagacctcggagatacacagtgttgtctgtgggccctggcggtctgagatccggccggctgcctctgcagcctagggtgcagctggatgaaagaggccggcagagaggagacttcagcctgtggctgagacctgccagaagagctgacgccggcgagtatagagccgccgtgcatctgcgggacagagctctgtcctgtagactgcggctgaggctgggacaggcctccatgaccgcttctcctcctggaagcctgagagccagcgactgggtgatcctgaactgctctttctctcgccctgaccggcctgcttccgtgcactggttccggaaccggggccagggcagagtgcctgtgcgggaatctccacaccaccacctggccgagtcattcctgttcctgcctcaggtgtctccgatggactccggcccttggggctgcatcctgacctacagagatggcttcaacgtgtctatcatgtacaatctgaccgtgctcggactggagcctcccacccctctgaccgtgtacgccggcgctggctccagagtgggcctgccttgcagactgcctgccggtgtcggcacccggtctttcctgacagccaagtggacccctccaggcggcggccccgacctgctggttacaggggacaacggagacttcacactgagactggaggacgtgtctcaggcccaggctggcacctacacatgccacatccacctgcaagagcagcagctgaatgctaccgtgacactggccatcatcaccgtcacacctaagagcttcggctcccccggctccctcggcaagctgctgtgcgaggtgacacccgtctccggacaggagagattcgtgtggtcctccctggacacaccttcccagcggtctttttctggaccttggctggaagcccaggaagcccaactgctgtctcagccttggcagtgccagctgtaccagggcgaaagactgctgggcgctgctgtgtacttcaccgagctctcatctcctggcggaggcggctccggcggcggcagtggaggcggaagtggcgaagtgcagctgctggagtctggcggcggcttggtgcagcctggcggcagcctgagactgtcctgcgcagcttccggctttaccttctcttcctatgccatgtcctgggtccggcaggccccgggcaagggcctggaatgggtgtctggcatctccggctccggcggctttacctactacgccgattctgtcaagggcagattcacaatttccagagacaactcgaagaataccctgtacctgcagatgaactccctccgggccgaggacaccgccgtatactactgcgccaaacctcctagaggctacaactacggccctttcgactactggggccaaggcaccctggtcaccgtgtcttctgcctccaccaaaggcccctccgtgttcccactggccccttgtagccggtctacctccgagtccaccgctgccctgggctgtctggtgaaggactacttccccgagcctgtgaccgtgtcttggaacagtggcgctctgacgtcaggagtgcacaccttccccgctgtgctgcagtccagtggactctacagcctgtccagcgtggtgaccgtgccttcttctagcctgggcaccaaaacctatacctgcaatgtggaccacaagccttctaataccaaggtggacaagcgggtggaatccaagtacggccctccctgtcctccttgtccagctcctgagttcctgggcggcccttccgtgtttctgtttcctcctaagcccaaggataccctgatgatctctagaacccctgaagtgacctgtgtggtggtggatgtgtctcaagaggatcctgaggtgcagttcaactggtacgtggacggcgtggaagtacacaacgccaagaccaaaccaagggaggaacaatttaacagcacctaccgggtggtgtctgttctgaccgtcctgcatcaggattggctgaacggcaaggaatataagtgcaaggtgagcaacaagggcctgccctcctccatcgagaaaaccatctccaaggccaagggccagcctagagagcctcaggtgtacactctccctccttctcaggaggagatgacaaagaaccaggtctccctcacctgcctggtgaagggcttctacccctcggacatcgccgtggagtgggagtccaacggacagcctgagaacaactacaagaccacccctccagttctcgacagcgatggctcttttttcctgtactctaggttaactgtggacaagtcgagatggcaagaaggcaacgtgttctcttgttctgtgatgcacgaggctttgcacaaccactacacccagaagtccctgagcctgtctctgggcgctggcggaggcggatccggcggcggcggctcgggaggcggcggctccggcggcggcggctcaggcgtcatccacgtgactaaagaagtgaaggaggtggctaccctgtcttgcggccacaacgtgtccgtcgaggaactggctcagacccgcatctactggcagaaagaaaagaagatggtgctgacaatgatgtctggcgacatgaacatttggcctgagtacaagaatcggaccatcttcgatatcaccaacaacctgtccatcgtgatcctggccctgagaccttccgatgagggcacatacgagtgcgtggttctgaagtacgagaaggacgccttcaagagagaacatctggccgaggtgaccctcagcgtgaaggcagattttccaacccccagtatctctgacttcgagatccctacctccaacatccggagaatcatctgctccacttctggcggcttccccgaacctcacctgtcctggctggaaaacggcgaagagctgaacgccatcaacaccacagtttcgcaggaccccgaaaccgagctgtacgccgtgtcctccaagctggacttcaacatgaccaccaaccacagcttcatgtgcctgatcaagtacggccacctgagagtgaaccagaccttcaactggaacaccaccaagcaagagcacttccctgacaac

SEQ ID NO: 174 - protein, 1118 aa, synthetic construct
  REGION 1..1118: note = AN_Bif_Abs_0061
MGWSCIILFLVATATGVHSLQPGAEVPVVWAQEGAPAQLPCSPTIPLQDLSLLRRAGVTWQHQPDSGPPAAAPGHPLAPGPHPAAPSSWGPRPRRYTVLSVGPGGLRSGRLPLQPRVQLDERGRQRGDFSLWLRPARRADAGEYRAAVHLRDRALSCRLRLRLGQASMTASPPGSLRASDWVILNCSFSRPDRPASVHWFRNRGQGRVPVRESPHHHLAESFLFLPQVSPMDSGPWGCILTYRDGFNVSIMYNLTVLGLEPPTPLTVYAGAGSRVGLPCRLPAGVGTRSFLTAKWTPPGGGPDLLVTGDNGDFTLRLEDVSQAQAGTYTCHIHLQEQQLNATVTLAIITVTPKSFGSPGSLGKLLCEVTPVSGQERFVWSSLDTPSQRSFSGPWLEAQEAQLLSQPWQCQLYQGERLLGAAVYFTELSSPGGGGSGGGGSGEVQLLESGGGLVQPGGSLRLSCAASGFTFSSYAMSWVRQAPGKGLEWVSGISGSGGFTYYADSVKGRFTISRDNSKNTLYLQMNSLRAEDTAVYYCAKPPRGYNYGPFDYWGQGTLVTVSSASTKGPSVFPLAPCSRSTSESTAALGCLVKDYFPEPVTVSWNSGALTSGVHTFPAVLQSSGLYSLSSVVTVPSSSLGTKTYTCNVDHKPSNTKVDKRVESKYGPPCPPCPAPEFLGGPSVFLFPPKPKDTLMISRTPEVTCVVVDVSQEDPEVQFNWYVDGVEVHNAKTKPREEQFNSTYRVVSVLTVLHQDWLNGKEYKCKVSNKGLPSSIEKTISKAKGQPREPQVYTLPPSQEEMTKNQVSLTCLVKGFYPSDIAVEWESNGQPENNYKTTPPVLDSDGSFFLYSRLTVDKSRWQEGNVFSCSVMHEALHNHYTQKSLSLSLGAGGGGSGGGGSGGGGSGGGGSGVIHVTKEVKEVATLSCGHNVSVEELAQTRIYWQKEKKMVLTMMSGDMNIWPEYKNRTIFDITNNLSIVILALRPSDEGTYECVVLKYEKDAFKREHLAEVTLSVKADFPTPSISDFEIPTSNIRRIICSTSGGFPEPHLSWLENGEELNAINTTVSQDPETELYAVSSKLDFNMTTNHSFMCLIKYGHLRVNQTFNWNTTKQEHFPDN

SEQ ID NO: 175 - DNA, 3354 bp, synthetic construct
  misc_feature 1..3354: note = AN_Bif_Abs_0061DNA
  source 1..3354: mol_type = other DNA
atgggttggagttgcatcatcctatttctagtggccaccgccacaggcgtgcactccctgcaaccaggcgctgaagtgcccgtcgtgtgggctcaagaaggcgcccctgcccagcttccttgttctcccaccatccccctccaggacctgtccctgctgcggagggccggcgtcacctggcagcaccagcccgattccggccctcctgctgccgcccctggccaccctctggcccctggacctcatcctgccgctcctagttcctggggccccagacctcggcggtacaccgtgctgtctgtgggacccggcggtctgagatccggccggctgcccctgcagcctagagtgcagctggatgaaagaggcagacagagaggcgacttctccctgtggctgcgcccggccagaagagccgacgccggcgagtaccgggccgccgtccacctgagagacagagccctgtcttgtagactgagactgcggctgggccaggcctccatgaccgcttcccctcccggctccctccgggcctctgactgggtgatcctgaactgcagcttctccagacctgaccggcctgcaagtgtgcactggttcagaaaccggggccagggcagagtgcctgtgcgggaaagccctcaccaccatctggctgagtcttttctgtttttaccccaagtgtcccctatggactctggcccttggggctgcatcctgacctacagagatggcttcaatgtgagcatcatgtacaacctgaccgtgctcggcctggagccacctacacctctgactgtctacgctggcgctggctccagagtgggcctgccttgccggctgcctgccggcgtgggcacaagatccttcctgacagctaagtggaccccacctggcggaggacctgatctgctggtgaccggcgataacggcgacttcaccctgagactggaggacgtgtctcaggcccaggctggcacctacacctgtcacatccacctgcaggagcagcagctgaacgctacagtgactctggccattatcaccgtgacccctaagagcttcggctctcctggctctctgggcaagctgctgtgcgaggtaacccctgtttcaggccaggagcggttcgtgtggtcctctctggacaccccctcccagcggtccttctccgggccttggctggaagctcaagaggctcagctgctgagccaaccttggcagtgccagctctaccagggggagagactgctgggcgccgctgtgtacttcaccgagctgtcttcccctggaggaggtggatctggcggcggcggctccggggaggtgcagctgttggagtccggaggcggactggtgcagcctggcggctctctgagactgtcctgcgccgcaagcggattcaccttttcctcctacgccatgtcttgggtgcgccaggctcctggcaaagggctggaatgggttagcggcatctctggcagcggcggcttcacctactacgccgactccgtcaaaggcaggttcaccatatccagagacaactccaagaacaccctgtacctgcagatgaactccctgcgggccgaggataccgccgtgtactattgcgctaagccccctcgtggctataactacggccctttcgactactggggccagggaaccctggtcaccgtgtcctccgcctctaccaagggaccgtcagtgttccccctggctccttgctctcggagcacatccgagtctaccgctgctctgggctgtctggtcaaagactacttccccgagcctgtcaccgtgtcttggaattccggcgctctgacatctggcgtgcacaccttccctgccgtgctgcagtcctctggcctgtactctctatcctccgtggtgacagtgccatcctccagcttaggaaccaagacctatacatgcaacgtggaccacaagccttccaacaccaaagtggataagagagtggaatccaagtacggccctccctgtcctccttgccccgcccctgagttcctgggcggcccatctgtatttctgttccctcctaagcctaaggacactctgatgatcagccggacccccgaggtgacctgcgtggtcgtggatgtgtctcaggaagaccccgaagtgcagttcaactggtacgtggacggcgtagaggtgcacaacgccaagaccaagcccagagaggaacaatttaacagcacctaccgggtggtatctgtgctgaccgtgctgcaccaggactggctgaacggcaaggaatacaagtgcaaggtgtccaacaagggcctgccatccagcatcgagaagaccatctccaaggccaagggccagccgagagagccccaggtgtacaccctgcctccttcccaggaagagatgaccaagaaccaggtttctctgacctgtctggtgaagggcttttacccatccgacatcgccgtggagtgggagtctaatggccaacctgagaacaactacaaaaccaccccacctgtgctggactccgatggatccttcttcctctactccagactgacagtggacaagtccagatggcaagagggcaacgtgttctcttgctctgtgatgcacgaggccctgcacaaccactacacccagaagtccctgtccctgtcactgggagccggcggcggaggctccggcgggggcggctccggcggcggcgggtcgggcggcggcggctctggcgtgatccacgtgacaaaggaagtgaaagaagtggctaccctgagttgcggccataacgtgtctgtggaagagctggctcagaccagaatctactggcagaaagagaaaaagatggtgctgaccatgatgtccggcgacatgaacatctggcctgagtacaagaacagaaccatcttcgacatcaccaataatctgtccatcgtgatcctggccctgaggcctagcgacgagggcacctatgagtgcgtggtcctgaagtacgagaaagatgccttcaagcgggagcacctggccgaagtgacactgagcgtgaaggccgatttccctaccccttctatctctgacttcgagatccctacctctaacatccggcggatcatctgctccaccagcggcggatttcctgaacctcacctgagctggctggaaaatggagaggaactgaatgctatcaacaccaccgtgtctcaggaccctgaaaccgagctgtatgctgtctcttctaagctggacttcaacatgaccaccaaccactctttcatgtgcctgatcaagtacggacatctgcgggtgaaccagacgttcaactggaacacaaccaagcaggaacacttccctgacaac

SEQ ID NO: 176 - protein, 1113 aa, synthetic construct
  REGION 1..1113: note = AN_Bif_Abs_0062
MGWSCIILFLVATATGVHSLQPGAEVPVVWAQEGAPAQLPCSPTIPLQDLSLLRRAGVTWQHQPDSGPPAAAPGHPLAPGPHPAAPSSWGPRPRRYTVLSVGPGGLRSGRLPLQPRVQLDERGRQRGDFSLWLRPARRADAGEYRAAVHLRDRALSCRLRLRLGQASMTASPPGSLRASDWVILNCSFSRPDRPASVHWFRNRGQGRVPVRESPHHHLAESFLFLPQVSPMDSGPWGCILTYRDGFNVSIMYNLTVLGLEPPTPLTVYAGAGSRVGLPCRLPAGVGTRSFLTAKWTPPGGGPDLLVTGDNGDFTLRLEDVSQAQAGTYTCHIHLQEQQLNATVTLAIITVTPKSFGSPGSLGKLLCEVTPVSGQERFVWSSLDTPSQRSFSGPWLEAQEAQLLSQPWQCQLYQGERLLGAAVYFTELSSPGGGGSGEVQLLESGGGLVQPGGSLRLSCAASGFTFSSYAMSWVRQAPGKGLEWVSGISGSGGFTYYADSVKGRFTISRDNSKNTLYLQMNSLRAEDTAVYYCAKPPRGYNYGPFDYWGQGTLVTVSSASTKGPSVFPLAPCSRSTSESTAALGCLVKDYFPEPVTVSWNSGALTSGVHTFPAVLQSSGLYSLSSVVTVPSSSLGTKTYTCNVDHKPSNTKVDKRVESKYGPPCPPCPAPEFLGGPSVFLFPPKPKDTLMISRTPEVTCVVVDVSQEDPEVQFNWYVDGVEVHNAKTKPREEQFNSTYRVVSVLTVLHQDWLNGKEYKCKVSNKGLPSSIEKTISKAKGQPREPQVYTLPPSQEEMTKNQVSLTCLVKGFYPSDIAVEWESNGQPENNYKTTPPVLDSDGSFFLYSRLTVDKSRWQEGNVFSCSVMHEALHNHYTQKSLSLSLGAGGGGSGGGGSGGGGSGGGGSGVIHVTKEVKEVATLSCGHNVSVEELAQTRIYWQKEKKMVLTMMSGDMNIWPEYKNRTIFDITNNLSIVILALRPSDEGTYECVVLKYEKDAFKREHLAEVTLSVKADFPTPSISDFEIPTSNIRRIICSTSGGFPEPHLSWLENGEELNAINTTVSQDPETELYAVSSKLDFNMTTNHSFMCLIKYGHLRVNQTFNWNTTKQEHFPDN

SEQ ID NO: 177 - DNA, 3339 bp, synthetic construct
  misc_feature 1..3339: note = AN_Bif_Abs_0062DNA
  source 1..3339: mol_type = other DNA
atgggttggagttgcatcatcctatttctagtggccaccgccacaggagtgcacagcctgcagccaggcgcggaggtgcctgtggtgtgggcccaggaaggcgctcccgcccagctgccctgctcccctaccattcctctgcaggacctgtcactgctgcggagagctggcgtaacctggcagcaccagcccgacagcggccctcctgctgctgctccaggccatcctctggcccctggccctcatcctgctgctcctagttcttggggacctcgtcctagacggtacacagtgctgtctgtgggcccgggcggtcttcggtctggtagactgccactgcagcctagagtgcagctggacgagcggggcagacagagaggcgacttttccctgtggctgagacctgccaggcgcgccgatgccggcgagtaccgggccgccgtgcacctcagagacagagccctgtcctgccggctgcggctgcggctgggccaggcctccatgaccgcctctcctccaggctctctcagagcctcggattgggtcatcctgaactgctctttctccagacctgatagacccgcctccgtgcactggttccggaacagaggccagggcagggtgcccgtgcgcgagtctccacaccatcacctggctgagagctttctgttcttgcctcaggtgtcccctatggactctggcccttggggctgcatcctgacttatcgagacggctttaatgtgtccatcatgtacaacctgaccgtgctgggactggaacctcctacacctctgaccgtgtacgccggcgctggctctagagtgggactgccctgcagactgcctgctggcgtgggcaccagatcttttctgaccgctaagtggaccccacctggcggcggcccggatctgctggtgaccggcgataatggcgacttcacactgcgtctggaagatgtgtcccaagcacaggccggcacctacacctgtcacatccacctgcaagagcagcagctgaacgctacagtcaccctcgctatcatcaccgttacccctaaatccttcggctctcccggctccctcggcaagctgctgtgcgaggtgacccctgtcagcggccaagaaagattcgtgtggtcctctctggacaccccttctcagcggtctttttccggcccttggctggaagcccaggaagctcaactgctgtctcagccctggcagtgccagctgtaccagggagagagactgctgggggccgccgtgtacttcaccgagctgtcctctccaggagggggaggctctggcgaggtgcaactgctggaatctggcggaggcctggttcagcctggaggttccctgagactgtcttgtgccgcctctggattcaccttttccagctacgccatgtcctgggtgcggcaggctcctggcaagggcctggagtgggtatcgggcatctccggctctggcggcttcacctactacgccgactccgtgaagggcagattcaccatcagccgggacaactccaagaacaccctgtacctgcagatgaactccttaagagccgaggacaccgccgtgtactactgcgccaagccccctagaggctacaactatggccccttcgactactggggccagggcaccctggtgaccgtgtcgtccgcttctacaaaaggcccttcagtgttccccctggccccctgttctcggtcaacatctgagagcaccgctgctctgggctgtctggtgaaggactacttcccagaacctgtgacagtgagctggaactccggcgctctgacctccggagttcacaccttccctgcagtgctgcagtcttctggcctgtactccctgtcgtctgtcgtcacggtgcctagttcctccctgggcaccaagacatatacctgcaatgtggaccacaagcctagcaataccaaggtggacaagagagtggaatccaagtacggccctccttgtcctccatgcccagcacccgagttcctaggcggcccctccgtgttcctgttcccacccaaacccaaggacaccctgatgatctcccggacccctgaggtcacctgtgtggtggtggacgtgtctcaggaggaccctgaggtgcagttcaattggtacgtggatggcgtggaggtgcacaacgctaagaccaagcccagagaggaacagttcaatagcacatacagagtcgtgtccgtcctgaccgtgctgcaccaggactggctgaacggtaaagagtacaagtgcaaggtttccaacaagggcctgccctcctctatcgagaaaaccatctctaaggccaagggtcagcctcgggagccccaagtgtacaccctccctcccagtcaagaggagatgaccaagaaccaggtgtccttgacctgcctggtcaagggcttctacccttccgacatcgccgtggaatgggagagcaacggccagcccgagaacaactacaagactacacctcctgtgttagattccgacggcagcttcttcctctattcccggctgacggtggacaagtccagatggcaagagggcaacgtgttctcttgctccgtgatgcacgaggccctgcacaaccactacacccagaagtctctgtccctgtccctgggcgctggaggcggaggctccggtggaggcggctctggaggaggcggctctggcggcggcggctccggcgtgatccacgtgaccaaagaagtgaaagaagtcgccacactgtcttgcggccataacgtgtctgtggaagagctggctcagacccggatctactggcagaaagagaagaagatggtgctgaccatgatgtctggggacatgaacatctggcctgagtacaagaaccggaccatcttcgacatcaccaacaacctgtctatcgtgatcctggctctgagaccttccgatgagggcacatacgagtgcgtggtgctgaagtacgagaaagacgccttcaagcgggaacacctggccgaggtgaccctatccgtgaaggccgacttccctaccccctccatctccgacttcgagatccctaccagcaacatccggagaatcatctgctctacctctggcggcttccccgagcctcatctgtcctggctggaaaacggcgaagaacttaacgccatcaacaccaccgtttcccaggatcctgaaaccgagctgtacgctgtgtcttctaagctggatttcaacatgaccaccaaccacagcttcatgtgcctgatcaagtacggccacctgagagtgaaccagaccttcaattggaacaccaccaagcaggagcacttccctgacaac

SEQ ID NO: 178 - protein, 707 aa, synthetic construct
  REGION 1..707: note = sugemalimab-ICOSLG
EVQLLESGGGLVQPGGSLRLSCAASGFTFSSYAMSWVRQAPGKGLEWVSGISGSGGFTYYADSVKGRFTISRDNSKNTLYLQMNSLRAEDTAVYYCAKPPRGYNYGPFDYWGQGTLVTVSSASTKGPSVFPLAPCSRSTSESTAALGCLVKDYFPEPVTVSWNSGALTSGVHTFPAVLQSSGLYSLSSVVTVPSSSLGTKTYTCNVDHKPSNTKVDKRVESKYGPPCPPCPAPEFLGGPSVFLFPPKPKDTLMISRTPEVTCVVVDVSQEDPEVQFNWYVDGVEVHNAKTKPREEQFNSTYRVVSVLTVLHQDWLNGKEYKCKVSNKGLPSSIEKTISKAKGQPREPQVYTLPPSQEEMTKNQVSLTCLVKGFYPSDIAVEWESNGQPENNYKTTPPVLDSDGSFFLYSRLTVDKSRWQEGNVFSCSVMHEALHNHYTQKSLSLSLGAGGGGSGGGGSGGGGSGGGGSGDTQEKEVRAMVGSDVELSCACPEGSRFDLNDVYVYWQTSESKTVVTYHIPQNSSLENVDSRYRNRALMSPAGMLRGDFSLRLFNVTPQDEQKFHCLVLSQSLGFQEVLSVEVTLHVAANFSVPVVSAPHSPSQDELTFTCTSINGYPRPNVYWINKTDNSLLDQALQNDTVFLNMRGLYDVVSVLRIARTPSVNIGCCIENVLLQQNLTVGSQTGNDIGERDKITENPVSTGEKNAAT

SEQ ID NO: 179 - DNA, 2121 bp, synthetic construct
  misc_feature 1..2121: note = sugemalimab-ICOSLG DNA
  source 1..2121: mol_type = other DNA
gaggttcagcttcttgaatctggaggtggtttggtgcaaccaggtgggagtttgcgactgtcatgtgcggcttcaggattcaccttctcatcttacgctatgagttgggttcgacaggcacctggaaagggcctggaatgggtgtcaggcatttccgggtctggtggcttcacttattatgcagattccgttaaagggagatttactatcagtagggacaattcaaagaatactctgtacctccagatgaacagtttgagagccgaggacactgccgtttactactgtgccaaaccacccagaggctacaattacggccctttcgactattggggccaggggactttggtcactgtgtctagcgcaagcacaaagggtccttccgtgtttccacttgccccctgttcacgcagcacctcagaatcaaccgctgccctcggatgtctcgtgaaggactacttccccgagcccgtgaccgtgagttggaattccggcgccctcacaagtggggtccataccttccccgcagtgttgcagagctctgggctgtattcactgtctagcgtggtgacagttccatcttcctccctgggcactaagacttacacttgtaacgtggaccataaacccagtaatactaaggtggataagcgcgtcgagtctaagtatggtcctccttgtccgccttgtcctgccccagaatttttgggtgggccctccgtgttcctctttcctcccaagcccaaggatactctgatgatctcccggactcctgaggtaacctgcgtggtcgtggatgttagtcaggaggaccccgaagtgcagttcaactggtatgtggatggtgtggaggtacataacgccaagactaaaccccgcgaggaacaattcaattcaacataccgcgtggtcagtgtgctcacagtcctgcaccaggactggctcaacgggaaagaatataaatgtaaggttagcaataagggactgcctagctcaatcgagaaaacaatttctaaagctaagggacagcctagagagccacaggtgtatactctgccaccgagccaggaggagatgactaagaaccaggtgtctctgacctgtcttgtcaaaggtttctacccaagtgatatcgcagtcgagtgggagagtaacggccagcccgaaaataattataaaaccaccccccccgtgctggattcagatggctctttctttctgtactcacgccttaccgtcgacaaatccagatggcaggaaggcaatgtgttcagctgcagtgtgatgcacgaggcgctgcacaatcactatacgcaaaagagcctgagcttgagcttgggtgctggaggtggaggatcaggtggtggaggaagtggaggaggaggtagtggtggcgggggatctggtgatacacaagaaaaggaagtacgggccatggtgggatctgacgttgaactgtcctgtgcctgtcctgaaggatccaggtttgacctgaatgatgtgtacgtgtactggcagaccagcgagagtaaaacagtggtgacctatcacattcctcagaatagcagcttggagaatgtggactcaagatacaggaatcgagccctgatgtcacccgcaggaatgttgcggggcgacttctccttgagactctttaacgtgactccgcaggatgaacagaaattccactgcctcgtgttgagtcagagcctggggtttcaagaggtcctgagcgtcgaagtgaccctgcacgtagctgccaactttagcgtgcccgtggtatccgcacctcatagcccgtcccaagacgaactcacgttcacatgtacctccattaacgggtatccccggccaaatgtgtattggattaataaaaccgacaatagcttgctggatcaggccctccaaaatgacacggtgtttctcaatatgcgaggattgtacgacgtggtatctgttctgcgcatcgctcgcaccccttctgtgaatatcggatgctgcatcgagaacgttctgttgcagcagaatctcaccgtaggctcacagacaggaaatgatatcggggaacgagacaagatcaccgagaaccctgtgtccactggcgagaagaacgctgccacc

SEQ ID NO: 180 - DNA, 2037 bp, synthetic construct
  misc_feature 1..2037: note = Avelumab-CD80 DNA
  source 1..2037: mol_type = other DNA
gaagttcagcttttggagtctggagggggtttggtacaaccgggtggaagccttagactgtcctgcgcagccagcgggtttaccttcagttcctatatcatgatgtgggttagacaggctcccggcaagggccttgaatgggtgagcagcatttacccttctgggggcatcacgttttatgctgacactgtcaaaggacgcttcacaatctcccgcgacaatagtaagaatacgctgtacctgcagatgaacagcctgcgggctgaagacaccgcagtctactactgcgctcggattaagctcggcacagttactacagtggactactggggacagggtacactggtgacagtaagttctgcatccaccaaaggccccagcgttttccctctggcaccgtctagtaagtctacatctgggggtaccgccgcgctcggttgtcttgttaaggactattttcctgaacctgtcacagtgagttggaattccggcgcactgacctccggtgtgcatacttttcccgccgttctgcagtcctccggcttgtactccctttcatctgtcgtgaccgtaccttcaagcagtctgggaacccagacttatatctgtaacgttaatcataagccttccaataccaaggtagacaagaaggtggagccgaaaagttgtgacaaaacccacacctgtcctccctgtcctgctcccgaacttttgggcggaccatccgtgttccttttcccccccaagccaaaagatactctgatgataagcagaacacccgaggtcacctgcgtggtggtggacgtttcacacgaggaccccgaggtgaaatttaattggtatgtggacggtgtcgaagtgcataatgccaaaaccaagcctagagaggaacaatacaattcaacttatagagtagtgagcgtgctgacagtgctccaccaggattggctcaacggcaaagagtacaagtgcaaggtgtctaacaaggcattgccagcacctatcgagaaaactatttccaaggcaaaggggcaaccacgggaaccgcaggtttatacattgccaccatcaagagacgagctcacgaaaaatcaggtctccctgacctgcctggtcaaaggtttttatccctctgacatcgccgtggaatgggagagcaatggccaacccgagaataattataagaccaccccacctgtattggatagcgacggctccttttttctgtatagcaaacttacagtggataagtctcgatggcaacagggcaacgtgttcagttgcagcgtgatgcatgaagctctccacaaccattatacacagaagagcctgtctctgtctcctggtgctggagggggaggaagtggtggaggaggatctgggggaggtggaagtggaggaggcggatcaggggtcatacacgtcactaaggaagttaaggaggtggccacgttgagttgtggccataacgtatctgtggaggaactggcccagaccagaatctactggcagaaggaaaagaaaatggtgctcaccatgatgagtggtgatatgaacatttggcctgagtacaaaaataggaccattttcgacattactaacaacctgagcattgtcattctcgccctgagaccaagtgatgagggcacatacgaatgcgtcgtgcttaagtatgagaaggacgcatttaaaagggagcacctggctgaggtgaccctgtctgtcaaggctgacttccctacaccttctataagtgattttgaaatccctacaagcaacattagacgaatcatttgcagcaccagcggcggttttccagagccacatctgtcctggctcgagaatggcgaagagctgaacgccatcaacacaactgtgtcccaggatcccgaaactgagctgtacgccgtgtccagcaagctggattttaatatgaccacgaatcattcattcatgtgtctgatcaagtacggacatctgagagtcaaccaaaccttcaactggaacacaaccaagcaggaacacttcccggacaat

SEQ ID NO: 181 - DNA, 2031 bp, synthetic construct
  misc_feature 1..2031: note = Atezolizumab-CD80 DNA
  source 1..2031: mol_type = other DNA
gaagttcagcttgttgaatcaggaggaggactggtccaacctggaggatctttgcgacttagttgcgccgcctcaggctttactttctccgactcttggatccactgggtgagacaggcaccaggaaaaggtctcgaatgggtggcctggatcagtccatacggcggcagcacctattacgccgactccgtaaagggtcgcttcaccatttccgctgacactagcaagaatacagcctacctgcaaatgaacagtctgagggctgaggatacagctgtctactattgtgccaggcggcattggcctggcggatttgactactggggtcagggcaccctggtgacagtgtcctctgcctctaccaaggggccttctgtcttccctctcgcccccagttcaaagtctacctcaggcggaacagctgcccttgggtgtctggtgaaggactatttcccggaaccggtgacagttagctggaactccggggcattgacttctggagtacatacattcccagccgtgcttcaaagcagcgggctgtattccttgagctcagtcgtcactgtccctagttccagcctggggacacagacatatatatgtaatgtgaatcataagcccagtaacacgaaggttgacaaaaaggtggagccgaagagctgcgataaaacccacacatgtcccccatgtccagcacccgagcttctcggaggaccttccgtcttcctgtttccacctaagcctaaggacactctgatgattagtcgcacccctgaagtgacctgtgtcgttgtcgacgtgagccatgaggacccagaagtgaaatttaattggtacgtggacggagttgaagtccataacgccaaaactaagcctcgcgaagagcaatatgccagtacatatcgagtagtatctgtgcttacggtgctccatcaggactggctgaacggaaaagaatataaatgcaaggtgtccaataaggctctccccgcccctatcgaaaaaaccatttccaaggctaaaggccagcctcgcgaaccgcaggtttatacactcccgccatctagagaagaaatgaccaagaaccaggtcagcctgacatgcctggttaagggcttctacccttctgatatagcagtggagtgggagtctaacggacagcctgagaacaactacaagaccactccgccagtgctggactccgatggctctttcttcctctatagtaagctcaccgtcgataagagtcgctggcagcagggcaatgtgttttcttgtagcgtgatgcatgaagccctgcacaaccattatacccagaagtcacttagtctgagtcctggagcaggaggtggtggtagtggtggaggcggttcaggaggagggggatctggtggaggtggatcaggtgtgatccacgtgacaaaagaagtaaaggaggtggcaacactgtcttgcggccataatgtttccgtggaagaactggcccagacacgaatctattggcagaaagaaaaaaaaatggtcctgaccatgatgagcggcgacatgaacatctggcctgaatataaaaacagaaccatcttcgacatcactaacaatctctcaattgtgatcctcgcactgcggccatcagacgaggggacttatgaatgtgtggttttgaagtatgagaaggacgcattcaaaagagagcatctcgctgaagtcacactcagtgtaaaggccgatttccctacgcctagcatttccgacttcgagattcctacgtccaatattcggagaatcatatgctctactagcggaggcttccctgagccacacctgtcctggctcgagaacggggaggagctcaatgctatcaacaccactgtcagccaggacccagaaacagaactgtatgccgtgagctccaaactggacttcaacatgactaccaatcattcattcatgtgtttgatcaagtatggtcatctgagagtgaaccagacctttaattggaacaccaccaaacaagagcacttcccagataac

SEQ ID NO: 182 - DNA, 2634 bp, synthetic construct
  misc_feature 1..2634: note = Durvalumab-LAG3 DNA
  source 1..2634: mol_type = other DNA
gaagtgcagcttgtggaatctggaggaggcttggtacaaccaggaggcagtcttaggctcagttgtgcagcaagcgggtttaccttttctaggtattggatgagttgggtgcgccaggcccctggaaaagggcttgagtgggtcgccaatattaagcaggacggctccgaaaaatactacgtggacagcgttaagggccgctttacaatttctcgcgacaatgccaagaattccttgtacctgcagatgaacagcctgagagctgaggacactgccgtttactactgcgctcgagagggcgggtggttcggagaactggcttttgattattgggggcaaggaaccctggttaccgtgtcttccgcctccacaaagggcccaagtgtattccccctggctccctcttccaaatctacatccggaggcaccgccgcattgggctgtttggtaaaggactatttcccagaacctgtcacagtctcttggaacagcggcgcattgacctccggcgtgcacacattccctgctgtcctgcagtcctctggactttactccctcagctccgtggtgaccgttccttccagctcactcggtactcagacttatatctgcaacgtgaatcacaagccaagtaatacgaaagtagataagcgggtcgaacccaagtcttgtgataagacccatacctgtccaccatgtcctgctccagagtttgagggaggccctagcgtcttcctgttcccaccaaaaccaaaggataccctgatgatcagccggacccctgaggtgacctgtgttgtggttgatgtctcccacgaggacccagaagtgaaatttaattggtatgtagatggggtggaggtgcataacgctaaaactaagcctcgcgaagagcagtataactcaacttatcgggttgtgagtgtcctgacagtccttcaccaggactggctgaatggtaaagagtataaatgcaaggtgtccaacaaggcactccctgcgagtatcgagaagacgataagcaaggccaaaggacagcctagggaaccacaggtgtacactttgcccccaagcagagaggaaatgaccaagaatcaagtgagtctgacctgcctggttaagggcttctaccctagcgacattgctgtggagtgggagtccaatgggcagccggaaaacaactacaagactacaccacctgtattggactccgatggctctttcttcctgtacagtaagctgacagtggacaaaagccggtggcagcagggcaatgtgttctcctgtagcgtgatgcacgaggcactgcacaatcactacacacaaaaatcactgtccctctcacctggagcaggtggaggaggatctggaggtgggggatcaggcggtggaggaagtggaggagggggatcaggtcttcaacctggagccgaagtcccggtcgtatgggcacaagagggagctccggcacagttgccatgctcccctactataccactgcaagacctgtctctccttaggagagccggcgttacatggcagcaccagccagactccggacctccagctgctgcaccaggacatcccctggcaccaggacctcatcctgctgctccatcttcttggggcccaagacccaggcggtacaccgttctttcagtagggcctggaggcctgagaagtggtcgccttcctctgcagcctcgcgtacaacttgatgagcggggaagacagcggggggatttttctctgtggttgagacctgcccgcagagccgatgcaggggaatatagagccgccgtgcacctcagagatagagccctgtcttgtcgacttagactgcggttggggcaggcttcaatgacagcttctcctcctgggagcctcagagcttctgactgggtcatcttgaattgctcattctcccggccagatagacctgcatcagttcactggtttcgaaatcggggacaggggagagtcccggtgagagaatccccccatcaccacctcgcggaaagtttcctgtttctgcctcaggtttctccaatggactctggcccctggggatgcatccttacctatagagatgggtttaatgtctccattatgtataacctgacagttcttggtctggaaccgcccacaccactgactgtctacgcaggagcaggttcaagagtcggacttccttgcagattgccggccggggttggaaccaggtcatttctgaccgctaaatggaccccaccagggggaggtccggatttgctggttactggggataacggcgacttcacactccggctggaagacgtgtcacaagcccaagcaggcacctatacctgccatatccatctgcaagagcagcaactcaatgcaacggtgaccttggccattattacagttacacccaagagctttggttctcccgggagcctgggcaaacttctttgcgaggtgacccctgtttcaggccaggaaaggttcgtgtggagttccctggatacaccttctcagagaagcttcagtgggccttggttggaagcccaggaagctcaactcctgagccagccctggcaatgccaactgtatcagggggaaagactgctgggagccgctgtgtattttacc

SEQ ID NO: 183 - DNA, 2361 bp, synthetic construct
  misc_feature 1..2361: note = Envafolimab-LAG3 DNA
  source 1..2361: mol_type = other DNA
caagtgcaattggttgaatcaggtggaggattggtgcagcctggagggtcattgaggctgagctgtgctgcatctggcaagatgtcatcacggcgctgcatggcatggttcaggcaagcacccggaaaagaaagagaaagagtggcaaaactgcttaccacgtcaggcagcacctacctggcagactccgtgaaaggccggttcactatcagcagggacaatagcaaaaacacagtgtatttgcagatgaactctctgagggccgaagacacagccgtctactattgtgcagccgacagctttgaagatcctacttgtaccctggtaacatcttccggagcctttcagtactggggccaaggaaccctggtgactgttagttcagaaccgaagagctccgacaaaacgcatacttgtccaccttgtccagcacccgagctgttgggaggcccttctgtatttctgttcccacctaagccaaaagacaccctgatgatctcccgcacccctgaagttacctgtgtagtggtagccgtttcacatgaggatccagaagtaaaattcaattggtacgtggacggcgtggaggttcataatgcaaagactaagccccgcgaagagcagtacaactcaacttatcgcgtcgtttctgtcctcaccgttctgcaccaagattggctcaatggcaaagaatacaagtgcaaagtatctaataaagctctcccagccggtatagagaagaccatatcaaaagcaaaggggcagcccagggaaccacaggtttatactctgcctccaagccgcgacgaactgacaaagaatcaggtcagtcttacctgccttgtgaaggggttttatccttcagacatagcagtggagtgggagagtaatggacagcctgaaaataactacaagacaacccctcctgtactggactctgacggttctttcttcctgtacagcaagctgaccgtcgataaatctcggtggcagcagggcaatgtgttctcttgtagcgttatgcatgaggcccttcataatcattatacccaaaagtccctctctctttcaccaggagcaggaggaggtggttcaggtggaggaggaagtggaggaggaggtagtggcggcggaggttctggtctccaacctggtgctgaggtaccggttgtgtgggctcaggaaggagcaccagcccagctgccttgttctcctacaattcctctgcaggatctgtcactcctcagaagggccggagttacttggcaacatcaacctgattcaggacctccagccgcagctcctggacatcctctcgcacctggccctcatccagcagctcctagctcttggggacctagacctaggcggtataccgtactgagcgtgggtccaggcggtttgcgctctggtaggctgccacttcaaccgcgggtgcaactggatgagcgaggaagacagcgaggtgacttttctctgtggcttagacctgcaagaagagccgatgctggggaatatagagccgcagtgcatctgcgcgatagagctctgtcatgtaggttgagattgaggctgggtcaggcttctatgaccgcatctccccctggctcattgcgagcttcagattgggtgattctgaactgctcattttcacggccagacagacctgctagcgtgcactggttccgaaatcggggacaaggccgagttccagtgagggagtcaccacatcaccatctggcggagagcttccttttcttgccacaggtctctcctatggactctggcccctgggggtgcattctgacttacagagatggttttaacgtgtccatcatgtacaatcttaccgttttgggcctggagccaccaacacccttgacggtttacgcaggagctggatcccgagtgggattgccatgcagacttccagcaggcgtaggtacaagaagctttctgacagcaaaatggacacctcctgggggaggtccagaccttctggtaactggagataacggagatttcaccctgaggctggaggacgtttcacaggctcaggctggtacttatacttgccacattcacttgcaggagcagcagcttaatgcgaccgtcaccttggctattatcacagttacacctaagtcattcggttctcccggcagtctgggaaagctgctgtgcgaggtgacacctgtgtccgggcaagagagatttgtgtggtcctccctggatacaccctcccaaagatccttcagtggtccctggctggaagctcaggaggctcagctgctctcacagccctggcagtgtcaactgtatcagggagaaaggctgctgggagctgcagtttacttcacc

SEQ ID NO: 184 - DNA, 3045 bp, synthetic construct
  misc_feature 1..3045: note = LAG3-Envafolimab-CD80 DNA
  source 1..3045: mol_type = other DNA
ttgcaacctggagctgaagttccggttgtatgggcacaggaaggtgcgcctgctcagttgccatgtagccccacaattccgctgcaagatcttagcctccttcgcagagctggcgtgacatggcaacatcaaccagattctggaccaccagctgctgctccaggacatcctcttgcacctggcccacatccagctgcacctagctcatggggccctagaccaagacgctacactgttctctctgttggccccggagggttgaggagtggtagactgccactgcagcctcgcgttcaattggacgaacgaggtcgccaaagaggcgattttagtctctggctgagacccgctcggagagctgatgcgggtgaataccgggccgctgttcacctgcgggatagagcactgtcatgtaggctgcgcctcagactgggacaggcaagcatgacggcttctcctcccgggtctttgagggcgagtgactgggtaatccttaactgcagtttctctagacctgaccgaccggcgtccgtacattggttcaggaacagaggccagggaagggtgcccgtcagggaatctccccatcatcatttggcagagtctttcctgtttctgccccaggtgagccctatggactctggcccttggggctgtattctgacctatagagatggtttcaatgtgagcatcatgtacaacttgaccgttttgggactggaaccacccacccctctgacagtgtatgctggagcaggttccagggtaggtctgccctgtagactgccagccggagtaggaacccgaagtttcctcactgccaaatggaccccgccaggtggaggtcctgatctcctcgtgacaggcgataatggagacttcacactcagactcgaggacgtgtcacaggcacaagccggtacctacacctgccacatccacctgcaggagcagcagttgaatgccacagtcactctggccatcattaccgtcacaccaaaaagcttcggatctcccggatcattgggcaagttgctgtgtgaggtgaccccagtttctgggcaggagaggtttgtgtggtcctccctcgatactccatcccagaggagttttagcggtccttggctggaggcccaagaagcccagcttctgtcccaaccgtggcaatgtcaactgtaccagggagaaaggctgcttggagcagccgtgtattttactggaggaggaggcagtggtggaggtggttctggtggtgggggatctggtggtggatcaggtcaggtacagttggtggaaagcggaggcgggttggtacagcctggaggatcattgcgattgtcatgtgccgcctccggaaagatgagctctcggaggtgcatggcttggttccgccaggctcccggaaaggagagagagagggtcgctaagttgctcactacatcaggcagcacgtacttggccgatagcgtaaaaggaagattcacgattagccgcgataactccaaaaacaccgtttacctgcagatgaactccttgagagccgaagacaccgcagtttactactgtgccgccgacagtttcgaggatccgacctgtacgctggttaccagttcaggcgcctttcaatactggggccaaggaacactggtgaccgtcagctctgaaccaaaaagttccgataagactcatacgtgtccaccttgtccagccccagaattgctgggaggtcctagcgtgttcctgttcccaccgaagccaaaagataccctgatgattagcaggacaccagaagtgacttgcgtggtcgttgccgtcagtcacgaggatcctgaggtgaaatttaactggtacgtggatggcgtcgaggtgcataatgcgaaaacaaagcctcgagaagagcaatacaatagtacctatagagtcgtgtctgtcctgaccgtgcttcatcaggactggctgaatggcaaggagtataagtgtaaagtaagcaacaaggcactgcccgcaggcattgagaagaccatctcaaaggccaaagggcagccacgcgaaccacaagtatacactctgccaccgagccgcgacgagctgactaagaaccaggtgagtctgacatgcttggtcaagggattttacccctctgatatagctgttgagtgggaatcaaacggccaacccgaaaataactataagacaaccccccccgtcctcgattccgatggatcctttttcctttactctaagcttacagtagacaagtcaagatggcagcagggaaatgtgttttcatgttctgtcatgcacgaagccctccataatcactacactcagaaatctctttcactctctccaggtgcaggtggaggagggtctggtggaggaggatcaggtggtggaggcagtggaggtggtggaagcggagtgattcacgtcacaaaggaggttaaagaagtcgctacacttagctgtggtcataatgtctccgtggaagaactggcccagacccgcatatattggcagaaggagaaaaaaatggtgctgacaatgatgtccggggacatgaatatttggcccgagtacaagaaccgcaccatttttgacatcacaaataatctttcaatcgtgatcttggccctgcgaccctccgacgaaggtacgtatgagtgtgtggtgcttaaatatgaaaaagacgcctttaagcgcgagcacctcgctgaagtcacactgtccgtgaaagccgacttccctacgccttccatcagcgacttcgaaattcctacaagtaacatccggaggatcatctgctctacatccggcggattccccgagccacatctcagctggctcgaaaacggggaggaactgaacgcaatcaacaccaccgtgagccaggatcctgagactgagctttatgctgtcagttctaaattggacttcaatatgaccacaaaccattcatttatgtgcctgatcaaatatggccatctccgagtgaaccagacattcaactggaacaccacaaaacaggaacactttcctgacaat

SEQ ID NO: 185 - DNA, 3309 bp, synthetic construct
  misc_feature 1..3309: note = CD80-sugemalimab-LAG3 DNA
  source 1..3309: mol_type = other DNA
gtaatacacgtgacaaaagaggttaaagaggtggccactctctcctgtgggcataacgttagtgtcgaggagttggcccagaccaggatctactggcagaaggaaaagaaaatggtccttaccatgatgagcggagatatgaacatctggcctgaatataagaatcgaaccatttttgacatcacaaacaacctttctattgtcatcctggcgctgaggccctcagacgaaggcacatatgaatgcgtggtcctgaaatatgagaaggacgcctttaaacgagagcatctcgccgaagtgacccttagcgtcaaggcagactttcctactccttctataagcgatttcgaaatcccaactagcaacatccggcggattatctgttctactagcggcggattccctgaacctcacttgagttggctggaaaacggtgaagagctgaacgccatcaacactactgtgtcacaggacccagaaaccgagctctacgccgtatcatccaagcttgacttcaatatgacgaccaaccactcatttatgtgcctcatcaaatatggtcacctgagagttaaccagaccttcaactggaacaccaccaagcaggagcactttcctgacaacggtgggggaggtagcggcggaggcggctctggagggggaggttctggcggcgggtcaggggaagtgcaactgctggaaagcggcggaggccttgtgcagcctggcggttctctgagactcagctgcgccgcgagcgggttcacgttcagttcttacgcaatgagctgggttaggcaggctcctgggaaggggctcgagtgggtctccgggatctctggcagcggcggcttcacatattacgcagatagtgtcaaaggacggttcacaattagccgagataactctaaaaacacactgtaccttcagatgaattcactgcgggccgaagacaccgccgtgtactactgcgccaagccccctcgcggatacaattacggtcccttcgactattggggccagggcacactggtgacagtgtccagtgcttctacgaagggaccttccgtgttccctcttgccccctgcagcaggtctacatctgagtccacagcagccctgggatgcctggttaaagactacttccccgagcccgtgacagtatcttggaactccggagccctgacgagtggggtgcacacattccctgccgttttgcagagctctggcttgtatagtctgtccagcgtcgtgaccgtgcccagctccagcctcggcacgaaaacctacacttgcaatgtggaccataaaccgtccaatactaaggttgacaagagagtcgagtcaaagtacggacccccatgccccccatgtccggctcccgaatttctcgggggccccagcgtgtttttgtttcctccaaaacccaaggacacattgatgatatcaaggactcccgaggtgacatgcgtagttgtggacgtttctcaggaagatccggaggtccaatttaattggtatgtggacggcgtggaggttcataatgctaagactaagccaagagaagagcagttcaactcaacctacagggttgtgtctgtcctcaccgtgctgcaccaggactggctgaacggaaaggagtacaaatgcaaagtgtcaaacaaggggctgccatcaagcatcgaaaagaccatcagcaaggcaaaggggcaaccccgcgaacctcaggtgtacacactccctccttctcaggaagaaatgaccaaaaatcaggtgagcctcacatgtttggtgaagggtttttacccatccgatattgccgttgagtgggagagtaacggacaacccgaaaataactataaaacaaccccacccgtcctcgatagtgacggatccttctttctgtacagcaggttgacagtggacaagtcccggtggcaggagggcaacgtgttctcttgttccgttatgcatgaagccctgcataaccattatacacagaaatcactcagcctgagtctcggagccggagggggaggaagcggaggaggagggagcggtggaggaggcagtggtggaggcggctcaggcctccagccaggcgccgaagtgcctgttgtgtgggcccaggaaggcgcccccgcacagctcccctgcagccctactattcccctgcaggatctctccctgctgcgcagagccggcgttacatggcaacatcagcctgattctggccctccagcagcggctcctgggcatcccctcgctcctggaccccatccagcagcccctagctcctggggaccacgcccaaggagatacaccgtgctcagcgtcggcccgggcggcttgaggtcagggaggctgcccctgcagccacgggttcagttggacgaacggggacgccagagaggagacttttcactctggttgcggcctgcccgcagggccgacgctggagagtatcgggccgccgtgcacctccgagaccgcgccctgtcttgccgattgagactgcggctgggtcaggcctccatgactgcttcacctccggggagtctgcgcgcatcagactgggttatactcaattgttcattctcccggccagaccgcccggcttcagttcactggtttcgaaaccggggacagggccgggtccctgtgcgggagagcccacaccatcacttggcggaatcttttctctttctgccacaggtgagccctatggactctggaccctggggctgcatcctcacatacagggatggcttcaatgtaagcattatgtacaacttgaccgtgttgggcctggaacctcccactccccttacggtgtacgccggcgccggctctagagttgggctgccgtgccggctgccagctggagttggcacacgcagctttctgacagctaaatggacccccccagggggagggcctgacctcctggtaacaggtgacaacggcgattttaccctccggctcgaagatgtttcacaggctcaggcgggcacctacacctgccatattcatctgcaggaacagcaactgaatgcaacagtgaccctcgccatcattacagtcacccccaaatcatttgggagtcctggttccctcggcaagctcctttgcgaagtgactccagtgtcaggtcaagagaggttcgtctggtccagtctggacacccctagtcagcggtcattctccggcccatggctggaggcccaagaggcccagctgctgtctcagccctggcaatgccagctgtaccagggcgagcgcttgctcggagctgccgtgtacttcact

SEQ ID NO: 186 - DNA, 1869 bp, synthetic construct
  misc_feature 1..1869: note = Envafolimab-LAG3 IgD1/D2 DNA
  source 1..1869: mol_type = other DNA
caagtacagctggtagaaagtggaggaggcttggtacaacctggggggagtctgagattgagctgcgctgcctcaggcaaaatgagttcccggagatgtatggcctggtttagacaggccccaggaaaagaacgggagcgggtggcaaaactcctgaccacatctgggtcaacatacctcgctgatagtgtgaagggcaggttcaccatcagcagggataactctaaaaacactgtgtacttgcagatgaactctcttcgcgccgaggacactgccgtgtactactgtgccgcagacagcttcgaggatcccacatgcacgctggtgaccagctcaggcgcctttcagtattggggacagggcactctggtgaccgtgagttctgagcccaaatcctccgataagacgcatacctgtcctccttgccctgcgccagagttgcttggtggacctagtgttttcctgttcccacctaagcctaaagacacgctgatgatctcacgcacccctgaggtgacttgcgtggtggtggcggttagccatgaagaccctgaagtgaagttcaattggtatgtggatggggtagaggtgcataatgccaagactaaaccacgggaagagcaatataattccacataccgggtggttagcgttctcacggttcttcaccaggactggcttaacggaaaagagtacaagtgcaaggtgtctaacaaagccctgcccgccggaatcgagaagacaataagcaaggcaaaggggcagcctagagagccgcaggtctacactttgcccccaagcagagacgagcttactaaaaatcaggtttccctgacgtgcctggttaaaggattttatccctctgatatcgccgtggagtgggagtccaatggtcagcctgaaaacaactacaagaccacgcctcccgtccttgactctgatggcagcttcttcctgtattcaaagctgacggtcgataaatctagatggcagcagggcaatgtcttttcctgctccgtgatgcacgaggctctgcacaaccactatacccagaagtccctgtctctcagcccaggagctggaggaggaggttcaggtggtggtggatcaggaggaggcggatctggtggagggggatctggactccaaccaggtgcagaggtcccagtcgtatgggctcaagaaggagccccagcacagctcccatgtagccctaccattcccttgcaagacctcagcttgctgagaagagccggagtcacctggcagcatcagcctgattctggacctcctgctgcagcaccaggacatccattggctcctggaccccatcctgccgctccttcaagctggggtcctagacccagaagatacacagttctgtccgtgggaccgggtgggctgagatcaggacgactgccactgcagcctagagtccaactggatgagcgcggacgccagaggggagattttagtttgtggttgaggccggccagaagagctgatgctggggagtatagagccgcagtgcacttgagagacagggccctgagctgcagacttagactgcggcttggccaggcctcaatgacagcatcaccaccaggttcactgagagctagcgactgggtgatcctgaattgttccttctccaggcctgatcgccctgcttccgtccactggtttagaaatagaggccaggggagggtgccagtcagagaatccccccatcatcatctggcagaaagcttcctgttcctgcctcaggtgtcccctatggacagtggaccatggggatgtatcctgacctatcgcgacgggttcaatgtgtcaatcatgtataatctgaccgtcttgggccttgaaccg

SEQ ID NO: 187 - DNA, 2118 bp, synthetic construct
  misc_feature 1..2118: note = Envafolimab-LAG3 IgD1/D2/D3 DNA
  source 1..2118: mol_type = other DNA
caggttcagcttgtagaatctggaggaggcttggtgcaacctggtggatctctccggttgtcatgtgccgcttcaggcaagatgagttcacgaagatgtatggcatggttcaggcaggctcctggcaaagaaagggaacgggttgcaaagctgcttaccaccagtggttcaacgtacttggcggactcagtgaaaggtcggttcacgatctcaagggataatagtaaaaacaccgtgtacctccagatgaattccctgcgggctgaggacaccgctgtctactactgtgctgctgactctttcgaagatccgacctgcactcttgtgaccagtagcggcgcttttcagtactggggacaagggacattggtcacagtgtccagtgagcccaagagtagtgataaaacacatacttgtcccccatgtcctgctcctgagttgctgggaggaccttctgtgtttctgttcccaccgaagcctaaggacactctgatgattagcaggactccagaagtgacctgcgtggtagtggccgtctctcacgaagatcccgaggtgaagtttaactggtatgtcgacggagtggaggtgcacaacgctaagactaaacctagggaggaacaatacaacagcacctaccgggtggtttctgtactcactgtcctgcatcaggattggctgaatggcaaagagtacaagtgtaaggtcagtaacaaggccctcccagccggaattgagaaaacaatctccaaagccaagggtcagcctagggaaccccaagtgtacaccttgccacccagtcgggatgagctgacaaaaaatcaggtgtcactcacctgcttggtcaagggcttctaccctagcgatattgccgtggagtgggaatccaacggccagccagaaaacaattacaagaccacaccacctgttcttgactctgatggaagcttttttctgtatagcaagttgaccgtagacaagtccagatggcagcagggcaacgtattttcatgcagcgtgatgcacgaagctctgcacaaccactacacacagaaatctttgtccctgtctcctggagctggaggtggagggtctggaggtggaggttcaggcggaggaggatctggcggaggaggatcaggtttgcaacctggagccgaagtgccagtggtttgggcacaggaaggtgctccagcgcagcttccttgttcacctactataccacttcaggacctgagtctgctgcgcagagccggagtgacctggcaacaccaaccagatagcggtcctccagcagctgcaccaggtcacccactggctccaggaccacaccctgctgcaccaagttcatggggcccacgacccagaagatacacagtgttgagtgtaggtccgggtgggcttaggagtgggagactgccattgcagcccagagttcagctggacgagagaggcagacagagaggtgatttttctctgtggctgagaccagctagacgcgcagatgccggggagtatagagctgccgtgcatctccgcgatagggctctgtcctgtaggctgagattgagattgggacaagcatcaatgacagcatctccaccaggttctttgcgggcctcagactgggttatcttgaattgcagtttcagcagaccagaccgcccagcctctgtacactggtttcgcaataggggccagggaagggttcccgtgagggaatctccccatcatcatctggccgaatctttcttgttcttgccacaggtgagccctatggattctgggccatggggatgcattcttacataccgagatgggttcaacgttagtattatgtataatctgacggtgctgggactcgaacctccaactccacttaccgtatacgccggcgcaggtagtagagttgggctcccttgtagacttcccgctggtgtgggaacaagaagctttctgactgctaaatggacacctcctggaggcggtcctgatcttctggtcacaggagacaatggtgatttcaccttgcggctcgaagacgtgtcacaagctcaggccgggacttatacctgtcacattcatctgcaggagcaacagcttaacgctaccgtcacc

SEQ ID NO: 188 - DNA, 648 bp, synthetic construct
  misc_feature 1..648: note = Avelumab(MSB0010718C) DNA
  source 1..648: mol_type = other DNA
caatcagcccttacgcaaccggcatcagtttctggatcacctggtcagagcatcaccatcagttgtaccggcacatcctcagacgtgggaggatacaattacgtttcctggtaccagcagcaccctggaaaggccccgaaactcatgatttacgatgtgagcaacagacctagcggggtgagcaaccgcttcagtggctctaagtctgggaatacagcttcactgacaatcagtggcctgcaggccgaagacgaagccgactattactgttcatcatatacatcttcaagcacccgggtgttcgggaccggtacaaaggtgaccgtgctcggccaacccaaagccaaccccactgtcacgctgtttcctcctagcagcgaggagctccaggccaacaaggccaccctggtttgtctcattagcgatttttatcctggagctgtcacggtggcatggaaagctgatggctctcccgtgaaagctggcgtggaaactaccaaaccttcaaagcagtctaataacaagtacgccgcgagctcttatttgagtctgacacccgagcagtggaaatcacatcgctcttactcatgtcaagttacccatgaagggagtaccgtggagaagacagtggctccaacagagtgtagc

SEQ ID NO: 189 - DNA, 642 bp, synthetic construct
  misc_feature 1..642: note = atezolizumabMPDL3280A DNA
  source 1..642: mol_type = other DNA
gacattcagatgactcaatcaccatctagcttgtccgcctctgtgggtgaccgggtgacaattacctgccgcgcctcacaggatgtgtccaccgctgtggcctggtatcagcagaagccaggaaaggcgccaaagttgctcatctactcagccagcttcctctactcaggagtgccatcaaggttcagtggctcaggaagcggcacagactttactctgaccatctcatcacttcagcccgaagactttgccacatactactgccagcaatacctgtatcatcccgcaacgttcgggcaaggcacaaaggttgagattaagaggaccgtcgcagcaccaagtgtctttattttcccacccagcgatgagcagctgaaatcaggcaccgcctccgtggtgtgtctgctcaataatttctaccctagggaggcaaaagttcagtggaaagtagataatgccttgcagtccggcaactctcaggagagtgtgaccgagcaagactctaaggactccacctactccctgtcatccaccctgacactgtccaaggccgattacgaaaaacacaaggtctacgcttgcgaggtgactcaccaaggactctcttccccagtgacaaagtcctttaacaggggcgaatgc

SEQ ID NO: 190 - DNA, 645 bp, synthetic construct
  misc_feature 1..645: note = Durvalumab(MEDI4736) DNA
  source 1..645: mol_type = other DNA
gaaatcgtgcttactcagagtcctggcactctgagtctgtctccaggggaaagggccaccctgtcatgcagagcttcacagcgcgtgtcaagctcttatctggcttggtatcaacagaaacctggccaggctccccgattgcttatctatgatgcgtcatcacgggcaacagggatccccgataggttcagcgggagtggcagtggcaccgactttacactcacaatctctaggctggaaccagaggacttcgctgtgtactactgccagcagtacgggtccctcccatggacctttggacaaggaactaaggtggagatcaagcgaacagtggcagctcctagcgtgttcatctttccaccatcagatgagcagctcaagtcagggactgcctcagtggtttgcctgttgaacaacttttacccacgcgaggctaaagtccagtggaaagtcgataatgccctgcaatccgggaacagccaggaatctgttaccgagcaggactctaaggatagtacctactccttgtcaagcaccctgactctgagtaaggcagactacgagaagcacaaggtttatgcgtgtgaggtgacacaccagggactgtcaagccctgtgacaaaatctttcaaccggggcgaatgt